European Patent Application EP 4 374 872 A1, published May 29, 2024. Title: PDE enhanced CAR-T cells. Applicant: Koninklijke Philips N.V. Application EP. The sequence listing filed with the application follows.

SEQUENCE LISTING (122 sequences)

SEQ ID NO: 1 - DNA, 4829 bp, Homo sapiens
  source 1..4829: mol_type = other DNA
gtcagagtcttccctcagctttgtacatcagcactgttttgatagataagagaggctactgtataagtgtgtaagatttgtaatggactgaggaatgcttgttctagctgctgaaactgactgtaactgtattgtcttaggagcatcatcatggggtctagtgccacagagattgaagaattggaaaacaccacttttaagtatcttacaggagaacagactgaaaaaatgtggcagcgcctgaaaggaatactaagatgcttggtgaagcagctggaaagaggtgatgttaacgtcgtcgacttaaagaagaatattgaatatgcggcatctgtgctggaagcagtttatatcgatgaaacaagaagacttctggatactgaagatgagctcagtgacattcagactgactcagtcccatctgaagtccgggactggttggcttctacctttacacggaaaatggggatgacaaaaaagaaacctgaggaaaaaccaaaatttcggagcattgtgcatgctgttcaagctggaatttttgtggaaagaatgtaccgaaaaacatatcatatggttggtttggcatatccagcagctgtcatcgtaacattaaaggatgttgataaatggtctttcgatgtatttgccctaaatgaagcaagtggagagcatagtctgaagtttatgatttatgaactgtttaccagatatgatcttatcaaccgtttcaagattcctgtttcttgcctaatcacctttgcagaagctttagaagttggttacagcaagtacaaaaatccatatcacaatttgattcatgcagctgatgtcactcaaactgtgcattacataatgcttcatacaggtatcatgcactggctcactgaactggaaattttagcaatggtctttgctgctgccattcatgattatgagcatacagggacaacaaacaactttcacattcagacaaggtcagatgttgccattttgtataatgatcgctctgtccttgagaatcaccacgtgagtgcagcttatcgacttatgcaagaagaagaaatgaatatcttgataaatttatccaaagatgactggagggatcttcggaacctagtgattgaaatggttttatctacagacatgtcaggtcacttccagcaaattaaaaatataagaaacagtttgcagcagcctgaagggattgacagagccaaaaccatgtccctgattctccacgcagcagacatcagccacccagccaaatcctggaagctgcattatcggtggaccatggccctaatggaggagtttttcctgcagggagataaagaagctgaattagggcttccattttccccactttgtgatcggaagtcaaccatggtggcccagtcacaaataggtttcatcgatttcatagtagagccaacattttctcttctgacagactcaacagagaaaattgttattcctcttatagaggaagcctcaaaagccgaaacttcttcctatgtggcaagcagctcaaccaccattgtggggttacacattgctgatgcactaagacgatcaaatacaaaaggctccatgagtgatgggtcctattccccagactactcccttgcagcagtggacctgaagagtttcaagaacaacctggtggacatcattcagcagaacaaagagaggtggaaagagttagctgcacaaggtgaatctgatcttcataagaactcagaagacttagtaaatgctgaagaaaaacatgatgagacacattcataggcccgaaacaccttaaagacttctgtcattttaaacatgagaggacaatgaaatcagcatgaaaacatcctaaattctcaactttccacaaagctatggctcttctttcaacatagaattggattgggccattttaattgactcctatacaaggaattaagaagaacataaattttgagctagtaactctggccaaataaatacactcaagtttttatcagagtttttggccagtgcttctgccatttttttccctccacaatttggccttcttcaatcaagccagataaatttttgagacaaaagtcagacagtttttaatttttcttgctttgaaccctgtcataatgactgtgcaatacatgtgcagaagatgaggtattttaaaatttacttccttgcactgtcttacacagagtgctataactataaatttttcaaggtcttaaataaaaggaagcaaaaacaaaattattgaaaaattttttttgttgtgctggggaatatactatttagattgtccttcttattttaaatgcatgggaacagaatgacaggtgggatgctgaggagctggttgaagcatcagagcaatgctacagtccaacaatggagcattagatccccagctaggtgacctgatgaacacctttgtaaactctcatactgggaaatggcagtgaaacctttttctgaacccgtggaccagcctgcgtccgtccccatggtttcaaagcacgaatgcattacctccatggttgtggttacaagcaagtcacatgctatctacagttcatgataacaagaccgtcaaccattgctggagacagacactagaatggaaaatgaaatttgccagcgggatgtttatcccatcagaatgtaacaaaatatattaccagccaagagataagagacaagaatgtgtgtgtgtgtgtgtgtgtgtgtgtgtgtgtgttcaaaaatgtctatgaaaatgaaaacccacacttttctgtacagataacattatttgatgtgacttttatattttactacacagaaacaaactgcagccctcagaggccctgcttccttgtcatgttttgcctgagcatgtgcaaagtctttcctttgcttaaagctgaaaaactacctttatgcattgttagctgacaagaaagatcaagcacaattagatgttgtaacttttcactgtacaagcattgcaatgattgtgagcttcagtgaatttatctttgtgaaaggtaaaaattggctggaaagaatcaggagtagccataaattaaatcatgcaaaggaggatccatgcatcctaacaagttttctgctgcatctgcttccttcctgggctccacaatgttaagcaatattttagaaaagggtacaattggaagcttttaagcctgagtggtgagattttataactcacaacttagatctcttttaatgtgtaagccatattctatatgcatatttattatgcatcattgtaatttaagatatatttggatgtaggctgtataaatgcttttaattgttctgtgaatagatccttagctttagtttcacctgaatcttgtgcaaaacacagctaaataattgaattgtattatagacattatgaggtaattgatcttttaaatgtaaggagtaagattgatctataataatgtgctggggaaaacatttatagatatgtacatcatggttactttttgtcctttcaaatggactttttatttctatttatggagagactgtaactactgcttttaatgtctttttaaagcaagctatttaccagcttgaaaatatcatgcatttaaaatagaatctatctggggagtctaattactattgttcctatttgagccagttgtctttcagtaaagctatagaatctctcaaagaagtaaatagaaatactacttcttaaatgtcataggaagcatatccactttgtttctattagtactttaagatctataagaccttattactaaaaagtagaggaatataaagaattcatcaatttctgtatatgggctttaacctaattttccaggttatgcgacttataaagcactgtgaccaaacttccagagacagtaaaaaaaaaaaaaagaaaaaaaagttttactccttcagaagtattgtcatgctactgctgtacttattttcctaatctctctctatctgctatactccctccttttctttctttttcttttaagcttttatatttattccttcctttgttttcctctctgtaagacagctactactgagcactaattagtagaaagtcagagtggaggttatctgtgcatgtctttctgcaaacattactgttgaggccatctgaagagagggattgataggttaggctgttgcaccgtgaatgtcctgctttgcatttttaacctcagctccccaacatatatatcttgcagtttatatgccttttcatttaaccgaaacctcttttatttaatttttaacataacaacctacaattcttgtgtttttattatgctgtatttttctgtgtttcttattacatgtgattgctaaataaatcatatttgagggaaaacattgtgaaacatttggtgttttatgcaattcaatttagtgaggcattgaaaagttggagaaattgggggaaacccaaaggagaccaacttaaaaattgatatgagtttggtaagaaagtgctttttgttccattaaataaatactgattgaattacttattattatacctattattcataagctcctggctggaagcatggtgcatatatgcatatggcaatatttcctctagaaatttcaagtcttataaaggagataatctacacagactgtaatttatacctaataactagaatgccacataaaaaagtaaccagttgcaaataaaatgcacctatgtatatttgaggaggtaaaaaactgcttctgtcttcagagctttcaggactaagtggtgcatcagttggcatttagtaaataaaaacaagtttataaacatt

SEQ ID NO: 2 - protein, 545 aa, Homo sapiens
MGSSATEIEELENTTFKYLTGEQTEKMWQRLKGILRCLVKQLERGDVNVVDLKKNIEYAASVLEAVYIDETRRLLDTEDELSDIQTDSVPSEVRDWLASTFTRKMGMTKKKPEEKPKFRSIVHAVQAGIFVERMYRKTYHMVGLAYPAAVIVTLKDVDKWSFDVFALNEASGEHSLKFMIYELFTRYDLINRFKIPVSCLITFAEALEVGYSKYKNPYHNLIHAADVTQTVHYIMLHTGIMHWLTELEILAMVFAAAIHDYEHTGTTNNFHIQTRSDVAILYNDRSVLENHHVSAAYRLMQEEEMNILINLSKDDWRDLRNLVIEMVLSTDMSGHFQQIKNIRNSLQQPEGIDRAKTMSLILHAADISHPAKSWKLHYRWTMALMEEFFLQGDKEAELGLPFSPLCDRKSTMVAQSQIGFIDFIVEPTFSLLTDSTEKIVIPLIEEASKAETSSYVASSSTTIVGLHIADALRRSNTKGSMSDGSYSPDYSLAAVDLKSFKNNLVDIIQQNKERWKELAAQGESDLHKNSEDLVNAEEKHDETHS

SEQ ID NO: 3 - DNA, 3193 bp, Homo sapiens
  source 1..3193: mol_type = other DNA
agcgcgcggcggcggcggcggtagcggcagcagcagcggcggtgcggagagcttggactgggagcccaaagctcggctgggcagcgggagaggaggagccgcaggagctgcagctctgccagcttgggccgagcctagagacaccggcctggctggtccacgccagccgcagaccgtggctgagcatggagctgtccccccgcagtcctccggagatgctggaggagtcggattgcccgtcacccctggagctgaagtcagcccccagcaagaagatgtggattaagcttcggtctctgctgcgctacatggtgaagcagttggagaatggggagataaacattgaggagctgaagaaaaatctggagtacacagcttctctgctggaagccgtctacatagatgagacacggcaaatcttggacacggaggacgagctgcaggagctgcggtcagatgccgtgccttcggaggtgcgggactggctggcctccaccttcacccagcaggcccgggccaaaggccgccgagcagaggagaagcccaagttccgaagcattgtgcacgctgtgcaggctgggatcttcgtggaacggatgttccggagaacatacacctctgtgggccccacttactctactgcggttctcaactgtctcaagaacctggatctctggtgctttgatgtcttttccttgaaccaggcagcagatgaccatgccctgaggaccattgtttttgagttgctgactcggcataacctcatcagccgcttcaagattcccactgtgtttttgatgagtttcctggatgccttggagacaggctatgggaagtacaagaatccttaccacaaccagatccacgcagccgatgttacccagacagtccattgcttcttgctccgcacagggatggtgcactgcctgtcggagattgagctcctggccatcatctttgctgcagctatccatgattatgagcacacgggcactaccaacagcttccacatccagaccaagtcagaatgtgccatcgtgtacaatgatcgttcagtgctggagaatcaccacatcagctctgttttccgattgatgcaggatgatgagatgaacattttcatcaacctcaccaaggatgagtttgtagaactccgagccctggtcattgagatggtgttggccacagacatgtcctgccatttccagcaagtgaagaccatgaagacagccttgcaacagctggagaggattgacaagcccaaggccctgtctctactgctccatgctgctgacatcagccacccaaccaagcagtggttggtccacagccgttggaccaaggccctcatggaggaattcttccgtcagggtgacaaggaggcagagttgggcctgcccttttctccactctgtgaccgcacttccactctagtggcacagtctcagatagggttcatcgacttcattgtggagcccacattctctgtgctgactgacgtggcagagaagagtgttcagcccctggcggatgaggactccaagtctaaaaaccagcccagctttcagtggcgccagccctctctggatgtggaagtgggagaccccaaccctgatgtggtcagctttcgttccacctgggtcaagcgcattcaggagaataagcagaaatggaaggaacgggcagcaagtggcatcaccaaccagatgtccattgacgagctgtccccctgtgaagaagaggcccccccatcccctgccgaagatgaacacaaccagaatgggaatctggattagccctggggctggcccaggtcttcattgagtccaaagtgtttgatgtcatcagcaccatccatcaggactggctcccccatctgctccaagggagcgtggtcgtggaagaaacaacccacctgaaggccaaatgccagagatttggggttggggaaagggcccctccccacctgacacccactggggtgcactttaatgttccggcagcaagactggggaacttcaggctcccagtggtcactgtgcccatccctcagcctctggattctcttcatggccaggtggctgccagggagcggggagcttcctggaggcttcccagggccttggggaagggtcagagatgccagccccctgggacctcccccatcctttttgcctccaagtttctaagcaatacattttgggggttccctcagccccccaccccagatcttagctggcaggtctgggtgccccttttcctcccctgggaagggctggaataggatagaaagctgggggttttcagagccctatgtgtggggaggggagtggattccttcagggcatggtacctttctaggacctgggaatggggtggagaggacatcctcttcaccccagaattgcgctgcttcagccccatctccagcctgatcctctgaatcttccttccctccctttctgatacagtgactggggcaaaaggagccattgtgaccaggggctgcgggaggcctttcctgggaccttccttgggactggtctgggcccctggggcttgtcgcctgccctgagtccggagccctttgcctccttcctctcccctggggctgggaggctccatccgaccaatgtctgtaaagtgctttgaggatctccccagcaaagcaccttcagaatgtatcgacaccagctgggttagggtcaagggtgcctggggagggtgagtaatcctgcattgctaaaagagagggtctgtcccctcctctccacgtcccagaactggcccagctgcaggcactaagaagctcctcccctgagacaagtgaggggtagtcggtgaaaggcagatggacaaggggctcagggctgctgccttcctgtcctctggagagaacccagccaggcgcggtgccccttcctctcctcaggctcctccttgcccccaccttgccccaggaaaggccaaagtccaggtgactgccctccttctttcttgtaaataccaaccatgcatttgtacagtgggccctgttcatgcgaaatccacatccatggtctcctagacctgctaccctggtacttccaccctaccccaccccgagaagggcagagacgcatgtgactcacccctgcccttggtttcccagacccctgctatagccagagaacaataaagaagggagaccagg

SEQ ID NO: 4 - protein, 536 aa, Homo sapiens
MELSPRSPPEMLEESDCPSPLELKSAPSKKMWIKLRSLLRYMVKQLENGEINIEELKKNLEYTASLLEAVYIDETRQILDTEDELQELRSDAVPSEVRDWLASTFTQQARAKGRRAEEKPKFRSIVHAVQAGIFVERMFRRTYTSVGPTYSTAVLNCLKNLDLWCFDVFSLNQAADDHALRTIVFELLTRHNLISRFKIPTVFLMSFLDALETGYGKYKNPYHNQIHAADVTQTVHCFLLRTGMVHCLSEIELLAIIFAAAIHDYEHTGTTNSFHIQTKSECAIVYNDRSVLENHHISSVFRLMQDDEMNIFINLTKDEFVELRALVIEMVLATDMSCHFQQVKTMKTALQQLERIDKPKALSLLLHAADISHPTKQWLVHSRWTKALMEEFFRQGDKEAELGLPFSPLCDRTSTLVAQSQIGFIDFIVEPTFSVLTDVAEKSVQPLADEDSKSKNQPSFQWRQPSLDVEVGDPNPDVVSFRSTWVKRIQENKQKWKERAASGITNQMSIDELSPCEEEAPPSPAEDEHNQNGNLD

SEQ ID NO: 5 - DNA, 9123 bp, Homo sapiens
  source 1..9123: mol_type = other DNA
cggctcccgctttgctcagccgccgcttttctctcccttctcactttctctcctccccacccagccctccttttcacctccaaaccctttagctgcgcgctgatcgcttctgtggctttgtttgggggtagggggagaatacgaatagacccgaggtgctttctcttggagctggagtccaatcccaatccctatctctatccctatccctgtgcttatccctgggcattagcccgggaccatggctggttcccgcagctgcctccggagcgcacctggggccatggtttgccgcgatcggagtccgctctaagtcggagtctgggggcgcagaagggggagcgcgccgagaaagtgccgggcaaacgcgcgccgcgcctggctgggcatcgcgagctgggcgaggagacggggaggggacagcccaaactatctcagcttcaccgccagtggtcacctacctgcagctatggagtcgccaaccaaggagattgaagaatttgagagcaactctctgaaatacctgcaaccggaacagatcgagaaaatctggcttcggctccgcgggctgaggaaatataagaaaacgtcccagagattacggtctttggtcaaacaattagagagaggggaagcttcagtggtagatcttaagaagaatttggaatatgcagccacagtgcttgaatctgtgtatattgatgaaacaaggagactcctggatacagaggatgagctcagtgacattcagtcagatgctgtgccttctgaggtccgagactggctggcctccaccttcacgcggcagatggggatgatgctcaggaggagcgacgagaagccccggttcaagagcatcgttcacgcagtgcaggctgggatatttgtggagagaatgtatagacggacatcaaacatggttggactgagctatccaccagctgttattgaggcattaaaggatgtggacaagtggtcctttgacgtcttttccctcaatgaggccagtggggatcatgcactgaaatttattttctatgaactactcacacgttatgatctgatcagccgtttcaagatccccatttctgcacttgtctcatttgtggaggccctggaagtgggatacagcaagcacaaaaatccttaccataacttaatgcacgctgccgatgttacacagacagtgcattacctcctctataagacaggagtggcgaactggctgacggagctggagatctttgctataatcttctcagctgccatccatgactacgagcataccggaaccaccaacaatttccacattcagactcggtctgatccagctattctgtataatgacagatctgtactggagaatcaccatttaagtgcagcttatcgccttctgcaagatgacgaggaaatgaatattttgattaacctctcaaaggatgactggagggagtttcgaaccttggtaattgaaatggtgatggccacagatatgtcttgtcacttccaacaaatcaaagcaatgaagactgctctgcagcagccagaagccattgaaaagccaaaagccttatcccttatgctgcatacagcagatattagccatccagcaaaagcatgggacctccatcatcgctggacaatgtcactcctggaggagttcttcagacagggtgacagagaagcagagctggggctgcctttttctcctctgtgtgaccgaaagtccactatggttgctcagtcacaagtaggtttcattgatttcatcgtggaacccaccttcactgtgcttacggacatgaccgagaagattgtgagtccattaatcgatgaaacctctcaaactggtgggacaggacagaggcgttcgagtttgaatagcatcagctcgtcagatgccaagcgatcaggtgtcaagacctctggttcagagggaagtgccccgatcaacaattctgtcatctccgttgactataagagctttaaagctacttggacggaagtggtgcacatcaatcgggagagatggagggccaaggtacccaaagaggagaaggccaagaaggaagcagaggaaaaggctcgcctggccgcagaggagcagcaaaaggaaatggaagccaaaagccaggctgaagaaggcgcatctggcaaagctgagaaaaagacgtctggagaaactaagaatcaagtcaatggaacacgggcaaacaaaagtgacaaccctcgtgggaaaaactccaaagccgagaagtcatcaggagaacagcaacagaatggtgacttcaaagatggtaaaaataagacagacaagaaggatcactctaacatcggaaatgattcaaagaaaacagatgattcacaagagtaaaaaagacctcatagacaataaaagaggctgccagtgtcttgcatcattctagctgagcttcttcattctccttcttctccttcttccacaaagacccatatctggagaaggtgtacaactttcaaacacaagccccccaccccctgacccttggccttccctcacaccatctccttccaggggatgaatctttgggggttggtttgaggtcttagaactctgggggatattcccctgagcaaaacaaacaacgtgagatttttactcaaacagaaacaaaacatgaaggggcatcctcaaaatcctttgctaatgacctggctttcaaggcatctgtctggcctgatgagaatggacatcctggatatgctgggagaggcctgaaaaaagccacacacacagtaattgccattttatgactgtcaatgccgttactttaaatgttgtcatttttgcactggctactgatgatacagccatgctgacattcatcaccgcaaagatgatgattccagtctctggttcctttcctgagtcaggaacatttgttttctccaatttcctttcagacttaaaattgttcttatgctttttttcccacttctgtaatacagaattctgtttgttttctaaaaaagattattctataggaatctttatttgatggctaatttattttctctgtgcattcattagtataaacctgaatgttcagctggtgactgtactgttgagtgggaacccattgtttccactggtagcattgataactaagtggttactgaaatttttaccactggctggacatcttcttttggatatctgtggttttatttcatcactcttctttttattcagtaaagtgctaagggaattagtatcagggagatatggcagataattctttgcattttagtgagtttttaaaaatacaagatagaagtggattaatagcacgaataaaaaataagaatagtagatgtagcatggaaagagaataacattgcagcccccttgagaccaaattacaggtgggatctaagggagtgcaagtaaagtgggattttatgagtctaaatgatgtgatttagataaaagtgattcttaaaatgtggttattggtcacacaggaatctctgagtccttcccaagagtgaagcacatgaatatgctgatgatgaagtggggattagtaatagaaagagagctaggcaataggtttaagtgtattccccactacagatttaatttctacatgaaaaagcacgagaacagatatttaaacgtccttttattactaaggtgaaatattggcattttttcaggcagaaagaaagagactgtatgtggtcttcctggacctttgccttgccaaaatgttccccaacagaaagatctgaagaactttgtagtatcgaatgcacaacagcatgctgatatttgaacagatttcttctgtcagctttacattttgccttggagaaacacttagatttttctgttgtgctccctgtgttcataacaatgacctcaccacataatgtggccagaaattcaaatgacttcaggggcctagcaggtcaagtaaatgaataaagcaagccatgtaatatcacagtcattgtggtaaatggcaattcatagtgggcctttgtatcagcaagacaggaaggagcaatggggactgtgagaaattggagagggtgggtgctgtcaaaacagggtagttggtaggcagcaactgaatttgagctgtgtggggatgggggtcctagatacctaggatttgatataagctctctccaaatttttacatattgacaactaactcaaaaacttacaaacactgtgctaatcaaatgaaacatgcctgtgagctgcattcaatccatggggcattggtttgcaagctatgttcttagaggtggtatgattttgtattgaaattaaatataaccaagagtatgtcaatttttgaccttggaacctggaccttttacctcatttatattctgtatttttgtatgtggggctttttggccagtcaaaatagaaagtctacagcttccattttataatctaacaagcaacaagaaacaacatttgaaaaagaaacaggaatatagccattttttctagcaccaataaaaatggaaatgtttttcatttgctttaagtcattaatcagctgaaaaagaatagaaagagaatttcattccataaagaacttcacctaaaactctcagtgaagcaaaacaaaactccatgtaactcactcttagctttaaatctttaaaaagtgtttcgaagggatattgagtaaaaatgcagttatctattaaaaatacaaaatgctatattatatgatgctatgaattgatactggagctgataaaacattaaagtaattattccaaatcagtgctgactgcaaaagcaatatttccaaagctctagcttattttctgcggtcttttaattcccttgaaatagctttcttcaagttgagcagcaatttgggacaaacattattctattgcacagattatggcatcttactctggtttacacacacagagcaagggcttacacacctgaattaagaattaactagcatgtggggacagcaatagggatagtcctaccacagacgaaaccatgcgctctacacgtccctggataaaatgtgacaagttagcccttgaatttgggtccccatgtcaccaaatagctctatatttaagttgtgttaatgtggtacgtttcagtggcataatgacccattcttatcgaggcctttgttccatattttatttgtgccaatctttcttaggttatgagccctaatagtttatggcagcagacaagagactcatttctaacccattaaattcaaatggactttcttccactgtccatttcatttttggagctgttataaactaccgaaaacatttgacaggatcccattgtggatctgatacacttaaacagtaaaatgatatctaaacatctgaaagccaaagaataacctagtgcacgtgttcattcatttgtagaatttaagccattgtattatattttccacttggaaccatgcctttagatacaaaagtgtaaagtaaaaagcaacattatcatgggatgtgagacggtaatccaaaagttgaagaccaatttttgttatccatattttggaagtatggatactgtttattttaatatcacttctctcatgggtcacttttccttagataggtaggtaggtagatagatagatagatagatgatagatagatagatagatagatagatagatagatagatagatagatagatagatagatagataatataatatattttcttctttcttaacctatgagcagagactttgatgatggaaattactttgtaacattccccatggagcctaggaaaaacaatagaaaaaaagcatgaaatctttttctcatagtgaaatagagaagattctaagattggaaatctgtgtatgtggtgttctatcccaaataaagagaatttagggaattcaggcaacaatttttttcctaattggaaactttgttctgatcctgagatgcccacacaccccacaggagacgcagtgctggcccaccacagtgtttggaacacggtcagcattcaggaaacacattcaaaatcgtctaactgaattccactatccacttgtgaatgcaaacaaaattcaaatttccctgaaaatttattcaacttctatatgccaagcacactgctaaaggcttatcttctaagtatatgcaggcataccctactcacacaaatagcttattaccagagataggaaattgcaggtaatttgggagaaattgtcatagccaaatttatggaaaaaataaaataaaaacttctctatggcctcttgatttaagaaaaaaacagaacaatacaaaaaaaaaaaagcactaaaacaggatttatctgagaatgtctttccaaaagggaagatgacaccaatctatataaaacgtcagtggatttactgagaatccgagtggaaacttttaaaaccttaaacagactctcctacagcaaatagattctctatgtgcagcatgaggaatcactgcatagttctgctccaccaataatatgattggtacagcaccaaaccatggcaaagttagatgttaaagaacataatgttgcaataatgatgttatattggatcttatgcatgaacaaatggaaagtaataatttatcaactgtgatccatgattaaaggcctcattatcactaagaaaatgaacttaatgaaaaaaattataatgagcaatgacaatattcctataaaacctccctctgggtatcaagagacatattacctgccaaggccagattttactttttaaggtttcctctctctcaccaaagacactagtgggcacagaggtgacactagagttagaatgttaccagagtcatttgcattagacagtttatctgatcatgaacatgttcccagggagattagaaaaatgggaagcaggcctctaaagatcctccttggacatttgtaaaaaggctggctgcttctccaggaatgtctgaattaagcaagaattgtgccactgaaatagcttcttgtttttatattaaacaaggaacgattgtgcagtggatgacctggactgaaagatgtatgatggtcaagtttaaacatattaattcctgattgttttcttaaatacccaccctagtcattttttggaaaatattgccagacatatttgacatgaattcatgtttattctggcttctgttcccaagcagaagtggattaaccctggcaatggctggcttcactaactgtacttgcacccagcctgggctgccatctgctcagccaggagaagcagggagtggggtgtgggccctttaagttcgctcagggcacactcattcagtctcccctgaggagaccttgtccccctttgtggggtgaatgctggctgttgcaggccagaggcagtgccaactggagactcatcctctcagctttggtcagcttcagccacgtattcttcatgagtgctggcttctgaacctgcaggatcatttctcagtcagtttatggtgcagggtaattcatttaaaataaagcccattaaaaccccatggctatagaatgggttttaaatagattgtcctggagacacatcattgtatagtctttgcttccctctcatgacctatcttggagtagaatttgtgtactactgtccttgtctttgagtgggtatatgtgtgatggtacagaaatacagtcacatattatattaatatatatagatggataggaaaaacctacagccataggtattgtccaataactgattctagaggtagaactatagagtatacatttccttttttcttgctttgatgatatttttatacaattttatatgctataaaattttcaaaaatatatttgctattttcatttgtagagcttggttaggtttttatcagctcttgtgcccactgtacaaccagattcccctcatctaatttaaatgtcttccctttttcaaactctcctttatgttttcctttttttttcctcccatttttctacccttcacaaattccttcttttgcttctgtccaggtaacccattctgcttgcagtatcattttagcacgtacaaacacaaaataatgggaaaaataaaagcaccttgttccatgcaattcgtatgggaaagttttgggtgtcaaaggtcgctggggatagatggggaggcagaaatagcttgggaaaaggaagcaggaaaaaaggaaatctttatgggaaatcaattacccaaagcaaggtgagtcacctagaggtgaatatgatgttgttattgtcctcccttagtgtacagcacagtttttgctctcacagggtttttctctttaggatgcgtagcaccctatgcattaaatacatagcatcctaaagacaccctactcaccatgagtctgtaggctctttcctgatgagggcactggccatatatgaatggaaaactcaactcatctcctcagctttagatgttgctgctgttcagctggatttgtgagaaatatctggattactatcaagaacatttagcaagactcaaaagagagaggcaagcagaaccaaaacccaaacctcaaccaatgactagctgaataaacaattctttggaggaataaggaaggtatttctggatgtattctgagaatgctcttccaaaagggaagatggtaataatggacttgttttgatttcatggttgtgatagaatgtacttccatgatgtgaaatacacttctggcagataaaatgcaggttgtaatttgcatttgtacatcacagggtaaaagaatggccatccattctgaggaagagtgttctgttctctaagatgctgcttaaccaatgttatccaaatgccatagcatcatatctccaaatacaagattaaatcataaggattcatgtaaaacagagtatactgagctgttctcagaaaaattaatgatgtgtttattgtaaatctttattgcacagatgagcctgacagtccttcaatgtataattttcccccagcatctagtaatgcataagtacttgtatgttcttctgattaccaaataaaaacaatgagttaacctcttaattggaattggaaaaaaaaaaaaaaaaaa

SEQ ID NO: 6 - protein, 634 aa, Homo sapiens
MESPTKEIEEFESNSLKYLQPEQIEKIWLRLRGLRKYKKTSQRLRSLVKQLERGEASVVDLKKNLEYAATVLESVYIDETRRLLDTEDELSDIQSDAVPSEVRDWLASTFTRQMGMMLRRSDEKPRFKSIVHAVQAGIFVERMYRRTSNMVGLSYPPAVIEALKDVDKWSFDVFSLNEASGDHALKFIFYELLTRYDLISRFKIPISALVSFVEALEVGYSKHKNPYHNLMHAADVTQTVHYLLYKTGVANWLTELEIFAIIFSAAIHDYEHTGTTNNFHIQTRSDPAILYNDRSVLENHHLSAAYRLLQDDEEMNILINLSKDDWREFRTLVIEMVMATDMSCHFQQIKAMKTALQQPEAIEKPKALSLMLHTADISHPAKAWDLHHRWTMSLLEEFFRQGDREAELGLPFSPLCDRKSTMVAQSQVGFIDFIVEPTFTVLTDMTEKIVSPLIDETSQTGGTGQRRSSLNSISSSDAKRSGVKTSGSEGSAPINNSVISVDYKSFKATWTEVVHINRERWRAKVPKEEKAKKEAEEKARLAAEEQQKEMEAKSQAEEGASGKAEKKTSGETKNQVNGTRANKSDNPRGKNSKAEKSSGEQQQNGDFKDGKNKTDKKDHSNIGNDSKKTDDSQE

SEQ ID NO: 7 - DNA, 4177 bp, Homo sapiens
  source 1..4177: mol_type = other DNA
gaagctgtcgcggacgcgctgaccgagcgcagcggccgggccggcgggcgggcgggcggctgcgagcatggtcctggtgctgcaccacatcctcatcgctgttgtccaattcctcaggcggggccagcaggtcttcctcaagccggacgagccgccgccgccgccgcagccatgcgccgacagcctgcagccagcctggacccccttgcaaaggagccaggacccccagggagtagagacgaccgactggaggacgccttgctgagtctgggctctgtcatcgacatttcaggcctgcaacgtgctgtcaaggaggccctgtcagctgtgctcccccgagtggaaactgtctacacctacctactggatggtgagtcccagctggtgtgtgaggaccccccacatgagctgccccaggaggggaaagtccgggaggctatcatctcccagaagcggctgggctgcaatgggctgggcttctcagacctgccagggaagcccttggccaggctggtggctccactggctcctgatacccaagtgctggtcatgccgctagcggacaaggaggctggggccgtggcagctgtcatcttggtgcactgtggccagctgagtgataatgaggaatggagcctgcaggcggtggagaagcataccctggtcgccctgcggagggtgcaggtcctgcagcagcgcgggcccagggaggctccccgagccgtccagaaccccccggaggggacggcggaagaccagaagggcggggcggcgtacaccgaccgcgaccgcaagatcctccaactgtgcggggaactctacgacctggatgcctcttccctgcagctcaaagtgctccaatacctgcagcaggagacccgggcatcccgctgctgcctcctgctggtgtcggaggacaatctccagctttcttgcaaggtcatcggagacaaagtgctcggggaagaggtcagctttcccttgacaggatgcctgggccaggtggtggaagacaagaagtccatccagctgaaggacctcacctccgaggatgtacaacagctgcagagcatgttgggctgtgagctgcaggccatgctctgtgtccctgtcatcagccgggccactgaccaggtggtggccttggcctgcgccttcaacaagctagaaggagacttgttcaccgacgaggacgagcatgtgatccagcactgcttccactacaccagcaccgtgctcaccagcaccctggccttccagaaggaacagaaactcaagtgtgagtgccaggctcttctccaagtggcaaagaacctcttcacccacctggatgacgtctctgtcctgctccaggagatcatcacggaggccagaaacctcagcaacgcagagatctgctctgtgttcctgctggatcagaatgagctggtggccaaggtgttcgacgggggcgtggtggatgatgagagctatgagatccgcatcccggccgatcagggcatcgcgggacacgtggcgaccacgggccagatcctgaacatccctgacgcatatgcccatccgcttttctaccgcggcgtggacgacagcaccggcttccgcacgcgcaacatcctctgcttccccatcaagaacgagaaccaggaggtcatcggtgtggccgagctggtgaacaagatcaatgggccatggttcagcaagttcgacgaggacctggcgacggccttctccatctactgcggcatcagcatcgcccattctctcctatacaaaaaagtgaatgaggctcagtatcgcagccacctggccaatgagatgatgatgtaccacatgaaggtctccgatgatgagtataccaaacttctccatgatgggatccagcctgtggctgccattgactccaattttgcaagtttcacctatacccctcgttccctgcccgaggatgacacgtccatggccatcctgagcatgctgcaggacatgaatttcatcaacaactacaaaattgactgcccgaccctggcccggttctgtttgatggtgaagaagggctaccgggatcccccctaccacaactggatgcacgccttttctgtctcccacttctgctacctgctctacaagaacctggagctcaccaactacctcgaggacatcgagatctttgccttgtttatttcctgcatgtgtcatgacctggaccacagaggcacaaacaactctttccaggtggcctcgaaatctgtgctggctgcgctctacagctctgagggctccgtcatggagaggcaccactttgctcaggccatcgccatcctcaacacccacggctgcaacatctttgatcatttctcccggaaggactatcagcgcatgctggatctgatgcgggacatcatcttggccacagacctggcccaccatctccgcatcttcaaggacctccagaagatggctgaggtgggctacgaccgaaacaacaagcagcaccacagacttctcctctgcctcctcatgacctcctgtgacctctctgaccagaccaagggctggaagactacgagaaagatcgcggagctgatctacaaagaattcttctcccagggagacctggagaaggccatgggcaacaggccgatggagatgatggaccgggagaaggcctatatccctgagctgcaaatcagcttcatggagcacattgcaatgcccatctacaagctgttgcaggacctgttccccaaagcggcagagctgtacgagcgcgtggcctccaaccgtgagcactggaccaaggtgtcccacaagttcaccatccgcggcctcccaagtaacaactcgctggacttcctggatgaggagtacgaggtgcctgatctggatggcactagggcccccatcaatggctgctgcagccttgatgctgagtgatcccctccagggacacttccctgcccaggccacctcccacagccctccactggtctggccagatgcactgggaacagagccacgggtcctgggtcctagaccaggacttcctgtgtgaccctggacaagtactaccttcctgggcctcagctttctcgtctgtataatggaagcaagacttccaacctcacggagactttgtaatttgttttctgagagcacaggggtgaccaatgagcagtgggccctactctgcacctctgaccacaccttggcaagtctttcccaagccattctttgtctgagcagcttgatggtttctccttgccccatttctgccccaccagatctttgctcctttccctttgaggactcccaccctttggggtctccaggatcctcatggaaggggaaggtgagacatctgagtgagcagagtgtggcatcttggaaacagtccttagttctgtgggaggactagaaacagccgcggggcgaaggccccctgaggaccactactatactgatggtgggattgggacctgggggatacaggggccccaggaagaagctgccagaggggcagctcagtgctctgcagagaggggccctggggagaagcaggatgggattgatgggcaggagggatccccgcactgggagacaggcccaggtatgaatgagccagccatgcttcctcctgcctgtgtgacgctgggcgagtctcttcccctgtctgggccaaacagggagcgggtaagacaatccatgctctaagatccattttagatcaatgtctaaaatagctctatcgctctgcggagtcccagcagaggctatggaatgtttctgcaaccctaaggcacagagagcccaaccctgagtgtctcagaggccccctgagtgttccccttggcctgagccccttacccattcctgcagccagtgagagacctggcctcagccctggcagggctctctcttcaaggccatatccacctgtgccctggggcttgggagaccccatagggccgggactcttgggtcagcccggccactggcttctctctttttctctgtttcattctgtgtgcgttgtggggtgggggagggggtccacctgccttacctttctgagttgcctttagagagatgcgtttttctaggactctgtgcaactgtcgtatatggtcccgtgggctgaccgctttgtacatgagaataaatctatttctttctacca

SEQ ID NO: 8 - protein, 920 aa, Homo sapiens
MRRQPAASLDPLAKEPGPPGSRDDRLEDALLSLGSVIDISGLQRAVKEALSAVLPRVETVYTYLLDGESQLVCEDPPHELPQEGKVREAIISQKRLGCNGLGFSDLPGKPLARLVAPLAPDTQVLVMPLADKEAGAVAAVILVHCGQLSDNEEWSLQAVEKHTLVALRRVQVLQQRGPREAPRAVQNPPEGTAEDQKGGAAYTDRDRKILQLCGELYDLDASSLQLKVLQYLQQETRASRCCLLLVSEDNLQLSCKVIGDKVLGEEVSFPLTGCLGQVVEDKKSIQLKDLTSEDVQQLQSMLGCELQAMLCVPVISRATDQVVALACAFNKLEGDLFTDEDEHVIQHCFHYTSTVLTSTLAFQKEQKLKCECQALLQVAKNLFTHLDDVSVLLQEIITEARNLSNAEICSVFLLDQNELVAKVFDGGVVDDESYEIRIPADQGIAGHVATTGQILNIPDAYAHPLFYRGVDDSTGFRTRNILCFPIKNENQEVIGVAELVNKINGPWFSKFDEDLATAFSIYCGISIAHSLLYKKVNEAQYRSHLANEMMMYHMKVSDDEYTKLLHDGIQPVAAIDSNFASFTYTPRSLPEDDTSMAILSMLQDMNFINNYKIDCPTLARFCLMVKKGYRDPPYHNWMHAFSVSHFCYLLYKNLELTNYLEDIEIFALFISCMCHDLDHRGTNNSFQVASKSVLAALYSSEGSVMERHHFAQAIAILNTHGCNIFDHFSRKDYQRMLDLMRDIILATDLAHHLRIFKDLQKMAEVGYDRNNKQHHRLLLCLLMTSCDLSDQTKGWKTTRKIAELIYKEFFSQGDLEKAMGNRPMEMMDREKAYIPELQISFMEHIAMPIYKLLQDLFPKAAELYERVASNREHWTKVSHKFTIRGLPSNNSLDFLDEEYEVPDLDGTRAPINGCCSLDAE

SEQ ID NO: 9 - DNA, 4115 bp, Homo sapiens
  source 1..4115: mol_type = other DNA
gaagctgtcgcggacgcgctgaccgagcgcagcggccgggccggcgggcgggcgggcggctgcgagcatggtcctggtgctgcaccacatcctcatcgctgttgtccaattcctcaggcggggccagcaggtcttcctcaagccggacgagccgccgccgccgccgcagccatgcgccgacagcctgcaggacgccttgctgagtctgggctctgtcatcgacatttcaggcctgcaacgtgctgtcaaggaggccctgtcagctgtgctcccccgagtggaaactgtctacacctacctactggatggtgagtcccagctggtgtgtgaggaccccccacatgagctgccccaggaggggaaagtccgggaggctatcatctcccagaagcggctgggctgcaatgggctgggcttctcagacctgccagggaagcccttggccaggctggtggctccactggctcctgatacccaagtgctggtcatgccgctagcggacaaggaggctggggccgtggcagctgtcatcttggtgcactgtggccagctgagtgataatgaggaatggagcctgcaggcggtggagaagcataccctggtcgccctgcggagggtgcaggtcctgcagcagcgcgggcccagggaggctccccgagccgtccagaaccccccggaggggacggcggaagaccagaagggcggggcggcgtacaccgaccgcgaccgcaagatcctccaactgtgcggggaactctacgacctggatgcctcttccctgcagctcaaagtgctccaatacctgcagcaggagacccgggcatcccgctgctgcctcctgctggtgtcggaggacaatctccagctttcttgcaaggtcatcggagacaaagtgctcggggaagaggtcagctttcccttgacaggatgcctgggccaggtggtggaagacaagaagtccatccagctgaaggacctcacctccgaggatgtacaacagctgcagagcatgttgggctgtgagctgcaggccatgctctgtgtccctgtcatcagccgggccactgaccaggtggtggccttggcctgcgccttcaacaagctagaaggagacttgttcaccgacgaggacgagcatgtgatccagcactgcttccactacaccagcaccgtgctcaccagcaccctggccttccagaaggaacagaaactcaagtgtgagtgccaggctcttctccaagtggcaaagaacctcttcacccacctggatgacgtctctgtcctgctccaggagatcatcacggaggccagaaacctcagcaacgcagagatctgctctgtgttcctgctggatcagaatgagctggtggccaaggtgttcgacgggggcgtggtggatgatgagagctatgagatccgcatcccggccgatcagggcatcgcgggacacgtggcgaccacgggccagatcctgaacatccctgacgcatatgcccatccgcttttctaccgcggcgtggacgacagcaccggcttccgcacgcgcaacatcctctgcttccccatcaagaacgagaaccaggaggtcatcggtgtggccgagctggtgaacaagatcaatgggccatggttcagcaagttcgacgaggacctggcgacggccttctccatctactgcggcatcagcatcgcccattctctcctatacaaaaaagtgaatgaggctcagtatcgcagccacctggccaatgagatgatgatgtaccacatgaaggtctccgatgatgagtataccaaacttctccatgatgggatccagcctgtggctgccattgactccaattttgcaagtttcacctatacccctcgttccctgcccgaggatgacacgtccatggccatcctgagcatgctgcaggacatgaatttcatcaacaactacaaaattgactgcccgaccctggcccggttctgtttgatggtgaagaagggctaccgggatcccccctaccacaactggatgcacgccttttctgtctcccacttctgctacctgctctacaagaacctggagctcaccaactacctcgaggacatcgagatctttgccttgtttatttcctgcatgtgtcatgacctggaccacagaggcacaaacaactctttccaggtggcctcgaaatctgtgctggctgcgctctacagctctgagggctccgtcatggagaggcaccactttgctcaggccatcgccatcctcaacacccacggctgcaacatctttgatcatttctcccggaaggactatcagcgcatgctggatctgatgcgggacatcatcttggccacagacctggcccaccatctccgcatcttcaaggacctccagaagatggctgaggtgggctacgaccgaaacaacaagcagcaccacagacttctcctctgcctcctcatgacctcctgtgacctctctgaccagaccaagggctggaagactacgagaaagatcgcggagctgatctacaaagaattcttctcccagggagacctggagaaggccatgggcaacaggccgatggagatgatggaccgggagaaggcctatatccctgagctgcaaatcagcttcatggagcacattgcaatgcccatctacaagctgttgcaggacctgttccccaaagcggcagagctgtacgagcgcgtggcctccaaccgtgagcactggaccaaggtgtcccacaagttcaccatccgcggcctcccaagtaacaactcgctggacttcctggatgaggagtacgaggtgcctgatctggatggcactagggcccccatcaatggctgctgcagccttgatgctgagtgatcccctccagggacacttccctgcccaggccacctcccacagccctccactggtctggccagatgcactgggaacagagccacgggtcctgggtcctagaccaggacttcctgtgtgaccctggacaagtactaccttcctgggcctcagctttctcgtctgtataatggaagcaagacttccaacctcacggagactttgtaatttgttttctgagagcacaggggtgaccaatgagcagtgggccctactctgcacctctgaccacaccttggcaagtctttcccaagccattctttgtctgagcagcttgatggtttctccttgccccatttctgccccaccagatctttgctcctttccctttgaggactcccaccctttggggtctccaggatcctcatggaaggggaaggtgagacatctgagtgagcagagtgtggcatcttggaaacagtccttagttctgtgggaggactagaaacagccgcggggcgaaggccccctgaggaccactactatactgatggtgggattgggacctgggggatacaggggccccaggaagaagctgccagaggggcagctcagtgctctgcagagaggggccctggggagaagcaggatgggattgatgggcaggagggatccccgcactgggagacaggcccaggtatgaatgagccagccatgcttcctcctgcctgtgtgacgctgggcgagtctcttcccctgtctgggccaaacagggagcgggtaagacaatccatgctctaagatccattttagatcaatgtctaaaatagctctatcgctctgcggagtcccagcagaggctatggaatgtttctgcaaccctaaggcacagagagcccaaccctgagtgtctcagaggccccctgagtgttccccttggcctgagccccttacccattcctgcagccagtgagagacctggcctcagccctggcagggctctctcttcaaggccatatccacctgtgccctggggcttgggagaccccatagggccgggactcttgggtcagcccggccactggcttctctctttttctctgtttcattctgtgtgcgttgtggggtgggggagggggtccacctgccttacctttctgagttgcctttagagagatgcgtttttctaggactctgtgcaactgtcgtatatggtcccgtgggctgaccgctttgtacatgagaataaatctatttctttctacca

SEQ ID NO: 10 - protein, 934 aa, Homo sapiens
MVLVLHHILIAVVQFLRRGQQVFLKPDEPPPPPQPCADSLQDALLSLGSVIDISGLQRAVKEALSAVLPRVETVYTYLLDGESQLVCEDPPHELPQEGKVREAIISQKRLGCNGLGFSDLPGKPLARLVAPLAPDTQVLVMPLADKEAGAVAAVILVHCGQLSDNEEWSLQAVEKHTLVALRRVQVLQQRGPREAPRAVQNPPEGTAEDQKGGAAYTDRDRKILQLCGELYDLDASSLQLKVLQYLQQETRASRCCLLLVSEDNLQLSCKVIGDKVLGEEVSFPLTGCLGQVVEDKKSIQLKDLTSEDVQQLQSMLGCELQAMLCVPVISRATDQVVALACAFNKLEGDLFTDEDEHVIQHCFHYTSTVLTSTLAFQKEQKLKCECQALLQVAKNLFTHLDDVSVLLQEIITEARNLSNAEICSVFLLDQNELVAKVFDGGVVDDESYEIRIPADQGIAGHVATTGQILNIPDAYAHPLFYRGVDDSTGFRTRNILCFPIKNENQEVIGVAELVNKINGPWFSKFDEDLATAFSIYCGISIAHSLLYKKVNEAQYRSHLANEMMMYHMKVSDDEYTKLLHDGIQPVAAIDSNFASFTYTPRSLPEDDTSMAILSMLQDMNFINNYKIDCPTLARFCLMVKKGYRDPPYHNWMHAFSVSHFCYLLYKNLELTNYLEDIEIFALFISCMCHDLDHRGTNNSFQVASKSVLAALYSSEGSVMERHHFAQAIAILNTHGCNIFDHFSRKDYQRMLDLMRDIILATDLAHHLRIFKDLQKMAEVGYDRNNKQHHRLLLCLLMTSCDLSDQTKGWKTTRKIAELIYKEFFSQGDLEKAMGNRPMEMMDREKAYIPELQISFMEHIAMPIYKLLQDLFPKAAELYERVASNREHWTKVSHKFTIRGLPSNNSLDFLDEEYEVPDLDGTRAPINGCCSLDAE

SEQ ID NO: 11 - DNA, 4284 bp, Homo sapiens
  source 1..4284: mol_type = other DNA
agagccagccgagcagcagaggcagtggcagcgggagaggcgggagcagcggggcagcagagctggattggggtgttgagtccaggctgagtagggggcagcccactgctcttggtccctgtgcctgctgggggtgccctgccctgaactccaggcagcggggacagggcgaggtgccaccttagtctggctggggaggcggacgatgaggagtgatggggcaggcatgcggccactccatcctctgcaggagccagcagtacccggcagcgcgaccggctgagccgcggggccagcaggtcttcctcaagccggacgagccgccgccgccgccgcagccatgcgccgacagcctgcaggacgccttgctgagtctgggctctgtcatcgacatttcaggcctgcaacgtgctgtcaaggaggccctgtcagctgtgctcccccgagtggaaactgtctacacctacctactggatggtgagtcccagctggtgtgtgaggaccccccacatgagctgccccaggaggggaaagtccgggaggctatcatctcccagaagcggctgggctgcaatgggctgggcttctcagacctgccagggaagcccttggccaggctggtggctccactggctcctgatacccaagtgctggtcatgccgctagcggacaaggaggctggggccgtggcagctgtcatcttggtgcactgtggccagctgagtgataatgaggaatggagcctgcaggcggtggagaagcataccctggtcgccctgcggagggtgcaggtcctgcagcagcgcgggcccagggaggctccccgagccgtccagaaccccccggaggggacggcggaagaccagaagggcggggcggcgtacaccgaccgcgaccgcaagatcctccaactgtgcggggaactctacgacctggatgcctcttccctgcagctcaaagtgctccaatacctgcagcaggagacccgggcatcccgctgctgcctcctgctggtgtcggaggacaatctccagctttcttgcaaggtcatcggagacaaagtgctcggggaagaggtcagctttcccttgacaggatgcctgggccaggtggtggaagacaagaagtccatccagctgaaggacctcacctccgaggatgtacaacagctgcagagcatgttgggctgtgagctgcaggccatgctctgtgtccctgtcatcagccgggccactgaccaggtggtggccttggcctgcgccttcaacaagctagaaggagacttgttcaccgacgaggacgagcatgtgatccagcactgcttccactacaccagcaccgtgctcaccagcaccctggccttccagaaggaacagaaactcaagtgtgagtgccaggctcttctccaagtggcaaagaacctcttcacccacctggatgacgtctctgtcctgctccaggagatcatcacggaggccagaaacctcagcaacgcagagatctgctctgtgttcctgctggatcagaatgagctggtggccaaggtgttcgacgggggcgtggtggatgatgagagctatgagatccgcatcccggccgatcagggcatcgcgggacacgtggcgaccacgggccagatcctgaacatccctgacgcatatgcccatccgcttttctaccgcggcgtggacgacagcaccggcttccgcacgcgcaacatcctctgcttccccatcaagaacgagaaccaggaggtcatcggtgtggccgagctggtgaacaagatcaatgggccatggttcagcaagttcgacgaggacctggcgacggccttctccatctactgcggcatcagcatcgcccattctctcctatacaaaaaagtgaatgaggctcagtatcgcagccacctggccaatgagatgatgatgtaccacatgaaggtctccgatgatgagtataccaaacttctccatgatgggatccagcctgtggctgccattgactccaattttgcaagtttcacctatacccctcgttccctgcccgaggatgacacgtccatggccatcctgagcatgctgcaggacatgaatttcatcaacaactacaaaattgactgcccgaccctggcccggttctgtttgatggtgaagaagggctaccgggatcccccctaccacaactggatgcacgccttttctgtctcccacttctgctacctgctctacaagaacctggagctcaccaactacctcgaggacatcgagatctttgccttgtttatttcctgcatgtgtcatgacctggaccacagaggcacaaacaactctttccaggtggcctcgaaatctgtgctggctgcgctctacagctctgagggctccgtcatggagaggcaccactttgctcaggccatcgccatcctcaacacccacggctgcaacatctttgatcatttctcccggaaggactatcagcgcatgctggatctgatgcgggacatcatcttggccacagacctggcccaccatctccgcatcttcaaggacctccagaagatggctgaggtgggctacgaccgaaacaacaagcagcaccacagacttctcctctgcctcctcatgacctcctgtgacctctctgaccagaccaagggctggaagactacgagaaagatcgcggagctgatctacaaagaattcttctcccagggagacctggagaaggccatgggcaacaggccgatggagatgatggaccgggagaaggcctatatccctgagctgcaaatcagcttcatggagcacattgcaatgcccatctacaagctgttgcaggacctgttccccaaagcggcagagctgtacgagcgcgtggcctccaaccgtgagcactggaccaaggtgtcccacaagttcaccatccgcggcctcccaagtaacaactcgctggacttcctggatgaggagtacgaggtgcctgatctggatggcactagggcccccatcaatggctgctgcagccttgatgctgagtgatcccctccagggacacttccctgcccaggccacctcccacagccctccactggtctggccagatgcactgggaacagagccacgggtcctgggtcctagaccaggacttcctgtgtgaccctggacaagtactaccttcctgggcctcagctttctcgtctgtataatggaagcaagacttccaacctcacggagactttgtaatttgttttctgagagcacaggggtgaccaatgagcagtgggccctactctgcacctctgaccacaccttggcaagtctttcccaagccattctttgtctgagcagcttgatggtttctccttgccccatttctgccccaccagatctttgctcctttccctttgaggactcccaccctttggggtctccaggatcctcatggaaggggaaggtgagacatctgagtgagcagagtgtggcatcttggaaacagtccttagttctgtgggaggactagaaacagccgcggggcgaaggccccctgaggaccactactatactgatggtgggattgggacctgggggatacaggggccccaggaagaagctgccagaggggcagctcagtgctctgcagagaggggccctggggagaagcaggatgggattgatgggcaggagggatccccgcactgggagacaggcccaggtatgaatgagccagccatgcttcctcctgcctgtgtgacgctgggcgagtctcttcccctgtctgggccaaacagggagcgggtaagacaatccatgctctaagatccattttagatcaatgtctaaaatagctctatcgctctgcggagtcccagcagaggctatggaatgtttctgcaaccctaaggcacagagagcccaaccctgagtgtctcagaggccccctgagtgttccccttggcctgagccccttacccattcctgcagccagtgagagacctggcctcagccctggcagggctctctcttcaaggccatatccacctgtgccctggggcttgggagaccccatagggccgggactcttgggtcagcccggccactggcttctctctttttctctgtttcattctgtgtgcgttgtggggtgggggagggggtccacctgccttacctttctgagttgcctttagagagatgcgtttttctaggactctgtgcaactgtcgtatatggtcccgtgggctgaccgctttgtacatgagaataaatctatttctttctacca

SEQ ID NO: 12 - protein, 940 aa, Homo sapiens
MGQACGHSILCRSQQYPAARPAEPRGQQVFLKPDEPPPPPQPCADSLQDALLSLGSVIDISGLQRAVKEALSAVLPRVETVYTYLLDGESQLVCEDPPHELPQEGKVREAIISQKRLGCNGLGFSDLPGKPLARLVAPLAPDTQVLVMPLADKEAGAVAAVILVHCGQLSDNEEWSLQAVEKHTLVALRRVQVLQQRGPREAPRAVQNPPEGTAEDQKGGAAYTDRDRKILQLCGELYDLDASSLQLKVLQYLQQETRASRCCLLLVSEDNLQLSCKVIGDKVLGEEVSFPLTGCLGQVVEDKKSIQLKDLTSEDVQQLQSMLGCELQAMLCVPVISRATDQVVALACAFNKLEGDLFTDEDEHVIQHCFHYTSTVLTSTLAFQKEQKLKCECQALLQVAKNLFTHLDDVSVLLQEIITEARNLSNAEICSVFLLDQNELVAKVFDGGVVDDESYEIRIPADQGIAGHVATTGQILNIPDAYAHPLFYRGVDDSTGFRTRNILCFPIKNENQEVIGVAELVNKINGPWFSKFDEDLATAFSIYCGISIAHSLLYKKVNEAQYRSHLANEMMMYHMKVSDDEYTKLLHDGIQPVAAIDSNFASFTYTPRSLPEDDTSMAILSMLQDMNFINNYKIDCPTLARFCLMVKKGYRDPPYHNWMHAFSVSHFCYLLYKNLELTNYLEDIEIFALFISCMCHDLDHRGTNNSFQVASKSVLAALYSSEGSVMERHHFAQAIAILNTHGCNIFDHFSRKDYQRMLDLMRDIILATDLAHHLRIFKDLQKMAEVGYDRNNKQHHRLLLCLLMTSCDLSDQTKGWKTTRKIAELIYKEFFSQGDLEKAMGNRPMEMMDREKAYIPELQISFMEHIAMPIYKLLQDLFPKAAELYERVASNREHWTKVSHKFTIRGLPSNNSLDFLDEEYEVPDLDGTRAPINGCCSLDA

SEQ ID NO: 13 - DNA, 4182 bp, Homo sapiens
  source 1..4182: mol_type = other DNA
gaagaatctggaagtgcagagcttagcccctggcatgcggcaggtgctcacaaagaagtttacagcttcctgagcactgtttccacacctgtgatctcatttaatcctcaccacaaacccaagagactgctgttttctggatgaagaaacagaggatccaggaggggaaatcgcttgcccacaggcggggccagcaggtcttcctcaagccggacgagccgccgccgccgccgcagccatgcgccgacagcctgcaggacgccttgctgagtctgggctctgtcatcgacatttcaggcctgcaacgtgctgtcaaggaggccctgtcagctgtgctcccccgagtggaaactgtctacacctacctactggatggtgagtcccagctggtgtgtgaggaccccccacatgagctgccccaggaggggaaagtccgggaggctatcatctcccagaagcggctgggctgcaatgggctgggcttctcagacctgccagggaagcccttggccaggctggtggctccactggctcctgatacccaagtgctggtcatgccgctagcggacaaggaggctggggccgtggcagctgtcatcttggtgcactgtggccagctgagtgataatgaggaatggagcctgcaggcggtggagaagcataccctggtcgccctgcggagggtgcaggtcctgcagcagcgcgggcccagggaggctccccgagccgtccagaaccccccggaggggacggcggaagaccagaagggcggggcggcgtacaccgaccgcgaccgcaagatcctccaactgtgcggggaactctacgacctggatgcctcttccctgcagctcaaagtgctccaatacctgcagcaggagacccgggcatcccgctgctgcctcctgctggtgtcggaggacaatctccagctttcttgcaaggtcatcggagacaaagtgctcggggaagaggtcagctttcccttgacaggatgcctgggccaggtggtggaagacaagaagtccatccagctgaaggacctcacctccgaggatgtacaacagctgcagagcatgttgggctgtgagctgcaggccatgctctgtgtccctgtcatcagccgggccactgaccaggtggtggccttggcctgcgccttcaacaagctagaaggagacttgttcaccgacgaggacgagcatgtgatccagcactgcttccactacaccagcaccgtgctcaccagcaccctggccttccagaaggaacagaaactcaagtgtgagtgccaggctcttctccaagtggcaaagaacctcttcacccacctggatgacgtctctgtcctgctccaggagatcatcacggaggccagaaacctcagcaacgcagagatctgctctgtgttcctgctggatcagaatgagctggtggccaaggtgttcgacgggggcgtggtggatgatgagagctatgagatccgcatcccggccgatcagggcatcgcgggacacgtggcgaccacgggccagatcctgaacatccctgacgcatatgcccatccgcttttctaccgcggcgtggacgacagcaccggcttccgcacgcgcaacatcctctgcttccccatcaagaacgagaaccaggaggtcatcggtgtggccgagctggtgaacaagatcaatgggccatggttcagcaagttcgacgaggacctggcgacggccttctccatctactgcggcatcagcatcgcccattctctcctatacaaaaaagtgaatgaggctcagtatcgcagccacctggccaatgagatgatgatgtaccacatgaaggtctccgatgatgagtataccaaacttctccatgatgggatccagcctgtggctgccattgactccaattttgcaagtttcacctatacccctcgttccctgcccgaggatgacacgtccatggccatcctgagcatgctgcaggacatgaatttcatcaacaactacaaaattgactgcccgaccctggcccggttctgtttgatggtgaagaagggctaccgggatcccccctaccacaactggatgcacgccttttctgtctcccacttctgctacctgctctacaagaacctggagctcaccaactacctcgaggacatcgagatctttgccttgtttatttcctgcatgtgtcatgacctggaccacagaggcacaaacaactctttccaggtggcctcgaaatctgtgctggctgcgctctacagctctgagggctccgtcatggagaggcaccactttgctcaggccatcgccatcctcaacacccacggctgcaacatctttgatcatttctcccggaaggactatcagcgcatgctggatctgatgcgggacatcatcttggccacagacctggcccaccatctccgcatcttcaaggacctccagaagatggctgaggtgggctacgaccgaaacaacaagcagcaccacagacttctcctctgcctcctcatgacctcctgtgacctctctgaccagaccaagggctggaagactacgagaaagatcgcggagctgatctacaaagaattcttctcccagggagacctggagaaggccatgggcaacaggccgatggagatgatggaccgggagaaggcctatatccctgagctgcaaatcagcttcatggagcacattgcaatgcccatctacaagctgttgcaggacctgttccccaaagcggcagagctgtacgagcgcgtggcctccaaccgtgagcactggaccaaggtgtcccacaagttcaccatccgcggcctcccaagtaacaactcgctggacttcctggatgaggagtacgaggtgcctgatctggatggcactagggcccccatcaatggctgctgcagccttgatgctgagtgatcccctccagggacacttccctgcccaggccacctcccacagccctccactggtctggccagatgcactgggaacagagccacgggtcctgggtcctagaccaggacttcctgtgtgaccctggacaagtactaccttcctgggcctcagctttctcgtctgtataatggaagcaagacttccaacctcacggagactttgtaatttgttttctgagagcacaggggtgaccaatgagcagtgggccctactctgcacctctgaccacaccttggcaagtctttcccaagccattctttgtctgagcagcttgatggtttctccttgccccatttctgccccaccagatctttgctcctttccctttgaggactcccaccctttggggtctccaggatcctcatggaaggggaaggtgagacatctgagtgagcagagtgtggcatcttggaaacagtccttagttctgtgggaggactagaaacagccgcggggcgaaggccccctgaggaccactactatactgatggtgggattgggacctgggggatacaggggccccaggaagaagctgccagaggggcagctcagtgctctgcagagaggggccctggggagaagcaggatgggattgatgggcaggagggatccccgcactgggagacaggcccaggtatgaatgagccagccatgcttcctcctgcctgtgtgacgctgggcgagtctcttcccctgtctgggccaaacagggagcgggtaagacaatccatgctctaagatccattttagatcaatgtctaaaatagctctatcgctctgcggagtcccagcagaggctatggaatgtttctgcaaccctaaggcacagagagcccaaccctgagtgtctcagaggccccctgagtgttccccttggcctgagccccttacccattcctgcagccagtgagagacctggcctcagccctggcagggctctctcttcaaggccatatccacctgtgccctggggcttgggagaccccatagggccgggactcttgggtcagcccggccactggcttctctctttttctctgtttcattctgtgtgcgttgtggggtgggggagggggtccacctgccttacctttctgagttgcctttagagagatgcgtttttctaggactctgtgcaactgtcgtatatggtcccgtgggctgaccgctttgtacatgagaataaatctatttctttctacca

SEQ ID NO: 14 - protein, 932 aa, Homo sapiens
MKKQRIQEGKSLAHRRGQQVFLKPDEPPPPPQPCADSLQDALLSLGSVIDISGLQRAVKEALSAVLPRVETVYTYLLDGESQLVCEDPPHELPQEGKVREAIISQKRLGCNGLGFSDLPGKPLARLVAPLAPDTQVLVMPLADKEAGAVAAVILVHCGQLSDNEEWSLQAVEKHTLVALRRVQVLQQRGPREAPRAVQNPPEGTAEDQKGGAAYTDRDRKILQLCGELYDLDASSLQLKVLQYLQQETRASRCCLLLVSEDNLQLSCKVIGDKVLGEEVSFPLTGCLGQVVEDKKSIQLKDLTSEDVQQLQSMLGCELQAMLCVPVISRATDQVVALACAFNKLEGDLFTDEDEHVIQHCFHYTSTVLTSTLAFQKEQKLKCECQALLQVAKNLFTHLDDVSVLLQEIITEARNLSNAEICSVFLLDQNELVAKVFDGGVVDDESYEIRIPADQGIAGHVATTGQILNIPDAYAHPLFYRGVDDSTGFRTRNILCFPIKNENQEVIGVAELVNKINGPWFSKFDEDLATAFSIYCGISIAHSLLYKKVNEAQYRSHLANEMMMYHMKVSDDEYTKLLHDGIQPVAAIDSNFASFTYTPRSLPEDDTSMAILSMLQDMNFINNYKIDCPTLARFCLMVKKGYRDPPYHNWMHAFSVSHFCYLLYKNLELTNYLEDIEIFALFISCMCHDLDHRGTNNSFQVASKSVLAALYSSEGSVMERHHFAQAIAILNTHGCNIFDHFSRKDYQRMLDLMRDIILATDLAHHLRIFKDLQKMAEVGYDRNNKQHHRLLLCLLMTSCDLSDQTKGWKTTRKIAELIYKEFFSQGDLEKAMGNRPMEMMDREKAYIPELQISFMEHIAMPIYKLLQDLFPKAAELYERVASNREHWTKVSHKFTIRGLPSNNSLDFLDEEYEVPDLDGTRAPINGCCSLDAE

SEQ ID NO: 15 - DNA, 12486 bp, Homo sapiens
  source 1..12486: mol_type = other DNA
gctagtctctcggtctggctctctctccgacgggacttagcaacttcttatttctcagccccttgtccatttttttttttccatcctttgccatgaattggattgacagaggcgggggaggctttgctttctgccccagggaatggcgattcgcgtcctggggccgtgccggggagaatcggccgaggagaaagaaagagtgatagaaaaagagctgcaggaaggaggagaagggagacctccatctgccgcgggcccggcgcgctgcagcgcagcgcagcgccgagctgcgcctcggaatggcccggagcccgccctgcgcccccggctcctccagcgtcagcggctcctgcgcgcgggatgcattgggcaatttttgaaatcctgaagtaggaagagaccccggaggatataagtcgggggtgggggtggagcagagaatctgtgaaagatattcaaagagagaaaaggggaatcctgatcgtttctgcccgtgcttgttttcaacttgagcgtgctagcctttaacttgaagaagtctcattggagcatctagcattctccaggagttattcgaaagctgaaactttcagtggattgtgggcctggggagaagaaggattccgagggtggaattgggaagagcgtgcgtgcgtgtgtgtgtgtgtgtgtgtgcgcgcgcgcgcgtgggtcggggcgggggcgtcggggggccactgggaattcagtgaagagggcaccctataccatggcagtgcccggcgacgctgcacgagtcagggacaagcccgtccacagtggggtgagtcaagcccccacggcgggccgggactgccaccatcgtgcggaccccgcatcgccgcgggactcgggctgccgtggctgctggggagacctggtgctgcagccgctccggagctctcggaaactttcctccgcgctgtgcgcgggctccctgtcctttctgctggcgctgctggtgaggctggtccgcggggaggtcggctgtgacctggagcagtgtaaggaggcggcggcggcggaggaggaggaagcagccccgggagcagaagggggcgtcttcccggggcctcggggaggtgctcccgggggcggtgcgcggctcagcccctggctgcagccctcggcgctgctcttcagtctcctgtgtgccttcttctggatgggcttgtacctcctgcgcgccggggtgcgcctgcctctggctgtcgcgctgctggccgcctgctgcgggggggaagcgctcgtccagattgggctgggcgtcggggaggatcacttactctcactccccgccgcgggggtggtgctcagctgcttggccgccgcgacatggctggtgctgaggctgaggctgggcgtcctcatgatcgccttgactagcgcggtcaggaccgtgtccctcatttccttagagaggttcaaggtcgcctggagaccttacctggcgtacctggccggcgtgctggggatcctcttggccaggtacgtggaacaaatcttgccgcagtccgcggaggcggctccaagggagcatttggggtcccagctgattgctgggaccaaggaagatatcccggtgtttaagaggaggaggcggtccagctccgtcgtgtccgccgagatgtccggctgcagcagcaagtcccatcggaggacctccctgccctgtataccgagggaacagctcatggggcattcagaatgggaccacaaacgagggccaagaggatcacagtcttcaggaaccagtattactgtggacatcgccgtcatgggcgaggcccacggcctcattaccgacctcctggcagacccttctcttccaccaaacgtgtgcacatccttgagagccgtgagcaacttgctcagcacacagctcaccttccaggccattcacaagcccagagtgaatcccgtcacttcgctcagtgaaaactatacctgttctgactctgaagagagctctgaaaaagacaagcttgctattccaaagcgcctgagaaggagtttgcctcctggcttgttgagacgagtttcttccacttggaccaccaccacctcggccacaggtctacccaccttggagcctgcaccagtacggagagaccgcagcaccagcatcaaactgcaggaagcaccttcatccagtcctgattcttggaataatccagtgatgatgaccctcaccaaaagcagatcctttacttcatcctatgctatttctgcagctaaccatgtaaaggctaaaaagcaaagtcgaccaggtgccctcgctaaaatttcacctctttcatcgccctgctcctcacctctccaagggactcctgccagcagcctggtcagcaaaatttctgcagtgcagtttccagaatctgctgacacaactgccaaacaaagcctaggttctcacagggccttaacttacactcagagtgccccagacctatcccctcaaatcctgactccacctgttatatgtagcagctgtggcagaccatattcccaagggaatcctgctgatgagcccctggagagaagtggggtagccactcggacaccaagtagaacagatgacactgctcaagttacctctgattatgaaaccaataacaacagtgacagcagtgacattgtacagaatgaagatgaaacagagtgcctgagagagcctctgaggaaagcatcggcttgcagcacctatgctcctgagaccatgatgtttctggacaaaccaattcttgctcccgaacctcttgtcatggataacctggactcaattatggagcagctaaatacttggaattttccaatttttgatttagtggaaaatataggaagaaaatgtggccgtattcttagtcaggtatcttacagactttttgaagacatgggcctctttgaagcttttaaaattccaattagggaatttatgaattattttcatgctttggagattggatatagggatattccttatcataacagaatccatgccactgatgttttacatgctgtttggtatcttactacacagcctattccaggcctctcaactgtgattaatgatcatggttcaaccagtgattcagattctgacagtggatttacacatggacatatgggatatgtattctcaaaaacgtataatgtgacagatgataaatacggatgtctgtctgggaatatccctgccttggagttgatggcgctgtatgtggctgcagccatgcacgattatgatcatccaggaaggactaatgctttcctggttgcaactagtgctcctcaggcggtgctatataacgatcgttcagttttggagaatcatcacgcagctgctgcatggaatcttttcatgtcccggccagagtataacttcttaattaaccttgaccatgtggaatttaagcatttccgtttccttgtcattgaagcaattttggccactgacctgaagaaacactttgacttcgtagccaaatttaatggcaaggtaaatgatgatgttggaatagattggaccaatgaaaatgatcgtctactggtttgtcaaatgtgtataaagttggctgatatcaatggtccagctaaatgtaaagaactccatcttcagtggacagatggtattgtcaatgaattttatgaacagggtgatgaagaggccagccttggattacccataagccccttcatggatcgttctgctcctcagctggccaaccttcaggaatccttcatctctcacattgtggggcctctgtgcaactcctatgattcagcaggactaatgcctggaaaatgggtggaagacagcgatgagtcaggagatactgatgacccagaagaagaggaggaagaagcaccagcaccaaatgaagaggaaacctgtgaaaataatgaatctccaaaaaagaagactttcaaaaggagaaaaatctactgccaaataactcagcacctcttacagaaccacaagatgtggaagaaagtcattgaagaggagcaacggttggcaggcatagaaaatcaatccctggaccagacccctcagtcgcactcttcagaacagatccaggctatcaaggaagaagaagaagagaaagggaaaccaagaggcgaggagataccaacccaaaagccagaccagtgacaatggatagaatgggctgtgtttccaaacagattgacttgtcaaagactctcttcaagccagcacaacatttagacacaacactgtagaaatttgagatgggcaaatggctattgcattttgggattcttcgcattttgtgtgtatatttttacagtgaggtacattgttaaaaactttttgctcaaagaagctttcacattgcaacaccagcttctaaggattttttaaggagggaatatatatgtgtgtgtgtatataagctcccacatagatacatgtaaaacatattcacacccatgcacgcacacacatacacactgaaggccacgattgctggctccacaatttagtaacatttatattaagatatatatatagtggtcactgtgatataataaatcataaaggaaaccaaatcacaaaggagatggtgtggcttagcaaggaaacagtgcaggaaatgtaggttaccaactaagcagcttttgctcttagtactgagggatgaaagttccagagcattatttgaattctgatacatcctgccaacactgtgtgtgtgtgtgtgtgtgtgtgtgtgtgtgtgtgtgtgtgtgaaagagagacagaagggaatggtttgagagggtgcttgtgtgcatgtgtgtgcatatgtaaagagatttttgtggtttaagtaactcagaatagctgtagcaaatgactgaatacatgtgaacaaacagaaggaagttcactctggagtgtctttgggaggcagccattccaaatgccctcctccatttagcttcaataaagggccttttgctgatggagggcactcaagggctgggtgagagggccacgtgtttggtattacattactgctatgcaccacttgaaggagctctatcaccagcctcaaacccgaaagactgaggcattttccagtctacttgcctaatgaatgtataggaactgtctatgagtatggatgtcactcaactaagatcaaatcaccatttaaggggatggcattctttatacctaaacacctaagagctgaagtcaggtcttttaatcaggttagaattctaaatgatgccagagaaggcttgggaaattgtacttcagcgtgatagcctgtgtcttcttaatttgctgcaaaatatgtggtagagaaagaaaaggaaacagaaaaatcactctgggttatatagcaagagatgaaggagaatatttcaacacagggtttttgtgttgacataggaaaagcctgattcttggcaactgttgtagtttgtctttcaggggtgaaggtcccactgacaacccctgttgtggtgttccacacgctgtttgttggggtagcttccatcggcagtctggcccattgtcagtcatgcttcttctggccggggagattatagagagattgtttgaagattgggttattattgaaagtctttttttttgtttgttttgttttggtttgtttgtttatctacacttgtttatgctgtgagccaaacctctatttaaaaagttgatactcactttcaatattttatttcatattattatatatgtcatgatagttatcttgatgtaaatatgaagatttttttgtttctgtagatagtaaactctttttttaaaaaaggaaaagggaaacatttttataaagttatattttaatcaccatttttatacattgtagttctctccaagcccagtaagagaatgatgattcatttgcatggaggtcgatggacaaccaatcatctaccttttctaatttaaatgataatctgatatagttttattgccagttaaatgaggatgctgcaaagcatgttttttcactagtaacttttgctaactgaatgaattctgggtccatatctcccagatgaaaaactgttaaccaataccatattttatagttggtgtccatttctttccaacactgtttgttatgattcttccttgagtacttatatacagacctgctcattatctaaacaatcttaccttctaagtaaaccttgattgtgatttccagtttttattttctctgacgtagtagaaaggaatgtttacattaaaaatacttttgtttctcataaatggatattgtactcccccctttcaaagcattattttacaataattcatggcattttaaaaaataaggcaaagataatacgacaaaaaatatacatggtttcaaggcaaattctccaataagttggaaaatgtaaaaaggatcaagtggatgcagcctctacctaaataattaaaatatatttcagtatatttctgaattaacaccaggtcttcattatttagaacttactaaattgttttcattttcttagttttacctgtgtatctccatgtttgcaaaaattactataagtcaaattttgccagtgaatttaactatttttctttccttgcaattaaggggaaaaaagcatttatcttatcttctcataccccttgcatctaagtacttagcaaagtcaatattttcccattttccaaatgcgtccatctctaacataaatattaattgaacatagagctatgtttggagtgagtggactggcaggacagttggaagtccatcacagtctattgacagtttcatcaaagctgtatagtccaactagtggggcagcttggctactatggtggaagtctcagcaaactgcctggttttgtttgtttgttttgttttaaggtacaggaaataagaggaataatagtggccaaagcaattagaacatcttcattccagaactgtgttcagcaatccaggcagattgatacatttttctttaaaaataaattgctattacagctagacgtcaattgggataaataaagggatgaagatccactaagtttgtgactttcatacacacccagtacatctcaaaggatgctaagggacattttctgccagtagagttctccccctttttggtgacagcaatattattatgttcacatctaactccagagcttacttcctgtggtgccaatgtatttgttgcaatttactacatttttatatgagcctatttataggtgccattaaactcaggtctttcaaatgaaagagtttctagcccacttagggaaaaagataattgtttagaaaaccataaaatcaatggtaggaaaagttggaactggttacctggatgccatggttctctgttaaataaagtaagagaccaggtgtattctgagtgtcatcagtgttattttcagcatgctaataaatgtctttccggttatatatctatctaaattaacctttaaaatattggtttccttgataaaagcaccacttttgcttttgttagctgtaatattttttgtcatttagataagacctggtttggctctcaataaaagatgaagacagtagctctgtacagggatatatctatattagtcttcatctgatgaatgaagaaattttctcatattatgttcaagaaagtatttacttcctaaaaatagaattcccgattctgtctattttggttgaataccagaacaaatctttccgttgcaatcccagtaaaacgaaagaaaaggaatatcttacagactgttcatattagatgtatgtagactgttaatttgcaatttccccatatttcctgcctatcttacccagataactttctttgaaggtaaaagctgtgcaaaaggcatgagactcaggcctactctttgtttaaatgatggaaaaatataaattattttctaagtaataaaagtataaaaattatcattataaataaagtctaaagtttgaaattattaatttataaaagtgaactaattgtgtgattatcaaatcctgattaatgagaagtgaataatctaaaaatcatttatattctactgtgggaggtattcttggtgcttccatgtcagtatcgggctctccattgtcctcatcatttatagtacttctaaaataataatggaaacctcaataagggtcttgtcctcttctgtcatcctaaccctgattctagtttaatgcctttcctgacttatatgccatttgtaaataaacttcctttcaaactgttagaacgctccaataaaacaaagttctatgaactttcatagtctagaaaaaccaacaagatcccccttatttagagattattagctaatgtgtgaaagaaatatcaatagaagttcaaatgctaatagctcaattccagataattgaaagctaaaatatctatgtactttgaagccaaactgagtttatttcattgatcgaacaagcagcaacacattttatgaccattgtcctaggtcgtttgtgtctttatgaatttgctgatattgtcagtccattttttaaatcttcaacaaaattcaattttaagattaagaaatcagcaattttaggtaaagaatattccaagattaaattgttctttttaagaaatatatcagttttaggtcctatgttcacacatcaatttgttcatctggaagatattcaaattcttattgggaatgaattacactacaaacaatgagttgagctaaaaactatacataacttaaattgagatttgcatacgtatttgtgtgtttcacaccaaagacccatgctcagagaatggtaacatattttccagtctatgttatgcaccatggatgttaggcaatgtgtgctattgccaacacatggtatttgttgaaatacatgttgctttgaccttacctaatggtgcttttacctaacttgaagtgctttttgtgttcccaccagcaaatcattctaacagcaggctaacaatggtgaagtaaaatgaacatttttgggccgggcgcagtggctcacgcctgtaatcccagcactttgggaggccaaggctggtggatcacctgaggtcgggagttcgacaccagcctgaccaacacggagaaaccccgtctttactaaaaatacaaaatgattcaggtgtggtggcgcatgtctgtaatcccagctacccaggaggctgaggcagaatcgcttgaacctgggaggcagaggttatggtgagctgagattgcaccattgcactccagcctgggcaacaggagttaaattttgcctcaaaaaaaaaaaaaaaaaaaaaaagaacattttttggcaaaatatgaagacacgaaactgaagataaaggcttcatttccatagtggaaatcagtgtttacctgctgattcaaaaatactgacctagtatcagtgtaggtaagaccataaaatacagtgtatagaattatatataaatggaaaacaaaattagcttttgacatatgtttaagtctctaaaaggaatccacattttctttccagatacagctagtttttctccacatgtttttaaggttgatttccttgacacacattggtatccttgggtttctgcttccttgaaaagttgtggagcacagaagaaaagccttctctttacagataaaaaatgttgaacatgttcatgttctgacaatgaagcaatgatttcctcattgctttgcattaagaagtggttctttagttatgcaaataattcaataaccaaaaatgcttcaaagagtaataataaatcaccataggtaagtattctcaagaatgtttaaatttggtttattttcttgaagcaaagttatttaattttttaatttttaacttaaaatgaaacccacaaaatgacattccgtggtactgagtattttcacataatcagaactgtaaactactgattattttcatatactcagaggctgaatattttgatataataagaactagtatcatataacagaaaactagaaagaaggtttaattctttttctaatattctacaagcctcatggggaaaatgttttatgaaggattcaaatacattagataaaaattagtgtcaataatttaactttgtacaaattatagtctgagatcttctgagttttcctaagacaaaggagtgtattatccagcaatttattgttttgtgttgttataaaataaatgttctattaatgtatattttattttactaagttctaacacaaaaggccaaatacttatctttcctactaagaaaaattaaaccttactaatcttgactttcacagatgaaacactgaccagtcaataaacaacagccactgcattaatctgcccagcatgatcagatagtaggttagaatttgaaattcattaataaaaaattaataacaaaactttgtaagccttaatggtttaatatttccgtgtcattgaaagttcctatttcaaattaaacaaactacagcaggatatttttcctttcctgtttcaaaacaaaaaccagatgaagaaaaaacaaagacaaactcataggaggaaagcatggcttctcttcaattatacttctcttactcaatattagtaaccaaaaaataagcagaaattctcctctgccataattaaaagaaagaatggccttcgacttaagttctagttcctcaagcctgctttccttgtaaagtccatggtactaagaagcaaaaaatgcagagctgtggattgggagtgaacactacataaaatttgcagggtatcccaggacacccctcagtctttaatacaaaccaatttagttactctggagtgaaatgacttgtggatacactgttcaaccatgacttcctttatgacaaggagcacttatacatgtttccaaatgtgaattagcccttgaattagtttgaaaactgctacttgaataacttttgaagagaaagattttctttccggtaattttactccctaaaaaaggcaaaatactcagatgttcaatgtgaaattacaaatagttgtttgaagtatatatacttcaataaatagttctttgtgtatataaagtgttggttcatagcagtttccttgtcccttttctttttaaaattcccaactgattatgggtcaaaaactccatcttatatcagcgatgatttcattttaactatttataaggataatttagtattatagtattgctaactttaataattctaccatatctatatattacctgttagtgaggttttaatggctttacttaatacatatttgttcatcagcttaaaaaatcactaaattttttatactctgtaaaatatttgcatgggaattttagcttattatgtttgcttaactggtgtttttttcacttatgactgtcagtttatgtcttaatgtattctcacagaagaatgcataccatttttgttccaacaagaacaatctgttagttgataagcactggtaataaatatcactgaacccacccaccccctgatatttcttcctcaagttttctatcatgcaaatcacaaaatgaaaattggtgcttttacaaatatttgaaagctctcaatgcaaaataataaaaatgagattctccctggctttctataatatattaggatatgtgactgaaggaaatttaatctgaatttagagtgttttaggttttggttggtttgaataatttgatttgcattttggtattaaaatgtgctctgatttctgcgggcatttgttctgaccagtcattacctcttcccaacagaaaaaaaaaaaaaaaaaaaaaaactggcattggcaagttttaattaatatggcccaaaaatttgaccttgaaggatatttgtaaaccagagagtatttaattaactaaatttactgtttctgaaaagcaatattttcaaataactgccaaccaaagtgacactatagggatgtcatttgtacatgacaatttttaacaatgtaattcttaccactctcgacagacctgaatatgtttactaataactttgccaaatttttcaacttctagaaaaacaagagtgagtcttttgaacttcatcattttgcaattgaaataaatcttgtcctttcacctatatcttccatttaatatatgtagcaatacttagtatcatcccatcacaagtattgttaggcgacttagtggcggagaaatgtttgtaaaaagtagaatctgtacagaaaaaaaactagatcaattgtatttatttttattattttttagcttagatactatgttgatgctccctttttgccagaattactggaagtgcctcttggttttatatatataatatataaatattacagtaaatatatactcaaaattattaaaattatgtcctagattatctatgtcgatgttatgagtgaagataatgtataatataaaaataattctgcagta

SEQ ID NO: 16 - protein, 1141 aa, Homo sapiens
MAVPGDAARVRDKPVHSGVSQAPTAGRDCHHRADPASPRDSGCRGCWGDLVLQPLRSSRKLSSALCAGSLSFLLALLVRLVRGEVGCDLEQCKEAAAAEEEEAAPGAEGGVFPGPRGGAPGGGARLSPWLQPSALLFSLLCAFFWMGLYLLRAGVRLPLAVALLAACCGGEALVQIGLGVGEDHLLSLPAAGVVLSCLAAATWLVLRLRLGVLMIALTSAVRTVSLISLERFKVAWRPYLAYLAGVLGILLARYVEQILPQSAEAAPREHLGSQLIAGTKEDIPVFKRRRRSSSVVSAEMSGCSSKSHRRTSLPCIPREQLMGHSEWDHKRGPRGSQSSGTSITVDIAVMGEAHGLITDLLADPSLPPNVCTSLRAVSNLLSTQLTFQAIHKPRVNPVTSLSENYTCSDSEESSEKDKLAIPKRLRRSLPPGLLRRVSSTWTTTTSATGLPTLEPAPVRRDRSTSIKLQEAPSSSPDSWNNPVMMTLTKSRSFTSSYAISAANHVKAKKQSRPGALAKISPLSSPCSSPLQGTPASSLVSKISAVQFPESADTTAKQSLGSHRALTYTQSAPDLSPQILTPPVICSSCGRPYSQGNPADEPLERSGVATRTPSRTDDTAQVTSDYETNNNSDSSDIVQNEDETECLREPLRKASACSTYAPETMMFLDKPILAPEPLVMDNLDSIMEQLNTWNFPIFDLVENIGRKCGRILSQVSYRLFEDMGLFEAFKIPIREFMNYFHALEIGYRDIPYHNRIHATDVLHAVWYLTTQPIPGLSTVINDHGSTSDSDSDSGFTHGHMGYVFSKTYNVTDDKYGCLSGNIPALELMALYVAAAMHDYDHPGRTNAFLVATSAPQAVLYNDRSVLENHHAAAAWNLFMSRPEYNFLINLDHVEFKHFRFLVIEAILATDLKKHFDFVAKFNGKVNDDVGIDWTNENDRLLVCQMCIKLADINGPAKCKELHLQWTDGIVNEFYEQGDEEASLGLPISPFMDRSAPQLANLQESFISHIVGPLCNSYDSAGLMPGKWVEDSDESGDTDDPEEEEEEAPAPNEEETCENNESPKKKTFKRRKIYCQITQHLLQNHKMWKKVIEEEQRLAGIENQSLDQTPQSHSSEQIQAIKEEEEEKGKPRGEEIPTQKPDQ

SEQ ID NO: 17 - DNA, 5995 bp, Homo sapiens
  source 1..5995: mol_type = other DNA
agtcccgagaggtgcccgagggaaaaggaggcggcagctaaactggtcctggagagaagccccttccgcccctctcctcagccagcatgtcccggactccgccgctcctcagtccgcgcggtggggaccccgggccgtggcggccggcgcagccctgacgggttgcgaaccagggggcgccccgaacgcgggggttggggtctgggagcgcgagcggccgctacggtacgagcggggtgtgctgagtcccgtggccacccccggccccagccatgaggagggacgagcgagacgccaaagccatgcggtccctgcagccgccggatggggccggctcgccccccgagagtctgaggaacggctacgtgaagagctgcgtgagccccttgcggcaggaccctccgcgcggcttcttcttccacctctgccgcttctgcaacgtggagctgcggccgccgccggcctctccccagcagccgcggcgctgctcccccttctgccgggcgcgcctctcgctgggcgccctggctgcctttgtcctcgccctgctgctgggcgcggaacccgagagctgggctgccggggccgcctggctgcggacgctgctgagcgtgtgttcgcacagcttgagccccctcttcagcatcgcctgtgccttcttcttcctcacctgcttcctcacccggaccaagcggggacccggcccgggccggagctgcggctcctggtggctgctggcgctgcccgcctgctgttacctgggggacttcttggtgtggcagtggtggtcttggccttggggggatggcgacgcagggtccgcggccccgcacacgcccccggaggcggcagcgggcaggttgctgctggtgctgagctgcgtagggctgctgctgacgctcgcgcacccgctgcggctccggcactgcgttctggtgctgctcctggccagcttcgtctggtgggtctccttcaccagcctcgggtcgctgccctccgccctcaggccgctgctctccggcctggtggggggcgctggctgcctgctggccctggggttggatcacttctttcaaatcagggaagcgcctcttcatcctcgactgtccagtgccgccgaagaaaaagtgcctgtgatccgaccccggaggaggtccagctgcgtgtcgttaggagaaactgcagccagttactatggcagttgcaaaatattcaggagaccgtcgttgccttgtatttccagagaacagatgattctttgggattgggacttaaaacaatggtataagcctcattatcaaaattctggaggtggaaatggagttgatctttcagtgctaaatgaggctcgcaatatggtgtcagatcttctgactgatccaagccttccaccacaagtcatttcctctctacggagtattagtagcttaatgggtgctttctcaggttcctgtaggccaaagattaatcctctcacaccatttcctggattttacccctgttctgaaatagaggacccagctgagaaaggggatagaaaacttaacaagggactaaataggaatagtttgccaactccacagctgaggagaagctcaggaacttcaggattgctacctgttgaacagtcttcaaggtgggatcgtaataatggcaaaagacctcaccaagaatttggcatttcaagtcaaggatgctatctaaatgggccttttaattcaaatctactgactatcccgaagcaaaggtcatcttctgtatcactgactcaccatgtaggtctcagaagagctggtgttttgtccagtctgagtcctgtgaattcttccaaccatggaccagtgtctactggctctctaactaatcgatcacccatagaatttcctgatactgctgattttcttaataagccaagcgttatcttgcagagatctctgggcaatgcacctaatactccagatttttatcagcaacttagaaattctgatagcaatctgtgtaacagctgtggacatcaaatgctgaaatatgtttcaacatctgaatcagatggtacagattgctgcagtggaaaatcaggtgaagaagaaaacattttctcgaaagaatcattcaaacttatggaaactcaacaagaagaggaaacagagaagaaagacagcagaaaattatttcaggaaggtgataagtggctaacagaagaggcacagagtgaacagcaaacaaatattgaacaggaagtatcactggacctgattttagtagaagagtatgactcattaatagaaaagatgagcaactggaattttccaatttttgaacttgtagaaaagatgggagagaaatcaggaaggattctcagtcaggttatgtataccttatttcaagacactggtttattggaaatatttaaaattcccactcaacaatttatgaactattttcgtgcattagaaaatggctatcgagacattccttatcacaatcgtatacatgccacagatgtgctacatgcagtttggtatctgacaacacggccagttcctggcttacagcagatccacaatggttgtggaacaggaaatgaaacagattctgatggtagaattaaccatgggcgaattgcttatatttcttcgaagagctgctctaatcctgatgagagttatggctgcctgtcttcaaacattcctgcattagaattgatggctctatacgtggcagctgccatgcatgattatgatcacccagggaggacaaatgcatttctagtggctacaaatgcccctcaggcagttttatacaatgacagatctgttctggaaaatcatcatgctgcgtcagcttggaatctatatctttctcgcccagaatacaacttccttcttcatcttgatcatgtggaattcaagcgctttcgttttttagtcattgaagcaatccttgctacggatcttaaaaagcattttgattttctcgcagaattcaatgccaaggcaaatgatgtaaatagtaatggcatagaatggagtaatgaaaatgatcgcctcttggtatgccaggtgtgcatcaaactggcagatataaatggcccagcaaaagttcgagacttgcatttgaaatggacagaaggcattgtcaatgaattttatgagcagggagatgaagaagcaaatcttggtctgcccatcagtccattcatggatcgttcttctcctcaactagcaaaactccaagaatcttttatcacccacatagtgggtcccctgtgtaactcctatgatgctgctggtttgctaccaggtcagtggttagaagcagaagaggataatgatactgaaagtggtgatgatgaagacggtgaagaattagatacagaagatgaagaaatggaaaacaatctaaatccaaaaccaccaagaaggaaaagcagacggcgaatattttgtcagctaatgcaccacctcactgaaaaccacaagatatggaaggaaatcgtagaggaagaagaaaaatgtaaagctgatgggaataaactgcaggtggagaattcctccttacctcaagcagatgagattcaggtaattgaagaggcagatgaagaggaatagcgacagtttgagtaaaagaaaagtcatattgaagaagcccagagggttgtgcccaggggcagaaatcattgcctagtgttcaccggctgactctcaactgaccattcccatgtggacaggccttaatactgtgagaggatccttgctctgctggcagtttcccactcctatgcactttcacaggaactagaaaactattcttaaaccaaaaataccatccgtgttgacccatgttgcagagcccttacttaaatccttcactggtgtatgaatactttgtcataatgctgctttgctgggtagtgagctcttatttttcactgggggtcagctataactaaaaactcaagtgacatatttcagttaccaaagtggccaggaactttttgcttttatgaaaatagattcatattgtatttcccagtgtgtcttttatgtctttgaatgttttggagaaaagtctatgcctgtctaaaaatgaatccagtgttgcctttctgagggatttctgctcaatgcaatacactgttcagtgctattctcccagctaggtttatccatgaaggactgagtgacctttgttgtatttaacaaaatccaggtgcatcaatttctgatgctttttactattgtgtattatctactatgtgtgttttatttctgctgagagtattcaggtttgccatggacatcagaagtttgaattccagtcttatcttatgttccatggctgaattttaaagctgtttaggtttaacaatgaagggatttattctttagtcaaaattgttgtttttactctagctcaggattcgtatttttaaagatttagttaatatgaacacagcacagatttgttagaagaaaaaaaatttgctgtaataccaaaactaacctcatcaaagatacagaaaaaaagaaatatagtgagccctaaaggacacatacattgaataaataattggaacatgtggttatctttagatccacatcttagctgtcatttgttcactctaaaactgatgttcatctttctgttaatttccctctgcctaaagactacatgacagaaatgacctatcactacttattatttctgaagcctaactgcaagactgatttctgagaacaagtaaagaactggaatacttatttttcatataaaaatctaaatgtgttaataaatcatttcatacaaaagtacattattaaataaccacattattaaaataattgcaagaaaatggaccatatttacaatgttttgtaaacttgctagtgtgtggatatgtaccctacttgtgaaatacatttgaagatataaagagcagccaaaatgatggcaaaatggtaggctaatattttctattattattggagaacatatcatattttggaatcatgcaattttgcacacagtgaaaccattaattttccaaggtaattcctttagaatatggtattggcatgcagtttcttacttatctagaatatttggcttatctgaaagatatcaatttaagatctctggaagtgttagaatttttgatccttcacagtgtcaatatttaatgaatcactaagctttatttattagacgtgttgagtgagtgctgagttccttgctgccacttttgttaccattgtcacacactatgtgtaaaccagtcccaccacttattactaataaaattttgactgataatttatatttgcacttacaatatatatatcctgtccttatatttctctagagtacattttccatcatgtttaagtgtatttctgctattatttcctctcctgcagaatacatacaagtgtatgtgtataaagtcatacatgtacaagcatgcatattgagattgaatcacatttccatactgtctgttattttattgggttttatattgggtttctttagtttatgttgttttctcaaaagcagcattttaaattacgaatactggacttattggatttaattataaatccaattactactggaaactcatttttacataatatagtccttaaattatttaacccttgctaagtaattgacatatgtaacaataactagcctaaagaaacccaaaaaagtatctctcccgagctgaaacttaaaaattcgtaagtgtaagaaagaatgtgagaatatattaaatgcacactgtaccattagatgaaatcttacttgagaaattgccataagccatattacagatcttactttgttactgaatcagattaatttcttgttataataattttcatcataaattttctatttttaaagccgctggtactagaaatattcttttaatgctatatctatgtacctactgacacatttttctccataaaagtacttttaaaaatta

SEQ ID NO: 18 - protein, 1112 aa, Homo sapiens
MRRDERDAKAMRSLQPPDGAGSPPESLRNGYVKSCVSPLRQDPPRGFFFHLCRFCNVELRPPPASPQQPRRCSPFCRARLSLGALAAFVLALLLGAEPESWAAGAAWLRTLLSVCSHSLSPLFSIACAFFFLTCFLTRTKRGPGPGRSCGSWWLLALPACCYLGDFLVWQWWSWPWGDGDAGSAAPHTPPEAAAGRLLLVLSCVGLLLTLAHPLRLRHCVLVLLLASFVWWVSFTSLGSLPSALRPLLSGLVGGAGCLLALGLDHFFQIREAPLHPRLSSAAEEKVPVIRPRRRSSCVSLGETAASYYGSCKIFRRPSLPCISREQMILWDWDLKQWYKPHYQNSGGGNGVDLSVLNEARNMVSDLLTDPSLPPQVISSLRSISSLMGAFSGSCRPKINPLTPFPGFYPCSEIEDPAEKGDRKLNKGLNRNSLPTPQLRRSSGTSGLLPVEQSSRWDRNNGKRPHQEFGISSQGCYLNGPFNSNLLTIPKQRSSSVSLTHHVGLRRAGVLSSLSPVNSSNHGPVSTGSLTNRSPIEFPDTADFLNKPSVILQRSLGNAPNTPDFYQQLRNSDSNLCNSCGHQMLKYVSTSESDGTDCCSGKSGEEENIFSKESFKLMETQQEEETEKKDSRKLFQEGDKWLTEEAQSEQQTNIEQEVSLDLILVEEYDSLIEKMSNWNFPIFELVEKMGEKSGRILSQVMYTLFQDTGLLEIFKIPTQQFMNYFRALENGYRDIPYHNRIHATDVLHAVWYLTTRPVPGLQQIHNGCGTGNETDSDGRINHGRIAYISSKSCSNPDESYGCLSSNIPALELMALYVAAAMHDYDHPGRTNAFLVATNAPQAVLYNDRSVLENHHAASAWNLYLSRPEYNFLLHLDHVEFKRFRFLVIEAILATDLKKHFDFLAEFNAKANDVNSNGIEWSNENDRLLVCQVCIKLADINGPAKVRDLHLKWTEGIVNEFYEQGDEEANLGLPISPFMDRSSPQLAKLQESFITHIVGPLCNSYDAAGLLPGQWLEAEEDNDTESGDDEDGEELDTEDEEMENNLNPKPPRRKSRRRIFCQLMHHLTENHKIWKEIVEEEEKCKADGNKLQVENSSLPQADEIQVIEEADEEE

SEQ ID NO: 19 - DNA, 4897 bp, Homo sapiens
  source 1..4897: mol_type = other DNA
gagcgccgccgggcactgagcagagctccaggcgccgaaaggaagctgcagagcccggcccgggggcgattggcccgcagcgcccccgggtctgtccccggggcgccatggccctaccgcggccgggcgcacccgcggggccctgggctcgctggcttgcgcgcagctgagcggggtgtaggttggaagggccagggccccctggggcgcaagtgggggccggcgccatggaacccccgaccgtcccctcggaaaggagcctgtctctgtcactgcccgggccccgggagggccaggccaccctgaagcctcccccgcagcacctgtggcggcagcctcggacccccatccgtatccagcagcgcggctactccgacagcgcggagcgcgccgagcgggagcggcagccgcaccggcccatagagcgcgccgatgccatggacaccagcgaccggcccggcctgcgcacgacccgcatgtcctggccctcgtccttccatggcactggcaccggcagcggcggcgcgggcggaggcagcagcaggcgcttcgaggcagagaatgggccgacaccatctcctggccgcagccccctggactcgcaggcgagcccaggactcgtgctgcacgccggggcggccaccagccagcgccgggagtccttcctgtaccgctcagacagcgactatgacatgtcacccaagaccatgtcccggaactcatcggtcaccagcgaggcgcacgctgaagacctcatcgtaacaccatttgctcaggtgctggccagcctccggagcgtccgtagcaacttctcactcctgaccaatgtgcccgttcccagtaacaagcggtccccgctgggcggccccacccctgtctgcaaggccacgctgtcagaagaaacgtgtcagcagttggcccgggagactctggaggagctggactggtgtctggagcagctggagaccatgcagacctatcgctctgtcagcgagatggcctcgcacaagttcaaaaggatgttgaaccgtgagctcacacacctgtcagaaatgagcaggtccggaaaccaggtctcagagtacatttccacaacattcctggacaaacagaatgaagtggagatcccatcacccacgatgaaggaacgagaaaaacagcaagcgccgcgaccaagaccctcccagccgcccccgccccctgtaccacacttacagcccatgtcccaaatcacagggttgaaaaagttgatgcatagtaacagcctgaacaactctaacattccccgatttggggtgaagaccgatcaagaagagctcctggcccaagaactggagaacctgaacaagtggggcctgaacatcttttgcgtgtcggattacgctggaggccgctcactcacctgcatcatgtacatgatattccaggagcgggacctgctgaagaaattccgcatccctgtggacacgatggtgacatacatgctgacgctggaggatcactaccacgctgacgtggcctaccataacagcctgcacgcagctgacgtgctgcagtccacccacgtactgctggccacgcctgcactagatgcagtgttcacggacctggagattctcgccgccctcttcgcggctgccatccacgatgtggatcaccctggggtctccaaccagttcctcatcaacaccaattcggagctggcgctcatgtacaacgatgagtcggtgctcgagaatcaccacctggccgtgggcttcaagctgctgcaggaggacaactgcgacatcttccagaacctcagcaagcgccagcggcagagcctacgcaagatggtcatcgacatggtgctggccacggacatgtccaagcacatgaccctcctggctgacctgaagaccatggtggagaccaagaaagtgaccagctcaggggtcctcctgctagataactactccgaccgcatccaggtcctccggaacatggtgcactgtgccgacctcagcaaccccaccaagccgctggagctgtaccgccagtggacagaccgcatcatggccgagttcttccagcagggtgaccgagagcgcgagcgtggcatggaaatcagccccatgtgtgacaagcacactgcctccgtggagaagtctcaggtgggttttattgactacattgtgcacccattgtgggagacctgggcggaccttgtccacccagatgcccaggagatcttggacactttggaggacaaccgggactggtactacagcgccatccggcagagcccatctccgccacccgaggaggagtcaagggggccaggccacccacccctgcctgacaagttccagtttgagctgacgctggaggaggaagaggaggaagaaatatcaatggcccagataccgtgcacagcccaagaggcattgactgcgcagggattgtcaggagtcgaggaagctctggatgcaaccatagcctgggaggcatccccggcccaggagtcgttggaagttatggcacaggaagcatccctggaggccgagctggaggcagtgtatttgacacagcaggcacagtccacaggcagtgcacctgtggctccggatgagttctcgtcccgggaggaattcgtggttgctgtaagccacagcagcccctctgccctggctcttcaaagcccccttctccctgcttggaggaccctgtctgtttcagagcatgccccgggcctcccgggcctcccctccacggcggccgaggtggaggcccaacgagagcaccaggctgccaagagggcttgcagtgcctgcgcagggacatttggggaggacacatccgcactcccagctcctggtggcggggggtcaggtggagaccctacctgatccccagacctctgtccctgttcccctccactcctcccctcactcccctgctcccccgaccacctcctcctctgcctcaaagactcttgtcctcttgtccctcctgagaaaaaagaaaacgaaaagtggggtttttttctgttttctttttttcccctttccccctgcccccacccacggggcctttttttggaggtgggggctggggaatgaggggctgaggtcccggaagggattttatttttttgaattttaattgtaacatttttagaaaaagaacaaaaaaagaaaaaaaaaagaaagaaacacagcaactgtagatgctcctgttcctggttcccgctttccacttccaaatccctcccctcaccttcccccactgccccccaagttccaggctcagtcttccagccgcctggggagtctctacctgggcccaagcaggtgtggggcctccttctgggcttttcttctgaatttagaggatttctagaacgtggtcaggaatagccattctaggcggggctggggccagggtggggggcagtcactgtgggaggtcccagctccagcccccctctggtttgctgcctcctctcccctctaaaaaagtcttccgcttgattttgcacaatcccggcgatactcctggcgatactgactagaaagtcagggagctgggggagctgttcactttaggatacgggggtggtatggaagggagcgttcacaccgccagcctcgggcctgggatttgaggagggccctagacctcctccactctccatcccctttcccttccactttgggttcactttgaattttctccgttttttggggcagtggctctgatccactcacccccccgccccccgccccacttctagctgcttctcctcttgtttctgccttaataattcccacggccacaggcaagggggttgcagtggccgcctgcaccttggatgaggcagggccaggcgcccagaacccccatcctggccgcacccccctttccagggtcctccggaccccaccttccacactctgatcacagcccccctaccttttgccctaggaggaagcaataatggtgtataccctcattctcattcctgggcagcccttccttccaccctggcaccaaaataatttctcctccatccgtaccttgcctagcctctccctctcccccagctagtccctgagcaatacggcagacagatgcaagaccatttttctccaagccatgggggactgtttggaaggaaagccccctctctccctcctcccctcgccctcggcctggttctgcagctggaccgacctcattcatcgcctgccccctacccaattctgagcacacggtactgtagcccccagttcctccctagccttccatccctctgtccaccccagggggaggtaaccccgcactcacactcccttgatgctgtctgtacagggttcatattttgtagcgaaagtcgtttttgtcccagccggcgatcggagtgggccttttctttctttttgttcattctttacctttttttcttttctttctttcttttttgtacatactgtaaggttggtttgtaaattattctacggaggcaaaaagggaaaataaaaacttgcccttccctggctgacccagtcgggaaggtagggaaggaggtctcccgttgggagagtctctgttcctgctgtattatacaaactgtaccatagtcctgggaaaagggtggactcaccgctgttgttttatgggaagtcgtgtcatcctaggggttggggctgggcagagcctgtcccctccccccttctccaggagccagggggtgactggagagacagacccacccccaagcagggctcctctccccagggtgagcacaggacctctgtaagctgcttgtgtattgtccactttgacgatcagtcattcggtccgttgatcaataatccttcgatcttgtctccaattaaaccgaggctttcaccga

SEQ ID NO: 20 - protein, 886 aa, Homo sapiens
MEPPTVPSERSLSLSLPGPREGQATLKPPPQHLWRQPRTPIRIQQRGYSDSAERAERERQPHRPIERADAMDTSDRPGLRTTRMSWPSSFHGTGTGSGGAGGGSSRRFEAENGPTPSPGRSPLDSQASPGLVLHAGAATSQRRESFLYRSDSDYDMSPKTMSRNSSVTSEAHAEDLIVTPFAQVLASLRSVRSNFSLLTNVPVPSNKRSPLGGPTPVCKATLSEETCQQLARETLEELDWCLEQLETMQTYRSVSEMASHKFKRMLNRELTHLSEMSRSGNQVSEYISTTFLDKQNEVEIPSPTMKEREKQQAPRPRPSQPPPPPVPHLQPMSQITGLKKLMHSNSLNNSNIPRFGVKTDQEELLAQELENLNKWGLNIFCVSDYAGGRSLTCIMYMIFQERDLLKKFRIPVDTMVTYMLTLEDHYHADVAYHNSLHAADVLQSTHVLLATPALDAVFTDLEILAALFAAAIHDVDHPGVSNQFLINTNSELALMYNDESVLENHHLAVGFKLLQEDNCDIFQNLSKRQRQSLRKMVIDMVLATDMSKHMTLLADLKTMVETKKVTSSGVLLLDNYSDRIQVLRNMVHCADLSNPTKPLELYRQWTDRIMAEFFQQGDRERERGMEISPMCDKHTASVEKSQVGFIDYIVHPLWETWADLVHPDAQEILDTLEDNRDWYYSAIRQSPSPPPEEESRGPGHPPLPDKFQFELTLEEEEEEEISMAQIPCTAQEALTAQGLSGVEEALDATIAWEASPAQESLEVMAQEASLEAELEAVYLTQQAQSTGSAPVAPDEFSSREEFVVAVSHSSPSALALQSPLLPAWRTLSVSEHAPGLPGLPSTAAEVEAQREHQAAKRACSACAGTFGEDTSALPAPGGGGSGGDPT

SEQ ID NO: 21 - DNA, 4608 bp, Homo sapiens
  source 1..4608: mol_type = other DNA
atggcgcggccgcgcggcctaggccgcatcccggagctgcaactggtggccttcccggtggcggtggcggctgaggacgaggcgttcctgcccgagcccctggccccgcgcgcgccccgccgcccgcgttcgccgccctcctcgcccgtcttcttcgccagcccgtccccaactttccgcagacgccttcggcttctccgcagctgccaggatttgggccgccaggcttgggctggggctggcttcgaggcagagaatgggccgacaccatctcctggccgcagccccctggactcgcaggcgagcccaggactcgtgctgcacgccggggcggccaccagccagcgccgggagtccttcctgtaccgctcagacagcgactatgacatgtcacccaagaccatgtcccggaactcatcggtcaccagcgaggcgcacgctgaagacctcatcgtaacaccatttgctcaggtgctggccagcctccggagcgtccgtagcaacttctcactcctgaccaatgtgcccgttcccagtaacaagcggtccccgctgggcggccccacccctgtctgcaaggccacgctgtcagaagaaacgtgtcagcagttggcccgggagactctggaggagctggactggtgtctggagcagctggagaccatgcagacctatcgctctgtcagcgagatggcctcgcacaagttcaaaaggatgttgaaccgtgagctcacacacctgtcagaaatgagcaggtccggaaaccaggtctcagagtacatttccacaacattcctggacaaacagaatgaagtggagatcccatcacccacgatgaaggaacgagaaaaacagcaagcgccgcgaccaagaccctcccagccgcccccgccccctgtaccacacttacagcccatgtcccaaatcacagggttgaaaaagttgatgcatagtaacagcctgaacaactctaacattccccgatttggggtgaagaccgatcaagaagagctcctggcccaagaactggagaacctgaacaagtggggcctgaacatcttttgcgtgtcggattacgctggaggccgctcactcacctgcatcatgtacatgatattccaggagcgggacctgctgaagaaattccgcatccctgtggacacgatggtgacatacatgctgacgctggaggatcactaccacgctgacgtggcctaccataacagcctgcacgcagctgacgtgctgcagtccacccacgtactgctggccacgcctgcactagatgcagtgttcacggacctggagattctcgccgccctcttcgcggctgccatccacgatgtggatcaccctggggtctccaaccagttcctcatcaacaccaattcggagctggcgctcatgtacaacgatgagtcggtgctcgagaatcaccacctggccgtgggcttcaagctgctgcaggaggacaactgcgacatcttccagaacctcagcaagcgccagcggcagagcctacgcaagatggtcatcgacatggtgctggccacggacatgtccaagcacatgaccctcctggctgacctgaagaccatggtggagaccaagaaagtgaccagctcaggggtcctcctgctagataactactccgaccgcatccaggtcctccggaacatggtgcactgtgccgacctcagcaaccccaccaagccgctggagctgtaccgccagtggacagaccgcatcatggccgagttcttccagcagggtgaccgagagcgcgagcgtggcatggaaatcagccccatgtgtgacaagcacactgcctccgtggagaagtctcaggtgggttttattgactacattgtgcacccattgtgggagacctgggcggaccttgtccacccagatgcccaggagatcttggacactttggaggacaaccgggactggtactacagcgccatccggcagagcccatctccgccacccgaggaggagtcaagggggccaggccacccacccctgcctgacaagttccagtttgagctgacgctggaggaggaagaggaggaagaaatatcaatggcccagataccgtgcacagcccaagaggcattgactgcgcagggattgtcaggagtcgaggaagctctggatgcaaccatagcctgggaggcatccccggcccaggagtcgttggaagttatggcacaggaagcatccctggaggccgagctggaggcagtgtatttgacacagcaggcacagtccacaggcagtgcacctgtggctccggatgagttctcgtcccgggaggaattcgtggttgctgtaagccacagcagcccctctgccctggctcttcaaagcccccttctccctgcttggaggaccctgtctgtttcagagcatgccccgggcctcccgggcctcccctccacggcggccgaggtggaggcccaacgagagcaccaggctgccaagagggcttgcagtgcctgcgcagggacatttggggaggacacatccgcactcccagctcctggtggcggggggtcaggtggagaccctacctgatccccagacctctgtccctgttcccctccactcctcccctcactcccctgctcccccgaccacctcctcctctgcctcaaagactcttgtcctcttgtccctcctgagaaaaaagaaaacgaaaagtggggtttttttctgttttctttttttcccctttccccctgcccccacccacggggcctttttttggaggtgggggctggggaatgaggggctgaggtcccggaagggattttatttttttgaattttaattgtaacatttttagaaaaagaacaaaaaaagaaaaaaaaaagaaagaaacacagcaactgtagatgctcctgttcctggttcccgctttccacttccaaatccctcccctcaccttcccccactgccccccaagttccaggctcagtcttccagccgcctggggagtctctacctgggcccaagcaggtgtggggcctccttctgggcttttcttctgaatttagaggatttctagaacgtggtcaggaatagccattctaggcggggctggggccagggtggggggcagtcactgtgggaggtcccagctccagcccccctctggtttgctgcctcctctcccctctaaaaaagtcttccgcttgattttgcacaatcccggcgatactcctggcgatactgactagaaagtcagggagctgggggagctgttcactttaggatacgggggtggtatggaagggagcgttcacaccgccagcctcgggcctgggatttgaggagggccctagacctcctccactctccatcccctttcccttccactttgggttcactttgaattttctccgttttttggggcagtggctctgatccactcacccccccgccccccgccccacttctagctgcttctcctcttgtttctgccttaataattcccacggccacaggcaagggggttgcagtggccgcctgcaccttggatgaggcagggccaggcgcccagaacccccatcctggccgcacccccctttccagggtcctccggaccccaccttccacactctgatcacagcccccctaccttttgccctaggaggaagcaataatggtgtataccctcattctcattcctgggcagcccttccttccaccctggcaccaaaataatttctcctccatccgtaccttgcctagcctctccctctcccccagctagtccctgagcaatacggcagacagatgcaagaccatttttctccaagccatgggggactgtttggaaggaaagccccctctctccctcctcccctcgccctcggcctggttctgcagctggaccgacctcattcatcgcctgccccctacccaattctgagcacacggtactgtagcccccagttcctccctagccttccatccctctgtccaccccagggggaggtaaccccgcactcacactcccttgatgctgtctgtacagggttcatattttgtagcgaaagtcgtttttgtcccagccggcgatcggagtgggccttttctttctttttgttcattctttacctttttttcttttctttctttcttttttgtacatactgtaaggttggtttgtaaattattctacggaggcaaaaagggaaaataaaaacttgcccttccctggctgacccagtcgggaaggtagggaaggaggtctcccgttgggagagtctctgttcctgctgtattatacaaactgtaccatagtcctgggaaaagggtggactcaccgctgttgttttatgggaagtcgtgtcatcctaggggttggggctgggcagagcctgtcccctccccccttctccaggagccagggggtgactggagagacagacccacccccaagcagggctcctctccccagggtgagcacaggacctctgtaagctgcttgtgtattgtccactttgacgatcagtcattcggtccgttgatcaataatccttcgatcttgtctccaattaaaccgaggctttcaccgataaaaaaaaaaaaaaa

SEQ ID NO: 22 - protein, 860 aa, Homo sapiens
MARPRGLGRIPELQLVAFPVAVAAEDEAFLPEPLAPRAPRRPRSPPSSPVFFASPSPTFRRRLRLLRSCQDLGRQAWAGAGFEAENGPTPSPGRSPLDSQASPGLVLHAGAATSQRRESFLYRSDSDYDMSPKTMSRNSSVTSEAHAEDLIVTPFAQVLASLRSVRSNFSLLTNVPVPSNKRSPLGGPTPVCKATLSEETCQQLARETLEELDWCLEQLETMQTYRSVSEMASHKFKRMLNRELTHLSEMSRSGNQVSEYISTTFLDKQNEVEIPSPTMKEREKQQAPRPRPSQPPPPPVPHLQPMSQITGLKKLMHSNSLNNSNIPRFGVKTDQEELLAQELENLNKWGLNIFCVSDYAGGRSLTCIMYMIFQERDLLKKFRIPVDTMVTYMLTLEDHYHADVAYHNSLHAADVLQSTHVLLATPALDAVFTDLEILAALFAAAIHDVDHPGVSNQFLINTNSELALMYNDESVLENHHLAVGFKLLQEDNCDIFQNLSKRQRQSLRKMVIDMVLATDMSKHMTLLADLKTMVETKKVTSSGVLLLDNYSDRIQVLRNMVHCADLSNPTKPLELYRQWTDRIMAEFFQQGDRERERGMEISPMCDKHTASVEKSQVGFIDYIVHPLWETWADLVHPDAQEILDTLEDNRDWYYSAIRQSPSPPPEEESRGPGHPPLPDKFQFELTLEEEEEEEISMAQIPCTAQEALTAQGLSGVEEALDATIAWEASPAQESLEVMAQEASLEAELEAVYLTQQAQSTGSAPVAPDEFSSREEFVVAVSHSSPSALALQSPLLPAWRTLSVSEHAPGLPGLPSTAAEVEAQREHQAAKRACSACAGTFGEDTSALPAPGGGGSGGDPT

SEQ ID NO: 23 - DNA, 4503 bp, Homo sapiens
  source 1..4503: mol_type = other DNA
atgcgctccggtgcagcgccccgggcccggccccggccccctgccctggcactgccccccacgggccccgagtccctgacccacttccccttcagcgatgaggacacccgtcggcaccctccgggcagatctgtcagcttcgaggcagagaatgggccgacaccatctcctggccgcagccccctggactcgcaggcgagcccaggactcgtgctgcacgccggggcggccaccagccagcgccgggagtccttcctgtaccgctcagacagcgactatgacatgtcacccaagaccatgtcccggaactcatcggtcaccagcgaggcgcacgctgaagacctcatcgtaacaccatttgctcaggtgctggccagcctccggagcgtccgtagcaacttctcactcctgaccaatgtgcccgttcccagtaacaagcggtccccgctgggcggccccacccctgtctgcaaggccacgctgtcagaagaaacgtgtcagcagttggcccgggagactctggaggagctggactggtgtctggagcagctggagaccatgcagacctatcgctctgtcagcgagatggcctcgcacaagttcaaaaggatgttgaaccgtgagctcacacacctgtcagaaatgagcaggtccggaaaccaggtctcagagtacatttccacaacattcctggacaaacagaatgaagtggagatcccatcacccacgatgaaggaacgagaaaaacagcaagcgccgcgaccaagaccctcccagccgcccccgccccctgtaccacacttacagcccatgtcccaaatcacagggttgaaaaagttgatgcatagtaacagcctgaacaactctaacattccccgatttggggtgaagaccgatcaagaagagctcctggcccaagaactggagaacctgaacaagtggggcctgaacatcttttgcgtgtcggattacgctggaggccgctcactcacctgcatcatgtacatgatattccaggagcgggacctgctgaagaaattccgcatccctgtggacacgatggtgacatacatgctgacgctggaggatcactaccacgctgacgtggcctaccataacagcctgcacgcagctgacgtgctgcagtccacccacgtactgctggccacgcctgcactagatgcagtgttcacggacctggagattctcgccgccctcttcgcggctgccatccacgatgtggatcaccctggggtctccaaccagttcctcatcaacaccaattcggagctggcgctcatgtacaacgatgagtcggtgctcgagaatcaccacctggccgtgggcttcaagctgctgcaggaggacaactgcgacatcttccagaacctcagcaagcgccagcggcagagcctacgcaagatggtcatcgacatggtgctggccacggacatgtccaagcacatgaccctcctggctgacctgaagaccatggtggagaccaagaaagtgaccagctcaggggtcctcctgctagataactactccgaccgcatccaggtcctccggaacatggtgcactgtgccgacctcagcaaccccaccaagccgctggagctgtaccgccagtggacagaccgcatcatggccgagttcttccagcagggtgaccgagagcgcgagcgtggcatggaaatcagccccatgtgtgacaagcacactgcctccgtggagaagtctcaggtgggttttattgactacattgtgcacccattgtgggagacctgggcggaccttgtccacccagatgcccaggagatcttggacactttggaggacaaccgggactggtactacagcgccatccggcagagcccatctccgccacccgaggaggagtcaagggggccaggccacccacccctgcctgacaagttccagtttgagctgacgctggaggaggaagaggaggaagaaatatcaatggcccagataccgtgcacagcccaagaggcattgactgcgcagggattgtcaggagtcgaggaagctctggatgcaaccatagcctgggaggcatccccggcccaggagtcgttggaagttatggcacaggaagcatccctggaggccgagctggaggcagtgtatttgacacagcaggcacagtccacaggcagtgcacctgtggctccggatgagttctcgtcccgggaggaattcgtggttgctgtaagccacagcagcccctctgccctggctcttcaaagcccccttctccctgcttggaggaccctgtctgtttcagagcatgccccgggcctcccgggcctcccctccacggcggccgaggtggaggcccaacgagagcaccaggctgccaagagggcttgcagtgcctgcgcagggacatttggggaggacacatccgcactcccagctcctggtggcggggggtcaggtggagaccctacctgatccccagacctctgtccctgttcccctccactcctcccctcactcccctgctcccccgaccacctcctcctctgcctcaaagactcttgtcctcttgtccctcctgagaaaaaagaaaacgaaaagtggggtttttttctgttttctttttttcccctttccccctgcccccacccacggggcctttttttggaggtgggggctggggaatgaggggctgaggtcccggaagggattttatttttttgaattttaattgtaacatttttagaaaaagaacaaaaaaagaaaaaaaaaagaaagaaacacagcaactgtagatgctcctgttcctggttcccgctttccacttccaaatccctcccctcaccttcccccactgccccccaagttccaggctcagtcttccagccgcctggggagtctctacctgggcccaagcaggtgtggggcctccttctgggcttttcttctgaatttagaggatttctagaacgtggtcaggaatagccattctaggcggggctggggccagggtggggggcagtcactgtgggaggtcccagctccagcccccctctggtttgctgcctcctctcccctctaaaaaagtcttccgcttgattttgcacaatcccggcgatactcctggcgatactgactagaaagtcagggagctgggggagctgttcactttaggatacgggggtggtatggaagggagcgttcacaccgccagcctcgggcctgggatttgaggagggccctagacctcctccactctccatcccctttcccttccactttgggttcactttgaattttctccgttttttggggcagtggctctgatccactcacccccccgccccccgccccacttctagctgcttctcctcttgtttctgccttaataattcccacggccacaggcaagggggttgcagtggccgcctgcaccttggatgaggcagggccaggcgcccagaacccccatcctggccgcacccccctttccagggtcctccggaccccaccttccacactctgatcacagcccccctaccttttgccctaggaggaagcaataatggtgtataccctcattctcattcctgggcagcccttccttccaccctggcaccaaaataatttctcctccatccgtaccttgcctagcctctccctctcccccagctagtccctgagcaatacggcagacagatgcaagaccatttttctccaagccatgggggactgtttggaaggaaagccccctctctccctcctcccctcgccctcggcctggttctgcagctggaccgacctcattcatcgcctgccccctacccaattctgagcacacggtactgtagcccccagttcctccctagccttccatccctctgtccaccccagggggaggtaaccccgcactcacactcccttgatgctgtctgtacagggttcatattttgtagcgaaagtcgtttttgtcccagccggcgatcggagtgggccttttctttctttttgttcattctttacctttttttcttttctttctttcttttttgtacatactgtaaggttggtttgtaaattattctacggaggcaaaaagggaaaataaaaacttgcccttccctggctgacccagtcgggaaggtagggaaggaggtctcccgttgggagagtctctgttcctgctgtattatacaaactgtaccatagtcctgggaaaagggtggactcaccgctgttgttttatgggaagtcgtgtcatcctaggggttggggctgggcagagcctgtcccctccccccttctccaggagccagggggtgactggagagacagacccacccccaagcagggctcctctccccagggtgagcacaggacctctgtaagctgcttgtgtattgtccactttgacgatcagtcattcggtccgttgatcaataatccttcgatcttgtctccaattaaaccgaggctttcaccgataaaaaaaaaaaaaaa

SEQ ID NO: 24 - protein, 825 aa, Homo sapiens
MRSGAAPRARPRPPALALPPTGPESLTHFPFSDEDTRRHPPGRSVSFEAENGPTPSPGRSPLDSQASPGLVLHAGAATSQRRESFLYRSDSDYDMSPKTMSRNSSVTSEAHAEDLIVTPFAQVLASLRSVRSNFSLLTNVPVPSNKRSPLGGPTPVCKATLSEETCQQLARETLEELDWCLEQLETMQTYRSVSEMASHKFKRMLNRELTHLSEMSRSGNQVSEYISTTFLDKQNEVEIPSPTMKEREKQQAPRPRPSQPPPPPVPHLQPMSQITGLKKLMHSNSLNNSNIPRFGVKTDQEELLAQELENLNKWGLNIFCVSDYAGGRSLTCIMYMIFQERDLLKKFRIPVDTMVTYMLTLEDHYHADVAYHNSLHAADVLQSTHVLLATPALDAVFTDLEILAALFAAAIHDVDHPGVSNQFLINTNSELALMYNDESVLENHHLAVGFKLLQEDNCDIFQNLSKRQRQSLRKMVIDMVLATDMSKHMTLLADLKTMVETKKVTSSGVLLLDNYSDRIQVLRNMVHCADLSNPTKPLELYRQWTDRIMAEFFQQGDRERERGMEISPMCDKHTASVEKSQVGFIDYIVHPLWETWADLVHPDAQEILDTLEDNRDWYYSAIRQSPSPPPEEESRGPGHPPLPDKFQFELTLEEEEEEEISMAQIPCTAQEALTAQGLSGVEEALDATIAWEASPAQESLEVMAQEASLEAELEAVYLTQQAQSTGSAPVAPDEFSSREEFVVAVSHSSPSALALQSPLLPAWRTLSVSEHAPGLPGLPSTAAEVEAQREHQAAKRACSACAGTFGEDTSALPAPGGGGSGGDPT

SEQ ID NO: 25 - DNA, 4285 bp, Homo sapiens
  source 1..4285: mol_type = other DNA
acacacacgggtgcacacacagagctccgcagcctcctcctgggacccttgccctgcccccctcccatgggcacggaccccccaccgcctccacccactgccgcgggggggcccgttggggcccagggctggcgggccatgtaaccagggctgctgctgggagcgcggaggggaagggagcccccagccctgctgggccggcccaggcccctccgcggctcccccttccactacccacctgcccggcaccccctccccagtggttgttaaccccgggactccccaagcccagcctctgtgtgcagcagccccaggcgggctaagtctccaagatgcccttggtggatttcttctgcgagacctgctctaagccttggctggtgggctggtgggaccagttcaaaaggatgttgaaccgtgagctcacacacctgtcagaaatgagcaggtccggaaaccaggtctcagagtacatttccacaacattcctggacaaacagaatgaagtggagatcccatcacccacgatgaaggaacgagaaaaacagcaagcgccgcgaccaagaccctcccagccgcccccgccccctgtaccacacttacagcccatgtcccaaatcacagggttgaaaaagttgatgcatagtaacagcctgaacaactctaacattccccgatttggggtgaagaccgatcaagaagagctcctggcccaagaactggagaacctgaacaagtggggcctgaacatcttttgcgtgtcggattacgctggaggccgctcactcacctgcatcatgtacatgatattccaggagcgggacctgctgaagaaattccgcatccctgtggacacgatggtgacatacatgctgacgctggaggatcactaccacgctgacgtggcctaccataacagcctgcacgcagctgacgtgctgcagtccacccacgtactgctggccacgcctgcactagatgcagtgttcacggacctggagattctcgccgccctcttcgcggctgccatccacgatgtggatcaccctggggtctccaaccagttcctcatcaacaccaattcggagctggcgctcatgtacaacgatgagtcggtgctcgagaatcaccacctggccgtgggcttcaagctgctgcaggaggacaactgcgacatcttccagaacctcagcaagcgccagcggcagagcctacgcaagatggtcatcgacatggtgctggccacggacatgtccaagcacatgaccctcctggctgacctgaagaccatggtggagaccaagaaagtgaccagctcaggggtcctcctgctagataactactccgaccgcatccaggtcctccggaacatggtgcactgtgccgacctcagcaaccccaccaagccgctggagctgtaccgccagtggacagaccgcatcatggccgagttcttccagcagggtgaccgagagcgcgagcgtggcatggaaatcagccccatgtgtgacaagcacactgcctccgtggagaagtctcaggtgggttttattgactacattgtgcacccattgtgggagacctgggcggaccttgtccacccagatgcccaggagatcttggacactttggaggacaaccgggactggtactacagcgccatccggcagagcccatctccgccacccgaggaggagtcaagggggccaggccacccacccctgcctgacaagttccagtttgagctgacgctggaggaggaagaggaggaagaaatatcaatggcccagataccgtgcacagcccaagaggcattgactgcgcagggattgtcaggagtcgaggaagctctggatgcaaccatagcctgggaggcatccccggcccaggagtcgttggaagttatggcacaggaagcatccctggaggccgagctggaggcagtgtatttgacacagcaggcacagtccacaggcagtgcacctgtggctccggatgagttctcgtcccgggaggaattcgtggttgctgtaagccacagcagcccctctgccctggctcttcaaagcccccttctccctgcttggaggaccctgtctgtttcagagcatgccccgggcctcccgggcctcccctccacggcggccgaggtggaggcccaacgagagcaccaggctgccaagagggcttgcagtgcctgcgcagggacatttggggaggacacatccgcactcccagctcctggtggcggggggtcaggtggagaccctacctgatccccagacctctgtccctgttcccctccactcctcccctcactcccctgctcccccgaccacctcctcctctgcctcaaagactcttgtcctcttgtccctcctgagaaaaaagaaaacgaaaagtggggtttttttctgttttctttttttcccctttccccctgcccccacccacggggcctttttttggaggtgggggctggggaatgaggggctgaggtcccggaagggattttatttttttgaattttaattgtaacatttttagaaaaagaacaaaaaaagaaaaaaaaaagaaagaaacacagcaactgtagatgctcctgttcctggttcccgctttccacttccaaatccctcccctcaccttcccccactgccccccaagttccaggctcagtcttccagccgcctggggagtctctacctgggcccaagcaggtgtggggcctccttctgggcttttcttctgaatttagaggatttctagaacgtggtcaggaatagccattctaggcggggctggggccagggtggggggcagtcactgtgggaggtcccagctccagcccccctctggtttgctgcctcctctcccctctaaaaaagtcttccgcttgattttgcacaatcccggcgatactcctggcgatactgactagaaagtcagggagctgggggagctgttcactttaggatacgggggtggtatggaagggagcgttcacaccgccagcctcgggcctgggatttgaggagggccctagacctcctccactctccatcccctttcccttccactttgggttcactttgaattttctccgttttttggggcagtggctctgatccactcacccccccgccccccgccccacttctagctgcttctcctcttgtttctgccttaataattcccacggccacaggcaagggggttgcagtggccgcctgcaccttggatgaggcagggccaggcgcccagaacccccatcctggccgcacccccctttccagggtcctccggaccccaccttccacactctgatcacagcccccctaccttttgccctaggaggaagcaataatggtgtataccctcattctcattcctgggcagcccttccttccaccctggcaccaaaataatttctcctccatccgtaccttgcctagcctctccctctcccccagctagtccctgagcaatacggcagacagatgcaagaccatttttctccaagccatgggggactgtttggaaggaaagccccctctctccctcctcccctcgccctcggcctggttctgcagctggaccgacctcattcatcgcctgccccctacccaattctgagcacacggtactgtagcccccagttcctccctagccttccatccctctgtccaccccagggggaggtaaccccgcactcacactcccttgatgctgtctgtacagggttcatattttgtagcgaaagtcgtttttgtcccagccggcgatcggagtgggccttttctttctttttgttcattctttacctttttttcttttctttctttcttttttgtacatactgtaaggttggtttgtaaattattctacggaggcaaaaagggaaaataaaaacttgcccttccctggctgacccagtcgggaaggtagggaaggaggtctcccgttgggagagtctctgttcctgctgtattatacaaactgtaccatagtcctgggaaaagggtggactcaccgctgttgttttatgggaagtcgtgtcatcctaggggttggggctgggcagagcctgtcccctccccccttctccaggagccagggggtgactggagagacagacccacccccaagcagggctcctctccccagggtgagcacaggacctctgtaagctgcttgtgtattgtccactttgacgatcagtcattcggtccgttgatcaataatccttcgatcttgtctccaattaaaccgaggctttcaccga

SEQ ID NO: 26 - protein, 647 aa, Homo sapiens
MPLVDFFCETCSKPWLVGWWDQFKRMLNRELTHLSEMSRSGNQVSEYISTTFLDKQNEVEIPSPTMKEREKQQAPRPRPSQPPPPPVPHLQPMSQITGLKKLMHSNSLNNSNIPRFGVKTDQEELLAQELENLNKWGLNIFCVSDYAGGRSLTCIMYMIFQERDLLKKFRIPVDTMVTYMLTLEDHYHADVAYHNSLHAADVLQSTHVLLATPALDAVFTDLEILAALFAAAIHDVDHPGVSNQFLINTNSELALMYNDESVLENHHLAVGFKLLQEDNCDIFQNLSKRQRQSLRKMVIDMVLATDMSKHMTLLADLKTMVETKKVTSSGVLLLDNYSDRIQVLRNMVHCADLSNPTKPLELYRQWTDRIMAEFFQQGDRERERGMEISPMCDKHTASVEKSQVGFIDYIVHPLWETWADLVHPDAQEILDTLEDNRDWYYSAIRQSPSPPPEEESRGPGHPPLPDKFQFELTLEEEEEEEISMAQIPCTAQEALTAQGLSGVEEALDATIAWEASPAQESLEVMAQEASLEAELEAVYLTQQAQSTGSAPVAPDEFSSREEFVVAVSHSSPSALALQSPLLPAWRTLSVSEHAPGLPGLPSTAAEVEAQREHQAAKRACSACAGTFGEDTSALPAPGGGGSGGDPT

SEQ ID NO: 27 - DNA, 4688 bp, Homo sapiens
  source 1..4688: mol_type = other DNA
cgtcacgccccaggagaggcaataggaggccctggccctgccgacatggccaccgcagtcccaacggcgcgctaggttggcgagatgaagaggagtcgcagtgccctgtccgtggcagggaccggggacgagaggtcgagggagacccccgaatccgaccgtgccaacatgctgggggccgacctgcgtcgccctcgccgccgcctctcgtccggtcctggcctgggctgggcccagcctgagccctcggaccctggggtccctctgccgccacggcccaccaccctgccgctgctgatcccaccgcggatttccatcaccagggccgagaacgacagcttcgaggcagagaatgggccgacaccatctcctggccgcagccccctggactcgcaggcgagcccaggactcgtgctgcacgccggggcggccaccagccagcgccgggagtccttcctgtaccgctcagacagcgactatgacatgtcacccaagaccatgtcccggaactcatcggtcaccagcgaggcgcacgctgaagacctcatcgtaacaccatttgctcaggtgctggccagcctccggagcgtccgtagcaacttctcactcctgaccaatgtgcccgttcccagtaacaagcggtccccgctgggcggccccacccctgtctgcaaggccacgctgtcagaagaaacgtgtcagcagttggcccgggagactctggaggagctggactggtgtctggagcagctggagaccatgcagacctatcgctctgtcagcgagatggcctcgcacaagttcaaaaggatgttgaaccgtgagctcacacacctgtcagaaatgagcaggtccggaaaccaggtctcagagtacatttccacaacattcctggacaaacagaatgaagtggagatcccatcacccacgatgaaggaacgagaaaaacagcaagcgccgcgaccaagaccctcccagccgcccccgccccctgtaccacacttacagcccatgtcccaaatcacagggttgaaaaagttgatgcatagtaacagcctgaacaactctaacattccccgatttggggtgaagaccgatcaagaagagctcctggcccaagaactggagaacctgaacaagtggggcctgaacatcttttgcgtgtcggattacgctggaggccgctcactcacctgcatcatgtacatgatattccaggagcgggacctgctgaagaaattccgcatccctgtggacacgatggtgacatacatgctgacgctggaggatcactaccacgctgacgtggcctaccataacagcctgcacgcagctgacgtgctgcagtccacccacgtactgctggccacgcctgcactagatgcagtgttcacggacctggagattctcgccgccctcttcgcggctgccatccacgatgtggatcaccctggggtctccaaccagttcctcatcaacaccaattcggagctggcgctcatgtacaacgatgagtcggtgctcgagaatcaccacctggccgtgggcttcaagctgctgcaggaggacaactgcgacatcttccagaacctcagcaagcgccagcggcagagcctacgcaagatggtcatcgacatggtgctggccacggacatgtccaagcacatgaccctcctggctgacctgaagaccatggtggagaccaagaaagtgaccagctcaggggtcctcctgctagataactactccgaccgcatccaggtcctccggaacatggtgcactgtgccgacctcagcaaccccaccaagccgctggagctgtaccgccagtggacagaccgcatcatggccgagttcttccagcagggtgaccgagagcgcgagcgtggcatggaaatcagccccatgtgtgacaagcacactgcctccgtggagaagtctcaggtgggttttattgactacattgtgcacccattgtgggagacctgggcggaccttgtccacccagatgcccaggagatcttggacactttggaggacaaccgggactggtactacagcgccatccggcagagcccatctccgccacccgaggaggagtcaagggggccaggccacccacccctgcctgacaagttccagtttgagctgacgctggaggaggaagaggaggaagaaatatcaatggcccagataccgtgcacagcccaagaggcattgactgcgcagggattgtcaggagtcgaggaagctctggatgcaaccatagcctgggaggcatccccggcccaggagtcgttggaagttatggcacaggaagcatccctggaggccgagctggaggcagtgtatttgacacagcaggcacagtccacaggcagtgcacctgtggctccggatgagttctcgtcccgggaggaattcgtggttgctgtaagccacagcagcccctctgccctggctcttcaaagcccccttctccctgcttggaggaccctgtctgtttcagagcatgccccgggcctcccgggcctcccctccacggcggccgaggtggaggcccaacgagagcaccaggctgccaagagggcttgcagtgcctgcgcagggacatttggggaggacacatccgcactcccagctcctggtggcggggggtcaggtggagaccctacctgatccccagacctctgtccctgttcccctccactcctcccctcactcccctgctcccccgaccacctcctcctctgcctcaaagactcttgtcctcttgtccctcctgagaaaaaagaaaacgaaaagtggggtttttttctgttttctttttttcccctttccccctgcccccacccacggggcctttttttggaggtgggggctggggaatgaggggctgaggtcccggaagggattttatttttttgaattttaattgtaacatttttagaaaaagaacaaaaaaagaaaaaaaaaagaaagaaacacagcaactgtagatgctcctgttcctggttcccgctttccacttccaaatccctcccctcaccttcccccactgccccccaagttccaggctcagtcttccagccgcctggggagtctctacctgggcccaagcaggtgtggggcctccttctgggcttttcttctgaatttagaggatttctagaacgtggtcaggaatagccattctaggcggggctggggccagggtggggggcagtcactgtgggaggtcccagctccagcccccctctggtttgctgcctcctctcccctctaaaaaagtcttccgcttgattttgcacaatcccggcgatactcctggcgatactgactagaaagtcagggagctgggggagctgttcactttaggatacgggggtggtatggaagggagcgttcacaccgccagcctcgggcctgggatttgaggagggccctagacctcctccactctccatcccctttcccttccactttgggttcactttgaattttctccgttttttggggcagtggctctgatccactcacccccccgccccccgccccacttctagctgcttctcctcttgtttctgccttaataattcccacggccacaggcaagggggttgcagtggccgcctgcaccttggatgaggcagggccaggcgcccagaacccccatcctggccgcacccccctttccagggtcctccggaccccaccttccacactctgatcacagcccccctaccttttgccctaggaggaagcaataatggtgtataccctcattctcattcctgggcagcccttccttccaccctggcaccaaaataatttctcctccatccgtaccttgcctagcctctccctctcccccagctagtccctgagcaatacggcagacagatgcaagaccatttttctccaagccatgggggactgtttggaaggaaagccccctctctccctcctcccctcgccctcggcctggttctgcagctggaccgacctcattcatcgcctgccccctacccaattctgagcacacggtactgtagcccccagttcctccctagccttccatccctctgtccaccccagggggaggtaaccccgcactcacactcccttgatgctgtctgtacagggttcatattttgtagcgaaagtcgtttttgtcccagccggcgatcggagtgggccttttctttctttttgttcattctttacctttttttcttttctttctttcttttttgtacatactgtaaggttggtttgtaaattattctacggaggcaaaaagggaaaataaaaacttgcccttccctggctgacccagtcgggaaggtagggaaggaggtctcccgttgggagagtctctgttcctgctgtattatacaaactgtaccatagtcctgggaaaagggtggactcaccgctgttgttttatgggaagtcgtgtcatcctaggggttggggctgggcagagcctgtcccctccccccttctccaggagccagggggtgactggagagacagacccacccccaagcagggctcctctccccagggtgagcacaggacctctgtaagctgcttgtgtattgtccactttgacgatcagtcattcggtccgttgatcaataatccttcgatcttgtctccaattaaaccgaggctttcaccga

SEQ ID NO: 28 - protein, 864 aa, Homo sapiens
MKRSRSALSVAGTGDERSRETPESDRANMLGADLRRPRRRLSSGPGLGWAQPEPSDPGVPLPPRPTTLPLLIPPRISITRAENDSFEAENGPTPSPGRSPLDSQASPGLVLHAGAATSQRRESFLYRSDSDYDMSPKTMSRNSSVTSEAHAEDLIVTPFAQVLASLRSVRSNFSLLTNVPVPSNKRSPLGGPTPVCKATLSEETCQQLARETLEELDWCLEQLETMQTYRSVSEMASHKFKRMLNRELTHLSEMSRSGNQVSEYISTTFLDKQNEVEIPSPTMKEREKQQAPRPRPSQPPPPPVPHLQPMSQITGLKKLMHSNSLNNSNIPRFGVKTDQEELLAQELENLNKWGLNIFCVSDYAGGRSLTCIMYMIFQERDLLKKFRIPVDTMVTYMLTLEDHYHADVAYHNSLHAADVLQSTHVLLATPALDAVFTDLEILAALFAAAIHDVDHPGVSNQFLINTNSELALMYNDESVLENHHLAVGFKLLQEDNCDIFQNLSKRQRQSLRKMVIDMVLATDMSKHMTLLADLKTMVETKKVTSSGVLLLDNYSDRIQVLRNMVHCADLSNPTKPLELYRQWTDRIMAEFFQQGDRERERGMEISPMCDKHTASVEKSQVGFIDYIVHPLWETWADLVHPDAQEILDTLEDNRDWYYSAIRQSPSPPPEEESRGPGHPPLPDKFQFELTLEEEEEEEISMAQIPCTAQEALTAQGLSGVEEALDATIAWEASPAQESLEVMAQEASLEAELEAVYLTQQAQSTGSAPVAPDEFSSREEFVVAVSHSSPSALALQSPLLPAWRTLSVSEHAPGLPGLPSTAAEVEAQREHQAAKRACSACAGTFGEDTSALPAPGGGGSGGDPT

SEQ ID NO: 29 - DNA, 4531 bp, Homo sapiens
  source 1..4531: mol_type = other DNA
agaggacgagagaagagctgaggggcgcgtcgccagcgcctgtgtctccctggcgcgggttccccaggctagcccgctggcccgtccgcgcgcgcgcccccggcccgcgcgccccttcccggggctcctggcctcgcctcagcggctgcaggctcttcgtcgcgggccgggctgcacgcgagcgccctccgggcagactttcgtcccccacccccgggagcgcggaaggctcactcgcagcgcatggtctacccgcgccgggcggagccccggcgtccagagcgctgcggccgcggcggtgcagcagaggcgcctcgggcaggaggagggcggcttctgcgagggcagcctgaggtattaaaaagtgtcagcaaactgcattgaataacagacatcctaagaggggatattttccacctctataatgaagaaaagcaggagtgtgatgacggtgatggctgatgataatgttaaagattattttgaatgtagcttgagtaaatcctacagttcttccagtaacacacttgggatcgacctctggagagggagaaggtgttgctcaggaaacttacagttaccaccactgtctcaaagacagagtgaaagggcaaggactcctgagggagatggtatttccaggccgaccacactgcctttgacaacgcttccaagcattgctattacaactgtaagccaggagtgctttgatgtggaaaatggcccttccccaggtcggagtccactggatccccaggccagctcttccgctgggctggtacttcacgccacctttcctgggcacagccagcgcagagagtcatttctctacagatcagacagcgactatgacttgtcaccaaaggcgatgtcgagaaactcttctcttccaagcgagcaacacggcgatgacttgattgtaactccttttgcccaggtccttgccagcttgcgaagtgtgagaaacaacttcactatactgacaaaccttcatggtacatctaacaagaggtccccagctgctagtcagcctcctgtctccagagtcaacccacaagaagaatcttatcaaaaattagcaatggaaacgctggaggaattagactggtgtttagaccagctagagaccatacagacctaccggtctgtcagtgagatggcttctaacaagttcaaaagaatgctgaaccgggagctgacacacctctcagagatgagccgatcagggaaccaggtgtctgaatacatttcaaatactttcttagacaagcagaatgatgtggagatcccatctcctacccagaaagacagggagaaaaagaaaaagcagcagctcatgacccagataagtggagtgaagaaattaatgcatagttcaagcctaaacaatacaagcatctcacgctttggagtcaacactgaaaatgaagatcacctggccaaggagctggaagacctgaacaaatggggtcttaacatctttaatgtggctggatattctcacaatagacccctaacatgcatcatgtatgctatattccaggaaagagacctcctaaagacattcagaatctcatctgacacatttataacctacatgatgactttagaagaccattaccattctgacgtggcatatcacaacagcctgcacgctgctgatgtagcccagtcgacccatgttctcctttctacaccagcattagacgctgtcttcacagatttggagatcctggctgccatttttgcagctgccatccatgacgttgatcatcctggagtctccaatcagtttctcatcaacacaaattcagaacttgctttgatgtataatgatgaatctgtgttggaaaatcatcaccttgctgtgggtttcaaactgctgcaagaagaacactgtgacatcttcatgaatctcaccaagaagcagcgtcagacactcaggaagatggttattgacatggtgttagcaactgatatgtctaaacatatgagcctgctggcagacctgaagacaatggtagaaacgaagaaagttacaagttcaggcgttcttctcctagacaactataccgatcgcattcaggtccttcgcaacatggtacactgtgcagacctgagcaaccccaccaagtccttggaattgtatcggcaatggacagaccgcatcatggaggaatttttccagcagggagacaaagagcgggagaggggaatggaaattagcccaatgtgtgataaacacacagcttctgtggaaaaatcccaggttggtttcatcgactacattgtccatccattgtgggagacatgggcagatttggtacagcctgatgctcaggacattctcgataccttagaagataacaggaactggtatcagagcatgatacctcaaagtccctcaccaccactggacgagcagaacagggactgccagggtctgatggagaagtttcagtttgaactgactctcgatgaggaagattctgaaggacctgagaaggagggagagggacacagctatttcagcagcacaaagacgctttgtgtgattgatccagaaaacagagattccctgggagagactgacatagacattgcaacagaagacaagtcccccgtggatacataatccccctctccctgtggagatgaacattctatccttgatgagcatgccagctatgtggtagggccagcccaccatgggggccaagacctgcacaggacaagggccacctggcctttcagttacttgagtttggagtcagaaagcaagaccaggaagcaaatagcagctcaggaaatcccacggttgacttgccttgatggcaagcttggtggagagggctgaagctgttgctgggggccgattctgatcaagacacatggcttgaaaatggaagacacaaaactgagagatcattctgcactaagtttcgggaacttatccccgacagtgactgaactcactgactaataacttcatttatgaatcttctcacttgtccctttgtctgccaacctgtgtgccttttttgtaaaacattttcatgtctttaaaatgcctgttgaatacctggagtttagtatcaacttctacacagataagctttcaaagttgacaaacttttttgactctttctggaaaagggaaagaaaatagtcttccttctttcttgggcaatatccttcactttactacagttacttttgcaaacagacagaaaggatacacttctaaccacattttacttccttcccctgttgtccagtccaactccacagtcactcttaaaacttctctctgtttgcctgcctccaacagtacttttaactttttgctgtaaacagaataaaattgaacaaattagggggtagaaaggagcagtggtgtcgttcaccgtgagagtctgcatagaactcagcagtgtgccctgctgtgtcttggaccctgccccccacaggagttgtacagtccctggccctgttccctacctcctctcttcaccccgttaggctgttttcaatgtaatgctgccgtccttctcttgcactgccttctgcgctaacacctccattcctgtttataaccgtgtatttattacttaatgtatataatgtaatgttttgtaagttattaatttatatatctaacattgcctgccaatggtggtgttaaatttgtgtagaaaactctgcctaagagttacgactttttcttgtaatgttttgtattgtgtattatataacccaaacgtcacttagtagagacatatggcccccttggcagagaggacaggggtgggcttttgttcaaagggtctgccctttccctgcctgagttgctacttctgcacaacccctttatgaaccagttttggaaacaatattctcacattagatactaaatggtttatactgagcttttacttttgtatagcttgataggggcagggggcaatgggatgtagtttttacccaggttctatccaaatctatgtgggcatgagttgggttataactggatcctactatcattgtggctttggttcaaaaggaaacactacatttgctcacagatgattcttctgaatgctcccgaactactgactttgaagaggtagcctcctgcctgccattaagcaggaatgtcatgttccagttcattacaaaagaaaacaataaaacaatgtgaatttttataataaaatgtgaactgatgtagcaaattacgcaaatgtgaagcctcttctgataacacttgttaggcctcttactgatgtcagtttcagtttgtaaaatatgtttcatgctttcagttcagcattgtgactcagtaattacagaaaatggcacaaatgtgcatgaccaatgtatgtctatgaacactgcattgtttcaggtggacattttatcattttcaaatgtttctcacaatgtatgttatagtattattattatatattgtgttcaaatgcattctaaagagacttttatatgaggtgaataaagaaaagcatgatta

SEQ ID NO: 30 - protein, 736 aa, Homo sapiens
MKKSRSVMTVMADDNVKDYFECSLSKSYSSSSNTLGIDLWRGRRCCSGNLQLPPLSQRQSERARTPEGDGISRPTTLPLTTLPSIAITTVSQECFDVENGPSPGRSPLDPQASSSAGLVLHATFPGHSQRRESFLYRSDSDYDLSPKAMSRNSSLPSEQHGDDLIVTPFAQVLASLRSVRNNFTILTNLHGTSNKRSPAASQPPVSRVNPQEESYQKLAMETLEELDWCLDQLETIQTYRSVSEMASNKFKRMLNRELTHLSEMSRSGNQVSEYISNTFLDKQNDVEIPSPTQKDREKKKKQQLMTQISGVKKLMHSSSLNNTSISRFGVNTENEDHLAKELEDLNKWGLNIFNVAGYSHNRPLTCIMYAIFQERDLLKTFRISSDTFITYMMTLEDHYHSDVAYHNSLHAADVAQSTHVLLSTPALDAVFTDLEILAAIFAAAIHDVDHPGVSNQFLINTNSELALMYNDESVLENHHLAVGFKLLQEEHCDIFMNLTKKQRQTLRKMVIDMVLATDMSKHMSLLADLKTMVETKKVTSSGVLLLDNYTDRIQVLRNMVHCADLSNPTKSLELYRQWTDRIMEEFFQQGDKERERGMEISPMCDKHTASVEKSQVGFIDYIVHPLWETWADLVQPDAQDILDTLEDNRNWYQSMIPQSPSPPLDEQNRDCQGLMEKFQFELTLDEEDSEGPEKEGEGHSYFSSTKTLCVIDPENRDSLGETDIDIATEDKSPVDT

SEQ ID NO: 31 - DNA, 3884 bp, Homo sapiens
  source 1..3884: mol_type = other DNA
atcacataccctaaagaaccctgggatgactaaggcagagagagtctgagaaaactctttggtgcttctgcctttagttttaggacacatttatgcagatgagcttataagagaccgttccctccgccttcttcctcagaggaagtttcttggtagatcaccgacacctcatccaggcggggggttggggggaaacttggcaccagccatcccaggcagagcaccactgtgatttgttctcctggtggagagagctggaaggaaggagccagcgtgcaaataatgaaggagcacgggggcaccttcagtagcaccggaatcagcggtggtagcggtgactctgctatggacagcctgcagccgctccagcctaactacatgcctgtgtgtttgtttgcagaagaatcttatcaaaaattagcaatggaaacgctggaggaattagactggtgtttagaccagctagagaccatacagacctaccggtctgtcagtgagatggcttctaacaagttcaaaagaatgctgaaccgggagctgacacacctctcagagatgagccgatcagggaaccaggtgtctgaatacatttcaaatactttcttagacaagcagaatgatgtggagatcccatctcctacccagaaagacagggagaaaaagaaaaagcagcagctcatgacccagataagtggagtgaagaaattaatgcatagttcaagcctaaacaatacaagcatctcacgctttggagtcaacactgaaaatgaagatcacctggccaaggagctggaagacctgaacaaatggggtcttaacatctttaatgtggctggatattctcacaatagacccctaacatgcatcatgtatgctatattccaggaaagagacctcctaaagacattcagaatctcatctgacacatttataacctacatgatgactttagaagaccattaccattctgacgtggcatatcacaacagcctgcacgctgctgatgtagcccagtcgacccatgttctcctttctacaccagcattagacgctgtcttcacagatttggagatcctggctgccatttttgcagctgccatccatgacgttgatcatcctggagtctccaatcagtttctcatcaacacaaattcagaacttgctttgatgtataatgatgaatctgtgttggaaaatcatcaccttgctgtgggtttcaaactgctgcaagaagaacactgtgacatcttcatgaatctcaccaagaagcagcgtcagacactcaggaagatggttattgacatggtgttagcaactgatatgtctaaacatatgagcctgctggcagacctgaagacaatggtagaaacgaagaaagttacaagttcaggcgttcttctcctagacaactataccgatcgcattcaggtccttcgcaacatggtacactgtgcagacctgagcaaccccaccaagtccttggaattgtatcggcaatggacagaccgcatcatggaggaatttttccagcagggagacaaagagcgggagaggggaatggaaattagcccaatgtgtgataaacacacagcttctgtggaaaaatcccaggttggtttcatcgactacattgtccatccattgtgggagacatgggcagatttggtacagcctgatgctcaggacattctcgataccttagaagataacaggaactggtatcagagcatgatacctcaaagtccctcaccaccactggacgagcagaacagggactgccagggtctgatggagaagtttcagtttgaactgactctcgatgaggaagattctgaaggacctgagaaggagggagagggacacagctatttcagcagcacaaagacgctttgtgtgattgatccagaaaacagagattccctgggagagactgacatagacattgcaacagaagacaagtcccccgtggatacataatccccctctccctgtggagatgaacattctatccttgatgagcatgccagctatgtggtagggccagcccaccatgggggccaagacctgcacaggacaagggccacctggcctttcagttacttgagtttggagtcagaaagcaagaccaggaagcaaatagcagctcaggaaatcccacggttgacttgccttgatggcaagcttggtggagagggctgaagctgttgctgggggccgattctgatcaagacacatggcttgaaaatggaagacacaaaactgagagatcattctgcactaagtttcgggaacttatccccgacagtgactgaactcactgactaataacttcatttatgaatcttctcacttgtccctttgtctgccaacctgtgtgccttttttgtaaaacattttcatgtctttaaaatgcctgttgaatacctggagtttagtatcaacttctacacagataagctttcaaagttgacaaacttttttgactctttctggaaaagggaaagaaaatagtcttccttctttcttgggcaatatccttcactttactacagttacttttgcaaacagacagaaaggatacacttctaaccacattttacttccttcccctgttgtccagtccaactccacagtcactcttaaaacttctctctgtttgcctgcctccaacagtacttttaactttttgctgtaaacagaataaaattgaacaaattagggggtagaaaggagcagtggtgtcgttcaccgtgagagtctgcatagaactcagcagtgtgccctgctgtgtcttggaccctgccccccacaggagttgtacagtccctggccctgttccctacctcctctcttcaccccgttaggctgttttcaatgtaatgctgccgtccttctcttgcactgccttctgcgctaacacctccattcctgtttataaccgtgtatttattacttaatgtatataatgtaatgttttgtaagttattaatttatatatctaacattgcctgccaatggtggtgttaaatttgtgtagaaaactctgcctaagagttacgactttttcttgtaatgttttgtattgtgtattatataacccaaacgtcacttagtagagacatatggcccccttggcagagaggacaggggtgggcttttgttcaaagggtctgccctttccctgcctgagttgctacttctgcacaacccctttatgaaccagttttggaaacaatattctcacattagatactaaatggtttatactgagcttttacttttgtatagcttgataggggcagggggcaatgggatgtagtttttacccaggttctatccaaatctatgtgggcatgagttgggttataactggatcctactatcattgtggctttggttcaaaaggaaacactacatttgctcacagatgattcttctgaatgctcccgaactactgactttgaagaggtagcctcctgcctgccattaagcaggaatgtcatgttccagttcattacaaaagaaaacaataaaacaatgtgaatttttataataaaatgtgaactgatgtagcaaattacgcaaatgtgaagcctcttctgataacacttgttaggcctcttactgatgtcagtttcagtttgtaaaatatgtttcatgctttcagttcagcattgtgactcagtaattacagaaaatggcacaaatgtgcatgaccaatgtatgtctatgaacactgcattgtttcaggtggacattttatcattttcaaatgtttctcacaatgtatgttatagtattattattatatattgtgttcaaatgcattctaaagagacttttatatgaggtgaataaagaaaagcatgattagattaaaaaaa

SEQ ID NO: 32 - protein, 564 aa, Homo sapiens
MKEHGGTFSSTGISGGSGDSAMDSLQPLQPNYMPVCLFAEESYQKLAMETLEELDWCLDQLETIQTYRSVSEMASNKFKRMLNRELTHLSEMSRSGNQVSEYISNTFLDKQNDVEIPSPTQKDREKKKKQQLMTQISGVKKLMHSSSLNNTSISRFGVNTENEDHLAKELEDLNKWGLNIFNVAGYSHNRPLTCIMYAIFQERDLLKTFRISSDTFITYMMTLEDHYHSDVAYHNSLHAADVAQSTHVLLSTPALDAVFTDLEILAAIFAAAIHDVDHPGVSNQFLINTNSELALMYNDESVLENHHLAVGFKLLQEEHCDIFMNLTKKQRQTLRKMVIDMVLATDMSKHMSLLADLKTMVETKKVTSSGVLLLDNYTDRIQVLRNMVHCADLSNPTKSLELYRQWTDRIMEEFFQQGDKERERGMEISPMCDKHTASVEKSQVGFIDYIVHPLWETWADLVQPDAQDILDTLEDNRNWYQSMIPQSPSPPLDEQNRDCQGLMEKFQFELTLDEEDSEGPEKEGEGHSYFSSTKTLCVIDPENRDSLGETDIDIATEDKSPVDT

SEQ ID NO: 33 - DNA, 4234 bp, Homo sapiens
  source 1..4234: mol_type = other DNA
attcttcgagtatgctgctcttgctctaagacgctcatacattggagtcacagcttcgtaaattaaactggaaatagtttgcagacttatcagtcttctgacctgcagcagtgtctctgctatgtttgagatttttgttttggatggtgaaagctagcactccttacaagacatgacagcaaaagattcttcaaaggaacttactgcttctgaacctgaggtttgcataaagactttcaaggagcaaatgcatttagaacttgagcttccgagattaccaggaaacagacctacatctcctaaaatttctccacgcagttcaccaaggaactcaccatgctttttcagaaagttgctggtgaataaaagcattcggcagcgtcgtcgcttcactgtggctcatacatgctttgatgtggaaaatggcccttccccaggtcggagtccactggatccccaggccagctcttccgctgggctggtacttcacgccacctttcctgggcacagccagcgcagagagtcatttctctacagatcagacagcgactatgacttgtcaccaaaggcgatgtcgagaaactcttctcttccaagcgagcaacacggcgatgacttgattgtaactccttttgcccaggtccttgccagcttgcgaagtgtgagaaacaacttcactatactgacaaaccttcatggtacatctaacaagaggtccccagctgctagtcagcctcctgtctccagagtcaacccacaagaagaatcttatcaaaaattagcaatggaaacgctggaggaattagactggtgtttagaccagctagagaccatacagacctaccggtctgtcagtgagatggcttctaacaagttcaaaagaatgctgaaccgggagctgacacacctctcagagatgagccgatcagggaaccaggtgtctgaatacatttcaaatactttcttagacaagcagaatgatgtggagatcccatctcctacccagaaagacagggagaaaaagaaaaagcagcagctcatgacccagataagtggagtgaagaaattaatgcatagttcaagcctaaacaatacaagcatctcacgctttggagtcaacactgaaaatgaagatcacctggccaaggagctggaagacctgaacaaatggggtcttaacatctttaatgtggctggatattctcacaatagacccctaacatgcatcatgtatgctatattccaggaaagagacctcctaaagacattcagaatctcatctgacacatttataacctacatgatgactttagaagaccattaccattctgacgtggcatatcacaacagcctgcacgctgctgatgtagcccagtcgacccatgttctcctttctacaccagcattagacgctgtcttcacagatttggagatcctggctgccatttttgcagctgccatccatgacgttgatcatcctggagtctccaatcagtttctcatcaacacaaattcagaacttgctttgatgtataatgatgaatctgtgttggaaaatcatcaccttgctgtgggtttcaaactgctgcaagaagaacactgtgacatcttcatgaatctcaccaagaagcagcgtcagacactcaggaagatggttattgacatggtgttagcaactgatatgtctaaacatatgagcctgctggcagacctgaagacaatggtagaaacgaagaaagttacaagttcaggcgttcttctcctagacaactataccgatcgcattcaggtccttcgcaacatggtacactgtgcagacctgagcaaccccaccaagtccttggaattgtatcggcaatggacagaccgcatcatggaggaatttttccagcagggagacaaagagcgggagaggggaatggaaattagcccaatgtgtgataaacacacagcttctgtggaaaaatcccaggttggtttcatcgactacattgtccatccattgtgggagacatgggcagatttggtacagcctgatgctcaggacattctcgataccttagaagataacaggaactggtatcagagcatgatacctcaaagtccctcaccaccactggacgagcagaacagggactgccagggtctgatggagaagtttcagtttgaactgactctcgatgaggaagattctgaaggacctgagaaggagggagagggacacagctatttcagcagcacaaagacgctttgtgtgattgatccagaaaacagagattccctgggagagactgacatagacattgcaacagaagacaagtcccccgtggatacataatccccctctccctgtggagatgaacattctatccttgatgagcatgccagctatgtggtagggccagcccaccatgggggccaagacctgcacaggacaagggccacctggcctttcagttacttgagtttggagtcagaaagcaagaccaggaagcaaatagcagctcaggaaatcccacggttgacttgccttgatggcaagcttggtggagagggctgaagctgttgctgggggccgattctgatcaagacacatggcttgaaaatggaagacacaaaactgagagatcattctgcactaagtttcgggaacttatccccgacagtgactgaactcactgactaataacttcatttatgaatcttctcacttgtccctttgtctgccaacctgtgtgccttttttgtaaaacattttcatgtctttaaaatgcctgttgaatacctggagtttagtatcaacttctacacagataagctttcaaagttgacaaacttttttgactctttctggaaaagggaaagaaaatagtcttccttctttcttgggcaatatccttcactttactacagttacttttgcaaacagacagaaaggatacacttctaaccacattttacttccttcccctgttgtccagtccaactccacagtcactcttaaaacttctctctgtttgcctgcctccaacagtacttttaactttttgctgtaaacagaataaaattgaacaaattagggggtagaaaggagcagtggtgtcgttcaccgtgagagtctgcatagaactcagcagtgtgccctgctgtgtcttggaccctgccccccacaggagttgtacagtccctggccctgttccctacctcctctcttcaccccgttaggctgttttcaatgtaatgctgccgtccttctcttgcactgccttctgcgctaacacctccattcctgtttataaccgtgtatttattacttaatgtatataatgtaatgttttgtaagttattaatttatatatctaacattgcctgccaatggtggtgttaaatttgtgtagaaaactctgcctaagagttacgactttttcttgtaatgttttgtattgtgtattatataacccaaacgtcacttagtagagacatatggcccccttggcagagaggacaggggtgggcttttgttcaaagggtctgccctttccctgcctgagttgctacttctgcacaacccctttatgaaccagttttggaaacaatattctcacattagatactaaatggtttatactgagcttttacttttgtatagcttgataggggcagggggcaatgggatgtagtttttacccaggttctatccaaatctatgtgggcatgagttgggttataactggatcctactatcattgtggctttggttcaaaaggaaacactacatttgctcacagatgattcttctgaatgctcccgaactactgactttgaagaggtagcctcctgcctgccattaagcaggaatgtcatgttccagttcattacaaaagaaaacaataaaacaatgtgaatttttataataaaatgtgaactgatgtagcaaattacgcaaatgtgaagcctcttctgataacacttgttaggcctcttactgatgtcagtttcagtttgtaaaatatgtttcatgctttcagttcagcattgtgactcagtaattacagaaaatggcacaaatgtgcatgaccaatgtatgtctatgaacactgcattgtttcaggtggacattttatcattttcaaatgtttctcacaatgtatgttatagtattattattatatattgtgttcaaatgcattctaaagagacttttatatgaggtgaataaagaaaagcatgatta

SEQ ID NO: 34 - protein, 721 aa, Homo sapiens
MTAKDSSKELTASEPEVCIKTFKEQMHLELELPRLPGNRPTSPKISPRSSPRNSPCFFRKLLVNKSIRQRRRFTVAHTCFDVENGPSPGRSPLDPQASSSAGLVLHATFPGHSQRRESFLYRSDSDYDLSPKAMSRNSSLPSEQHGDDLIVTPFAQVLASLRSVRNNFTILTNLHGTSNKRSPAASQPPVSRVNPQEESYQKLAMETLEELDWCLDQLETIQTYRSVSEMASNKFKRMLNRELTHLSEMSRSGNQVSEYISNTFLDKQNDVEIPSPTQKDREKKKKQQLMTQISGVKKLMHSSSLNNTSISRFGVNTENEDHLAKELEDLNKWGLNIFNVAGYSHNRPLTCIMYAIFQERDLLKTFRISSDTFITYMMTLEDHYHSDVAYHNSLHAADVAQSTHVLLSTPALDAVFTDLEILAAIFAAAIHDVDHPGVSNQFLINTNSELALMYNDESVLENHHLAVGFKLLQEEHCDIFMNLTKKQRQTLRKMVIDMVLATDMSKHMSLLADLKTMVETKKVTSSGVLLLDNYTDRIQVLRNMVHCADLSNPTKSLELYRQWTDRIMEEFFQQGDKERERGMEISPMCDKHTASVEKSQVGFIDYIVHPLWETWADLVQPDAQDILDTLEDNRNWYQSMIPQSPSPPLDEQNRDCQGLMEKFQFELTLDEEDSEGPEKEGEGHSYFSSTKTLCVIDPENRDSLGETDIDIATEDKSPVDT

SEQ ID NO: 35 - DNA, 4059 bp, Homo sapiens
  source 1..4059: mol_type = other DNA
gtgcgtaatccttcagctctggtggtaagggagatgcagtgagctcccggctgggagagagggttattttgcaaaactcccctggtaccgtgcccgcggaatattgcaggaggtctgtgaggtattaaaaagtgtcagcaaactgcattgaataacagacatcctaagaggggatattttccacctctataatgaagaaaagcaggagtgtgatgacggtgatggctgatgatctttgatgtggaaaatggcccttccccaggtcggagtccactggatccccaggccagctcttccgctgggctggtacttcacgccacctttcctgggcacagccagcgcagagagtcatttctctacagatcagacagcgactatgacttgtcaccaaaggcgatgtcgagaaactcttctcttccaagcgagcaacacggcgatgacttgattgtaactccttttgcccaggtccttgccagcttgcgaagtgtgagaaacaacttcactatactgacaaaccttcatggtacatctaacaagaggtccccagctgctagtcagcctcctgtctccagagtcaacccacaagaagaatcttatcaaaaattagcaatggaaacgctggaggaattagactggtgtttagaccagctagagaccatacagacctaccggtctgtcagtgagatggcttctaacaagttcaaaagaatgctgaaccgggagctgacacacctctcagagatgagccgatcagggaaccaggtgtctgaatacatttcaaatactttcttagacaagcagaatgatgtggagatcccatctcctacccagaaagacagggagaaaaagaaaaagcagcagctcatgacccagataagtggagtgaagaaattaatgcatagttcaagcctaaacaatacaagcatctcacgctttggagtcaacactgaaaatgaagatcacctggccaaggagctggaagacctgaacaaatggggtcttaacatctttaatgtggctggatattctcacaatagacccctaacatgcatcatgtatgctatattccaggaaagagacctcctaaagacattcagaatctcatctgacacatttataacctacatgatgactttagaagaccattaccattctgacgtggcatatcacaacagcctgcacgctgctgatgtagcccagtcgacccatgttctcctttctacaccagcattagacgctgtcttcacagatttggagatcctggctgccatttttgcagctgccatccatgacgttgatcatcctggagtctccaatcagtttctcatcaacacaaattcagaacttgctttgatgtataatgatgaatctgtgttggaaaatcatcaccttgctgtgggtttcaaactgctgcaagaagaacactgtgacatcttcatgaatctcaccaagaagcagcgtcagacactcaggaagatggttattgacatggtgttagcaactgatatgtctaaacatatgagcctgctggcagacctgaagacaatggtagaaacgaagaaagttacaagttcaggcgttcttctcctagacaactataccgatcgcattcaggtccttcgcaacatggtacactgtgcagacctgagcaaccccaccaagtccttggaattgtatcggcaatggacagaccgcatcatggaggaatttttccagcagggagacaaagagcgggagaggggaatggaaattagcccaatgtgtgataaacacacagcttctgtggaaaaatcccaggttggtttcatcgactacattgtccatccattgtgggagacatgggcagatttggtacagcctgatgctcaggacattctcgataccttagaagataacaggaactggtatcagagcatgatacctcaaagtccctcaccaccactggacgagcagaacagggactgccagggtctgatggagaagtttcagtttgaactgactctcgatgaggaagattctgaaggacctgagaaggagggagagggacacagctatttcagcagcacaaagacgctttgtgtgattgatccagaaaacagagattccctgggagagactgacatagacattgcaacagaagacaagtcccccgtggatacataatccccctctccctgtggagatgaacattctatccttgatgagcatgccagctatgtggtagggccagcccaccatgggggccaagacctgcacaggacaagggccacctggcctttcagttacttgagtttggagtcagaaagcaagaccaggaagcaaatagcagctcaggaaatcccacggttgacttgccttgatggcaagcttggtggagagggctgaagctgttgctgggggccgattctgatcaagacacatggcttgaaaatggaagacacaaaactgagagatcattctgcactaagtttcgggaacttatccccgacagtgactgaactcactgactaataacttcatttatgaatcttctcacttgtccctttgtctgccaacctgtgtgccttttttgtaaaacattttcatgtctttaaaatgcctgttgaatacctggagtttagtatcaacttctacacagataagctttcaaagttgacaaacttttttgactctttctggaaaagggaaagaaaatagtcttccttctttcttgggcaatatccttcactttactacagttacttttgcaaacagacagaaaggatacacttctaaccacattttacttccttcccctgttgtccagtccaactccacagtcactcttaaaacttctctctgtttgcctgcctccaacagtacttttaactttttgctgtaaacagaataaaattgaacaaattagggggtagaaaggagcagtggtgtcgttcaccgtgagagtctgcatagaactcagcagtgtgccctgctgtgtcttggaccctgccccccacaggagttgtacagtccctggccctgttccctacctcctctcttcaccccgttaggctgttttcaatgtaatgctgccgtccttctcttgcactgccttctgcgctaacacctccattcctgtttataaccgtgtatttattacttaatgtatataatgtaatgttttgtaagttattaatttatatatctaacattgcctgccaatggtggtgttaaatttgtgtagaaaactctgcctaagagttacgactttttcttgtaatgttttgtattgtgtattatataacccaaacgtcacttagtagagacatatggcccccttggcagagaggacaggggtgggcttttgttcaaagggtctgccctttccctgcctgagttgctacttctgcacaacccctttatgaaccagttttggaaacaatattctcacattagatactaaatggtttatactgagcttttacttttgtatagcttgataggggcagggggcaatgggatgtagtttttacccaggttctatccaaatctatgtgggcatgagttgggttataactggatcctactatcattgtggctttggttcaaaaggaaacactacatttgctcacagatgattcttctgaatgctcccgaactactgactttgaagaggtagcctcctgcctgccattaagcaggaatgtcatgttccagttcattacaaaagaaaacaataaaacaatgtgaatttttataataaaatgtgaactgatgtagcaaattacgcaaatgtgaagcctcttctgataacacttgttaggcctcttactgatgtcagtttcagtttgtaaaatatgtttcatgctttcagttcagcattgtgactcagtaattacagaaaatggcacaaatgtgcatgaccaatgtatgtctatgaacactgcattgtttcaggtggacattttatcattttcaaatgtttctcacaatgtatgttatagtattattattatatattgtgttcaaatgcattctaaagagacttttatatgaggtgaataaagaaaagcatgatta

SEQ ID NO: 36 - protein, 644 aa, Homo sapiens
MIFDVENGPSPGRSPLDPQASSSAGLVLHATFPGHSQRRESFLYRSDSDYDLSPKAMSRNSSLPSEQHGDDLIVTPFAQVLASLRSVRNNFTILTNLHGTSNKRSPAASQPPVSRVNPQEESYQKLAMETLEELDWCLDQLETIQTYRSVSEMASNKFKRMLNRELTHLSEMSRSGNQVSEYISNTFLDKQNDVEIPSPTQKDREKKKKQQLMTQISGVKKLMHSSSLNNTSISRFGVNTENEDHLAKELEDLNKWGLNIFNVAGYSHNRPLTCIMYAIFQERDLLKTFRISSDTFITYMMTLEDHYHSDVAYHNSLHAADVAQSTHVLLSTPALDAVFTDLEILAAIFAAAIHDVDHPGVSNQFLINTNSELALMYNDESVLENHHLAVGFKLLQEEHCDIFMNLTKKQRQTLRKMVIDMVLATDMSKHMSLLADLKTMVETKKVTSSGVLLLDNYTDRIQVLRNMVHCADLSNPTKSLELYRQWTDRIMEEFFQQGDKERERGMEISPMCDKHTASVEKSQVGFIDYIVHPLWETWADLVQPDAQDILDTLEDNRNWYQSMIPQSPSPPLDEQNRDCQGLMEKFQFELTLDEEDSEGPEKEGEGHSYFSSTKTLCVIDPENRDSLGETDIDIATEDKSPVDT

SEQ ID NO: 37 - DNA, 3963 bp, Homo sapiens
  source 1..3963: mol_type = other DNA
gtattaaaaagtgtcagcaaactgcattgaataacagacatcctaagaggggatattttccacctctataatgaagaaaagcaggagtgtgatgacggtgatggctgatgatgtaattttaaagaactttgatgtggaaaatggcccttccccaggtcggagtccactggatccccaggccagctcttccgctgggctggtacttcacgccacctttcctgggcacagccagcgcagagagtcatttctctacagatcagacagcgactatgacttgtcaccaaaggcgatgtcgagaaactcttctcttccaagcgagcaacacggcgatgacttgattgtaactccttttgcccaggtccttgccagcttgcgaagtgtgagaaacaacttcactatactgacaaaccttcatggtacatctaacaagaggtccccagctgctagtcagcctcctgtctccagagtcaacccacaagaagaatcttatcaaaaattagcaatggaaacgctggaggaattagactggtgtttagaccagctagagaccatacagacctaccggtctgtcagtgagatggcttctaacaagttcaaaagaatgctgaaccgggagctgacacacctctcagagatgagccgatcagggaaccaggtgtctgaatacatttcaaatactttcttagacaagcagaatgatgtggagatcccatctcctacccagaaagacagggagaaaaagaaaaagcagcagctcatgacccagataagtggagtgaagaaattaatgcatagttcaagcctaaacaatacaagcatctcacgctttggagtcaacactgaaaatgaagatcacctggccaaggagctggaagacctgaacaaatggggtcttaacatctttaatgtggctggatattctcacaatagacccctaacatgcatcatgtatgctatattccaggaaagagacctcctaaagacattcagaatctcatctgacacatttataacctacatgatgactttagaagaccattaccattctgacgtggcatatcacaacagcctgcacgctgctgatgtagcccagtcgacccatgttctcctttctacaccagcattagacgctgtcttcacagatttggagatcctggctgccatttttgcagctgccatccatgacgttgatcatcctggagtctccaatcagtttctcatcaacacaaattcagaacttgctttgatgtataatgatgaatctgtgttggaaaatcatcaccttgctgtgggtttcaaactgctgcaagaagaacactgtgacatcttcatgaatctcaccaagaagcagcgtcagacactcaggaagatggttattgacatggtgttagcaactgatatgtctaaacatatgagcctgctggcagacctgaagacaatggtagaaacgaagaaagttacaagttcaggcgttcttctcctagacaactataccgatcgcattcaggtccttcgcaacatggtacactgtgcagacctgagcaaccccaccaagtccttggaattgtatcggcaatggacagaccgcatcatggaggaatttttccagcagggagacaaagagcgggagaggggaatggaaattagcccaatgtgtgataaacacacagcttctgtggaaaaatcccaggttggtttcatcgactacattgtccatccattgtgggagacatgggcagatttggtacagcctgatgctcaggacattctcgataccttagaagataacaggaactggtatcagagcatgatacctcaaagtccctcaccaccactggacgagcagaacagggactgccagggtctgatggagaagtttcagtttgaactgactctcgatgaggaagattctgaaggacctgagaaggagggagagggacacagctatttcagcagcacaaagacgctttgtgtgattgatccagaaaacagagattccctgggagagactgacatagacattgcaacagaagacaagtcccccgtggatacataatccccctctccctgtggagatgaacattctatccttgatgagcatgccagctatgtggtagggccagcccaccatgggggccaagacctgcacaggacaagggccacctggcctttcagttacttgagtttggagtcagaaagcaagaccaggaagcaaatagcagctcaggaaatcccacggttgacttgccttgatggcaagcttggtggagagggctgaagctgttgctgggggccgattctgatcaagacacatggcttgaaaatggaagacacaaaactgagagatcattctgcactaagtttcgggaacttatccccgacagtgactgaactcactgactaataacttcatttatgaatcttctcacttgtccctttgtctgccaacctgtgtgccttttttgtaaaacattttcatgtctttaaaatgcctgttgaatacctggagtttagtatcaacttctacacagataagctttcaaagttgacaaacttttttgactctttctggaaaagggaaagaaaatagtcttccttctttcttgggcaatatccttcactttactacagttacttttgcaaacagacagaaaggatacacttctaaccacattttacttccttcccctgttgtccagtccaactccacagtcactcttaaaacttctctctgtttgcctgcctccaacagtacttttaactttttgctgtaaacagaataaaattgaacaaattagggggtagaaaggagcagtggtgtcgttcaccgtgagagtctgcatagaactcagcagtgtgccctgctgtgtcttggaccctgccccccacaggagttgtacagtccctggccctgttccctacctcctctcttcaccccgttaggctgttttcaatgtaatgctgccgtccttctcttgcactgccttctgcgctaacacctccattcctgtttataaccgtgtatttattacttaatgtatataatgtaatgttttgtaagttattaatttatatatctaacattgcctgccaatggtggtgttaaatttgtgtagaaaactctgcctaagagttacgactttttcttgtaatgttttgtattgtgtattatataacccaaacgtcacttagtagagacatatggcccccttggcagagaggacaggggtgggcttttgttcaaagggtctgccctttccctgcctgagttgctacttctgcacaacccctttatgaaccagttttggaaacaatattctcacattagatactaaatggtttatactgagcttttacttttgtatagcttgataggggcagggggcaatgggatgtagtttttacccaggttctatccaaatctatgtgggcatgagttgggttataactggatcctactatcattgtggctttggttcaaaaggaaacactacatttgctcacagatgattcttctgaatgctcccgaactactgactttgaagaggtagcctcctgcctgccattaagcaggaatgtcatgttccagttcattacaaaagaaaacaataaaacaatgtgaatttttataataaaatgtgaactgatgtagcaaattacgcaaatgtgaagcctcttctgataacacttgttaggcctcttactgatgtcagtttcagtttgtaaaatatgtttcatgctttcagttcagcattgtgactcagtaattacagaaaatggcacaaatgtgcatgaccaatgtatgtctatgaacactgcattgtttcaggtggacattttatcattttcaaatgtttctcacaatgtatgttatagtattattattatatattgtgttcaaatgcattctaaagagacttttatatgaggtgaataaagaaaagcatgattagattaaaaaaa

SEQ ID NO: 38 - protein, 661 aa, Homo sapiens
MKKSRSVMTVMADDVILKNFDVENGPSPGRSPLDPQASSSAGLVLHATFPGHSQRRESFLYRSDSDYDLSPKAMSRNSSLPSEQHGDDLIVTPFAQVLASLRSVRNNFTILTNLHGTSNKRSPAASQPPVSRVNPQEESYQKLAMETLEELDWCLDQLETIQTYRSVSEMASNKFKRMLNRELTHLSEMSRSGNQVSEYISNTFLDKQNDVEIPSPTQKDREKKKKQQLMTQISGVKKLMHSSSLNNTSISRFGVNTENEDHLAKELEDLNKWGLNIFNVAGYSHNRPLTCIMYAIFQERDLLKTFRISSDTFITYMMTLEDHYHSDVAYHNSLHAADVAQSTHVLLSTPALDAVFTDLEILAAIFAAAIHDVDHPGVSNQFLINTNSELALMYNDESVLENHHLAVGFKLLQEEHCDIFMNLTKKQRQTLRKMVIDMVLATDMSKHMSLLADLKTMVETKKVTSSGVLLLDNYTDRIQVLRNMVHCADLSNPTKSLELYRQWTDRIMEEFFQQGDKERERGMEISPMCDKHTASVEKSQVGFIDYIVHPLWETWADLVQPDAQDILDTLEDNRNWYQSMIPQSPSPPLDEQNRDCQGLMEKFQFELTLDEEDSEGPEKEGEGHSYFSSTKTLCVIDPENRDSLGETDIDIATEDKSPVDT

SEQ ID NO: 39 - DNA, 3720 bp, Homo sapiens
  source 1..3720: mol_type = other DNA
ataagtgcttcaaaccagccagctgaatacatttggacaggctcttgctccttcgtgcaattcctgatttcattactctcttctgccaggaaataagcagggagcataggcttcttgcaagaatggagtgcgaagatgggctttgtttggcttaggaaatgccatacattttggaggtttttgtcttttctaagttttgattattttatcactgaatctgcagggctttcctgatcctttcgggattgctctctcagaactgtgaattctttcaaagggatttgtggattgtggcaaggagagcattccaaaatgcctgaggcaaattatttgttatctgtatcttggggttacatcaagttcaaaagaatgctgaaccgggagctgacacacctctcagagatgagccgatcagggaaccaggtgtctgaatacatttcaaatactttcttagacaagcagaatgatgtggagatcccatctcctacccagaaagacagggagaaaaagaaaaagcagcagctcatgacccagataagtggagtgaagaaattaatgcatagttcaagcctaaacaatacaagcatctcacgctttggagtcaacactgaaaatgaagatcacctggccaaggagctggaagacctgaacaaatggggtcttaacatctttaatgtggctggatattctcacaatagacccctaacatgcatcatgtatgctatattccaggaaagagacctcctaaagacattcagaatctcatctgacacatttataacctacatgatgactttagaagaccattaccattctgacgtggcatatcacaacagcctgcacgctgctgatgtagcccagtcgacccatgttctcctttctacaccagcattagacgctgtcttcacagatttggagatcctggctgccatttttgcagctgccatccatgacgttgatcatcctggagtctccaatcagtttctcatcaacacaaattcagaacttgctttgatgtataatgatgaatctgtgttggaaaatcatcaccttgctgtgggtttcaaactgctgcaagaagaacactgtgacatcttcatgaatctcaccaagaagcagcgtcagacactcaggaagatggttattgacatggtgttagcaactgatatgtctaaacatatgagcctgctggcagacctgaagacaatggtagaaacgaagaaagttacaagttcaggcgttcttctcctagacaactataccgatcgcattcaggtccttcgcaacatggtacactgtgcagacctgagcaaccccaccaagtccttggaattgtatcggcaatggacagaccgcatcatggaggaatttttccagcagggagacaaagagcgggagaggggaatggaaattagcccaatgtgtgataaacacacagcttctgtggaaaaatcccaggttggtttcatcgactacattgtccatccattgtgggagacatgggcagatttggtacagcctgatgctcaggacattctcgataccttagaagataacaggaactggtatcagagcatgatacctcaaagtccctcaccaccactggacgagcagaacagggactgccagggtctgatggagaagtttcagtttgaactgactctcgatgaggaagattctgaaggacctgagaaggagggagagggacacagctatttcagcagcacaaagacgctttgtgtgattgatccagaaaacagagattccctgggagagactgacatagacattgcaacagaagacaagtcccccgtggatacataatccccctctccctgtggagatgaacattctatccttgatgagcatgccagctatgtggtagggccagcccaccatgggggccaagacctgcacaggacaagggccacctggcctttcagttacttgagtttggagtcagaaagcaagaccaggaagcaaatagcagctcaggaaatcccacggttgacttgccttgatggcaagcttggtggagagggctgaagctgttgctgggggccgattctgatcaagacacatggcttgaaaatggaagacacaaaactgagagatcattctgcactaagtttcgggaacttatccccgacagtgactgaactcactgactaataacttcatttatgaatcttctcacttgtccctttgtctgccaacctgtgtgccttttttgtaaaacattttcatgtctttaaaatgcctgttgaatacctggagtttagtatcaacttctacacagataagctttcaaagttgacaaacttttttgactctttctggaaaagggaaagaaaatagtcttccttctttcttgggcaatatccttcactttactacagttacttttgcaaacagacagaaaggatacacttctaaccacattttacttccttcccctgttgtccagtccaactccacagtcactcttaaaacttctctctgtttgcctgcctccaacagtacttttaactttttgctgtaaacagaataaaattgaacaaattagggggtagaaaggagcagtggtgtcgttcaccgtgagagtctgcatagaactcagcagtgtgccctgctgtgtcttggaccctgccccccacaggagttgtacagtccctggccctgttccctacctcctctcttcaccccgttaggctgttttcaatgtaatgctgccgtccttctcttgcactgccttctgcgctaacacctccattcctgtttataaccgtgtatttattacttaatgtatataatgtaatgttttgtaagttattaatttatatatctaacattgcctgccaatggtggtgttaaatttgtgtagaaaactctgcctaagagttacgactttttcttgtaatgttttgtattgtgtattatataacccaaacgtcacttagtagagacatatggcccccttggcagagaggacaggggtgggcttttgttcaaagggtctgccctttccctgcctgagttgctacttctgcacaacccctttatgaaccagttttggaaacaatattctcacattagatactaaatggtttatactgagcttttacttttgtatagcttgataggggcagggggcaatgggatgtagtttttacccaggttctatccaaatctatgtgggcatgagttgggttataactggatcctactatcattgtggctttggttcaaaaggaaacactacatttgctcacagatgattcttctgaatgctcccgaactactgactttgaagaggtagcctcctgcctgccattaagcaggaatgtcatgttccagttcattacaaaagaaaacaataaaacaatgtgaatttttataataaaatgtgaactgatgtagcaaattacgcaaatgtgaagcctcttctgataacacttgttaggcctcttactgatgtcagtttcagtttgtaaaatatgtttcatgctttcagttcagcattgtgactcagtaattacagaaaatggcacaaatgtgcatgaccaatgtatgtctatgaacactgcattgtttcaggtggacattttatcattttcaaatgtttctcacaatgtatgttatagtattattattatatattgtgttcaaatgcattctaaagagacttttatatgaggtgaataaagaaaagcatgatta

SEQ ID NO: 40 - protein, 503 aa, Homo sapiens
MPEANYLLSVSWGYIKFKRMLNRELTHLSEMSRSGNQVSEYISNTFLDKQNDVEIPSPTQKDREKKKKQQLMTQISGVKKLMHSSSLNNTSISRFGVNTENEDHLAKELEDLNKWGLNIFNVAGYSHNRPLTCIMYAIFQERDLLKTFRISSDTFITYMMTLEDHYHSDVAYHNSLHAADVAQSTHVLLSTPALDAVFTDLEILAAIFAAAIHDVDHPGVSNQFLINTNSELALMYNDESVLENHHLAVGFKLLQEEHCDIFMNLTKKQRQTLRKMVIDMVLATDMSKHMSLLADLKTMVETKKVTSSGVLLLDNYTDRIQVLRNMVHCADLSNPTKSLELYRQWTDRIMEEFFQQGDKERERGMEISPMCDKHTASVEKSQVGFIDYIVHPLWETWADLVQPDAQDILDTLEDNRNWYQSMIPQSPSPPLDEQNRDCQGLMEKFQFELTLDEEDSEGPEKEGEGHSYFSSTKTLCVIDPENRDSLGETDIDIATEDKSPVDT

SEQ ID NO: 41 - DNA, 4298 bp, Homo sapiens
  source 1..4298: mol_type = other DNA
gtgcgtaatccttcagctctggtggtaagggagatgcagtgagctcccggctgggagagagggttattttgcaaaactcccctggtaccgtgcccgcggaatattgcaggaggtctgtgaggtattaaaaagtgtcagcaaactgcattgaataacagacatcctaagaggggatattttccacctctataatgaagaaaagcaggagtgtgatgacggtgatggctgatgataatgttaaagattattttgaatgtagcttgagtaaatcctacagttcttccagtaacacacttgggatcgacctctggagagggagaaggtgttgctcaggaaacttacagttaccaccactgtctcaaagacagagtgaaagggcaaggactcctgagggagatggtatttccaggccgaccacactgcctttgacaacgcttccaagcattgctattacaactgtaagccaggagtgctttgatgtggaaaatggcccttccccaggtcggagtccactggatccccaggccagctcttccgctgggctggtacttcacgccacctttcctgggcacagccagcgcagagagtcatttctctacagatcagacagcgactatgacttgtcaccaaaggcgatgtcgagaaactcttctcttccaagcgagcaacacggcgatgacttgattgtaactccttttgcccaggtccttgccagcttgcgaagtgtgagaaacaacttcactatactgacaaaccttcatggtacatctaacaagaggtccccagctgctagtcagcctcctgtctccagagtcaacccacaagaagaatcttatcaaaaattagcaatggaaacgctggaggaattagactggtgtttagaccagctagagaccatacagacctaccggtctgtcagtgagatggcttctaacaagttcaaaagaatgctgaaccgggagctgacacacctctcagagatgagccgatcagggaaccaggtgtctgaatacatttcaaatactttcttagacaagcagaatgatgtggagatcccatctcctacccagaaagacagggagaaaaagaaaaagcagcagctcatgacccagataagtggagtgaagaaattaatgcatagttcaagcctaaacaatacaagcatctcacgctttggagtcaacactgaaaatgaagatcacctggccaaggagctggaagacctgaacaaatggggtcttaacatctttaatgtggctggatattctcacaatagacccctaacatgcatcatgtatgctatattccaggaaagagacctcctaaagacattcagaatctcatctgacacatttataacctacatgatgactttagaagaccattaccattctgacgtggcatatcacaacagcctgcacgctgctgatgtagcccagtcgacccatgttctcctttctacaccagcattagacgctgtcttcacagatttggagatcctggctgccatttttgcagctgccatccatgacgttgatcatcctggagtctccaatcagtttctcatcaacacaaattcagaacttgctttgatgtataatgatgaatctgtgttggaaaatcatcaccttgctgtgggtttcaaactgctgcaagaagaacactgtgacatcttcatgaatctcaccaagaagcagcgtcagacactcaggaagatggttattgacatggtgttagcaactgatatgtctaaacatatgagcctgctggcagacctgaagacaatggtagaaacgaagaaagttacaagttcaggcgttcttctcctagacaactataccgatcgcattcaggtccttcgcaacatggtacactgtgcagacctgagcaaccccaccaagtccttggaattgtatcggcaatggacagaccgcatcatggaggaatttttccagcagggagacaaagagcgggagaggggaatggaaattagcccaatgtgtgataaacacacagcttctgtggaaaaatcccaggttggtttcatcgactacattgtccatccattgtgggagacatgggcagatttggtacagcctgatgctcaggacattctcgataccttagaagataacaggaactggtatcagagcatgatacctcaaagtccctcaccaccactggacgagcagaacagggactgccagggtctgatggagaagtttcagtttgaactgactctcgatgaggaagattctgaaggacctgagaaggagggagagggacacagctatttcagcagcacaaagacgctttgtgtgattgatccagaaaacagagattccctgggagagactgacatagacattgcaacagaagacaagtcccccgtggatacataatccccctctccctgtggagatgaacattctatccttgatgagcatgccagctatgtggtagggccagcccaccatgggggccaagacctgcacaggacaagggccacctggcctttcagttacttgagtttggagtcagaaagcaagaccaggaagcaaatagcagctcaggaaatcccacggttgacttgccttgatggcaagcttggtggagagggctgaagctgttgctgggggccgattctgatcaagacacatggcttgaaaatggaagacacaaaactgagagatcattctgcactaagtttcgggaacttatccccgacagtgactgaactcactgactaataacttcatttatgaatcttctcacttgtccctttgtctgccaacctgtgtgccttttttgtaaaacattttcatgtctttaaaatgcctgttgaatacctggagtttagtatcaacttctacacagataagctttcaaagttgacaaacttttttgactctttctggaaaagggaaagaaaatagtcttccttctttcttgggcaatatccttcactttactacagttacttttgcaaacagacagaaaggatacacttctaaccacattttacttccttcccctgttgtccagtccaactccacagtcactcttaaaacttctctctgtttgcctgcctccaacagtacttttaactttttgctgtaaacagaataaaattgaacaaattagggggtagaaaggagcagtggtgtcgttcaccgtgagagtctgcatagaactcagcagtgtgccctgctgtgtcttggaccctgccccccacaggagttgtacagtccctggccctgttccctacctcctctcttcaccccgttaggctgttttcaatgtaatgctgccgtccttctcttgcactgccttctgcgctaacacctccattcctgtttataaccgtgtatttattacttaatgtatataatgtaatgttttgtaagttattaatttatatatctaacattgcctgccaatggtggtgttaaatttgtgtagaaaactctgcctaagagttacgactttttcttgtaatgttttgtattgtgtattatataacccaaacgtcacttagtagagacatatggcccccttggcagagaggacaggggtgggcttttgttcaaagggtctgccctttccctgcctgagttgctacttctgcacaacccctttatgaaccagttttggaaacaatattctcacattagatactaaatggtttatactgagcttttacttttgtatagcttgataggggcagggggcaatgggatgtagtttttacccaggttctatccaaatctatgtgggcatgagttgggttataactggatcctactatcattgtggctttggttcaaaaggaaacactacatttgctcacagatgattcttctgaatgctcccgaactactgactttgaagaggtagcctcctgcctgccattaagcaggaatgtcatgttccagttcattacaaaagaaaacaataaaacaatgtgaatttttataataaaatgtgaactgatgtagcaaattacgcaaatgtgaagcctcttctgataacacttgttaggcctcttactgatgtcagtttcagtttgtaaaatatgtttcatgctttcagttcagcattgtgactcagtaattacagaaaatggcacaaatgtgcatgaccaatgtatgtctatgaacactgcattgtttcaggtggacattttatcattttcaaatgtttctcacaatgtatgttatagtattattattatatattgtgttcaaatgcattctaaagagacttttatatgaggtgaataaagaaaagcatgatta

SEQ ID NO: 42 - protein, 736 aa, Homo sapiens; identical to SEQ ID NO: 30

SEQ ID NO: 43 - DNA, 5342 bp, Homo sapiens
  source 1..5342: mol_type = other DNA
atgggacccaggcaggactccgcagtggtgcaccatctgggcatcgacagctcctcggtgtcggccccaccttgagccccagttccaccttctaccgcttcagcacctccggcgcggacagctcctcgctgtcgcctccactcccggccctgggccggacccgggagcagacgctcctcggcgcccgctcacggggacgagtcctgctccctgctatcccagacccctttctctggcgcatggagaacctgggggtcggcgaaggggcagaggcttgcagcaggttgagtcgctctcgcggccgccacagcatgaccagagccccgaagcacctgtggcggcaaccccggcgccccatccgcatccaacagcgcttctattcggatccggacaagtccgcgggctgccgcgagagggacctgagcccgcggccggagctcaggaagtcgcggctctcctggcccgtttcctcctgcaggcgctttgacctggaaaatgggctctcgtgtgggaggagggccctggaccctcagtccagccctggcctgggccggattatgcaggctccagtcccgcacagccagcggcgcgagtccttcctgtaccgctcagatagcgactatgaactctcgcccaaggccatgtctcggaactcctctgtggccagcgacctacatggagaggacatgattgtgacgccctttgcccaggtcctggccagtctgcggaccgttcggagcaacgtggcggcccttgcccgccagcaatgcctaggagcagccaagcagggacccgtcggaaacccttcatccagcaatcagctccctcctgcagaggacacggggcagaagctggcattggagacgctagacgagctggactggtgcctggatcagttggagacgctgcagacccggcactcggtgggggagatggcctccaacaagttcaagcggatcctgaaccgggagttgacccacctgtccgaaaccagccgctccgggaaccaggtgtccgagtacatctcccggaccttcctggaccagcagaccgaggtggagctgcccaaggtgaccgctgaggaggccccacagcccatgtcccggatcagtggcctacatgggctctgccacagtgccagcctctcctcagccactgtcccacgctttggggtccagactgaccaggaggagcaactggccaaggagctagaagacaccaacaagtggggacttgatgtgttcaaggtggcggagctaagtgggaaccggcccctcacagctatcatattcagcatttttcaggagcgggacctgctgaagacattccagatcccagcagacacactggccacctacctgctgatgctggaaggtcactaccacgccaatgtggcctaccacaacagcctacatgccgccgacgtggcccagtccacgcatgtgctgctggctacgcccgccctcgaggctgtgttcacagacttggaaatcctggctgccctctttgcaagcgccatccacgacgtggaccatcctggggtctccaaccagtttctgattaacaccaactcagagctggcgcttatgtacaacgacgcctcggtgctggagaaccatcacctggctgtgggcttcaagctgctgcaggcagagaactgcgatatcttccagaacctcagcgccaagcagcgactgagtctgcgcaggatggtcattgacatggtgctggccacagacatgtccaaacacatgaacctcctggccgacctcaagaccatggtggagaccaagaaggtgacaagcctcggtgtcctcctcctggacaactattccgaccgaatccaggtcttgcagaacctggtgcactgtgctgatctgagcaaccccaccaagccgctgcccctgtaccgccagtggacggaccgcatcatggccgagttcttccagcagggagaccgcgagcgtgagtcgggcctggacatcagtcccatgtgtgacaagcatacggcctcagtggagaagtcccaggtgggtttcattgactacattgctcacccactgtgggagacttgggctgacctggtccacccagatgcacaggacctgctggacacgctggaggacaatcgagagtggtaccagagcaagatcccccgaagtccctcagacctcaccaaccccgagcgggacgggcctgacagattccagtttgaactgactctggaggaggcagaggaagaggatgaggaggaagaagaggagggggaagagacagctttagccaaagaggccttggagttgcctgacactgaactcctgtcccctgaagccggcccagaccctggggacttacccctcgacaaccagaggacttagggccagccctgcgtgaactgcaggggcaatggatggtaaagccctttggctcttggcaggcagactttccaggaagaggctccatgtggctcctgcttcactttcccacccatttagggagacaatcaagctcttagttataggtggctcccagggtctaattggaggcacctggctggggtccactctgaccctagacttgcctaaaagagctctctaaggggcagcctcttacgatgccctggtgtctttctcctgggcttctatccctgtgaggagaggtgctgtctgctggagcctctagtccaccctctccagtggtcactcttgagtcacatctgtcacttaattatttccttctttatcaaatatttattgctcatctacttcgtgccagctttctgcctctgtagtagccctgcacaaagggtggggagtcaggagaccatcccaaaggcatctccctgtcttcctctaccaagcggctctctgcaagagcatggaaatgtgagtggggaaaattttcagcaccaaagcttcactcatacccagttttgtttctgaaactacggtagggggcaggaagaggagcagaaaagaagggctgggcaaggcatagtggcttatgcctgtaatcccggtactttgggaggctgaggtgggaggactgcttaagctcaggagtttgagaccagcctgggcaacatagcaagacccccaccatctctgaaaaaaaaaattagccaggcatggtggtgtgcacctgagaatcccagctactcagaaggttgagacaaaggggatcgcttgagcccaggagttggaggctgaagagagctatgactgcatcactgcactccagcctgggcaacacagcaagatcctgtctaaaaataaaaagaaaagagaaggaaaggaaagagacggggctctgaggccgagcacagtggcccatgcctataatcccagcactttgggaggctgaggcaggtggatcacctgaggttaggagttcgagaccagcctggccaacatggtgaaaccccatctctactaaaaatacaaaaattggctgggcatggtggcgggtgcctgtaatcccagctactggggaggctgaggcaggagaatcacttgaattcaggaggtggaggttgcagtgagccgacatcatgccactgcactccagcctgggcgacagagcaagacactgtctcaaaaaagaaaagaaaaaaaaaaaagccgggccaggtggctcacgcctgtaatcctagcactttgggaggctgagtgggggtggatcgcctgagatcaggagttcaaaatcagcctggccaacatagtgaaaccctgtctctactaaaaatacaaaaaattagaggctgggtgcggcggctcacacctgtaatcccagaactttgggaggccgaggcgggtggatcacgaggtcaggagttcaagaccagcctggccaacacggtgaaaccccatctctactaaaaatacacaaattagctgggcatggtgttgggtgcctgaatcccagctactcgggaggctgaggcaggagaatcgcttgaatccgggaggcggggcttgcagtgagccgagatcgtgccattgcactccagcctgggtgacagagcaagactccgtctcaaaaagaaaaaaaaaaaattagccaggcatggtggcaggtgcctgtaatcccagctacttgagaggctgaggcaggagaatcgcttgaacccgggaggtggaggttgtggtgagccgaggtcgcgccactgcactccagcctgggcaacgacaacaacaataaaaagagggggctctgtgcccggcatgtctctgaagactgattgaacctatgcaccagttgttgctttaagtcgctttattttctgtctttggtgtctctggatgtaggagccccctgctttctctgtccgcagaactccatactgggtcccctacgtgttcctccttccctaggacagcaacaaaaacacacaattttccctctctagcaggtctctaagtctcctgattcctgaaactgcctcagactccccctagagggagggaggcccctgaggctttcttgccatcatagcctcttctgggcctcagtttcccctctgtaacctgatcctagtacttggataaactccgacgaggtgtggggggttgttgtctgtgacctccctgaaatatcttagacatttggggtactgagcatttatctggggttaaataaaatctttacatcttaagacattcgattgaccaaattgagtgtcctggccatttcactgatgaggaaactgaggcgcagagaggtcctcttgccagctcaaagtcaagcatctgggcgcccaatgttagccagcggcaccccctggtggcgggcgtgggagacacggcggggcgcgcttgtcgggggttggggggtgggtcggaggggtggcatcctccagccctgatggtcccacttaccgcacctcgccgggaagagctcgtcctgctggtcgggcctccgagcggactgggcagcaccatgctcaagcctagggttcgatccccgcctccggaagcctcagtatccatccctcccctctgcctccctcttcgcgtgcctgaatatttatacaagatacaggcgtcatcacagccgccctcggcttccagagcagctggcttcgttcataaatattataaccactcagaattcatcatcatcacagttaatgataaaattccacagtgccagaactaaaagtcatccgggttcacgaacttggtgcatttccttccagacttttaaaaagaagatatttagggaatttttttttcaagatttttccccccagtccgcttacaaagtaataccatgttcgctgtaaaaaatttggaaataatggaaatgtataaagaaggaaataaaattctgctgtatctcca

SEQ ID NO: 44 - protein, 712 aa, Homo sapiens
MENLGVGEGAEACSRLSRSRGRHSMTRAPKHLWRQPRRPIRIQQRFYSDPDKSAGCRERDLSPRPELRKSRLSWPVSSCRRFDLENGLSCGRRALDPQSSPGLGRIMQAPVPHSQRRESFLYRSDSDYELSPKAMSRNSSVASDLHGEDMIVTPFAQVLASLRTVRSNVAALARQQCLGAAKQGPVGNPSSSNQLPPAEDTGQKLALETLDELDWCLDQLETLQTRHSVGEMASNKFKRILNRELTHLSETSRSGNQVSEYISRTFLDQQTEVELPKVTAEEAPQPMSRISGLHGLCHSASLSSATVPRFGVQTDQEEQLAKELEDTNKWGLDVFKVAELSGNRPLTAIIFSIFQERDLLKTFQIPADTLATYLLMLEGHYHANVAYHNSLHAADVAQSTHVLLATPALEAVFTDLEILAALFASAIHDVDHPGVSNQFLINTNSELALMYNDASVLENHHLAVGFKLLQAENCDIFQNLSAKQRLSLRRMVIDMVLATDMSKHMNLLADLKTMVETKKVTSLGVLLLDNYSDRIQVLQNLVHCADLSNPTKPLPLYRQWTDRIMAEFFQQGDRERESGLDISPMCDKHTASVEKSQVGFIDYIAHPLWETWADLVHPDAQDLLDTLEDNREWYQSKIPRSPSDLTNPERDGPDRFQFELTLEEAEEEDEEEEEEGEETALAKEALELPDTELLSPEAGPDPGDLPLDNQRT

SEQ ID NO: 45 - DNA, 5120 bp, Homo sapiens
  source 1..5120: mol_type = other DNA
ttcgacgtgatcagacccaactcagacccggtcatacttggaccgaatgctgccaaatcccccacctctacccagatctgagcctacgcggggtgccgacccagctcgtggacggggatacggtgacctttgacccaaaagtcttggccgggaccagccggacactggccctcggccgggagctccgagtctcaggcggtcccggttgtcttcctgtcggtgccgcttccgcctgcccttcttgaaaacccacccccagctttgacctggaaaatgggctctcgtgtgggaggagggccctggaccctcagtccagccctggcctgggccggattatgcaggctccagtcccgcacagccagcggcgcgagtccttcctgtaccgctcagatagcgactatgaactctcgcccaaggccatgtctcggaactcctctgtggccagcgacctacatggagaggacatgattgtgacgccctttgcccaggtcctggccagtctgcggaccgttcggagcaacgtggcggcccttgcccgccagcaatgcctaggagcagccaagcagggacccgtcggaaacccttcatccagcaatcagctccctcctgcagaggacacggggcagaagctggcattggagacgctagacgagctggactggtgcctggatcagttggagacgctgcagacccggcactcggtgggggagatggcctccaacaagttcaagcggatcctgaaccgggagttgacccacctgtccgaaaccagccgctccgggaaccaggtgtccgagtacatctcccggaccttcctggaccagcagaccgaggtggagctgcccaaggtgaccgctgaggaggccccacagcccatgtcccggatcagtggcctacatgggctctgccacagtgccagcctctcctcagccactgtcccacgctttggggtccagactgaccaggaggagcaactggccaaggagctagaagacaccaacaagtggggacttgatgtgttcaaggtggcggagctaagtgggaaccggcccctcacagctatcatattcagcatttttcaggagcgggacctgctgaagacattccagatcccagcagacacactggccacctacctgctgatgctggaaggtcactaccacgccaatgtggcctaccacaacagcctacatgccgccgacgtggcccagtccacgcatgtgctgctggctacgcccgccctcgaggctgtgttcacagacttggaaatcctggctgccctctttgcaagcgccatccacgacgtggaccatcctggggtctccaaccagtttctgattaacaccaactcagagctggcgcttatgtacaacgacgcctcggtgctggagaaccatcacctggctgtgggcttcaagctgctgcaggcagagaactgcgatatcttccagaacctcagcgccaagcagcgactgagtctgcgcaggatggtcattgacatggtgctggccacagacatgtccaaacacatgaacctcctggccgacctcaagaccatggtggagaccaagaaggtgacaagcctcggtgtcctcctcctggacaactattccgaccgaatccaggtcttgcagaacctggtgcactgtgctgatctgagcaaccccaccaagccgctgcccctgtaccgccagtggacggaccgcatcatggccgagttcttccagcagggagaccgcgagcgtgagtcgggcctggacatcagtcccatgtgtgacaagcatacggcctcagtggagaagtcccaggtgggtttcattgactacattgctcacccactgtgggagacttgggctgacctggtccacccagatgcacaggacctgctggacacgctggaggacaatcgagagtggtaccagagcaagatcccccgaagtccctcagacctcaccaaccccgagcgggacgggcctgacagattccagtttgaactgactctggaggaggcagaggaagaggatgaggaggaagaagaggagggggaagagacagctttagccaaagaggccttggagttgcctgacactgaactcctgtcccctgaagccggcccagaccctggggacttacccctcgacaaccagaggacttagggccagccctgcgtgaactgcaggggcaatggatggtaaagccctttggctcttggcaggcagactttccaggaagaggctccatgtggctcctgcttcactttcccacccatttagggagacaatcaagctcttagttataggtggctcccagggtctaattggaggcacctggctggggtccactctgaccctagacttgcctaaaagagctctctaaggggcagcctcttacgatgccctggtgtctttctcctgggcttctatccctgtgaggagaggtgctgtctgctggagcctctagtccaccctctccagtggtcactcttgagtcacatctgtcacttaattatttccttctttatcaaatatttattgctcatctacttcgtgccagctttctgcctctgtagtagccctgcacaaagggtggggagtcaggagaccatcccaaaggcatctccctgtcttcctctaccaagcggctctctgcaagagcatggaaatgtgagtggggaaaattttcagcaccaaagcttcactcatacccagttttgtttctgaaactacggtagggggcaggaagaggagcagaaaagaagggctgggcaaggcatagtggcttatgcctgtaatcccggtactttgggaggctgaggtgggaggactgcttaagctcaggagtttgagaccagcctgggcaacatagcaagacccccaccatctctgaaaaaaaaaattagccaggcatggtggtgtgcacctgagaatcccagctactcagaaggttgagacaaaggggatcgcttgagcccaggagttggaggctgaagagagctatgactgcatcactgcactccagcctgggcaacacagcaagatcctgtctaaaaataaaaagaaaagagaaggaaaggaaagagacggggctctgaggccgagcacagtggcccatgcctataatcccagcactttgggaggctgaggcaggtggatcacctgaggttaggagttcgagaccagcctggccaacatggtgaaaccccatctctactaaaaatacaaaaattggctgggcatggtggcgggtgcctgtaatcccagctactggggaggctgaggcaggagaatcacttgaattcaggaggtggaggttgcagtgagccgacatcatgccactgcactccagcctgggcgacagagcaagacactgtctcaaaaaagaaaagaaaaaaaaaaaagccgggccaggtggctcacgcctgtaatcctagcactttgggaggctgagtgggggtggatcgcctgagatcaggagttcaaaatcagcctggccaacatagtgaaaccctgtctctactaaaaatacaaaaaattagaggctgggtgcggcggctcacacctgtaatcccagaactttgggaggccgaggcgggtggatcacgaggtcaggagttcaagaccagcctggccaacacggtgaaaccccatctctactaaaaatacacaaattagctgggcatggtgttgggtgcctgaatcccagctactcgggaggctgaggcaggagaatcgcttgaatccgggaggcggggcttgcagtgagccgagatcgtgccattgcactccagcctgggtgacagagcaagactccgtctcaaaaagaaaaaaaaaaaattagccaggcatggtggcaggtgcctgtaatcccagctacttgagaggctgaggcaggagaatcgcttgaacccgggaggtggaggttgtggtgagccgaggtcgcgccactgcactccagcctgggcaacgacaacaacaataaaaagagggggctctgtgcccggcatgtctctgaagactgattgaacctatgcaccagttgttgctttaagtcgctttattttctgtctttggtgtctctggatgtaggagccccctgctttctctgtccgcagaactccatactgggtcccctacgtgttcctccttccctaggacagcaacaaaaacacacaattttccctctctagcaggtctctaagtctcctgattcctgaaactgcctcagactccccctagagggagggaggcccctgaggctttcttgccatcatagcctcttctgggcctcagtttcccctctgtaacctgatcctagtacttggataaactccgacgaggtgtggggggttgttgtctgtgacctccctgaaatatcttagacatttggggtactgagcatttatctggggttaaataaaatctttacatcttaagacattcgattgaccaaattgagtgtcctggccatttcactgatgaggaaactgaggcgcagagaggtcctcttgccagctcaaagtcaagcatctgggcgcccaatgttagccagcggcaccccctggtggcgggcgtgggagacacggcggggcgcgcttgtcgggggttggggggtgggtcggaggggtggcatcctccagccctgatggtcccacttaccgcacctcgccgggaagagctcgtcctgctggtcgggcctccgagcggactgggcagcaccatgctcaagcctagggttcgatccccgcctccggaagcctcagtatccatccctcccctctgcctccctcttcgcgtgcctgaatatttatacaagatacaggcgtcatcacagccgccctcggcttccagagcagctggcttcgttcataaatattataaccactcagaattcatcatcatcacagttaatgataaaattccacagtgccagaactaaaagtcatccgggttcacgaacttggtgcatttccttccagacttttaaaaagaagatatttagggaatttttttttcaagatttttccccccagtccgcttacaaagtaataccatgttcgctgtaaaaaatttggaaataatggaaatgtataaagaaggaaataaaattctgctgtatctcca

SEQ ID NO: 46 - protein, 606 aa, Homo sapiens
MQAPVPHSQRRESFLYRSDSDYELSPKAMSRNSSVASDLHGEDMIVTPFAQVLASLRTVRSNVAALARQQCLGAAKQGPVGNPSSSNQLPPAEDTGQKLALETLDELDWCLDQLETLQTRHSVGEMASNKFKRILNRELTHLSETSRSGNQVSEYISRTFLDQQTEVELPKVTAEEAPQPMSRISGLHGLCHSASLSSATVPRFGVQTDQEEQLAKELEDTNKWGLDVFKVAELSGNRPLTAIIFSIFQERDLLKTFQIPADTLATYLLMLEGHYHANVAYHNSLHAADVAQSTHVLLATPALEAVFTDLEILAALFASAIHDVDHPGVSNQFLINTNSELALMYNDASVLENHHLAVGFKLLQAENCDIFQNLSAKQRLSLRRMVIDMVLATDMSKHMNLLADLKTMVETKKVTSLGVLLLDNYSDRIQVLQNLVHCADLSNPTKPLPLYRQWTDRIMAEFFQQGDRERESGLDISPMCDKHTASVEKSQVGFIDYIAHPLWETWADLVHPDAQDLLDTLEDNREWYQSKIPRSPSDLTNPERDGPDRFQFELTLEEAEEEDEEEEEEGEETALAKEALELPDTELLSPEAGPDPGDLPLDNQRT

SEQ ID NO: 47 - DNA, 5030 bp, Homo sapiens
  source 1..5030: mol_type = other DNA
ccagcctccacgcagtcctggcgatgcagggcccccccgcgcccgccccggtccccgggcccggctcccctcggggatccccgcgcggctcccccgggctcttcaggaagcttttggtgaatcagagcatccgcctgcagcggcgcttcacggtggcccatccgctgtgctttgacctggaaaatgggctctcgtgtgggaggagggccctggaccctcagtccagccctggcctgggccggattatgcaggctccagtcccgcacagccagcggcgcgagtccttcctgtaccgctcagatagcgactatgaactctcgcccaaggccatgtctcggaactcctctgtggccagcgacctacatggagaggacatgattgtgacgccctttgcccaggtcctggccagtctgcggaccgttcggagcaacgtggcggcccttgcccgccagcaatgcctaggagcagccaagcagggacccgtcggaaacccttcatccagcaatcagctccctcctgcagaggacacggggcagaagctggcattggagacgctagacgagctggactggtgcctggatcagttggagacgctgcagacccggcactcggtgggggagatggcctccaacaagttcaagcggatcctgaaccgggagttgacccacctgtccgaaaccagccgctccgggaaccaggtgtccgagtacatctcccggaccttcctggaccagcagaccgaggtggagctgcccaaggtgaccgctgaggaggccccacagcccatgtcccggatcagtggcctacatgggctctgccacagtgccagcctctcctcagccactgtcccacgctttggggtccagactgaccaggaggagcaactggccaaggagctagaagacaccaacaagtggggacttgatgtgttcaaggtggcggagctaagtgggaaccggcccctcacagctatcatattcagcatttttcaggagcgggacctgctgaagacattccagatcccagcagacacactggccacctacctgctgatgctggaaggtcactaccacgccaatgtggcctaccacaacagcctacatgccgccgacgtggcccagtccacgcatgtgctgctggctacgcccgccctcgaggctgtgttcacagacttggaaatcctggctgccctctttgcaagcgccatccacgacgtggaccatcctggggtctccaaccagtttctgattaacaccaactcagagctggcgcttatgtacaacgacgcctcggtgctggagaaccatcacctggctgtgggcttcaagctgctgcaggcagagaactgcgatatcttccagaacctcagcgccaagcagcgactgagtctgcgcaggatggtcattgacatggtgctggccacagacatgtccaaacacatgaacctcctggccgacctcaagaccatggtggagaccaagaaggtgacaagcctcggtgtcctcctcctggacaactattccgaccgaatccaggtcttgcagaacctggtgcactgtgctgatctgagcaaccccaccaagccgctgcccctgtaccgccagtggacggaccgcatcatggccgagttcttccagcagggagaccgcgagcgtgagtcgggcctggacatcagtcccatgtgtgacaagcatacggcctcagtggagaagtcccaggtgggtttcattgactacattgctcacccactgtgggagacttgggctgacctggtccacccagatgcacaggacctgctggacacgctggaggacaatcgagagtggtaccagagcaagatcccccgaagtccctcagacctcaccaaccccgagcgggacgggcctgacagattccagtttgaactgactctggaggaggcagaggaagaggatgaggaggaagaagaggagggggaagagacagctttagccaaagaggccttggagttgcctgacactgaactcctgtcccctgaagccggcccagaccctggggacttacccctcgacaaccagaggacttagggccagccctgcgtgaactgcaggggcaatggatggtaaagccctttggctcttggcaggcagactttccaggaagaggctccatgtggctcctgcttcactttcccacccatttagggagacaatcaagctcttagttataggtggctcccagggtctaattggaggcacctggctggggtccactctgaccctagacttgcctaaaagagctctctaaggggcagcctcttacgatgccctggtgtctttctcctgggcttctatccctgtgaggagaggtgctgtctgctggagcctctagtccaccctctccagtggtcactcttgagtcacatctgtcacttaattatttccttctttatcaaatatttattgctcatctacttcgtgccagctttctgcctctgtagtagccctgcacaaagggtggggagtcaggagaccatcccaaaggcatctccctgtcttcctctaccaagcggctctctgcaagagcatggaaatgtgagtggggaaaattttcagcaccaaagcttcactcatacccagttttgtttctgaaactacggtagggggcaggaagaggagcagaaaagaagggctgggcaaggcatagtggcttatgcctgtaatcccggtactttgggaggctgaggtgggaggactgcttaagctcaggagtttgagaccagcctgggcaacatagcaagacccccaccatctctgaaaaaaaaaattagccaggcatggtggtgtgcacctgagaatcccagctactcagaaggttgagacaaaggggatcgcttgagcccaggagttggaggctgaagagagctatgactgcatcactgcactccagcctgggcaacacagcaagatcctgtctaaaaataaaaagaaaagagaaggaaaggaaagagacggggctctgaggccgagcacagtggcccatgcctataatcccagcactttgggaggctgaggcaggtggatcacctgaggttaggagttcgagaccagcctggccaacatggtgaaaccccatctctactaaaaatacaaaaattggctgggcatggtggcgggtgcctgtaatcccagctactggggaggctgaggcaggagaatcacttgaattcaggaggtggaggttgcagtgagccgacatcatgccactgcactccagcctgggcgacagagcaagacactgtctcaaaaaagaaaagaaaaaaaaaaaagccgggccaggtggctcacgcctgtaatcctagcactttgggaggctgagtgggggtggatcgcctgagatcaggagttcaaaatcagcctggccaacatagtgaaaccctgtctctactaaaaatacaaaaaattagaggctgggtgcggcggctcacacctgtaatcccagaactttgggaggccgaggcgggtggatcacgaggtcaggagttcaagaccagcctggccaacacggtgaaaccccatctctactaaaaatacacaaattagctgggcatggtgttgggtgcctgaatcccagctactcgggaggctgaggcaggagaatcgcttgaatccgggaggcggggcttgcagtgagccgagatcgtgccattgcactccagcctgggtgacagagcaagactccgtctcaaaaagaaaaaaaaaaaattagccaggcatggtggcaggtgcctgtaatcccagctacttgagaggctgaggcaggagaatcgcttgaacccgggaggtggaggttgtggtgagccgaggtcgcgccactgcactccagcctgggcaacgacaacaacaataaaaagagggggctctgtgcccggcatgtctctgaagactgattgaacctatgcaccagttgttgctttaagtcgctttattttctgtctttggtgtctctggatgtaggagccccctgctttctctgtccgcagaactccatactgggtcccctacgtgttcctccttccctaggacagcaacaaaaacacacaattttccctctctagcaggtctctaagtctcctgattcctgaaactgcctcagactccccctagagggagggaggcccctgaggctttcttgccatcatagcctcttctgggcctcagtttcccctctgtaacctgatcctagtacttggataaactccgacgaggtgtggggggttgttgtctgtgacctccctgaaatatcttagacatttggggtactgagcatttatctggggttaaataaaatctttacatcttaagacattcgattgaccaaattgagtgtcctggccatttcactgatgaggaaactgaggcgcagagaggtcctcttgccagctcaaagtcaagcatctgggcgcccaatgttagccagcggcaccccctggtggcgggcgtgggagacacggcggggcgcgcttgtcgggggttggggggtgggtcggaggggtggcatcctccagccctgatggtcccacttaccgcacctcgccgggaagagctcgtcctgctggtcgggcctccgagcggactgggcagcaccatgctcaagcctagggttcgatccccgcctccggaagcctcagtatccatccctcccctctgcctccctcttcgcgtgcctgaatatttatacaagatacaggcgtcatcacagccgccctcggcttccagagcagctggcttcgttcataaatattataaccactcagaattcatcatcatcacagttaatgataaaattccacagtgccagaactaaaagtcatccgggttcacgaacttggtgcatttccttccagacttttaaaaagaagatatttagggaatttttttttcaagatttttccccccagtccgcttacaaagtaataccatgttcgctgtaaaaaatttggaaataatggaaatgtataaagaaggaaataaaattctgctgtatctcca

SEQ ID NO: 48 - protein, 680 aa, Homo sapiens
MQGPPAPAPVPGPGSPRGSPRGSPGLFRKLLVNQSIRLQRRFTVAHPLCFDLENGLSCGRRALDPQSSPGLGRIMQAPVPHSQRRESFLYRSDSDYELSPKAMSRNSSVASDLHGEDMIVTPFAQVLASLRTVRSNVAALARQQCLGAAKQGPVGNPSSSNQLPPAEDTGQKLALETLDELDWCLDQLETLQTRHSVGEMASNKFKRILNRELTHLSETSRSGNQVSEYISRTFLDQQTEVELPKVTAEEAPQPMSRISGLHGLCHSASLSSATVPRFGVQTDQEEQLAKELEDTNKWGLDVFKVAELSGNRPLTAIIFSIFQERDLLKTFQIPADTLATYLLMLEGHYHANVAYHNSLHAADVAQSTHVLLATPALEAVFTDLEILAALFASAIHDVDHPGVSNQFLINTNSELALMYNDASVLENHHLAVGFKLLQAENCDIFQNLSAKQRLSLRRMVIDMVLATDMSKHMNLLADLKTMVETKKVTSLGVLLLDNYSDRIQVLQNLVHCADLSNPTKPLPLYRQWTDRIMAEFFQQGDRERESGLDISPMCDKHTASVEKSQVGFIDYIAHPLWETWADLVHPDAQDLLDTLEDNREWYQSKIPRSPSDLTNPERDGPDRFQFELTLEEAEEEDEEEEEEGEETALAKEALELPDTELLSPEAGPDPGDLPLDNQRT

SEQ ID NO: 49 - DNA, 4980 bp, Homo sapiens
  source 1..4980: mol_type = other DNA
ccagcctccacgcagtcctggcgatgcagggcccccccgcgcccgccccggtccccgggcccggctcccctcggggatccccgcgcggctcccccgggctcttcaggaagcttttggtgaatcagagcatccgcctgcagcggcgcttcacggtggcccatccgctgtgctttgacctggaaaatgggctctcgtgtgggaggagggccctggaccctcagtccagccctggcctgggccggattatgcaggctccagtcccgcacagccagcggcgcgagtccttcctgtaccgctcagatagcgactatgaactctcgcccaaggccatgtctcggaactcctctgtggccagcgacctacatggagaggacatgattgtgacgccctttgcccaggtcctggccagtctgcggaccgttcggagcaacgtggcggcccttgcccgccagcaatgcctaggagcagccaaaggacacggggcagaagctggcattggagacgctagacgagctggactggtgcctggatcagttggagacgctgcagacccggcactcggtgggggagatggcctccaacaagttcaagcggatcctgaaccgggagttgacccacctgtccgaaaccagccgctccgggaaccaggtgtccgagtacatctcccggaccttcctggaccagcagaccgaggtggagctgcccaaggtgaccgctgaggaggccccacagcccatgtcccggatcagtggcctacatgggctctgccacagtgccagcctctcctcagccactgtcccacgctttggggtccagactgaccaggaggagcaactggccaaggagctagaagacaccaacaagtggggacttgatgtgttcaaggtggcggagctaagtgggaaccggcccctcacagctatcatattcagcatttttcaggagcgggacctgctgaagacattccagatcccagcagacacactggccacctacctgctgatgctggaaggtcactaccacgccaatgtggcctaccacaacagcctacatgccgccgacgtggcccagtccacgcatgtgctgctggctacgcccgccctcgaggctgtgttcacagacttggaaatcctggctgccctctttgcaagcgccatccacgacgtggaccatcctggggtctccaaccagtttctgattaacaccaactcagagctggcgcttatgtacaacgacgcctcggtgctggagaaccatcacctggctgtgggcttcaagctgctgcaggcagagaactgcgatatcttccagaacctcagcgccaagcagcgactgagtctgcgcaggatggtcattgacatggtgctggccacagacatgtccaaacacatgaacctcctggccgacctcaagaccatggtggagaccaagaaggtgacaagcctcggtgtcctcctcctggacaactattccgaccgaatccaggtcttgcagaacctggtgcactgtgctgatctgagcaaccccaccaagccgctgcccctgtaccgccagtggacggaccgcatcatggccgagttcttccagcagggagaccgcgagcgtgagtcgggcctggacatcagtcccatgtgtgacaagcatacggcctcagtggagaagtcccaggtgggtttcattgactacattgctcacccactgtgggagacttgggctgacctggtccacccagatgcacaggacctgctggacacgctggaggacaatcgagagtggtaccagagcaagatcccccgaagtccctcagacctcaccaaccccgagcgggacgggcctgacagattccagtttgaactgactctggaggaggcagaggaagaggatgaggaggaagaagaggagggggaagagacagctttagccaaagaggccttggagttgcctgacactgaactcctgtcccctgaagccggcccagaccctggggacttacccctcgacaaccagaggacttagggccagccctgcgtgaactgcaggggcaatggatggtaaagccctttggctcttggcaggcagactttccaggaagaggctccatgtggctcctgcttcactttcccacccatttagggagacaatcaagctcttagttataggtggctcccagggtctaattggaggcacctggctggggtccactctgaccctagacttgcctaaaagagctctctaaggggcagcctcttacgatgccctggtgtctttctcctgggcttctatccctgtgaggagaggtgctgtctgctggagcctctagtccaccctctccagtggtcactcttgagtcacatctgtcacttaattatttccttctttatcaaatatttattgctcatctacttcgtgccagctttctgcctctgtagtagccctgcacaaagggtggggagtcaggagaccatcccaaaggcatctccctgtcttcctctaccaagcggctctctgcaagagcatggaaatgtgagtggggaaaattttcagcaccaaagcttcactcatacccagttttgtttctgaaactacggtagggggcaggaagaggagcagaaaagaagggctgggcaaggcatagtggcttatgcctgtaatcccggtactttgggaggctgaggtgggaggactgcttaagctcaggagtttgagaccagcctgggcaacatagcaagacccccaccatctctgaaaaaaaaaattagccaggcatggtggtgtgcacctgagaatcccagctactcagaaggttgagacaaaggggatcgcttgagcccaggagttggaggctgaagagagctatgactgcatcactgcactccagcctgggcaacacagcaagatcctgtctaaaaataaaaagaaaagagaaggaaaggaaagagacggggctctgaggccgagcacagtggcccatgcctataatcccagcactttgggaggctgaggcaggtggatcacctgaggttaggagttcgagaccagcctggccaacatggtgaaaccccatctctactaaaaatacaaaaattggctgggcatggtggcgggtgcctgtaatcccagctactggggaggctgaggcaggagaatcacttgaattcaggaggtggaggttgcagtgagccgacatcatgccactgcactccagcctgggcgacagagcaagacactgtctcaaaaaagaaaagaaaaaaaaaaaagccgggccaggtggctcacgcctgtaatcctagcactttgggaggctgagtgggggtggatcgcctgagatcaggagttcaaaatcagcctggccaacatagtgaaaccctgtctctactaaaaatacaaaaaattagaggctgggtgcggcggctcacacctgtaatcccagaactttgggaggccgaggcgggtggatcacgaggtcaggagttcaagaccagcctggccaacacggtgaaaccccatctctactaaaaatacacaaattagctgggcatggtgttgggtgcctgaatcccagctactcgggaggctgaggcaggagaatcgcttgaatccgggaggcggggcttgcagtgagccgagatcgtgccattgcactccagcctgggtgacagagcaagactccgtctcaaaaagaaaaaaaaaaaattagccaggcatggtggcaggtgcctgtaatcccagctacttgagaggctgaggcaggagaatcgcttgaacccgggaggtggaggttgtggtgagccgaggtcgcgccactgcactccagcctgggcaacgacaacaacaataaaaagagggggctctgtgcccggcatgtctctgaagactgattgaacctatgcaccagttgttgctttaagtcgctttattttctgtctttggtgtctctggatgtaggagccccctgctttctctgtccgcagaactccatactgggtcccctacgtgttcctccttccctaggacagcaacaaaaacacacaattttccctctctagcaggtctctaagtctcctgattcctgaaactgcctcagactccccctagagggagggaggcccctgaggctttcttgccatcatagcctcttctgggcctcagtttcccctctgtaacctgatcctagtacttggataaactccgacgaggtgtggggggttgttgtctgtgacctccctgaaatatcttagacatttggggtactgagcatttatctggggttaaataaaatctttacatcttaagacattcgattgaccaaattgagtgtcctggccatttcactgatgaggaaactgaggcgcagagaggtcctcttgccagctcaaagtcaagcatctgggcgcccaatgttagccagcggcaccccctggtggcgggcgtgggagacacggcggggcgcgcttgtcgggggttggggggtgggtcggaggggtggcatcctccagccctgatggtcccacttaccgcacctcgccgggaagagctcgtcctgctggtcgggcctccgagcggactgggcagcaccatgctcaagcctagggttcgatccccgcctccggaagcctcagtatccatccctcccctctgcctccctcttcgcgtgcctgaatatttatacaagatacaggcgtcatcacagccgccctcggcttccagagcagctggcttcgttcataaatattataaccactcagaattcatcatcatcacagttaatgataaaattccacagtgccagaactaaaagtcatccgggttcacgaacttggtgcatttccttccagacttttaaaaagaagatatttagggaatttttttttcaagatttttccccccagtccgcttacaaagtaataccatgttcgctgtaaaaaatttggaaataatggaaatgtataaagaaggaaataaaattctgctgtatctcca

SEQ ID NO: 50 - protein, 481 aa, Homo sapiens
MASNKFKRILNRELTHLSETSRSGNQVSEYISRTFLDQQTEVELPKVTAEEAPQPMSRISGLHGLCHSASLSSATVPRFGVQTDQEEQLAKELEDTNKWGLDVFKVAELSGNRPLTAIIFSIFQERDLLKTFQIPADTLATYLLMLEGHYHANVAYHNSLHAADVAQSTHVLLATPALEAVFTDLEILAALFASAIHDVDHPGVSNQFLINTNSELALMYNDASVLENHHLAVGFKLLQAENCDIFQNLSAKQRLSLRRMVIDMVLATDMSKHMNLLADLKTMVETKKVTSLGVLLLDNYSDRIQVLQNLVHCADLSNPTKPLPLYRQWTDRIMAEFFQQGDRERESGLDISPMCDKHTASVEKSQVGFIDYIAHPLWETWADLVHPDAQDLLDTLEDNREWYQSKIPRSPSDLTNPERDGPDRFQFELTLEEAEEEDEEEEEEGEETALAKEALELPDTELLSPEAGPDPGDLPLDNQRT

SEQ ID NO: 51 - DNA, 5341 bp, Homo sapiens
  source 1..5341: mol_type = other DNA
ctcctgcctgtcctgagcttccacaaaagcaccatctgggcatcgacagctcctcggtgtcggccccaccttgagccccagttccaccttctaccgcttcagcacctccggcgcggacagctcctcgctgtcgcctccactcccggccctgggccggacccgggagcagacgctcctcggcgcccgctcacggggacgagtcctgctccctgctatcccagacccctttctctggcgcatggagaacctgggggtcggcgaaggggcagaggcttgcagcaggttgagtcgctctcgcggccgccacagcatgaccagagccccgaagcacctgtggcggcaaccccggcgccccatccgcatccaacagcgcttctattcggatccggacaagtccgcgggctgccgcgagagggacctgagcccgcggccggagctcaggaagtcgcggctctcctggcccgtttcctcctgcaggcgctttgacctggaaaatgggctctcgtgtgggaggagggccctggaccctcagtccagccctggcctgggccggattatgcaggctccagtcccgcacagccagcggcgcgagtccttcctgtaccgctcagatagcgactatgaactctcgcccaaggccatgtctcggaactcctctgtggccagcgacctacatggagaggacatgattgtgacgccctttgcccaggtcctggccagtctgcggaccgttcggagcaacgtggcggcccttgcccgccagcaatgcctaggagcagccaagcagggacccgtcggaaacccttcatccagcaatcagctccctcctgcagaggacacggggcagaagctggcattggagacgctagacgagctggactggtgcctggatcagttggagacgctgcagacccggcactcggtgggggagatggcctccaacaagttcaagcggatcctgaaccgggagttgacccacctgtccgaaaccagccgctccgggaaccaggtgtccgagtacatctcccggaccttcctggaccagcagaccgaggtggagctgcccaaggtgaccgctgaggaggccccacagcccatgtcccggatcagtggcctacatgggctctgccacagtgccagcctctcctcagccactgtcccacgctttggggtccagactgaccaggaggagcaactggccaaggagctagaagacaccaacaagtggggacttgatgtgttcaaggtggcggagctaagtgggaaccggcccctcacagctatcatattcagcatttttcaggagcgggacctgctgaagacattccagatcccagcagacacactggccacctacctgctgatgctggaaggtcactaccacgccaatgtggcctaccacaacagcctacatgccgccgacgtggcccagtccacgcatgtgctgctggctacgcccgccctcgaggctgtgttcacagacttggaaatcctggctgccctctttgcaagcgccatccacgacgtggaccatcctggggtctccaaccagtttctgattaacaccaactcagagctggcgcttatgtacaacgacgcctcggtgctggagaaccatcacctggctgtgggcttcaagctgctgcaggcagagaactgcgatatcttccagaacctcagcgccaagcagcgactgagtctgcgcaggatggtcattgacatggtgctggccacagacatgtccaaacacatgaacctcctggccgacctcaagaccatggtggagaccaagaaggtgacaagcctcggtgtcctcctcctggacaactattccgaccgaatccaggtcttgcagaacctggtgcactgtgctgatctgagcaaccccaccaagccgctgcccctgtaccgccagtggacggaccgcatcatggccgagttcttccagcagggagaccgcgagcgtgagtcgggcctggacatcagtcccatgtgtgacaagcatacggcctcagtggagaagtcccaggtgggtttcattgactacattgctcacccactgtgggagacttgggctgacctggtccacccagatgcacaggacctgctggacacgctggaggacaatcgagagtggtaccagagcaagatcccccgaagtccctcagacctcaccaaccccgagcgggacgggcctgacagattccagtttgaactgactctggaggaggcagaggaagaggatgaggaggaagaagaggagggggaagagacagctttagccaaagaggccttggagttgcctgacactgaactcctgtcccctgaagccggcccagaccctggggacttacccctcgacaaccagaggacttagggccagccctgcgtgaactgcaggggcaatggatggtaaagccctttggctcttggcaggcagactttccaggaagaggctccatgtggctcctgcttcactttcccacccatttagggagacaatcaagctcttagttataggtggctcccagggtctaattggaggcacctggctggggtccactctgaccctagacttgcctaaaagagctctctaaggggcagcctcttacgatgccctggtgtctttctcctgggcttctatccctgtgaggagaggtgctgtctgctggagcctctagtccaccctctccagtggtcactcttgagtcacatctgtcacttaattatttccttctttatcaaatatttattgctcatctacttcgtgccagctttctgcctctgtagtagccctgcacaaagggtggggagtcaggagaccatcccaaaggcatctccctgtcttcctctaccaagcggctctctgcaagagcatggaaatgtgagtggggaaaattttcagcaccaaagcttcactcatacccagttttgtttctgaaactacggtagggggcaggaagaggagcagaaaagaagggctgggcaaggcatagtggcttatgcctgtaatcccggtactttgggaggctgaggtgggaggactgcttaagctcaggagtttgagaccagcctgggcaacatagcaagacccccaccatctctgaaaaaaaaaattagccaggcatggtggtgtgcacctgagaatcccagctactcagaaggttgagacaaaggggatcgcttgagcccaggagttggaggctgaagagagctatgactgcatcactgcactccagcctgggcaacacagcaagatcctgtctaaaaataaaaagaaaagagaaggaaaggaaagagacggggctctgaggccgagcacagtggcccatgcctataatcccagcactttgggaggctgaggcaggtggatcacctgaggttaggagttcgagaccagcctggccaacatggtgaaaccccatctctactaaaaatacaaaaattggctgggcatggtggcgggtgcctgtaatcccagctactggggaggctgaggcaggagaatcacttgaattcaggaggtggaggttgcagtgagccgacatcatgccactgcactccagcctgggcgacagagcaagacactgtctcaaaaaagaaaagaaaaaaaaaaaagccgggccaggtggctcacgcctgtaatcctagcactttgggaggctgagtgggggtggatcgcctgagatcaggagttcaaaatcagcctggccaacatagtgaaaccctgtctctactaaaaatacaaaaaattagaggctgggtgcggcggctcacacctgtaatcccagaactttgggaggccgaggcgggtggatcacgaggtcaggagttcaagaccagcctggccaacacggtgaaaccccatctctactaaaaatacacaaattagctgggcatggtgttgggtgcctgaatcccagctactcgggaggctgaggcaggagaatcgcttgaatccgggaggcggggcttgcagtgagccgagatcgtgccattgcactccagcctgggtgacagagcaagactccgtctcaaaaagaaaaaaaaaaaattagccaggcatggtggcaggtgcctgtaatcccagctacttgagaggctgaggcaggagaatcgcttgaacccgggaggtggaggttgtggtgagccgaggtcgcgccactgcactccagcctgggcaacgacaacaacaataaaaagagggggctctgtgcccggcatgtctctgaagactgattgaacctatgcaccagttgttgctttaagtcgctttattttctgtctttggtgtctctggatgtaggagccccctgctttctctgtccgcagaactccatactgggtcccctacgtgttcctccttccctaggacagcaacaaaaacacacaattttccctctctagcaggtctctaagtctcctgattcctgaaactgcctcagactccccctagagggagggaggcccctgaggctttcttgccatcatagcctcttctgggcctcagtttcccctctgtaacctgatcctagtacttggataaactccgacgaggtgtggggggttgttgtctgtgacctccctgaaatatcttagacatttggggtactgagcatttatctggggttaaataaaatctttacatcttaagacattcgattgaccaaattgagtgtcctggccatttcactgatgaggaaactgaggcgcagagaggtcctcttgccagctcaaagtcaagcatctgggcgcccaatgttagccagcggcaccccctggtggcgggcgtgggagacacggcggggcgcgcttgtcgggggttggggggtgggtcggaggggtggcatcctccagccctgatggtcccacttaccgcacctcgccgggaagagctcgtcctgctggtcgggcctccgagcggactgggcagcaccatgctcaagcctagggttcgatccccgcctccggaagcctcagtatccatccctcccctctgcctccctcttcgcgtgcctgaatatttatacaagatacaggcgtcatcacagccgccctcggcttccagagcagctggcttcgttcataaatattataaccactcagaattcatcatcatcacagttaatgataaaattccacagtgccagaactaaaagtcatccgggttcacgaacttggtgcatttccttccagacttttaaaaagaagatatttagggaatttttttttcaagatttttccccccagtccgcttacaaagtaataccatgttcgctgtaaaaaatttggaaataatggaaatgtataaagaaggaaataaaattctgctgtatctcca

SEQ ID NO: 52 - protein, 712 aa, Homo sapiens; identical to SEQ ID NO: 44

SEQ ID NO: 53 - DNA, 5774 bp, Homo sapiens
  source 1..5774: mol_type = other DNA
ccagcctccacgcagtcctggcgatgcagggcccccccgcgcccgccccggtccccgggcccggctcccctcggggatccccgcgcggctcccccgggctcttcaggaagcttttggtgaatcagagcatccgcctgcagcggcgcttcacggtggcccatccgctgtggtgaggctggacagagggcctggcggggtcaccgggacgcccggtgtggaggtgggaagggcagggacagggacaaggccagggacagctggggccggggccggagtccgggcttggacgctctgcctctccctcgctttctctgtatctctctccctctaccctaccttaccctacttttgtctcgcagttggtgactctgtctctctctgtctccgtctgtctccacccgccgcctggatataggcccaggggaccagccgtctgtctccttccagctgtgaggcccagagtgggacgggctgaggctcacgtctcctcctgaccctcgccggcctggggcaggcaggctgtgcgtcctggcagtgggaggagggggaaggggcactccttcccttggtgccccctcccaccagcatcctgtcccagtgccagcaaagagatgccctgggggcctcacaatgaactctgggtgtccacggaggaagacctgaattgagggggttttcgaggcagggcgttcgggagtcccaggctgagcgcgcgcctgcgcccggcagctgcttgcgctgcatcctctaagcactcggtccacccctctgggttcgaatccctgcctttccagaaacgactgtgacctcgtggggagggatgggggcaaggctggggttcggagtggggcttgtgggcgccgactgtggctggcatcctgcgcttggtccgcgccgaattggcacccacttgctttgacctggaaaatgggctctcgtgtgggaggagggccctggaccctcagtccagccctggcctgggccggattatgcaggctccagtcccgcacagccagcggcgcgagtccttcctgtaccgctcagatagcgactatgaactctcgcccaaggccatgtctcggaactcctctgtggccagcgacctacatggagaggacatgattgtgacgccctttgcccaggtcctggccagtctgcggaccgttcggagcaacgtggcggcccttgcccgccagcaatgcctaggagcagccaagcagggacccgtcggaaacccttcatccagcaatcagctccctcctgcagaggacacggggcagaagctggcattggagacgctagacgagctggactggtgcctggatcagttggagacgctgcagacccggcactcggtgggggagatggcctccaacaagttcaagcggatcctgaaccgggagttgacccacctgtccgaaaccagccgctccgggaaccaggtgtccgagtacatctcccggaccttcctggaccagcagaccgaggtggagctgcccaaggtgaccgctgaggaggccccacagcccatgtcccggatcagtggcctacatgggctctgccacagtgccagcctctcctcagccactgtcccacgctttggggtccagactgaccaggaggagcaactggccaaggagctagaagacaccaacaagtggggacttgatgtgttcaaggtggcggagctaagtgggaaccggcccctcacagctatcatattcagcatttttcaggagcgggacctgctgaagacattccagatcccagcagacacactggccacctacctgctgatgctggaaggtcactaccacgccaatgtggcctaccacaacagcctacatgccgccgacgtggcccagtccacgcatgtgctgctggctacgcccgccctcgaggctgtgttcacagacttggaaatcctggctgccctctttgcaagcgccatccacgacgtggaccatcctggggtctccaaccagtttctgattaacaccaactcagagctggcgcttatgtacaacgacgcctcggtgctggagaaccatcacctggctgtgggcttcaagctgctgcaggcagagaactgcgatatcttccagaacctcagcgccaagcagcgactgagtctgcgcaggatggtcattgacatggtgctggccacagacatgtccaaacacatgaacctcctggccgacctcaagaccatggtggagaccaagaaggtgacaagcctcggtgtcctcctcctggacaactattccgaccgaatccaggtcttgcagaacctggtgcactgtgctgatctgagcaaccccaccaagccgctgcccctgtaccgccagtggacggaccgcatcatggccgagttcttccagcagggagaccgcgagcgtgagtcgggcctggacatcagtcccatgtgtgacaagcatacggcctcagtggagaagtcccaggtgggtttcattgactacattgctcacccactgtgggagacttgggctgacctggtccacccagatgcacaggacctgctggacacgctggaggacaatcgagagtggtaccagagcaagatcccccgaagtccctcagacctcaccaaccccgagcgggacgggcctgacagattccagtttgaactgactctggaggaggcagaggaagaggatgaggaggaagaagaggagggggaagagacagctttagccaaagaggccttggagttgcctgacactgaactcctgtcccctgaagccggcccagaccctggggacttacccctcgacaaccagaggacttagggccagccctgcgtgaactgcaggggcaatggatggtaaagccctttggctcttggcaggcagactttccaggaagaggctccatgtggctcctgcttcactttcccacccatttagggagacaatcaagctcttagttataggtggctcccagggtctaattggaggcacctggctggggtccactctgaccctagacttgcctaaaagagctctctaaggggcagcctcttacgatgccctggtgtctttctcctgggcttctatccctgtgaggagaggtgctgtctgctggagcctctagtccaccctctccagtggtcactcttgagtcacatctgtcacttaattatttccttctttatcaaatatttattgctcatctacttcgtgccagctttctgcctctgtagtagccctgcacaaagggtggggagtcaggagaccatcccaaaggcatctccctgtcttcctctaccaagcggctctctgcaagagcatggaaatgtgagtggggaaaattttcagcaccaaagcttcactcatacccagttttgtttctgaaactacggtagggggcaggaagaggagcagaaaagaagggctgggcaaggcatagtggcttatgcctgtaatcccggtactttgggaggctgaggtgggaggactgcttaagctcaggagtttgagaccagcctgggcaacatagcaagacccccaccatctctgaaaaaaaaaattagccaggcatggtggtgtgcacctgagaatcccagctactcagaaggttgagacaaaggggatcgcttgagcccaggagttggaggctgaagagagctatgactgcatcactgcactccagcctgggcaacacagcaagatcctgtctaaaaataaaaagaaaagagaaggaaaggaaagagacggggctctgaggccgagcacagtggcccatgcctataatcccagcactttgggaggctgaggcaggtggatcacctgaggttaggagttcgagaccagcctggccaacatggtgaaaccccatctctactaaaaatacaaaaattggctgggcatggtggcgggtgcctgtaatcccagctactggggaggctgaggcaggagaatcacttgaattcaggaggtggaggttgcagtgagccgacatcatgccactgcactccagcctgggcgacagagcaagacactgtctcaaaaaagaaaagaaaaaaaaaaaagccgggccaggtggctcacgcctgtaatcctagcactttgggaggctgagtgggggtggatcgcctgagatcaggagttcaaaatcagcctggccaacatagtgaaaccctgtctctactaaaaatacaaaaaattagaggctgggtgcggcggctcacacctgtaatcccagaactttgggaggccgaggcgggtggatcacgaggtcaggagttcaagaccagcctggccaacacggtgaaaccccatctctactaaaaatacacaaattagctgggcatggtgttgggtgcctgaatcccagctactcgggaggctgaggcaggagaatcgcttgaatccgggaggcggggcttgcagtgagccgagatcgtgccattgcactccagcctgggtgacagagcaagactccgtctcaaaaagaaaaaaaaaaaattagccaggcatggtggcaggtgcctgtaatcccagctacttgagaggctgaggcaggagaatcgcttgaacccgggaggtggaggttgtggtgagccgaggtcgcgccactgcactccagcctgggcaacgacaacaacaataaaaagagggggctctgtgcccggcatgtctctgaagactgattgaacctatgcaccagttgttgctttaagtcgctttattttctgtctttggtgtctctggatgtaggagccccctgctttctctgtccgcagaactccatactgggtcccctacgtgttcctccttccctaggacagcaacaaaaacacacaattttccctctctagcaggtctctaagtctcctgattcctgaaactgcctcagactccccctagagggagggaggcccctgaggctttcttgccatcatagcctcttctgggcctcagtttcccctctgtaacctgatcctagtacttggataaactccgacgaggtgtggggggttgttgtctgtgacctccctgaaatatcttagacatttggggtactgagcatttatctggggttaaataaaatctttacatcttaagacattcgattgaccaaattgagtgtcctggccatttcactgatgaggaaactgaggcgcagagaggtcctcttgccagctcaaagtcaagcatctgggcgcccaatgttagccagcggcaccccctggtggcgggcgtgggagacacggcggggcgcgcttgtcgggggttggggggtgggtcggaggggtggcatcctccagccctgatggtcccacttaccgcacctcgccgggaagagctcgtcctgctggtcgggcctccgagcggactgggcagcaccatgctcaagcctagggttcgatccccgcctccggaagcctcagtatccatccctcccctctgcctccctcttcgcgtgcctgaatatttatacaagatacaggcgtcatcacagccgccctcggcttccagagcagctggcttcgttcataaatattataaccactcagaattcatcatcatcacagttaatgataaaattccacagtgccagaactaaaagtcatccgggttcacgaacttggtgcatttccttccagacttttaaaaagaagatatttagggaatttttttttcaagatttttccccccagtccgcttacaaagtaataccatgttcgctgtaaaaaatttggaaataatggaaatgtataaagaaggaaataaaattctgctgtatctcca

SEQ ID NO: 54 - protein, 606 aa, Homo sapiens; identical to SEQ ID NO: 46

SEQ ID NO: 55 - DNA, 7753 bp, Homo sapiens
  source 1..7753: mol_type = other DNA
acttcaagtgccgtgcagaaggctcggcaggcggggcgggcgtggggccgcggctccgggttggggaccgaggagatccggctgtggaccagacgctcctctgcggggcgggcacccaagcgcgctcgccaccccctcgccatccgctagagccgggctcctggactgggactcgggcccgccgcacagttgaaaagtcgcatagtggtttttccgctcgcgtcgctgtgtgaaagttggctcgccgctctttgcacgccctccctggaggccgacccgagacgccaagctggagagaccgtgcctccccgaggccggccgccccgcgagcacagcctccgcccccgttgcactgccgggctgggcaatatgaaggagcagccctcatgtgccggcaccgggcatccgagcatggcggggtatggcaggatggccccctttgaactcgctagcggacccgtgaagcgcttgagaactgagtccccctttccctgtctcttcgcagaggaggcctaccagaaactggccagcgagaccctggaggagctggactggtgtctggaccagctagagaccctacagaccaggcactccgtcagtgagatggcctccaacaagtttaaaaggatgcttaatcgggagctcacccatctctctgaaatgagtcggtctggaaatcaagtgtcagagtttatatcaaacacattcttagataagcaacatgaagtggaaattccttctccaactcagaaggaaaaggagaaaaagaaaagaccaatgtctcagatcagtggagtcaagaaattgatgcacagctctagtctgactaattcaagtatcccaaggtttggagttaaaactgaacaagaagatgtccttgccaaggaactagaagatgtgaacaaatggggtcttcatgttttcagaatagcagagttgtctggtaaccggcccttgactgttatcatgcacaccatttttcaggaacgggatttattaaaaacatttaaaattccagtagatactttaattacatatcttatgactctcgaagaccattaccatgctgatgtggcctatcacaacaatatccatgctgcagatgttgtccagtctactcatgtgctattatctacacctgctttggaggctgtgtttacagatttggagattcttgcagcaatttttgccagtgcaatacatgatgtagatcatcctggtgtgtccaatcaatttctgatcaatacaaactctgaacttgccttgatgtacaatgattcctcagtcttagagaaccatcatttggctgtgggctttaaattgcttcaggaagaaaactgtgacattttccagaatttgaccaaaaaacaaagacaatctttaaggaaaatggtcattgacatcgtacttgcaacagatatgtcaaaacacatgaatctactggctgatttgaagactatggttgaaactaagaaagtgacaagctctggagttcttcttcttgataattattccgataggattcaggttcttcagaatatggtgcactgtgcagatctgagcaacccaacaaagcctctccagctgtaccgccagtggacggaccggataatggaggagttcttccgccaaggagaccgagagagggaacgtggcatggagataagccccatgtgtgacaagcacaatgcttccgtggaaaaatcacaggtgggcttcatagactatattgttcatcccctctgggagacatgggcagacctcgtccaccctgacgcccaggatattttggacactttggaggacaatcgtgaatggtaccagagcacaatccctcagagcccctctcctgcacctgatgacccagaggagggccggcagggtcaaactgagaaattccagtttgaactaactttagaggaagatggtgagtcagacacggaaaaggacagtggcagtcaagtggaagaagacactagctgcagtgactccaagactctttgtactcaagactcagagtctactgaaattccccttgatgaacaggttgaagaggaggcagtaggggaagaagaggaaagccagcctgaagcctgtgtcatagatgatcgttctcctgacacgtaacagtgcaaaaactttcatgccttttttttttttaagtagaaaaattgtttccaaagtgcatgtcacatgccacaaccacggtcacacctcactgtcatctgccaggacgtttgttgaacaaaactgaccttgactactcagtccagcgctcaggaatatcgtaaccagttttttcacctccatgtcatccgagcaaggtggacatcttcacgaacagcgtttttaacaagatttcagcttggtagagctgacaaagcagataaaatctactccaaattattttcaagagagtgtgactcatcaggcagcccaaaagtttattggacttggggtttctattcctttttatttgtttgcaatattttcagaagaaaggcattgcacagagtgaacttaatggacgaagcaacaaatatgtcaagaacaggacatagcacgaatctgttaccagtaggaggaggatgagccacagaaattgcataattttctaatttcaagtcttcctgatacatgactgaatagtgtggttcagtgagctgcactgacctctacattttgtatgatatgtaaaacagattttttgtagagcttacttttattattaaatgtattgaggtattatatttaaaaaaaactatgttcagaacttcatctgccactggttatttttttctaaggagtaacttgcaagttttcagtacaaatctgtgctacactggataaaaatctaatttatgaattttacttgcaccttatagttcatagcaattaactgatttgtagtgattcattgtttgttttatataccaatgacttccatattttaaaagagaaaaacaactttatgttgcaggaaaccctttttgtaagtctttattatttactttgcattttgtttcactctttccagataagcagagttgctcttcaccagtgtttttcttcatgtgcaaagtgactatttgttctataatacttttatgtgtgttatatcaaatgtgtcttaagcttcatgcaaactcagtcatcagttcgtgttgtctgaagcaagtgggagatatataaatacccagtagctaaaatggtcagtcttttttagatgttttcctacttagtatctcctaataacgttttgctgtgtcactagatgttcatttcacaagtgcatgtctttctaataatccacacatttcatgctctaataatccacacatttcatgctcatttttattgtttttacagccagttatagtaagaaaaaggtttttccccttgtgctgctttataatttagcgtgtgtctgaaccttatccatgtttgctagatgaggtcttgtcaaatatatcactaccattgtcaccggtgaaaagaaacaggtagttaagttagggttaacattcatttcaaccacgaggttgtatatcatgactagcttttactcttggtttacagagaaaagttaaacagccaactaggcagtttttaagaatattaacaatatattaacaaacaccaatacaactaatcctatttggttttaatgatttcaccatgggattaagaactatatcaggaacatccctgagaaacggttttaagtgtagcaactactcttccttaatggacagccacataacgtgtaggaagtcctttatcacttatcctcgatccataagcatatcttgcagaggggaactacttctttaaacacatggagggaaagaagatgatgccactggcaccagagggttagtactgtgatgcatcctaaaatatttattatattggtaaaaattctggttaaataaaaaattagagatcactcttggctgatttcagcaccaggaactgtattacagttttagagattaattcctagtgtttacctgattatagcagttggcatcatggggcatttaattctgactttatccccacgtcagccttaataaagtcttctttaccttctctatgaagactttaaagcccaaataatcatttttcacattgatattcaagaattgagatagatagaagccaaagtgggtatctgacaagtggaaaatcaaacgtttaagaagaattacaactctgaaaagcatttatatgtggaacttctcaaggagcctcctggggactggaaagtaagtcatcagccaggcaaatgactcatgctgaagagagtccccatttcagtcccctgagatctagctgatgcttagatcctttgaaataaaaattatgtctttataactctgatcttttacataaagcagaagaggaatcaactagttaattgcaaggtttctactctgtttcctctgtaaagatcagatggtaatctttcaaataagaaaaaaataaagacgtatgtttgaccaagtagtttcacaagaatatttgggaacttgtttcttttaattttatttgtccctgagtgaagtctagaaagaaaggtaaagagtctagagtttattcctctttccaaaacattctcattcctctcctccctacacttagtatttcccccacagagtgcctagaatcttaataatgaataaaataaaaagcagcaatatgtcattaacaaatccagacctgaaagggtaaagggtttataactgcactaataaagagaggctctttttttttcttccagtttgttggtttttaatggtaccgtgttgtaaagatacccactaatggacaatcaaattgcagaaaaggctcaatatccaagagacagggactaatgcactgtacaatctgcttatccttgcccttctctcttgccaaagtgtgcttcagaaatatatactgctttaaaaaagaataaaagaatatccttttacaagtggctttacatttcctaaaatgccataagaaaatgcaatatctgggtactgtatggggaaaaaaatgtccaagtttgtgtaaaaccagtgcatttcagcttgcaagttactgaacacaataatgctgttttaattttgttttatatcagttaaaattcacaataatgtagatagaacaaattacagacaaggaaagaaaaaacttgaatgaaatggattttacagaaagctttatgataatttttgaatgcattatttattttttgtgccatgcattttttttctcaccaaatgaccttacctgtaatacagtcttgtttgtctgtttacaaccatgtatttattgcaatgtacatactgtaatgttaattgtaaattatctgttcttattaaaacatcatcccatgatgggatggtgttgatatatttggaaactcttggtgagagaatgaatggtgtgtatacatactctgtacatttttcttttctcctgtaatatagtcttgtcaccttagagcttgtttatggaagattcaagaaaactataaaatacttaaagatatataaatttaaaaaaacatagctgcaggtctttggtcccagggctgtgccttaactttaaccaatattttcttctgttttgctgcatttgaaaggtaacagtggagctagggctgggcattttacatccaggcttttaattgattagaattctgccaataggtggattttacaaaaccacagacaacctctgaaagattctgagacccttttgagacagaagctcttaagtacttcttgccagggagcagcactgcatgtgtgatggttgtttgccatctgttgatcaggaactacttcagctacttgcatttgattatttcctttttttttttttttaactcggaaacacaactggggaaatatattctttcccagtgattataaacaatctttttcttttttttaagtccttttggcttctagagctcataggaaaatggacttgatttgaaattggagccagagtttactcgtgttggttatctattcatcagcttcctgacatgttaagagaatacattaaagagaaaatactgttttttaatcctaaaatttttcttccactaagataaaccaaatgtccttacatatatgtaaacccatctatttaaacgcaaaggtgggttgatgtcagtttacatagcagaaagcattcactatcctctaagatttgtttctgcaaaactttcattgctttagaattttaaaatttcaccttgtacaatggccagcccctaaagcaggaaacatttataatggattatatggaaacatcctcccagtacttgcccagcccttgaatcatgtggcttttcagtgaaaggaaagattctttttctaggaaaaatgagcctattttattttattttattttattttttgacacaaactgtagattttagcagccctggcccaaaggaatttgattacttttgttttaaacagtacaaaggggacactataattacaaaaacatccttaactgatttgagttgtttttatttctttggatatattttcagagtggtaaattgtgtgtgagaattacaaatgattattcttttagtggtttcttagcctctcttacagcccacggggatagtactgtacatcaataccttcatatgaaatttttatatgcaatgaaaataaaagcatgggttgattctgcctatttatgactcaatcttttacaaataaaagattattcattttaaattatagttcaatcagcatgtctcttaggatactgaacgtggttgaaatgaaaggatagtgacatcataagttagtactgatattcataaccaaataaagccaacttgagtaattttgctacattaaaaattaccaaaattacttagatggcctataagattaagcatggtgttttctaagcaagctttgaaaggggccttccatacttacttaattgaatattctgggatattgaaaattattcagatacttgacaattatttttggttacctactccgcaaactacaaagttttaaggactcaacaataagttaatgagacacagtgtttgctttcatggagcttacagtctggaggggacaaaggcttaaacaatactcatataattatatatgtgatcagtacaatgaaggagctcagtggggtaaataagcaggaacctgaacttgatctgttccggagggccacagaaggcttccttgaggccttgagaaagtgatttgcatctgagttctgaaggattgtaagaggtaactagggaaaaagttgacaggaagaggaaggggatccagacaagaaacatttgcaaagatcttgaggcataaatgagcttgagacatctggagaaactgaggaaaagtgagagagtaggcagggcctggagccgcagagccattgctaaccatcctgtgtgagatatcccccattctgtagctttattctcataaccctgctcaattttctttataacacttctcacagatttatatacgtgtttgtttttgttatctgtctctcccaccagaccacagctccatgagagcaaggtctttgcttaccaatatatcactagcacttaaaactatgcctggtacacagtaggttcttaatatgtgttgaatatagccatcaaattgatattggatataattcaatctgataagatattttgagatattaaagagtttttaacttgataccataaaaa

SEQ ID NO: 56 - protein, 585 aa, Homo sapiens
MKEQPSCAGTGHPSMAGYGRMAPFELASGPVKRLRTESPFPCLFAEEAYQKLASETLEELDWCLDQLETLQTRHSVSEMASNKFKRMLNRELTHLSEMSRSGNQVSEFISNTFLDKQHEVEIPSPTQKEKEKKKRPMSQISGVKKLMHSSSLTNSSIPRFGVKTEQEDVLAKELEDVNKWGLHVFRIAELSGNRPLTVIMHTIFQERDLLKTFKIPVDTLITYLMTLEDHYHADVAYHNNIHAADVVQSTHVLLSTPALEAVFTDLEILAAIFASAIHDVDHPGVSNQFLINTNSELALMYNDSSVLENHHLAVGFKLLQEENCDIFQNLTKKQRQSLRKMVIDIVLATDMSKHMNLLADLKTMVETKKVTSSGVLLLDNYSDRIQVLQNMVHCADLSNPTKPLQLYRQWTDRIMEEFFRQGDRERERGMEISPMCDKHNASVEKSQVGFIDYIVHPLWETWADLVHPDAQDILDTLEDNREWYQSTIPQSPSPAPDDPEEGRQGQTEKFQFELTLEEDGESDTEKDSGSQVEEDTSCSDSKTLCTQDSESTEIPLDEQVEEEAVGEEEESQPEACVIDDRSPDT

SEQ ID NO: 57 - DNA, 7666 bp, Homo sapiens
  source 1..7666: mol_type = other DNA
cttcaagtgccgtgcagaaggctcggcaggcggggcgggcgtggggccgcggctccgggttggggaccgaggagatccggctgtggaccagacgctcctctgcggggcgggcacccaagcgcgctcgccaccccctcgccatccgctagagccgggctcctggactgggactcgggcccgccgcacagttgaaaagtcgcatagtggtttttccgctcgcgtcgctgtgtgaaagttggctcgccgctctttgcacgccctccctggaggccgacccgagacgccaagctggagagaccgtgcctccccgaggccggccgccccgcgagcacagcctccgcccccgttgcactgccgggctgggcaatatgaaggagcagccctcatgtgccggcaccgggcatccgagcatggcgggaggaggcctaccagaaactggccagcgagaccctggaggagctggactggtgtctggaccagctagagaccctacagaccaggcactccgtcagtgagatggcctccaacaagtttaaaaggatgcttaatcgggagctcacccatctctctgaaatgagtcggtctggaaatcaagtgtcagagtttatatcaaacacattcttagataagcaacatgaagtggaaattccttctccaactcagaaggaaaaggagaaaaagaaaagaccaatgtctcagatcagtggagtcaagaaattgatgcacagctctagtctgactaattcaagtatcccaaggtttggagttaaaactgaacaagaagatgtccttgccaaggaactagaagatgtgaacaaatggggtcttcatgttttcagaatagcagagttgtctggtaaccggcccttgactgttatcatgcacaccatttttcaggaacgggatttattaaaaacatttaaaattccagtagatactttaattacatatcttatgactctcgaagaccattaccatgctgatgtggcctatcacaacaatatccatgctgcagatgttgtccagtctactcatgtgctattatctacacctgctttggaggctgtgtttacagatttggagattcttgcagcaatttttgccagtgcaatacatgatgtagatcatcctggtgtgtccaatcaatttctgatcaatacaaactctgaacttgccttgatgtacaatgattcctcagtcttagagaaccatcatttggctgtgggctttaaattgcttcaggaagaaaactgtgacattttccagaatttgaccaaaaaacaaagacaatctttaaggaaaatggtcattgacatcgtacttgcaacagatatgtcaaaacacatgaatctactggctgatttgaagactatggttgaaactaagaaagtgacaagctctggagttcttcttcttgataattattccgataggattcaggttcttcagaatatggtgcactgtgcagatctgagcaacccaacaaagcctctccagctgtaccgccagtggacggaccggataatggaggagttcttccgccaaggagaccgagagagggaacgtggcatggagataagccccatgtgtgacaagcacaatgcttccgtggaaaaatcacaggtgggcttcatagactatattgttcatcccctctgggagacatgggcagacctcgtccaccctgacgcccaggatattttggacactttggaggacaatcgtgaatggtaccagagcacaatccctcagagcccctctcctgcacctgatgacccagaggagggccggcagggtcaaactgagaaattccagtttgaactaactttagaggaagatggtgagtcagacacggaaaaggacagtggcagtcaagtggaagaagacactagctgcagtgactccaagactctttgtactcaagactcagagtctactgaaattccccttgatgaacaggttgaagaggaggcagtaggggaagaagaggaaagccagcctgaagcctgtgtcatagatgatcgttctcctgacacgtaacagtgcaaaaactttcatgccttttttttttttaagtagaaaaattgtttccaaagtgcatgtcacatgccacaaccacggtcacacctcactgtcatctgccaggacgtttgttgaacaaaactgaccttgactactcagtccagcgctcaggaatatcgtaaccagttttttcacctccatgtcatccgagcaaggtggacatcttcacgaacagcgtttttaacaagatttcagcttggtagagctgacaaagcagataaaatctactccaaattattttcaagagagtgtgactcatcaggcagcccaaaagtttattggacttggggtttctattcctttttatttgtttgcaatattttcagaagaaaggcattgcacagagtgaacttaatggacgaagcaacaaatatgtcaagaacaggacatagcacgaatctgttaccagtaggaggaggatgagccacagaaattgcataattttctaatttcaagtcttcctgatacatgactgaatagtgtggttcagtgagctgcactgacctctacattttgtatgatatgtaaaacagattttttgtagagcttacttttattattaaatgtattgaggtattatatttaaaaaaaactatgttcagaacttcatctgccactggttatttttttctaaggagtaacttgcaagttttcagtacaaatctgtgctacactggataaaaatctaatttatgaattttacttgcaccttatagttcatagcaattaactgatttgtagtgattcattgtttgttttatataccaatgacttccatattttaaaagagaaaaacaactttatgttgcaggaaaccctttttgtaagtctttattatttactttgcattttgtttcactctttccagataagcagagttgctcttcaccagtgtttttcttcatgtgcaaagtgactatttgttctataatacttttatgtgtgttatatcaaatgtgtcttaagcttcatgcaaactcagtcatcagttcgtgttgtctgaagcaagtgggagatatataaatacccagtagctaaaatggtcagtcttttttagatgttttcctacttagtatctcctaataacgttttgctgtgtcactagatgttcatttcacaagtgcatgtctttctaataatccacacatttcatgctctaataatccacacatttcatgctcatttttattgtttttacagccagttatagtaagaaaaaggtttttccccttgtgctgctttataatttagcgtgtgtctgaaccttatccatgtttgctagatgaggtcttgtcaaatatatcactaccattgtcaccggtgaaaagaaacaggtagttaagttagggttaacattcatttcaaccacgaggttgtatatcatgactagcttttactcttggtttacagagaaaagttaaacagccaactaggcagtttttaagaatattaacaatatattaacaaacaccaatacaactaatcctatttggttttaatgatttcaccatgggattaagaactatatcaggaacatccctgagaaacggttttaagtgtagcaactactcttccttaatggacagccacataacgtgtaggaagtcctttatcacttatcctcgatccataagcatatcttgcagaggggaactacttctttaaacacatggagggaaagaagatgatgccactggcaccagagggttagtactgtgatgcatcctaaaatatttattatattggtaaaaattctggttaaataaaaaattagagatcactcttggctgatttcagcaccaggaactgtattacagttttagagattaattcctagtgtttacctgattatagcagttggcatcatggggcatttaattctgactttatccccacgtcagccttaataaagtcttctttaccttctctatgaagactttaaagcccaaataatcatttttcacattgatattcaagaattgagatagatagaagccaaagtgggtatctgacaagtggaaaatcaaacgtttaagaagaattacaactctgaaaagcatttatatgtggaacttctcaaggagcctcctggggactggaaagtaagtcatcagccaggcaaatgactcatgctgaagagagtccccatttcagtcccctgagatctagctgatgcttagatcctttgaaataaaaattatgtctttataactctgatcttttacataaagcagaagaggaatcaactagttaattgcaaggtttctactctgtttcctctgtaaagatcagatggtaatctttcaaataagaaaaaaataaagacgtatgtttgaccaagtagtttcacaagaatatttgggaacttgtttcttttaattttatttgtccctgagtgaagtctagaaagaaaggtaaagagtctagagtttattcctctttccaaaacattctcattcctctcctccctacacttagtatttcccccacagagtgcctagaatcttaataatgaataaaataaaaagcagcaatatgtcattaacaaatccagacctgaaagggtaaagggtttataactgcactaataaagagaggctctttttttttcttccagtttgttggtttttaatggtaccgtgttgtaaagatacccactaatggacaatcaaattgcagaaaaggctcaatatccaagagacagggactaatgcactgtacaatctgcttatccttgcccttctctcttgccaaagtgtgcttcagaaatatatactgctttaaaaaagaataaaagaatatccttttacaagtggctttacatttcctaaaatgccataagaaaatgcaatatctgggtactgtatggggaaaaaaatgtccaagtttgtgtaaaaccagtgcatttcagcttgcaagttactgaacacaataatgctgttttaattttgttttatatcagttaaaattcacaataatgtagatagaacaaattacagacaaggaaagaaaaaacttgaatgaaatggattttacagaaagctttatgataatttttgaatgcattatttattttttgtgccatgcattttttttctcaccaaatgaccttacctgtaatacagtcttgtttgtctgtttacaaccatgtatttattgcaatgtacatactgtaatgttaattgtaaattatctgttcttattaaaacatcatcccatgatgggatggtgttgatatatttggaaactcttggtgagagaatgaatggtgtgtatacatactctgtacatttttcttttctcctgtaatatagtcttgtcaccttagagcttgtttatggaagattcaagaaaactataaaatacttaaagatatataaatttaaaaaaacatagctgcaggtctttggtcccagggctgtgccttaactttaaccaatattttcttctgttttgctgcatttgaaaggtaacagtggagctagggctgggcattttacatccaggcttttaattgattagaattctgccaataggtggattttacaaaaccacagacaacctctgaaagattctgagacccttttgagacagaagctcttaagtacttcttgccagggagcagcactgcatgtgtgatggttgtttgccatctgttgatcaggaactacttcagctacttgcatttgattatttcctttttttttttttttaactcggaaacacaactggggaaatatattctttcccagtgattataaacaatctttttcttttttttaagtccttttggcttctagagctcataggaaaatggacttgatttgaaattggagccagagtttactcgtgttggttatctattcatcagcttcctgacatgttaagagaatacattaaagagaaaatactgttttttaatcctaaaatttttcttccactaagataaaccaaatgtccttacatatatgtaaacccatctatttaaacgcaaaggtgggttgatgtcagtttacatagcagaaagcattcactatcctctaagatttgtttctgcaaaactttcattgctttagaattttaaaatttcaccttgtacaatggccagcccctaaagcaggaaacatttataatggattatatggaaacatcctcccagtacttgcccagcccttgaatcatgtggcttttcagtgaaaggaaagattctttttctaggaaaaatgagcctattttattttattttattttattttttgacacaaactgtagattttagcagccctggcccaaaggaatttgattacttttgttttaaacagtacaaaggggacactataattacaaaaacatccttaactgatttgagttgtttttatttctttggatatattttcagagtggtaaattgtgtgtgagaattacaaatgattattcttttagtggtttcttagcctctcttacagcccacggggatagtactgtacatcaataccttcatatgaaatttttatatgcaatgaaaataaaagcatgggttgattctgcctatttatgactcaatcttttacaaataaaagattattcattttaaattatagttcaatcagcatgtctcttaggatactgaacgtggttgaaatgaaaggatagtgacatcataagttagtactgatattcataaccaaataaagccaacttgagtaattttgctacattaaaaattaccaaaattacttagatggcctataagattaagcatggtgttttctaagcaagctttgaaaggggccttccatacttacttaattgaatattctgggatattgaaaattattcagatacttgacaattatttttggttacctactccgcaaactacaaagttttaaggactcaacaataagttaatgagacacagtgtttgctttcatggagcttacagtctggaggggacaaaggcttaaacaatactcatataattatatatgtgatcagtacaatgaaggagctcagtggggtaaataagcaggaacctgaacttgatctgttccggagggccacagaaggcttccttgaggccttgagaaagtgatttgcatctgagttctgaaggattgtaagaggtaactagggaaaaagttgacaggaagaggaaggggatccagacaagaaacatttgcaaagatcttgaggcataaatgagcttgagacatctggagaaactgaggaaaagtgagagagtaggcagggcctggagccgcagagccattgctaaccatcctgtgtgagatatcccccattctgtagctttattctcataaccctgctcaattttctttataacacttctcacagatttatatacgtgtttgtttttgttatctgtctctcccaccagaccacagctccatgagagcaaggtctttgcttaccaatatatcactagcacttaaaactatgcctggtacacagtaggttcttaatatgtgttgaatatagccatcaaattgatattggatataattcaatctgataagatattttgagatattaaagagtttttaacttgataccataaaaa

SEQ ID NO: 58 - protein, 507 aa, Homo sapiens
MASNKFKRMLNRELTHLSEMSRSGNQVSEFISNTFLDKQHEVEIPSPTQKEKEKKKRPMSQISGVKKLMHSSSLTNSSIPRFGVKTEQEDVLAKELEDVNKWGLHVFRIAELSGNRPLTVIMHTIFQERDLLKTFKIPVDTLITYLMTLEDHYHADVAYHNNIHAADVVQSTHVLLSTPALEAVFTDLEILAAIFASAIHDVDHPGVSNQFLINTNSELALMYNDSSVLENHHLAVGFKLLQEENCDIFQNLTKKQRQSLRKMVIDIVLATDMSKHMNLLADLKTMVETKKVTSSGVLLLDNYSDRIQVLQNMVHCADLSNPTKPLQLYRQWTDRIMEEFFRQGDRERERGMEISPMCDKHNASVEKSQVGFIDYIVHPLWETWADLVHPDAQDILDTLEDNREWYQSTIPQSPSPAPDDPEEGRQGQTEKFQFELTLEEDGESDTEKDSGSQVEEDTSCSDSKTLCTQDSESTEIPLDEQVEEEAVGEEEESQPEACVIDDRSPDT

SEQ ID NO: 59 - DNA, 7777 bp, Homo sapiens
  source 1..7777: mol_type = other DNA
ggattcaatacttgttgcaataattgcccacgatagctgctcaaacaagagagttggaattcatctgtaaaaatcactacatgtaacgtaggagacaagaaaaatattaatgacagaagatctgcgaacatgatgcacgtgaataattttccctttagaaggcattcctggatatgttttgatgtggacaatggcacatctgcgggacggagtcccttggatcccatgaccagcccaggatccgggctaattctccaagcaaattttgtccacagtcaacgacgggagtccttcctgtatcgatccgacagcgattatgacctctctccaaagtctatgtcccggaactcctccattgccagtgatatacacggagatgacttgattgtgactccatttgctcaggtcttggccagtctgcgaactgtacgaaacaactttgctgcattaactaatttgcaagatcgagcacctagcaaaagatcacccatgtgcaaccaaccatccatcaacaaagccaccataacagaggaggcctaccagaaactggccagcgagaccctggaggagctggactggtgtctggaccagctagagaccctacagaccaggcactccgtcagtgagatggcctccaacaagtttaaaaggatgcttaatcgggagctcacccatctctctgaaatgagtcggtctggaaatcaagtgtcagagtttatatcaaacacattcttagataagcaacatgaagtggaaattccttctccaactcagaaggaaaaggagaaaaagaaaagaccaatgtctcagatcagtggagtcaagaaattgatgcacagctctagtctgactaattcaagtatcccaaggtttggagttaaaactgaacaagaagatgtccttgccaaggaactagaagatgtgaacaaatggggtcttcatgttttcagaatagcagagttgtctggtaaccggcccttgactgttatcatgcacaccatttttcaggaacgggatttattaaaaacatttaaaattccagtagatactttaattacatatcttatgactctcgaagaccattaccatgctgatgtggcctatcacaacaatatccatgctgcagatgttgtccagtctactcatgtgctattatctacacctgctttggaggctgtgtttacagatttggagattcttgcagcaatttttgccagtgcaatacatgatgtagatcatcctggtgtgtccaatcaatttctgatcaatacaaactctgaacttgccttgatgtacaatgattcctcagtcttagagaaccatcatttggctgtgggctttaaattgcttcaggaagaaaactgtgacattttccagaatttgaccaaaaaacaaagacaatctttaaggaaaatggtcattgacatcgtacttgcaacagatatgtcaaaacacatgaatctactggctgatttgaagactatggttgaaactaagaaagtgacaagctctggagttcttcttcttgataattattccgataggattcaggttcttcagaatatggtgcactgtgcagatctgagcaacccaacaaagcctctccagctgtaccgccagtggacggaccggataatggaggagttcttccgccaaggagaccgagagagggaacgtggcatggagataagccccatgtgtgacaagcacaatgcttccgtggaaaaatcacaggtgggcttcatagactatattgttcatcccctctgggagacatgggcagacctcgtccaccctgacgcccaggatattttggacactttggaggacaatcgtgaatggtaccagagcacaatccctcagagcccctctcctgcacctgatgacccagaggagggccggcagggtcaaactgagaaattccagtttgaactaactttagaggaagatggtgagtcagacacggaaaaggacagtggcagtcaagtggaagaagacactagctgcagtgactccaagactctttgtactcaagactcagagtctactgaaattccccttgatgaacaggttgaagaggaggcagtaggggaagaagaggaaagccagcctgaagcctgtgtcatagatgatcgttctcctgacacgtaacagtgcaaaaactttcatgccttttttttttttaagtagaaaaattgtttccaaagtgcatgtcacatgccacaaccacggtcacacctcactgtcatctgccaggacgtttgttgaacaaaactgaccttgactactcagtccagcgctcaggaatatcgtaaccagttttttcacctccatgtcatccgagcaaggtggacatcttcacgaacagcgtttttaacaagatttcagcttggtagagctgacaaagcagataaaatctactccaaattattttcaagagagtgtgactcatcaggcagcccaaaagtttattggacttggggtttctattcctttttatttgtttgcaatattttcagaagaaaggcattgcacagagtgaacttaatggacgaagcaacaaatatgtcaagaacaggacatagcacgaatctgttaccagtaggaggaggatgagccacagaaattgcataattttctaatttcaagtcttcctgatacatgactgaatagtgtggttcagtgagctgcactgacctctacattttgtatgatatgtaaaacagattttttgtagagcttacttttattattaaatgtattgaggtattatatttaaaaaaaactatgttcagaacttcatctgccactggttatttttttctaaggagtaacttgcaagttttcagtacaaatctgtgctacactggataaaaatctaatttatgaattttacttgcaccttatagttcatagcaattaactgatttgtagtgattcattgtttgttttatataccaatgacttccatattttaaaagagaaaaacaactttatgttgcaggaaaccctttttgtaagtctttattatttactttgcattttgtttcactctttccagataagcagagttgctcttcaccagtgtttttcttcatgtgcaaagtgactatttgttctataatacttttatgtgtgttatatcaaatgtgtcttaagcttcatgcaaactcagtcatcagttcgtgttgtctgaagcaagtgggagatatataaatacccagtagctaaaatggtcagtcttttttagatgttttcctacttagtatctcctaataacgttttgctgtgtcactagatgttcatttcacaagtgcatgtctttctaataatccacacatttcatgctctaataatccacacatttcatgctcatttttattgtttttacagccagttatagtaagaaaaaggtttttccccttgtgctgctttataatttagcgtgtgtctgaaccttatccatgtttgctagatgaggtcttgtcaaatatatcactaccattgtcaccggtgaaaagaaacaggtagttaagttagggttaacattcatttcaaccacgaggttgtatatcatgactagcttttactcttggtttacagagaaaagttaaacagccaactaggcagtttttaagaatattaacaatatattaacaaacaccaatacaactaatcctatttggttttaatgatttcaccatgggattaagaactatatcaggaacatccctgagaaacggttttaagtgtagcaactactcttccttaatggacagccacataacgtgtaggaagtcctttatcacttatcctcgatccataagcatatcttgcagaggggaactacttctttaaacacatggagggaaagaagatgatgccactggcaccagagggttagtactgtgatgcatcctaaaatatttattatattggtaaaaattctggttaaataaaaaattagagatcactcttggctgatttcagcaccaggaactgtattacagttttagagattaattcctagtgtttacctgattatagcagttggcatcatggggcatttaattctgactttatccccacgtcagccttaataaagtcttctttaccttctctatgaagactttaaagcccaaataatcatttttcacattgatattcaagaattgagatagatagaagccaaagtgggtatctgacaagtggaaaatcaaacgtttaagaagaattacaactctgaaaagcatttatatgtggaacttctcaaggagcctcctggggactggaaagtaagtcatcagccaggcaaatgactcatgctgaagagagtccccatttcagtcccctgagatctagctgatgcttagatcctttgaaataaaaattatgtctttataactctgatcttttacataaagcagaagaggaatcaactagttaattgcaaggtttctactctgtttcctctgtaaagatcagatggtaatctttcaaataagaaaaaaataaagacgtatgtttgaccaagtagtttcacaagaatatttgggaacttgtttcttttaattttatttgtccctgagtgaagtctagaaagaaaggtaaagagtctagagtttattcctctttccaaaacattctcattcctctcctccctacacttagtatttcccccacagagtgcctagaatcttaataatgaataaaataaaaagcagcaatatgtcattaacaaatccagacctgaaagggtaaagggtttataactgcactaataaagagaggctctttttttttcttccagtttgttggtttttaatggtaccgtgttgtaaagatacccactaatggacaatcaaattgcagaaaaggctcaatatccaagagacagggactaatgcactgtacaatctgcttatccttgcccttctctcttgccaaagtgtgcttcagaaatatatactgctttaaaaaagaataaaagaatatccttttacaagtggctttacatttcctaaaatgccataagaaaatgcaatatctgggtactgtatggggaaaaaaatgtccaagtttgtgtaaaaccagtgcatttcagcttgcaagttactgaacacaataatgctgttttaattttgttttatatcagttaaaattcacaataatgtagatagaacaaattacagacaaggaaagaaaaaacttgaatgaaatggattttacagaaagctttatgataatttttgaatgcattatttattttttgtgccatgcattttttttctcaccaaatgaccttacctgtaatacagtcttgtttgtctgtttacaaccatgtatttattgcaatgtacatactgtaatgttaattgtaaattatctgttcttattaaaacatcatcccatgatgggatggtgttgatatatttggaaactcttggtgagagaatgaatggtgtgtatacatactctgtacatttttcttttctcctgtaatatagtcttgtcaccttagagcttgtttatggaagattcaagaaaactataaaatacttaaagatatataaatttaaaaaaacatagctgcaggtctttggtcccagggctgtgccttaactttaaccaatattttcttctgttttgctgcatttgaaaggtaacagtggagctagggctgggcattttacatccaggcttttaattgattagaattctgccaataggtggattttacaaaaccacagacaacctctgaaagattctgagacccttttgagacagaagctcttaagtacttcttgccagggagcagcactgcatgtgtgatggttgtttgccatctgttgatcaggaactacttcagctacttgcatttgattatttcctttttttttttttttaactcggaaacacaactggggaaatatattctttcccagtgattataaacaatctttttcttttttttaagtccttttggcttctagagctcataggaaaatggacttgatttgaaattggagccagagtttactcgtgttggttatctattcatcagcttcctgacatgttaagagaatacattaaagagaaaatactgttttttaatcctaaaatttttcttccactaagataaaccaaatgtccttacatatatgtaaacccatctatttaaacgcaaaggtgggttgatgtcagtttacatagcagaaagcattcactatcctctaagatttgtttctgcaaaactttcattgctttagaattttaaaatttcaccttgtacaatggccagcccctaaagcaggaaacatttataatggattatatggaaacatcctcccagtacttgcccagcccttgaatcatgtggcttttcagtgaaaggaaagattctttttctaggaaaaatgagcctattttattttattttattttattttttgacacaaactgtagattttagcagccctggcccaaaggaatttgattacttttgttttaaacagtacaaaggggacactataattacaaaaacatccttaactgatttgagttgtttttatttctttggatatattttcagagtggtaaattgtgtgtgagaattacaaatgattattcttttagtggtttcttagcctctcttacagcccacggggatagtactgtacatcaataccttcatatgaaatttttatatgcaatgaaaataaaagcatgggttgattctgcctatttatgactcaatcttttacaaataaaagattattcattttaaattatagttcaatcagcatgtctcttaggatactgaacgtggttgaaatgaaaggatagtgacatcataagttagtactgatattcataaccaaataaagccaacttgagtaattttgctacattaaaaattaccaaaattacttagatggcctataagattaagcatggtgttttctaagcaagctttgaaaggggccttccatacttacttaattgaatattctgggatattgaaaattattcagatacttgacaattatttttggttacctactccgcaaactacaaagttttaaggactcaacaataagttaatgagacacagtgtttgctttcatggagcttacagtctggaggggacaaaggcttaaacaatactcatataattatatatgtgatcagtacaatgaaggagctcagtggggtaaataagcaggaacctgaacttgatctgttccggagggccacagaaggcttccttgaggccttgagaaagtgatttgcatctgagttctgaaggattgtaagaggtaactagggaaaaagttgacaggaagaggaaggggatccagacaagaaacatttgcaaagatcttgaggcataaatgagcttgagacatctggagaaactgaggaaaagtgagagagtaggcagggcctggagccgcagagccattgctaaccatcctgtgtgagatatcccccattctgtagctttattctcataaccctgctcaattttctttataacacttctcacagatttatatacgtgtttgtttttgttatctgtctctcccaccagaccacagctccatgagagcaaggtctttgcttaccaatatatcactagcacttaaaactatgcctggtacacagtaggttcttaatatgtgttgaatatagccatcaaattgatattggatataattcaatctgataagatattttgagatattaaagagtttttaacttgataccataaaaa

SEQ ID NO: 60 - protein, 673 aa, Homo sapiens
MMHVNNFPFRRHSWICFDVDNGTSAGRSPLDPMTSPGSGLILQANFVHSQRRESFLYRSDSDYDLSPKSMSRNSSIASDIHGDDLIVTPFAQVLASLRTVRNNFAALTNLQDRAPSKRSPMCNQPSINKATITEEAYQKLASETLEELDWCLDQLETLQTRHSVSEMASNKFKRMLNRELTHLSEMSRSGNQVSEFISNTFLDKQHEVEIPSPTQKEKEKKKRPMSQISGVKKLMHSSSLTNSSIPRFGVKTEQEDVLAKELEDVNKWGLHVFRIAELSGNRPLTVIMHTIFQERDLLKTFKIPVDTLITYLMTLEDHYHADVAYHNNIHAADVVQSTHVLLSTPALEAVFTDLEILAAIFASAIHDVDHPGVSNQFLINTNSELALMYNDSSVLENHHLAVGFKLLQEENCDIFQNLTKKQRQSLRKMVIDIVLATDMSKHMNLLADLKTMVETKKVTSSGVLLLDNYSDRIQVLQNMVHCADLSNPTKPLQLYRQWTDRIMEEFFRQGDRERERGMEISPMCDKHNASVEKSQVGFIDYIVHPLWETWADLVHPDAQDILDTLEDNREWYQSTIPQSPSPAPDDPEEGRQGQTEKFQFELTLEEDGESDTEKDSGSQVEEDTSCSDSKTLCTQDSESTEIPLDEQVEEEAVGEEEESQPEACVIDDRSPDT

SEQ ID NO: 61 - DNA, 8160 bp, Homo sapiens
  source 1..8160: mol_type = other DNA
gcagaagcggcggcggcggcagcagcagcagcagcatcaggaaggcgctcgggccagcgcggtgaacccgggctgggcagcaggtcgcggagccgcgagccaggatggaggcagagggcagcagcgcgccggcccgggcgggcagcggagagggcagcgacagcgccggcggggccacgctcaaagcccccaagcatctctggaggcacgagcagcaccaccagtacccgctccggcagccccagttccgcctcctgcatccccatcaccacctgcccccgccgccgccaccctcgccccagccccagccccagtgtccgctacagccgccgccgccgccccccctgccgccgcccccgccgccgcccggggctgcccgcggccgctacgcctcgagcggggccaccggccgcgtccggcatcgcggctactcggacaccgagcgctacctgtactgtcgcgccatggaccgcacctcctacgcggtggagaccggccaccggcccggcctgaagaaatccaggatgtcctggccctcctcgttccagggactcaggcgttttgatgtggacaatggcacatctgcgggacggagtcccttggatcccatgaccagcccaggatccgggctaattctccaagcaaattttgtccacagtcaacgacgggagtccttcctgtatcgatccgacagcgattatgacctctctccaaagtctatgtcccggaactcctccattgccagtgatatacacggagatgacttgattgtgactccatttgctcaggtcttggccagtctgcgaactgtacgaaacaactttgctgcattaactaatttgcaagatcgagcacctagcaaaagatcacccatgtgcaaccaaccatccatcaacaaagccaccataacagaggaggcctaccagaaactggccagcgagaccctggaggagctggactggtgtctggaccagctagagaccctacagaccaggcactccgtcagtgagatggcctccaacaagtttaaaaggatgcttaatcgggagctcacccatctctctgaaatgagtcggtctggaaatcaagtgtcagagtttatatcaaacacattcttagataagcaacatgaagtggaaattccttctccaactcagaaggaaaaggagaaaaagaaaagaccaatgtctcagatcagtggagtcaagaaattgatgcacagctctagtctgactaattcaagtatcccaaggtttggagttaaaactgaacaagaagatgtccttgccaaggaactagaagatgtgaacaaatggggtcttcatgttttcagaatagcagagttgtctggtaaccggcccttgactgttatcatgcacaccatttttcaggaacgggatttattaaaaacatttaaaattccagtagatactttaattacatatcttatgactctcgaagaccattaccatgctgatgtggcctatcacaacaatatccatgctgcagatgttgtccagtctactcatgtgctattatctacacctgctttggaggctgtgtttacagatttggagattcttgcagcaatttttgccagtgcaatacatgatgtagatcatcctggtgtgtccaatcaatttctgatcaatacaaactctgaacttgccttgatgtacaatgattcctcagtcttagagaaccatcatttggctgtgggctttaaattgcttcaggaagaaaactgtgacattttccagaatttgaccaaaaaacaaagacaatctttaaggaaaatggtcattgacatcgtacttgcaacagatatgtcaaaacacatgaatctactggctgatttgaagactatggttgaaactaagaaagtgacaagctctggagttcttcttcttgataattattccgataggattcaggttcttcagaatatggtgcactgtgcagatctgagcaacccaacaaagcctctccagctgtaccgccagtggacggaccggataatggaggagttcttccgccaaggagaccgagagagggaacgtggcatggagataagccccatgtgtgacaagcacaatgcttccgtggaaaaatcacaggtgggcttcatagactatattgttcatcccctctgggagacatgggcagacctcgtccaccctgacgcccaggatattttggacactttggaggacaatcgtgaatggtaccagagcacaatccctcagagcccctctcctgcacctgatgacccagaggagggccggcagggtcaaactgagaaattccagtttgaactaactttagaggaagatggtgagtcagacacggaaaaggacagtggcagtcaagtggaagaagacactagctgcagtgactccaagactctttgtactcaagactcagagtctactgaaattccccttgatgaacaggttgaagaggaggcagtaggggaagaagaggaaagccagcctgaagcctgtgtcatagatgatcgttctcctgacacgtaacagtgcaaaaactttcatgccttttttttttttaagtagaaaaattgtttccaaagtgcatgtcacatgccacaaccacggtcacacctcactgtcatctgccaggacgtttgttgaacaaaactgaccttgactactcagtccagcgctcaggaatatcgtaaccagttttttcacctccatgtcatccgagcaaggtggacatcttcacgaacagcgtttttaacaagatttcagcttggtagagctgacaaagcagataaaatctactccaaattattttcaagagagtgtgactcatcaggcagcccaaaagtttattggacttggggtttctattcctttttatttgtttgcaatattttcagaagaaaggcattgcacagagtgaacttaatggacgaagcaacaaatatgtcaagaacaggacatagcacgaatctgttaccagtaggaggaggatgagccacagaaattgcataattttctaatttcaagtcttcctgatacatgactgaatagtgtggttcagtgagctgcactgacctctacattttgtatgatatgtaaaacagattttttgtagagcttacttttattattaaatgtattgaggtattatatttaaaaaaaactatgttcagaacttcatctgccactggttatttttttctaaggagtaacttgcaagttttcagtacaaatctgtgctacactggataaaaatctaatttatgaattttacttgcaccttatagttcatagcaattaactgatttgtagtgattcattgtttgttttatataccaatgacttccatattttaaaagagaaaaacaactttatgttgcaggaaaccctttttgtaagtctttattatttactttgcattttgtttcactctttccagataagcagagttgctcttcaccagtgtttttcttcatgtgcaaagtgactatttgttctataatacttttatgtgtgttatatcaaatgtgtcttaagcttcatgcaaactcagtcatcagttcgtgttgtctgaagcaagtgggagatatataaatacccagtagctaaaatggtcagtcttttttagatgttttcctacttagtatctcctaataacgttttgctgtgtcactagatgttcatttcacaagtgcatgtctttctaataatccacacatttcatgctctaataatccacacatttcatgctcatttttattgtttttacagccagttatagtaagaaaaaggtttttccccttgtgctgctttataatttagcgtgtgtctgaaccttatccatgtttgctagatgaggtcttgtcaaatatatcactaccattgtcaccggtgaaaagaaacaggtagttaagttagggttaacattcatttcaaccacgaggttgtatatcatgactagcttttactcttggtttacagagaaaagttaaacagccaactaggcagtttttaagaatattaacaatatattaacaaacaccaatacaactaatcctatttggttttaatgatttcaccatgggattaagaactatatcaggaacatccctgagaaacggttttaagtgtagcaactactcttccttaatggacagccacataacgtgtaggaagtcctttatcacttatcctcgatccataagcatatcttgcagaggggaactacttctttaaacacatggagggaaagaagatgatgccactggcaccagagggttagtactgtgatgcatcctaaaatatttattatattggtaaaaattctggttaaataaaaaattagagatcactcttggctgatttcagcaccaggaactgtattacagttttagagattaattcctagtgtttacctgattatagcagttggcatcatggggcatttaattctgactttatccccacgtcagccttaataaagtcttctttaccttctctatgaagactttaaagcccaaataatcatttttcacattgatattcaagaattgagatagatagaagccaaagtgggtatctgacaagtggaaaatcaaacgtttaagaagaattacaactctgaaaagcatttatatgtggaacttctcaaggagcctcctggggactggaaagtaagtcatcagccaggcaaatgactcatgctgaagagagtccccatttcagtcccctgagatctagctgatgcttagatcctttgaaataaaaattatgtctttataactctgatcttttacataaagcagaagaggaatcaactagttaattgcaaggtttctactctgtttcctctgtaaagatcagatggtaatctttcaaataagaaaaaaataaagacgtatgtttgaccaagtagtttcacaagaatatttgggaacttgtttcttttaattttatttgtccctgagtgaagtctagaaagaaaggtaaagagtctagagtttattcctctttccaaaacattctcattcctctcctccctacacttagtatttcccccacagagtgcctagaatcttaataatgaataaaataaaaagcagcaatatgtcattaacaaatccagacctgaaagggtaaagggtttataactgcactaataaagagaggctctttttttttcttccagtttgttggtttttaatggtaccgtgttgtaaagatacccactaatggacaatcaaattgcagaaaaggctcaatatccaagagacagggactaatgcactgtacaatctgcttatccttgcccttctctcttgccaaagtgtgcttcagaaatatatactgctttaaaaaagaataaaagaatatccttttacaagtggctttacatttcctaaaatgccataagaaaatgcaatatctgggtactgtatggggaaaaaaatgtccaagtttgtgtaaaaccagtgcatttcagcttgcaagttactgaacacaataatgctgttttaattttgttttatatcagttaaaattcacaataatgtagatagaacaaattacagacaaggaaagaaaaaacttgaatgaaatggattttacagaaagctttatgataatttttgaatgcattatttattttttgtgccatgcattttttttctcaccaaatgaccttacctgtaatacagtcttgtttgtctgtttacaaccatgtatttattgcaatgtacatactgtaatgttaattgtaaattatctgttcttattaaaacatcatcccatgatgggatggtgttgatatatttggaaactcttggtgagagaatgaatggtgtgtatacatactctgtacatttttcttttctcctgtaatatagtcttgtcaccttagagcttgtttatggaagattcaagaaaactataaaatacttaaagatatataaatttaaaaaaacatagctgcaggtctttggtcccagggctgtgccttaactttaaccaatattttcttctgttttgctgcatttgaaaggtaacagtggagctagggctgggcattttacatccaggcttttaattgattagaattctgccaataggtggattttacaaaaccacagacaacctctgaaagattctgagacccttttgagacagaagctcttaagtacttcttgccagggagcagcactgcatgtgtgatggttgtttgccatctgttgatcaggaactacttcagctacttgcatttgattatttcctttttttttttttttaactcggaaacacaactggggaaatatattctttcccagtgattataaacaatctttttcttttttttaagtccttttggcttctagagctcataggaaaatggacttgatttgaaattggagccagagtttactcgtgttggttatctattcatcagcttcctgacatgttaagagaatacattaaagagaaaatactgttttttaatcctaaaatttttcttccactaagataaaccaaatgtccttacatatatgtaaacccatctatttaaacgcaaaggtgggttgatgtcagtttacatagcagaaagcattcactatcctctaagatttgtttctgcaaaactttcattgctttagaattttaaaatttcaccttgtacaatggccagcccctaaagcaggaaacatttataatggattatatggaaacatcctcccagtacttgcccagcccttgaatcatgtggcttttcagtgaaaggaaagattctttttctaggaaaaatgagcctattttattttattttattttattttttgacacaaactgtagattttagcagccctggcccaaaggaatttgattacttttgttttaaacagtacaaaggggacactataattacaaaaacatccttaactgatttgagttgtttttatttctttggatatattttcagagtggtaaattgtgtgtgagaattacaaatgattattcttttagtggtttcttagcctctcttacagcccacggggatagtactgtacatcaataccttcatatgaaatttttatatgcaatgaaaataaaagcatgggttgattctgcctatttatgactcaatcttttacaaataaaagattattcattttaaattatagttcaatcagcatgtctcttaggatactgaacgtggttgaaatgaaaggatagtgacatcataagttagtactgatattcataaccaaataaagccaacttgagtaattttgctacattaaaaattaccaaaattacttagatggcctataagattaagcatggtgttttctaagcaagctttgaaaggggccttccatacttacttaattgaatattctgggatattgaaaattattcagatacttgacaattatttttggttacctactccgcaaactacaaagttttaaggactcaacaataagttaatgagacacagtgtttgctttcatggagcttacagtctggaggggacaaaggcttaaacaatactcatataattatatatgtgatcagtacaatgaaggagctcagtggggtaaataagcaggaacctgaacttgatctgttccggagggccacagaaggcttccttgaggccttgagaaagtgatttgcatctgagttctgaaggattgtaagaggtaactagggaaaaagttgacaggaagaggaaggggatccagacaagaaacatttgcaaagatcttgaggcataaatgagcttgagacatctggagaaactgaggaaaagtgagagagtaggcagggcctggagccgcagagccattgctaaccatcctgtgtgagatatcccccattctgtagctttattctcataaccctgctcaattttctttataacacttctcacagatttatatacgtgtttgtttttgttatctgtctctcccaccagaccacagctccatgagagcaaggtctttgcttaccaatatatcactagcacttaaaactatgcctggtacacagtaggttcttaatatgtgttgaatatagccatcaaattgatattggatataattcaatctgataagatattttgagatattaaagagtttttaacttgataccataaaaa

SEQ ID NO: 62 - protein, 809 aa, Homo sapiens
MEAEGSSAPARAGSGEGSDSAGGATLKAPKHLWRHEQHHQYPLRQPQFRLLHPHHHLPPPPPPSPQPQPQCPLQPPPPPPLPPPPPPPGAARGRYASSGATGRVRHRGYSDTERYLYCRAMDRTSYAVETGHRPGLKKSRMSWPSSFQGLRRFDVDNGTSAGRSPLDPMTSPGSGLILQANFVHSQRRESFLYRSDSDYDLSPKSMSRNSSIASDIHGDDLIVTPFAQVLASLRTVRNNFAALTNLQDRAPSKRSPMCNQPSINKATITEEAYQKLASETLEELDWCLDQLETLQTRHSVSEMASNKFKRMLNRELTHLSEMSRSGNQVSEFISNTFLDKQHEVEIPSPTQKEKEKKKRPMSQISGVKKLMHSSSLTNSSIPRFGVKTEQEDVLAKELEDVNKWGLHVFRIAELSGNRPLTVIMHTIFQERDLLKTFKIPVDTLITYLMTLEDHYHADVAYHNNIHAADVVQSTHVLLSTPALEAVFTDLEILAAIFASAIHDVDHPGVSNQFLINTNSELALMYNDSSVLENHHLAVGFKLLQEENCDIFQNLTKKQRQSLRKMVIDIVLATDMSKHMNLLADLKTMVETKKVTSSGVLLLDNYSDRIQVLQNMVHCADLSNPTKPLQLYRQWTDRIMEEFFRQGDRERERGMEISPMCDKHNASVEKSQVGFIDYIVHPLWETWADLVHPDAQDILDTLEDNREWYQSTIPQSPSPAPDDPEEGRQGQTEKFQFELTLEEDGESDTEKDSGSQVEEDTSCSDSKTLCTQDSESTEIPLDEQVEEEAVGEEEESQPEACVIDDRSPDT

SEQ ID NO: 63 - DNA, 8203 bp, Homo sapiens
  source 1..8203: mol_type = other DNA
gcggcgcattagttccaatagtttaacaggctgctttgtagcacggacaaagccgtgcgagcgcggtgctttccctccttgttcatttgctatgcgagcttgtcagtgatctttggcaggggcttgggagaggaggggtgacgtttaatacgcttccgcggaggagtgcgctcgcctcctctgcacccagccccaggctctacagagagactgaggcaggcgactgaatgcactaacagcagcaggctcagacctgcttccctggacatttccgggaccgtgagcgagggaaccacgttgccctggattcttgccagctgtacaaagttgaccaggaaaatggctcagcagacaagcccggacactttaacagtacctgaagtggataatccgcattgtccaaacccgtggctgaacgaagaccttgtgaaatccttgcgagaaaacctgttgcagcatgagaagtccaagacagcgaggaaatcggtttctcccaagctctctccagtgatctctccgagaaattcccccaggcttctgcgcagaatgcttctcagcagcaacatccccaaacagcggcgtttcacggtggcacatacatgttttgatgtggacaatggcacatctgcgggacggagtcccttggatcccatgaccagcccaggatccgggctaattctccaagcaaattttgtccacagtcaacgacgggagtccttcctgtatcgatccgacagcgattatgacctctctccaaagtctatgtcccggaactcctccattgccagtgatatacacggagatgacttgattgtgactccatttgctcaggtcttggccagtctgcgaactgtacgaaacaactttgctgcattaactaatttgcaagatcgagcacctagcaaaagatcacccatgtgcaaccaaccatccatcaacaaagccaccataacagaggaggcctaccagaaactggccagcgagaccctggaggagctggactggtgtctggaccagctagagaccctacagaccaggcactccgtcagtgagatggcctccaacaagtttaaaaggatgcttaatcgggagctcacccatctctctgaaatgagtcggtctggaaatcaagtgtcagagtttatatcaaacacattcttagataagcaacatgaagtggaaattccttctccaactcagaaggaaaaggagaaaaagaaaagaccaatgtctcagatcagtggagtcaagaaattgatgcacagctctagtctgactaattcaagtatcccaaggtttggagttaaaactgaacaagaagatgtccttgccaaggaactagaagatgtgaacaaatggggtcttcatgttttcagaatagcagagttgtctggtaaccggcccttgactgttatcatgcacaccatttttcaggaacgggatttattaaaaacatttaaaattccagtagatactttaattacatatcttatgactctcgaagaccattaccatgctgatgtggcctatcacaacaatatccatgctgcagatgttgtccagtctactcatgtgctattatctacacctgctttggaggctgtgtttacagatttggagattcttgcagcaatttttgccagtgcaatacatgatgtagatcatcctggtgtgtccaatcaatttctgatcaatacaaactctgaacttgccttgatgtacaatgattcctcagtcttagagaaccatcatttggctgtgggctttaaattgcttcaggaagaaaactgtgacattttccagaatttgaccaaaaaacaaagacaatctttaaggaaaatggtcattgacatcgtacttgcaacagatatgtcaaaacacatgaatctactggctgatttgaagactatggttgaaactaagaaagtgacaagctctggagttcttcttcttgataattattccgataggattcaggttcttcagaatatggtgcactgtgcagatctgagcaacccaacaaagcctctccagctgtaccgccagtggacggaccggataatggaggagttcttccgccaaggagaccgagagagggaacgtggcatggagataagccccatgtgtgacaagcacaatgcttccgtggaaaaatcacaggtgggcttcatagactatattgttcatcccctctgggagacatgggcagacctcgtccaccctgacgcccaggatattttggacactttggaggacaatcgtgaatggtaccagagcacaatccctcagagcccctctcctgcacctgatgacccagaggagggccggcagggtcaaactgagaaattccagtttgaactaactttagaggaagatggtgagtcagacacggaaaaggacagtggcagtcaagtggaagaagacactagctgcagtgactccaagactctttgtactcaagactcagagtctactgaaattccccttgatgaacaggttgaagaggaggcagtaggggaagaagaggaaagccagcctgaagcctgtgtcatagatgatcgttctcctgacacgtaacagtgcaaaaactttcatgccttttttttttttaagtagaaaaattgtttccaaagtgcatgtcacatgccacaaccacggtcacacctcactgtcatctgccaggacgtttgttgaacaaaactgaccttgactactcagtccagcgctcaggaatatcgtaaccagttttttcacctccatgtcatccgagcaaggtggacatcttcacgaacagcgtttttaacaagatttcagcttggtagagctgacaaagcagataaaatctactccaaattattttcaagagagtgtgactcatcaggcagcccaaaagtttattggacttggggtttctattcctttttatttgtttgcaatattttcagaagaaaggcattgcacagagtgaacttaatggacgaagcaacaaatatgtcaagaacaggacatagcacgaatctgttaccagtaggaggaggatgagccacagaaattgcataattttctaatttcaagtcttcctgatacatgactgaatagtgtggttcagtgagctgcactgacctctacattttgtatgatatgtaaaacagattttttgtagagcttacttttattattaaatgtattgaggtattatatttaaaaaaaactatgttcagaacttcatctgccactggttatttttttctaaggagtaacttgcaagttttcagtacaaatctgtgctacactggataaaaatctaatttatgaattttacttgcaccttatagttcatagcaattaactgatttgtagtgattcattgtttgttttatataccaatgacttccatattttaaaagagaaaaacaactttatgttgcaggaaaccctttttgtaagtctttattatttactttgcattttgtttcactctttccagataagcagagttgctcttcaccagtgtttttcttcatgtgcaaagtgactatttgttctataatacttttatgtgtgttatatcaaatgtgtcttaagcttcatgcaaactcagtcatcagttcgtgttgtctgaagcaagtgggagatatataaatacccagtagctaaaatggtcagtcttttttagatgttttcctacttagtatctcctaataacgttttgctgtgtcactagatgttcatttcacaagtgcatgtctttctaataatccacacatttcatgctctaataatccacacatttcatgctcatttttattgtttttacagccagttatagtaagaaaaaggtttttccccttgtgctgctttataatttagcgtgtgtctgaaccttatccatgtttgctagatgaggtcttgtcaaatatatcactaccattgtcaccggtgaaaagaaacaggtagttaagttagggttaacattcatttcaaccacgaggttgtatatcatgactagcttttactcttggtttacagagaaaagttaaacagccaactaggcagtttttaagaatattaacaatatattaacaaacaccaatacaactaatcctatttggttttaatgatttcaccatgggattaagaactatatcaggaacatccctgagaaacggttttaagtgtagcaactactcttccttaatggacagccacataacgtgtaggaagtcctttatcacttatcctcgatccataagcatatcttgcagaggggaactacttctttaaacacatggagggaaagaagatgatgccactggcaccagagggttagtactgtgatgcatcctaaaatatttattatattggtaaaaattctggttaaataaaaaattagagatcactcttggctgatttcagcaccaggaactgtattacagttttagagattaattcctagtgtttacctgattatagcagttggcatcatggggcatttaattctgactttatccccacgtcagccttaataaagtcttctttaccttctctatgaagactttaaagcccaaataatcatttttcacattgatattcaagaattgagatagatagaagccaaagtgggtatctgacaagtggaaaatcaaacgtttaagaagaattacaactctgaaaagcatttatatgtggaacttctcaaggagcctcctggggactggaaagtaagtcatcagccaggcaaatgactcatgctgaagagagtccccatttcagtcccctgagatctagctgatgcttagatcctttgaaataaaaattatgtctttataactctgatcttttacataaagcagaagaggaatcaactagttaattgcaaggtttctactctgtttcctctgtaaagatcagatggtaatctttcaaataagaaaaaaataaagacgtatgtttgaccaagtagtttcacaagaatatttgggaacttgtttcttttaattttatttgtccctgagtgaagtctagaaagaaaggtaaagagtctagagtttattcctctttccaaaacattctcattcctctcctccctacacttagtatttcccccacagagtgcctagaatcttaataatgaataaaataaaaagcagcaatatgtcattaacaaatccagacctgaaagggtaaagggtttataactgcactaataaagagaggctctttttttttcttccagtttgttggtttttaatggtaccgtgttgtaaagatacccactaatggacaatcaaattgcagaaaaggctcaatatccaagagacagggactaatgcactgtacaatctgcttatccttgcccttctctcttgccaaagtgtgcttcagaaatatatactgctttaaaaaagaataaaagaatatccttttacaagtggctttacatttcctaaaatgccataagaaaatgcaatatctgggtactgtatggggaaaaaaatgtccaagtttgtgtaaaaccagtgcatttcagcttgcaagttactgaacacaataatgctgttttaattttgttttatatcagttaaaattcacaataatgtagatagaacaaattacagacaaggaaagaaaaaacttgaatgaaatggattttacagaaagctttatgataatttttgaatgcattatttattttttgtgccatgcattttttttctcaccaaatgaccttacctgtaatacagtcttgtttgtctgtttacaaccatgtatttattgcaatgtacatactgtaatgttaattgtaaattatctgttcttattaaaacatcatcccatgatgggatggtgttgatatatttggaaactcttggtgagagaatgaatggtgtgtatacatactctgtacatttttcttttctcctgtaatatagtcttgtcaccttagagcttgtttatggaagattcaagaaaactataaaatacttaaagatatataaatttaaaaaaacatagctgcaggtctttggtcccagggctgtgccttaactttaaccaatattttcttctgttttgctgcatttgaaaggtaacagtggagctagggctgggcattttacatccaggcttttaattgattagaattctgccaataggtggattttacaaaaccacagacaacctctgaaagattctgagacccttttgagacagaagctcttaagtacttcttgccagggagcagcactgcatgtgtgatggttgtttgccatctgttgatcaggaactacttcagctacttgcatttgattatttcctttttttttttttttaactcggaaacacaactggggaaatatattctttcccagtgattataaacaatctttttcttttttttaagtccttttggcttctagagctcataggaaaatggacttgatttgaaattggagccagagtttactcgtgttggttatctattcatcagcttcctgacatgttaagagaatacattaaagagaaaatactgttttttaatcctaaaatttttcttccactaagataaaccaaatgtccttacatatatgtaaacccatctatttaaacgcaaaggtgggttgatgtcagtttacatagcagaaagcattcactatcctctaagatttgtttctgcaaaactttcattgctttagaattttaaaatttcaccttgtacaatggccagcccctaaagcaggaaacatttataatggattatatggaaacatcctcccagtacttgcccagcccttgaatcatgtggcttttcagtgaaaggaaagattctttttctaggaaaaatgagcctattttattttattttattttattttttgacacaaactgtagattttagcagccctggcccaaaggaatttgattacttttgttttaaacagtacaaaggggacactataattacaaaaacatccttaactgatttgagttgtttttatttctttggatatattttcagagtggtaaattgtgtgtgagaattacaaatgattattcttttagtggtttcttagcctctcttacagcccacggggatagtactgtacatcaataccttcatatgaaatttttatatgcaatgaaaataaaagcatgggttgattctgcctatttatgactcaatcttttacaaataaaagattattcattttaaattatagttcaatcagcatgtctcttaggatactgaacgtggttgaaatgaaaggatagtgacatcataagttagtactgatattcataaccaaataaagccaacttgagtaattttgctacattaaaaattaccaaaattacttagatggcctataagattaagcatggtgttttctaagcaagctttgaaaggggccttccatacttacttaattgaatattctgggatattgaaaattattcagatacttgacaattatttttggttacctactccgcaaactacaaagttttaaggactcaacaataagttaatgagacacagtgtttgctttcatggagcttacagtctggaggggacaaaggcttaaacaatactcatataattatatatgtgatcagtacaatgaaggagctcagtggggtaaataagcaggaacctgaacttgatctgttccggagggccacagaaggcttccttgaggccttgagaaagtgatttgcatctgagttctgaaggattgtaagaggtaactagggaaaaagttgacaggaagaggaaggggatccagacaagaaacatttgcaaagatcttgaggcataaatgagcttgagacatctggagaaactgaggaaaagtgagagagtaggcagggcctggagccgcagagccattgctaaccatcctgtgtgagatatcccccattctgtagctttattctcataaccctgctcaattttctttataacacttctcacagatttatatacgtgtttgtttttgttatctgtctctcccaccagaccacagctccatgagagcaaggtctttgcttaccaatatatcactagcacttaaaactatgcctggtacacagtaggttcttaatatgtgttgaatatagccatcaaattgatattggatataattcaatctgataagatattttgagatattaaagagtttttaacttgataccataaaaa

SEQ ID NO: 64 - protein, 745 aa, Homo sapiens
MAQQTSPDTLTVPEVDNPHCPNPWLNEDLVKSLRENLLQHEKSKTARKSVSPKLSPVISPRNSPRLLRRMLLSSNIPKQRRFTVAHTCFDVDNGTSAGRSPLDPMTSPGSGLILQANFVHSQRRESFLYRSDSDYDLSPKSMSRNSSIASDIHGDDLIVTPFAQVLASLRTVRNNFAALTNLQDRAPSKRSPMCNQPSINKATITEEAYQKLASETLEELDWCLDQLETLQTRHSVSEMASNKFKRMLNRELTHLSEMSRSGNQVSEFISNTFLDKQHEVEIPSPTQKEKEKKKRPMSQISGVKKLMHSSSLTNSSIPRFGVKTEQEDVLAKELEDVNKWGLHVFRIAELSGNRPLTVIMHTIFQERDLLKTFKIPVDTLITYLMTLEDHYHADVAYHNNIHAADVVQSTHVLLSTPALEAVFTDLEILAAIFASAIHDVDHPGVSNQFLINTNSELALMYNDSSVLENHHLAVGFKLLQEENCDIFQNLTKKQRQSLRKMVIDIVLATDMSKHMNLLADLKTMVETKKVTSSGVLLLDNYSDRIQVLQNMVHCADLSNPTKPLQLYRQWTDRIMEEFFRQGDRERERGMEISPMCDKHNASVEKSQVGFIDYIVHPLWETWADLVHPDAQDILDTLEDNREWYQSTIPQSPSPAPDDPEEGRQGQTEKFQFELTLEEDGESDTEKDSGSQVEEDTSCSDSKTLCTQDSESTEIPLDEQVEEEAVGEEEESQPEACVIDDRSPDT

SEQ ID NO: 65 - DNA, 7545 bp, Homo sapiens
  source 1..7545: mol_type = other DNA
ctttcttgcaactaagcatcttgacatacattattcattaagccctggagctcgggagagaaagatgcagacccttagatctttagatattcctttatcacgtggattttctttattcagaatagttgctgaattttgtgccattctggagtcttacaaatggcatgtattcgatgggaagacggctggatgggatttaatgcgaggctttcttatgtatacttaattaccaaaaatctttaaaaactcatactctgcgtggcttgtggaggttgttaaagtgtcgagattttgaagctaaatacattttagagcttactatatatatacatatatatatatatacatataatcaatcaaaaatgcctgaagcaaactatttactgtcagtgtcttggggctacataaagtttaaaaggatgcttaatcgggagctcacccatctctctgaaatgagtcggtctggaaatcaagtgtcagagtttatatcaaacacattcttagataagcaacatgaagtggaaattccttctccaactcagaaggaaaaggagaaaaagaaaagaccaatgtctcagatcagtggagtcaagaaattgatgcacagctctagtctgactaattcaagtatcccaaggtttggagttaaaactgaacaagaagatgtccttgccaaggaactagaagatgtgaacaaatggggtcttcatgttttcagaatagcagagttgtctggtaaccggcccttgactgttatcatgcacaccatttttcaggaacgggatttattaaaaacatttaaaattccagtagatactttaattacatatcttatgactctcgaagaccattaccatgctgatgtggcctatcacaacaatatccatgctgcagatgttgtccagtctactcatgtgctattatctacacctgctttggaggctgtgtttacagatttggagattcttgcagcaatttttgccagtgcaatacatgatgtagatcatcctggtgtgtccaatcaatttctgatcaatacaaactctgaacttgccttgatgtacaatgattcctcagtcttagagaaccatcatttggctgtgggctttaaattgcttcaggaagaaaactgtgacattttccagaatttgaccaaaaaacaaagacaatctttaaggaaaatggtcattgacatcgtacttgcaacagatatgtcaaaacacatgaatctactggctgatttgaagactatggttgaaactaagaaagtgacaagctctggagttcttcttcttgataattattccgataggattcaggttcttcagaatatggtgcactgtgcagatctgagcaacccaacaaagcctctccagctgtaccgccagtggacggaccggataatggaggagttcttccgccaaggagaccgagagagggaacgtggcatggagataagccccatgtgtgacaagcacaatgcttccgtggaaaaatcacaggtgggcttcatagactatattgttcatcccctctgggagacatgggcagacctcgtccaccctgacgcccaggatattttggacactttggaggacaatcgtgaatggtaccagagcacaatccctcagagcccctctcctgcacctgatgacccagaggagggccggcagggtcaaactgagaaattccagtttgaactaactttagaggaagatggtgagtcagacacggaaaaggacagtggcagtcaagtggaagaagacactagctgcagtgactccaagactctttgtactcaagactcagagtctactgaaattccccttgatgaacaggttgaagaggaggcagtaggggaagaagaggaaagccagcctgaagcctgtgtcatagatgatcgttctcctgacacgtaacagtgcaaaaactttcatgccttttttttttttaagtagaaaaattgtttccaaagtgcatgtcacatgccacaaccacggtcacacctcactgtcatctgccaggacgtttgttgaacaaaactgaccttgactactcagtccagcgctcaggaatatcgtaaccagttttttcacctccatgtcatccgagcaaggtggacatcttcacgaacagcgtttttaacaagatttcagcttggtagagctgacaaagcagataaaatctactccaaattattttcaagagagtgtgactcatcaggcagcccaaaagtttattggacttggggtttctattcctttttatttgtttgcaatattttcagaagaaaggcattgcacagagtgaacttaatggacgaagcaacaaatatgtcaagaacaggacatagcacgaatctgttaccagtaggaggaggatgagccacagaaattgcataattttctaatttcaagtcttcctgatacatgactgaatagtgtggttcagtgagctgcactgacctctacattttgtatgatatgtaaaacagattttttgtagagcttacttttattattaaatgtattgaggtattatatttaaaaaaaactatgttcagaacttcatctgccactggttatttttttctaaggagtaacttgcaagttttcagtacaaatctgtgctacactggataaaaatctaatttatgaattttacttgcaccttatagttcatagcaattaactgatttgtagtgattcattgtttgttttatataccaatgacttccatattttaaaagagaaaaacaactttatgttgcaggaaaccctttttgtaagtctttattatttactttgcattttgtttcactctttccagataagcagagttgctcttcaccagtgtttttcttcatgtgcaaagtgactatttgttctataatacttttatgtgtgttatatcaaatgtgtcttaagcttcatgcaaactcagtcatcagttcgtgttgtctgaagcaagtgggagatatataaatacccagtagctaaaatggtcagtcttttttagatgttttcctacttagtatctcctaataacgttttgctgtgtcactagatgttcatttcacaagtgcatgtctttctaataatccacacatttcatgctctaataatccacacatttcatgctcatttttattgtttttacagccagttatagtaagaaaaaggtttttccccttgtgctgctttataatttagcgtgtgtctgaaccttatccatgtttgctagatgaggtcttgtcaaatatatcactaccattgtcaccggtgaaaagaaacaggtagttaagttagggttaacattcatttcaaccacgaggttgtatatcatgactagcttttactcttggtttacagagaaaagttaaacagccaactaggcagtttttaagaatattaacaatatattaacaaacaccaatacaactaatcctatttggttttaatgatttcaccatgggattaagaactatatcaggaacatccctgagaaacggttttaagtgtagcaactactcttccttaatggacagccacataacgtgtaggaagtcctttatcacttatcctcgatccataagcatatcttgcagaggggaactacttctttaaacacatggagggaaagaagatgatgccactggcaccagagggttagtactgtgatgcatcctaaaatatttattatattggtaaaaattctggttaaataaaaaattagagatcactcttggctgatttcagcaccaggaactgtattacagttttagagattaattcctagtgtttacctgattatagcagttggcatcatggggcatttaattctgactttatccccacgtcagccttaataaagtcttctttaccttctctatgaagactttaaagcccaaataatcatttttcacattgatattcaagaattgagatagatagaagccaaagtgggtatctgacaagtggaaaatcaaacgtttaagaagaattacaactctgaaaagcatttatatgtggaacttctcaaggagcctcctggggactggaaagtaagtcatcagccaggcaaatgactcatgctgaagagagtccccatttcagtcccctgagatctagctgatgcttagatcctttgaaataaaaattatgtctttataactctgatcttttacataaagcagaagaggaatcaactagttaattgcaaggtttctactctgtttcctctgtaaagatcagatggtaatctttcaaataagaaaaaaataaagacgtatgtttgaccaagtagtttcacaagaatatttgggaacttgtttcttttaattttatttgtccctgagtgaagtctagaaagaaaggtaaagagtctagagtttattcctctttccaaaacattctcattcctctcctccctacacttagtatttcccccacagagtgcctagaatcttaataatgaataaaataaaaagcagcaatatgtcattaacaaatccagacctgaaagggtaaagggtttataactgcactaataaagagaggctctttttttttcttccagtttgttggtttttaatggtaccgtgttgtaaagatacccactaatggacaatcaaattgcagaaaaggctcaatatccaagagacagggactaatgcactgtacaatctgcttatccttgcccttctctcttgccaaagtgtgcttcagaaatatatactgctttaaaaaagaataaaagaatatccttttacaagtggctttacatttcctaaaatgccataagaaaatgcaatatctgggtactgtatggggaaaaaaatgtccaagtttgtgtaaaaccagtgcatttcagcttgcaagttactgaacacaataatgctgttttaattttgttttatatcagttaaaattcacaataatgtagatagaacaaattacagacaaggaaagaaaaaacttgaatgaaatggattttacagaaagctttatgataatttttgaatgcattatttattttttgtgccatgcattttttttctcaccaaatgaccttacctgtaatacagtcttgtttgtctgtttacaaccatgtatttattgcaatgtacatactgtaatgttaattgtaaattatctgttcttattaaaacatcatcccatgatgggatggtgttgatatatttggaaactcttggtgagagaatgaatggtgtgtatacatactctgtacatttttcttttctcctgtaatatagtcttgtcaccttagagcttgtttatggaagattcaagaaaactataaaatacttaaagatatataaatttaaaaaaacatagctgcaggtctttggtcccagggctgtgccttaactttaaccaatattttcttctgttttgctgcatttgaaaggtaacagtggagctagggctgggcattttacatccaggcttttaattgattagaattctgccaataggtggattttacaaaaccacagacaacctctgaaagattctgagacccttttgagacagaagctcttaagtacttcttgccagggagcagcactgcatgtgtgatggttgtttgccatctgttgatcaggaactacttcagctacttgcatttgattatttcctttttttttttttttaactcggaaacacaactggggaaatatattctttcccagtgattataaacaatctttttcttttttttaagtccttttggcttctagagctcataggaaaatggacttgatttgaaattggagccagagtttactcgtgttggttatctattcatcagcttcctgacatgttaagagaatacattaaagagaaaatactgttttttaatcctaaaatttttcttccactaagataaaccaaatgtccttacatatatgtaaacccatctatttaaacgcaaaggtgggttgatgtcagtttacatagcagaaagcattcactatcctctaagatttgtttctgcaaaactttcattgctttagaattttaaaatttcaccttgtacaatggccagcccctaaagcaggaaacatttataatggattatatggaaacatcctcccagtacttgcccagcccttgaatcatgtggcttttcagtgaaaggaaagattctttttctaggaaaaatgagcctattttattttattttattttattttttgacacaaactgtagattttagcagccctggcccaaaggaatttgattacttttgttttaaacagtacaaaggggacactataattacaaaaacatccttaactgatttgagttgtttttatttctttggatatattttcagagtggtaaattgtgtgtgagaattacaaatgattattcttttagtggtttcttagcctctcttacagcccacggggatagtactgtacatcaataccttcatatgaaatttttatatgcaatgaaaataaaagcatgggttgattctgcctatttatgactcaatcttttacaaataaaagattattcattttaaattatagttcaatcagcatgtctcttaggatactgaacgtggttgaaatgaaaggatagtgacatcataagttagtactgatattcataaccaaataaagccaacttgagtaattttgctacattaaaaattaccaaaattacttagatggcctataagattaagcatggtgttttctaagcaagctttgaaaggggccttccatacttacttaattgaatattctgggatattgaaaattattcagatacttgacaattatttttggttacctactccgcaaactacaaagttttaaggactcaacaataagttaatgagacacagtgtttgctttcatggagcttacagtctggaggggacaaaggcttaaacaatactcatataattatatatgtgatcagtacaatgaaggagctcagtggggtaaataagcaggaacctgaacttgatctgttccggagggccacagaaggcttccttgaggccttgagaaagtgatttgcatctgagttctgaaggattgtaagaggtaactagggaaaaagttgacaggaagaggaaggggatccagacaagaaacatttgcaaagatcttgaggcataaatgagcttgagacatctggagaaactgaggaaaagtgagagagtaggcagggcctggagccgcagagccattgctaaccatcctgtgtgagatatcccccattctgtagctttattctcataaccctgctcaattttctttataacacttctcacagatttatatacgtgtttgtttttgttatctgtctctcccaccagaccacagctccatgagagcaaggtctttgcttaccaatatatcactagcacttaaaactatgcctggtacacagtaggttcttaatatgtgttgaatatagccatcaaattgatattggatataattcaatctgataagatattttgagatattaaagagtttttaacttgataccataaaaa

SEQ ID NO: 66 - protein, 518 aa, Homo sapiens
MPEANYLLSVSWGYIKFKRMLNRELTHLSEMSRSGNQVSEFISNTFLDKQHEVEIPSPTQKEKEKKKRPMSQISGVKKLMHSSSLTNSSIPRFGVKTEQEDVLAKELEDVNKWGLHVFRIAELSGNRPLTVIMHTIFQERDLLKTFKIPVDTLITYLMTLEDHYHADVAYHNNIHAADVVQSTHVLLSTPALEAVFTDLEILAAIFASAIHDVDHPGVSNQFLINTNSELALMYNDSSVLENHHLAVGFKLLQEENCDIFQNLTKKQRQSLRKMVIDIVLATDMSKHMNLLADLKTMVETKKVTSSGVLLLDNYSDRIQVLQNMVHCADLSNPTKPLQLYRQWTDRIMEEFFRQGDRERERGMEISPMCDKHNASVEKSQVGFIDYIVHPLWETWADLVHPDAQDILDTLEDNREWYQSTIPQSPSPAPDDPEEGRQGQTEKFQFELTLEEDGESDTEKDSGSQVEEDTSCSDSKTLCTQDSESTEIPLDEQVEEEAVGEEEESQPEACVIDDRSPDT

SEQ ID NO: 67 - DNA, 8086 bp, Homo sapiens
  source 1..8086: mol_type = other DNA
ctatagttggcgtaccctgaggcctgccagttcctgccttaatgcatatgtagtcgtaattgagttctgacacggccttggatgtttctgtcctaaatagctgacattgcatcttcaagactgtcattccagttggcttttgagtggatacgtgcagtgagatcattgacactggaaacactagttcccattttaattacttaaaacaccacgatgaaaagaaatacctgtgatttgctttctcggagcaaaagtgcctctgaggaaacactacattccagtaatgaagaggaagaccctttccgcggaatggaaccctatcttgtccggagactttcatgtcgcaatattcagcttccccctctcgccttcagacagttggaacaagctgacttgaaaagtgaatcagagaacattcaacgaccaaccagcctccccctgaagattctgccgctgattgctatcacttctgcagaatccagtggttttgatgtggacaatggcacatctgcgggacggagtcccttggatcccatgaccagcccaggatccgggctaattctccaagcaaattttgtccacagtcaacgacgggagtccttcctgtatcgatccgacagcgattatgacctctctccaaagtctatgtcccggaactcctccattgccagtgatatacacggagatgacttgattgtgactccatttgctcaggtcttggccagtctgcgaactgtacgaaacaactttgctgcattaactaatttgcaagatcgagcacctagcaaaagatcacccatgtgcaaccaaccatccatcaacaaagccaccataacagaggaggcctaccagaaactggccagcgagaccctggaggagctggactggtgtctggaccagctagagaccctacagaccaggcactccgtcagtgagatggcctccaacaagtttaaaaggatgcttaatcgggagctcacccatctctctgaaatgagtcggtctggaaatcaagtgtcagagtttatatcaaacacattcttagataagcaacatgaagtggaaattccttctccaactcagaaggaaaaggagaaaaagaaaagaccaatgtctcagatcagtggagtcaagaaattgatgcacagctctagtctgactaattcaagtatcccaaggtttggagttaaaactgaacaagaagatgtccttgccaaggaactagaagatgtgaacaaatggggtcttcatgttttcagaatagcagagttgtctggtaaccggcccttgactgttatcatgcacaccatttttcaggaacgggatttattaaaaacatttaaaattccagtagatactttaattacatatcttatgactctcgaagaccattaccatgctgatgtggcctatcacaacaatatccatgctgcagatgttgtccagtctactcatgtgctattatctacacctgctttggaggctgtgtttacagatttggagattcttgcagcaatttttgccagtgcaatacatgatgtagatcatcctggtgtgtccaatcaatttctgatcaatacaaactctgaacttgccttgatgtacaatgattcctcagtcttagagaaccatcatttggctgtgggctttaaattgcttcaggaagaaaactgtgacattttccagaatttgaccaaaaaacaaagacaatctttaaggaaaatggtcattgacatcgtacttgcaacagatatgtcaaaacacatgaatctactggctgatttgaagactatggttgaaactaagaaagtgacaagctctggagttcttcttcttgataattattccgataggattcaggttcttcagaatatggtgcactgtgcagatctgagcaacccaacaaagcctctccagctgtaccgccagtggacggaccggataatggaggagttcttccgccaaggagaccgagagagggaacgtggcatggagataagccccatgtgtgacaagcacaatgcttccgtggaaaaatcacaggtgggcttcatagactatattgttcatcccctctgggagacatgggcagacctcgtccaccctgacgcccaggatattttggacactttggaggacaatcgtgaatggtaccagagcacaatccctcagagcccctctcctgcacctgatgacccagaggagggccggcagggtcaaactgagaaattccagtttgaactaactttagaggaagatggtgagtcagacacggaaaaggacagtggcagtcaagtggaagaagacactagctgcagtgactccaagactctttgtactcaagactcagagtctactgaaattccccttgatgaacaggttgaagaggaggcagtaggggaagaagaggaaagccagcctgaagcctgtgtcatagatgatcgttctcctgacacgtaacagtgcaaaaactttcatgccttttttttttttaagtagaaaaattgtttccaaagtgcatgtcacatgccacaaccacggtcacacctcactgtcatctgccaggacgtttgttgaacaaaactgaccttgactactcagtccagcgctcaggaatatcgtaaccagttttttcacctccatgtcatccgagcaaggtggacatcttcacgaacagcgtttttaacaagatttcagcttggtagagctgacaaagcagataaaatctactccaaattattttcaagagagtgtgactcatcaggcagcccaaaagtttattggacttggggtttctattcctttttatttgtttgcaatattttcagaagaaaggcattgcacagagtgaacttaatggacgaagcaacaaatatgtcaagaacaggacatagcacgaatctgttaccagtaggaggaggatgagccacagaaattgcataattttctaatttcaagtcttcctgatacatgactgaatagtgtggttcagtgagctgcactgacctctacattttgtatgatatgtaaaacagattttttgtagagcttacttttattattaaatgtattgaggtattatatttaaaaaaaactatgttcagaacttcatctgccactggttatttttttctaaggagtaacttgcaagttttcagtacaaatctgtgctacactggataaaaatctaatttatgaattttacttgcaccttatagttcatagcaattaactgatttgtagtgattcattgtttgttttatataccaatgacttccatattttaaaagagaaaaacaactttatgttgcaggaaaccctttttgtaagtctttattatttactttgcattttgtttcactctttccagataagcagagttgctcttcaccagtgtttttcttcatgtgcaaagtgactatttgttctataatacttttatgtgtgttatatcaaatgtgtcttaagcttcatgcaaactcagtcatcagttcgtgttgtctgaagcaagtgggagatatataaatacccagtagctaaaatggtcagtcttttttagatgttttcctacttagtatctcctaataacgttttgctgtgtcactagatgttcatttcacaagtgcatgtctttctaataatccacacatttcatgctctaataatccacacatttcatgctcatttttattgtttttacagccagttatagtaagaaaaaggtttttccccttgtgctgctttataatttagcgtgtgtctgaaccttatccatgtttgctagatgaggtcttgtcaaatatatcactaccattgtcaccggtgaaaagaaacaggtagttaagttagggttaacattcatttcaaccacgaggttgtatatcatgactagcttttactcttggtttacagagaaaagttaaacagccaactaggcagtttttaagaatattaacaatatattaacaaacaccaatacaactaatcctatttggttttaatgatttcaccatgggattaagaactatatcaggaacatccctgagaaacggttttaagtgtagcaactactcttccttaatggacagccacataacgtgtaggaagtcctttatcacttatcctcgatccataagcatatcttgcagaggggaactacttctttaaacacatggagggaaagaagatgatgccactggcaccagagggttagtactgtgatgcatcctaaaatatttattatattggtaaaaattctggttaaataaaaaattagagatcactcttggctgatttcagcaccaggaactgtattacagttttagagattaattcctagtgtttacctgattatagcagttggcatcatggggcatttaattctgactttatccccacgtcagccttaataaagtcttctttaccttctctatgaagactttaaagcccaaataatcatttttcacattgatattcaagaattgagatagatagaagccaaagtgggtatctgacaagtggaaaatcaaacgtttaagaagaattacaactctgaaaagcatttatatgtggaacttctcaaggagcctcctggggactggaaagtaagtcatcagccaggcaaatgactcatgctgaagagagtccccatttcagtcccctgagatctagctgatgcttagatcctttgaaataaaaattatgtctttataactctgatcttttacataaagcagaagaggaatcaactagttaattgcaaggtttctactctgtttcctctgtaaagatcagatggtaatctttcaaataagaaaaaaataaagacgtatgtttgaccaagtagtttcacaagaatatttgggaacttgtttcttttaattttatttgtccctgagtgaagtctagaaagaaaggtaaagagtctagagtttattcctctttccaaaacattctcattcctctcctccctacacttagtatttcccccacagagtgcctagaatcttaataatgaataaaataaaaagcagcaatatgtcattaacaaatccagacctgaaagggtaaagggtttataactgcactaataaagagaggctctttttttttcttccagtttgttggtttttaatggtaccgtgttgtaaagatacccactaatggacaatcaaattgcagaaaaggctcaatatccaagagacagggactaatgcactgtacaatctgcttatccttgcccttctctcttgccaaagtgtgcttcagaaatatatactgctttaaaaaagaataaaagaatatccttttacaagtggctttacatttcctaaaatgccataagaaaatgcaatatctgggtactgtatggggaaaaaaatgtccaagtttgtgtaaaaccagtgcatttcagcttgcaagttactgaacacaataatgctgttttaattttgttttatatcagttaaaattcacaataatgtagatagaacaaattacagacaaggaaagaaaaaacttgaatgaaatggattttacagaaagctttatgataatttttgaatgcattatttattttttgtgccatgcattttttttctcaccaaatgaccttacctgtaatacagtcttgtttgtctgtttacaaccatgtatttattgcaatgtacatactgtaatgttaattgtaaattatctgttcttattaaaacatcatcccatgatgggatggtgttgatatatttggaaactcttggtgagagaatgaatggtgtgtatacatactctgtacatttttcttttctcctgtaatatagtcttgtcaccttagagcttgtttatggaagattcaagaaaactataaaatacttaaagatatataaatttaaaaaaacatagctgcaggtctttggtcccagggctgtgccttaactttaaccaatattttcttctgttttgctgcatttgaaaggtaacagtggagctagggctgggcattttacatccaggcttttaattgattagaattctgccaataggtggattttacaaaaccacagacaacctctgaaagattctgagacccttttgagacagaagctcttaagtacttcttgccagggagcagcactgcatgtgtgatggttgtttgccatctgttgatcaggaactacttcagctacttgcatttgattatttcctttttttttttttttaactcggaaacacaactggggaaatatattctttcccagtgattataaacaatctttttcttttttttaagtccttttggcttctagagctcataggaaaatggacttgatttgaaattggagccagagtttactcgtgttggttatctattcatcagcttcctgacatgttaagagaatacattaaagagaaaatactgttttttaatcctaaaatttttcttccactaagataaaccaaatgtccttacatatatgtaaacccatctatttaaacgcaaaggtgggttgatgtcagtttacatagcagaaagcattcactatcctctaagatttgtttctgcaaaactttcattgctttagaattttaaaatttcaccttgtacaatggccagcccctaaagcaggaaacatttataatggattatatggaaacatcctcccagtacttgcccagcccttgaatcatgtggcttttcagtgaaaggaaagattctttttctaggaaaaatgagcctattttattttattttattttattttttgacacaaactgtagattttagcagccctggcccaaaggaatttgattacttttgttttaaacagtacaaaggggacactataattacaaaaacatccttaactgatttgagttgtttttatttctttggatatattttcagagtggtaaattgtgtgtgagaattacaaatgattattcttttagtggtttcttagcctctcttacagcccacggggatagtactgtacatcaataccttcatatgaaatttttatatgcaatgaaaataaaagcatgggttgattctgcctatttatgactcaatcttttacaaataaaagattattcattttaaattatagttcaatcagcatgtctcttaggatactgaacgtggttgaaatgaaaggatagtgacatcataagttagtactgatattcataaccaaataaagccaacttgagtaattttgctacattaaaaattaccaaaattacttagatggcctataagattaagcatggtgttttctaagcaagctttgaaaggggccttccatacttacttaattgaatattctgggatattgaaaattattcagatacttgacaattatttttggttacctactccgcaaactacaaagttttaaggactcaacaataagttaatgagacacagtgtttgctttcatggagcttacagtctggaggggacaaaggcttaaacaatactcatataattatatatgtgatcagtacaatgaaggagctcagtggggtaaataagcaggaacctgaacttgatctgttccggagggccacagaaggcttccttgaggccttgagaaagtgatttgcatctgagttctgaaggattgtaagaggtaactagggaaaaagttgacaggaagaggaaggggatccagacaagaaacatttgcaaagatcttgaggcataaatgagcttgagacatctggagaaactgaggaaaagtgagagagtaggcagggcctggagccgcagagccattgctaaccatcctgtgtgagatatcccccattctgtagctttattctcataaccctgctcaattttctttataacacttctcacagatttatatacgtgtttgtttttgttatctgtctctcccaccagaccacagctccatgagagcaaggtctttgcttaccaatatatcactagcacttaaaactatgcctggtacacagtaggttcttaatatgtgttgaatatagccatcaaattgatattggatataattcaatctgataagatattttgagatattaaagagtttttaacttgataccataaaaa

SEQ ID NO: 68 - protein, 748 aa, Homo sapiens
MKRNTCDLLSRSKSASEETLHSSNEEEDPFRGMEPYLVRRLSCRNIQLPPLAFRQLEQADLKSESENIQRPTSLPLKILPLIAITSAESSGFDVDNGTSAGRSPLDPMTSPGSGLILQANFVHSQRRESFLYRSDSDYDLSPKSMSRNSSIASDIHGDDLIVTPFAQVLASLRTVRNNFAALTNLQDRAPSKRSPMCNQPSINKATITEEAYQKLASETLEELDWCLDQLETLQTRHSVSEMASNKFKRMLNRELTHLSEMSRSGNQVSEFISNTFLDKQHEVEIPSPTQKEKEKKKRPMSQISGVKKLMHSSSLTNSSIPRFGVKTEQEDVLAKELEDVNKWGLHVFRIAELSGNRPLTVIMHTIFQERDLLKTFKIPVDTLITYLMTLEDHYHADVAYHNNIHAADVVQSTHVLLSTPALEAVFTDLEILAAIFASAIHDVDHPGVSNQFLINTNSELALMYNDSSVLENHHLAVGFKLLQEENCDIFQNLTKKQRQSLRKMVIDIVLATDMSKHMNLLADLKTMVETKKVTSSGVLLLDNYSDRIQVLQNMVHCADLSNPTKPLQLYRQWTDRIMEEFFRQGDRERERGMEISPMCDKHNASVEKSQVGFIDYIVHPLWETWADLVHPDAQDILDTLEDNREWYQSTIPQSPSPAPDDPEEGRQGQTEKFQFELTLEEDGESDTEKDSGSQVEEDTSCSDSKTLCTQDSESTEIPLDEQVEEEAVGEEEESQPEACVIDDRSPDT

SEQ ID NO: 69 - DNA, 7814 bp, Homo sapiens
  source 1..7814: mol_type = other DNA
acaaaggaaatgccctcactcagctacaagtgcctcctgctccgtgcggggcctcagggccccagagccccgcaccagctctgacttctcgtggttcctggggatcttggcatcgtccttaaaaatggcttttgtttgggatcctctgggagccacggtgccaggaccatctacaagagccaaatcaagattgcgtttctcaaagtcctacagttttgatgtggacaatggcacatctgcgggacggagtcccttggatcccatgaccagcccaggatccgggctaattctccaagcaaattttgtccacagtcaacgacgggagtccttcctgtatcgatccgacagcgattatgacctctctccaaagtctatgtcccggaactcctccattgccagtgatatacacggagatgacttgattgtgactccatttgctcaggtcttggccagtctgcgaactgtacgaaacaactttgctgcattaactaatttgcaagatcgagcacctagcaaaagatcacccatgtgcaaccaaccatccatcaacaaagccaccataacagaggaggcctaccagaaactggccagcgagaccctggaggagctggactggtgtctggaccagctagagaccctacagaccaggcactccgtcagtgagatggcctccaacaagtttaaaaggatgcttaatcgggagctcacccatctctctgaaatgagtcggtctggaaatcaagtgtcagagtttatatcaaacacattcttagataagcaacatgaagtggaaattccttctccaactcagaaggaaaaggagaaaaagaaaagaccaatgtctcagatcagtggagtcaagaaattgatgcacagctctagtctgactaattcaagtatcccaaggtttggagttaaaactgaacaagaagatgtccttgccaaggaactagaagatgtgaacaaatggggtcttcatgttttcagaatagcagagttgtctggtaaccggcccttgactgttatcatgcacaccatttttcaggaacgggatttattaaaaacatttaaaattccagtagatactttaattacatatcttatgactctcgaagaccattaccatgctgatgtggcctatcacaacaatatccatgctgcagatgttgtccagtctactcatgtgctattatctacacctgctttggaggctgtgtttacagatttggagattcttgcagcaatttttgccagtgcaatacatgatgtagatcatcctggtgtgtccaatcaatttctgatcaatacaaactctgaacttgccttgatgtacaatgattcctcagtcttagagaaccatcatttggctgtgggctttaaattgcttcaggaagaaaactgtgacattttccagaatttgaccaaaaaacaaagacaatctttaaggaaaatggtcattgacatcgtacttgcaacagatatgtcaaaacacatgaatctactggctgatttgaagactatggttgaaactaagaaagtgacaagctctggagttcttcttcttgataattattccgataggattcaggttcttcagaatatggtgcactgtgcagatctgagcaacccaacaaagcctctccagctgtaccgccagtggacggaccggataatggaggagttcttccgccaaggagaccgagagagggaacgtggcatggagataagccccatgtgtgacaagcacaatgcttccgtggaaaaatcacaggtgggcttcatagactatattgttcatcccctctgggagacatgggcagacctcgtccaccctgacgcccaggatattttggacactttggaggacaatcgtgaatggtaccagagcacaatccctcagagcccctctcctgcacctgatgacccagaggagggccggcagggtcaaactgagaaattccagtttgaactaactttagaggaagatggtgagtcagacacggaaaaggacagtggcagtcaagtggaagaagacactagctgcagtgactccaagactctttgtactcaagactcagagtctactgaaattccccttgatgaacaggttgaagaggaggcagtaggggaagaagaggaaagccagcctgaagcctgtgtcatagatgatcgttctcctgacacgtaacagtgcaaaaactttcatgccttttttttttttaagtagaaaaattgtttccaaagtgcatgtcacatgccacaaccacggtcacacctcactgtcatctgccaggacgtttgttgaacaaaactgaccttgactactcagtccagcgctcaggaatatcgtaaccagttttttcacctccatgtcatccgagcaaggtggacatcttcacgaacagcgtttttaacaagatttcagcttggtagagctgacaaagcagataaaatctactccaaattattttcaagagagtgtgactcatcaggcagcccaaaagtttattggacttggggtttctattcctttttatttgtttgcaatattttcagaagaaaggcattgcacagagtgaacttaatggacgaagcaacaaatatgtcaagaacaggacatagcacgaatctgttaccagtaggaggaggatgagccacagaaattgcataattttctaatttcaagtcttcctgatacatgactgaatagtgtggttcagtgagctgcactgacctctacattttgtatgatatgtaaaacagattttttgtagagcttacttttattattaaatgtattgaggtattatatttaaaaaaaactatgttcagaacttcatctgccactggttatttttttctaaggagtaacttgcaagttttcagtacaaatctgtgctacactggataaaaatctaatttatgaattttacttgcaccttatagttcatagcaattaactgatttgtagtgattcattgtttgttttatataccaatgacttccatattttaaaagagaaaaacaactttatgttgcaggaaaccctttttgtaagtctttattatttactttgcattttgtttcactctttccagataagcagagttgctcttcaccagtgtttttcttcatgtgcaaagtgactatttgttctataatacttttatgtgtgttatatcaaatgtgtcttaagcttcatgcaaactcagtcatcagttcgtgttgtctgaagcaagtgggagatatataaatacccagtagctaaaatggtcagtcttttttagatgttttcctacttagtatctcctaataacgttttgctgtgtcactagatgttcatttcacaagtgcatgtctttctaataatccacacatttcatgctctaataatccacacatttcatgctcatttttattgtttttacagccagttatagtaagaaaaaggtttttccccttgtgctgctttataatttagcgtgtgtctgaaccttatccatgtttgctagatgaggtcttgtcaaatatatcactaccattgtcaccggtgaaaagaaacaggtagttaagttagggttaacattcatttcaaccacgaggttgtatatcatgactagcttttactcttggtttacagagaaaagttaaacagccaactaggcagtttttaagaatattaacaatatattaacaaacaccaatacaactaatcctatttggttttaatgatttcaccatgggattaagaactatatcaggaacatccctgagaaacggttttaagtgtagcaactactcttccttaatggacagccacataacgtgtaggaagtcctttatcacttatcctcgatccataagcatatcttgcagaggggaactacttctttaaacacatggagggaaagaagatgatgccactggcaccagagggttagtactgtgatgcatcctaaaatatttattatattggtaaaaattctggttaaataaaaaattagagatcactcttggctgatttcagcaccaggaactgtattacagttttagagattaattcctagtgtttacctgattatagcagttggcatcatggggcatttaattctgactttatccccacgtcagccttaataaagtcttctttaccttctctatgaagactttaaagcccaaataatcatttttcacattgatattcaagaattgagatagatagaagccaaagtgggtatctgacaagtggaaaatcaaacgtttaagaagaattacaactctgaaaagcatttatatgtggaacttctcaaggagcctcctggggactggaaagtaagtcatcagccaggcaaatgactcatgctgaagagagtccccatttcagtcccctgagatctagctgatgcttagatcctttgaaataaaaattatgtctttataactctgatcttttacataaagcagaagaggaatcaactagttaattgcaaggtttctactctgtttcctctgtaaagatcagatggtaatctttcaaataagaaaaaaataaagacgtatgtttgaccaagtagtttcacaagaatatttgggaacttgtttcttttaattttatttgtccctgagtgaagtctagaaagaaaggtaaagagtctagagtttattcctctttccaaaacattctcattcctctcctccctacacttagtatttcccccacagagtgcctagaatcttaataatgaataaaataaaaagcagcaatatgtcattaacaaatccagacctgaaagggtaaagggtttataactgcactaataaagagaggctctttttttttcttccagtttgttggtttttaatggtaccgtgttgtaaagatacccactaatggacaatcaaattgcagaaaaggctcaatatccaagagacagggactaatgcactgtacaatctgcttatccttgcccttctctcttgccaaagtgtgcttcagaaatatatactgctttaaaaaagaataaaagaatatccttttacaagtggctttacatttcctaaaatgccataagaaaatgcaatatctgggtactgtatggggaaaaaaatgtccaagtttgtgtaaaaccagtgcatttcagcttgcaagttactgaacacaataatgctgttttaattttgttttatatcagttaaaattcacaataatgtagatagaacaaattacagacaaggaaagaaaaaacttgaatgaaatggattttacagaaagctttatgataatttttgaatgcattatttattttttgtgccatgcattttttttctcaccaaatgaccttacctgtaatacagtcttgtttgtctgtttacaaccatgtatttattgcaatgtacatactgtaatgttaattgtaaattatctgttcttattaaaacatcatcccatgatgggatggtgttgatatatttggaaactcttggtgagagaatgaatggtgtgtatacatactctgtacatttttcttttctcctgtaatatagtcttgtcaccttagagcttgtttatggaagattcaagaaaactataaaatacttaaagatatataaatttaaaaaaacatagctgcaggtctttggtcccagggctgtgccttaactttaaccaatattttcttctgttttgctgcatttgaaaggtaacagtggagctagggctgggcattttacatccaggcttttaattgattagaattctgccaataggtggattttacaaaaccacagacaacctctgaaagattctgagacccttttgagacagaagctcttaagtacttcttgccagggagcagcactgcatgtgtgatggttgtttgccatctgttgatcaggaactacttcagctacttgcatttgattatttcctttttttttttttttaactcggaaacacaactggggaaatatattctttcccagtgattataaacaatctttttcttttttttaagtccttttggcttctagagctcataggaaaatggacttgatttgaaattggagccagagtttactcgtgttggttatctattcatcagcttcctgacatgttaagagaatacattaaagagaaaatactgttttttaatcctaaaatttttcttccactaagataaaccaaatgtccttacatatatgtaaacccatctatttaaacgcaaaggtgggttgatgtcagtttacatagcagaaagcattcactatcctctaagatttgtttctgcaaaactttcattgctttagaattttaaaatttcaccttgtacaatggccagcccctaaagcaggaaacatttataatggattatatggaaacatcctcccagtacttgcccagcccttgaatcatgtggcttttcagtgaaaggaaagattctttttctaggaaaaatgagcctattttattttattttattttattttttgacacaaactgtagattttagcagccctggcccaaaggaatttgattacttttgttttaaacagtacaaaggggacactataattacaaaaacatccttaactgatttgagttgtttttatttctttggatatattttcagagtggtaaattgtgtgtgagaattacaaatgattattcttttagtggtttcttagcctctcttacagcccacggggatagtactgtacatcaataccttcatatgaaatttttatatgcaatgaaaataaaagcatgggttgattctgcctatttatgactcaatcttttacaaataaaagattattcattttaaattatagttcaatcagcatgtctcttaggatactgaacgtggttgaaatgaaaggatagtgacatcataagttagtactgatattcataaccaaataaagccaacttgagtaattttgctacattaaaaattaccaaaattacttagatggcctataagattaagcatggtgttttctaagcaagctttgaaaggggccttccatacttacttaattgaatattctgggatattgaaaattattcagatacttgacaattatttttggttacctactccgcaaactacaaagttttaaggactcaacaataagttaatgagacacagtgtttgctttcatggagcttacagtctggaggggacaaaggcttaaacaatactcatataattatatatgtgatcagtacaatgaaggagctcagtggggtaaataagcaggaacctgaacttgatctgttccggagggccacagaaggcttccttgaggccttgagaaagtgatttgcatctgagttctgaaggattgtaagaggtaactagggaaaaagttgacaggaagaggaaggggatccagacaagaaacatttgcaaagatcttgaggcataaatgagcttgagacatctggagaaactgaggaaaagtgagagagtaggcagggcctggagccgcagagccattgctaaccatcctgtgtgagatatcccccattctgtagctttattctcataaccctgctcaattttctttataacacttctcacagatttatatacgtgtttgtttttgttatctgtctctcccaccagaccacagctccatgagagcaaggtctttgcttaccaatatatcactagcacttaaaactatgcctggtacacagtaggttcttaatatgtgttgaatatagccatcaaattgatattggatataattcaatctgataagatattttgagatattaaagagtttttaacttgataccataaaaa

SEQ ID NO: 70 - protein, 687 aa, Homo sapiens
MAFVWDPLGATVPGPSTRAKSRLRFSKSYSFDVDNGTSAGRSPLDPMTSPGSGLILQANFVHSQRRESFLYRSDSDYDLSPKSMSRNSSIASDIHGDDLIVTPFAQVLASLRTVRNNFAALTNLQDRAPSKRSPMCNQPSINKATITEEAYQKLASETLEELDWCLDQLETLQTRHSVSEMASNKFKRMLNRELTHLSEMSRSGNQVSEFISNTFLDKQHEVEIPSPTQKEKEKKKRPMSQISGVKKLMHSSSLTNSSIPRFGVKTEQEDVLAKELEDVNKWGLHVFRIAELSGNRPLTVIMHTIFQERDLLKTFKIPVDTLITYLMTLEDHYHADVAYHNNIHAADVVQSTHVLLSTPALEAVFTDLEILAAIFASAIHDVDHPGVSNQFLINTNSELALMYNDSSVLENHHLAVGFKLLQEENCDIFQNLTKKQRQSLRKMVIDIVLATDMSKHMNLLADLKTMVETKKVTSSGVLLLDNYSDRIQVLQNMVHCADLSNPTKPLQLYRQWTDRIMEEFFRQGDRERERGMEISPMCDKHNASVEKSQVGFIDYIVHPLWETWADLVHPDAQDILDTLEDNREWYQSTIPQSPSPAPDDPEEGRQGQTEKFQFELTLEEDGESDTEKDSGSQVEEDTSCSDSKTLCTQDSESTEIPLDEQVEEEAVGEEEESQPEACVIDDRSPDT

SEQ ID NO: 71 - DNA, 8379 bp, Homo sapiens
  source 1..8379: mol_type = other DNA
cactgccctgcggtgttttgaactgccttcttacagacgtcatacagcccttgaggaatagtttctgcctggtgagattgaatgatagttctcattcacaaaaccctggattctaagcagggacacacagaaattactttcgcaggtaaatcagcccacccagccaaagtgtggagagatttgttccttggctgacttctttgctccacggagaggagtgttttcctgtgcttgccctgaaatggaacttccttgacagctctcccgtgttacagtacctcccggtcattttctttttctctctctctacctgcgctcttcgagtgtcagaaacctttaaagctgttactatggaattgcaaaaaagagatcaagtgactctttcactatgctggtttcccttgtgacccagatgaagaatcaattcagaattcagttcctcccttggcattgcaagacacagaagaaactgtcacttcctaacagcctagtactggagtaaattcagtatgaaggaagaaagcgctcctgcgtgttagaaccttgcccatgagctggaccgaggacaggagatggactccaggaaaattggatttcttcaagcagcctcccttggaaatggaatatctttaaaatcttctttgcagaaagacagttagaatgtattaatcagaatagttgaagacttattttcctttttattttttttcaaaatgagcattattatgaagccaagatcccgatctacaagttccctaaggactgcagaggcagtttgttttgatgtggacaatggcacatctgcgggacggagtcccttggatcccatgaccagcccaggatccgggctaattctccaagcaaattttgtccacagtcaacgacgggagtccttcctgtatcgatccgacagcgattatgacctctctccaaagtctatgtcccggaactcctccattgccagtgatatacacggagatgacttgattgtgactccatttgctcaggtcttggccagtctgcgaactgtacgaaacaactttgctgcattaactaatttgcaagatcgagcacctagcaaaagatcacccatgtgcaaccaaccatccatcaacaaagccaccataacagaggaggcctaccagaaactggccagcgagaccctggaggagctggactggtgtctggaccagctagagaccctacagaccaggcactccgtcagtgagatggcctccaacaagtttaaaaggatgcttaatcgggagctcacccatctctctgaaatgagtcggtctggaaatcaagtgtcagagtttatatcaaacacattcttagataagcaacatgaagtggaaattccttctccaactcagaaggaaaaggagaaaaagaaaagaccaatgtctcagatcagtggagtcaagaaattgatgcacagctctagtctgactaattcaagtatcccaaggtttggagttaaaactgaacaagaagatgtccttgccaaggaactagaagatgtgaacaaatggggtcttcatgttttcagaatagcagagttgtctggtaaccggcccttgactgttatcatgcacaccatttttcaggaacgggatttattaaaaacatttaaaattccagtagatactttaattacatatcttatgactctcgaagaccattaccatgctgatgtggcctatcacaacaatatccatgctgcagatgttgtccagtctactcatgtgctattatctacacctgctttggaggctgtgtttacagatttggagattcttgcagcaatttttgccagtgcaatacatgatgtagatcatcctggtgtgtccaatcaatttctgatcaatacaaactctgaacttgccttgatgtacaatgattcctcagtcttagagaaccatcatttggctgtgggctttaaattgcttcaggaagaaaactgtgacattttccagaatttgaccaaaaaacaaagacaatctttaaggaaaatggtcattgacatcgtacttgcaacagatatgtcaaaacacatgaatctactggctgatttgaagactatggttgaaactaagaaagtgacaagctctggagttcttcttcttgataattattccgataggattcaggttcttcagaatatggtgcactgtgcagatctgagcaacccaacaaagcctctccagctgtaccgccagtggacggaccggataatggaggagttcttccgccaaggagaccgagagagggaacgtggcatggagataagccccatgtgtgacaagcacaatgcttccgtggaaaaatcacaggtgggcttcatagactatattgttcatcccctctgggagacatgggcagacctcgtccaccctgacgcccaggatattttggacactttggaggacaatcgtgaatggtaccagagcacaatccctcagagcccctctcctgcacctgatgacccagaggagggccggcagggtcaaactgagaaattccagtttgaactaactttagaggaagatggtgagtcagacacggaaaaggacagtggcagtcaagtggaagaagacactagctgcagtgactccaagactctttgtactcaagactcagagtctactgaaattccccttgatgaacaggttgaagaggaggcagtaggggaagaagaggaaagccagcctgaagcctgtgtcatagatgatcgttctcctgacacgtaacagtgcaaaaactttcatgccttttttttttttaagtagaaaaattgtttccaaagtgcatgtcacatgccacaaccacggtcacacctcactgtcatctgccaggacgtttgttgaacaaaactgaccttgactactcagtccagcgctcaggaatatcgtaaccagttttttcacctccatgtcatccgagcaaggtggacatcttcacgaacagcgtttttaacaagatttcagcttggtagagctgacaaagcagataaaatctactccaaattattttcaagagagtgtgactcatcaggcagcccaaaagtttattggacttggggtttctattcctttttatttgtttgcaatattttcagaagaaaggcattgcacagagtgaacttaatggacgaagcaacaaatatgtcaagaacaggacatagcacgaatctgttaccagtaggaggaggatgagccacagaaattgcataattttctaatttcaagtcttcctgatacatgactgaatagtgtggttcagtgagctgcactgacctctacattttgtatgatatgtaaaacagattttttgtagagcttacttttattattaaatgtattgaggtattatatttaaaaaaaactatgttcagaacttcatctgccactggttatttttttctaaggagtaacttgcaagttttcagtacaaatctgtgctacactggataaaaatctaatttatgaattttacttgcaccttatagttcatagcaattaactgatttgtagtgattcattgtttgttttatataccaatgacttccatattttaaaagagaaaaacaactttatgttgcaggaaaccctttttgtaagtctttattatttactttgcattttgtttcactctttccagataagcagagttgctcttcaccagtgtttttcttcatgtgcaaagtgactatttgttctataatacttttatgtgtgttatatcaaatgtgtcttaagcttcatgcaaactcagtcatcagttcgtgttgtctgaagcaagtgggagatatataaatacccagtagctaaaatggtcagtcttttttagatgttttcctacttagtatctcctaataacgttttgctgtgtcactagatgttcatttcacaagtgcatgtctttctaataatccacacatttcatgctctaataatccacacatttcatgctcatttttattgtttttacagccagttatagtaagaaaaaggtttttccccttgtgctgctttataatttagcgtgtgtctgaaccttatccatgtttgctagatgaggtcttgtcaaatatatcactaccattgtcaccggtgaaaagaaacaggtagttaagttagggttaacattcatttcaaccacgaggttgtatatcatgactagcttttactcttggtttacagagaaaagttaaacagccaactaggcagtttttaagaatattaacaatatattaacaaacaccaatacaactaatcctatttggttttaatgatttcaccatgggattaagaactatatcaggaacatccctgagaaacggttttaagtgtagcaactactcttccttaatggacagccacataacgtgtaggaagtcctttatcacttatcctcgatccataagcatatcttgcagaggggaactacttctttaaacacatggagggaaagaagatgatgccactggcaccagagggttagtactgtgatgcatcctaaaatatttattatattggtaaaaattctggttaaataaaaaattagagatcactcttggctgatttcagcaccaggaactgtattacagttttagagattaattcctagtgtttacctgattatagcagttggcatcatggggcatttaattctgactttatccccacgtcagccttaataaagtcttctttaccttctctatgaagactttaaagcccaaataatcatttttcacattgatattcaagaattgagatagatagaagccaaagtgggtatctgacaagtggaaaatcaaacgtttaagaagaattacaactctgaaaagcatttatatgtggaacttctcaaggagcctcctggggactggaaagtaagtcatcagccaggcaaatgactcatgctgaagagagtccccatttcagtcccctgagatctagctgatgcttagatcctttgaaataaaaattatgtctttataactctgatcttttacataaagcagaagaggaatcaactagttaattgcaaggtttctactctgtttcctctgtaaagatcagatggtaatctttcaaataagaaaaaaataaagacgtatgtttgaccaagtagtttcacaagaatatttgggaacttgtttcttttaattttatttgtccctgagtgaagtctagaaagaaaggtaaagagtctagagtttattcctctttccaaaacattctcattcctctcctccctacacttagtatttcccccacagagtgcctagaatcttaataatgaataaaataaaaagcagcaatatgtcattaacaaatccagacctgaaagggtaaagggtttataactgcactaataaagagaggctctttttttttcttccagtttgttggtttttaatggtaccgtgttgtaaagatacccactaatggacaatcaaattgcagaaaaggctcaatatccaagagacagggactaatgcactgtacaatctgcttatccttgcccttctctcttgccaaagtgtgcttcagaaatatatactgctttaaaaaagaataaaagaatatccttttacaagtggctttacatttcctaaaatgccataagaaaatgcaatatctgggtactgtatggggaaaaaaatgtccaagtttgtgtaaaaccagtgcatttcagcttgcaagttactgaacacaataatgctgttttaattttgttttatatcagttaaaattcacaataatgtagatagaacaaattacagacaaggaaagaaaaaacttgaatgaaatggattttacagaaagctttatgataatttttgaatgcattatttattttttgtgccatgcattttttttctcaccaaatgaccttacctgtaatacagtcttgtttgtctgtttacaaccatgtatttattgcaatgtacatactgtaatgttaattgtaaattatctgttcttattaaaacatcatcccatgatgggatggtgttgatatatttggaaactcttggtgagagaatgaatggtgtgtatacatactctgtacatttttcttttctcctgtaatatagtcttgtcaccttagagcttgtttatggaagattcaagaaaactataaaatacttaaagatatataaatttaaaaaaacatagctgcaggtctttggtcccagggctgtgccttaactttaaccaatattttcttctgttttgctgcatttgaaaggtaacagtggagctagggctgggcattttacatccaggcttttaattgattagaattctgccaataggtggattttacaaaaccacagacaacctctgaaagattctgagacccttttgagacagaagctcttaagtacttcttgccagggagcagcactgcatgtgtgatggttgtttgccatctgttgatcaggaactacttcagctacttgcatttgattatttcctttttttttttttttaactcggaaacacaactggggaaatatattctttcccagtgattataaacaatctttttcttttttttaagtccttttggcttctagagctcataggaaaatggacttgatttgaaattggagccagagtttactcgtgttggttatctattcatcagcttcctgacatgttaagagaatacattaaagagaaaatactgttttttaatcctaaaatttttcttccactaagataaaccaaatgtccttacatatatgtaaacccatctatttaaacgcaaaggtgggttgatgtcagtttacatagcagaaagcattcactatcctctaagatttgtttctgcaaaactttcattgctttagaattttaaaatttcaccttgtacaatggccagcccctaaagcaggaaacatttataatggattatatggaaacatcctcccagtacttgcccagcccttgaatcatgtggcttttcagtgaaaggaaagattctttttctaggaaaaatgagcctattttattttattttattttattttttgacacaaactgtagattttagcagccctggcccaaaggaatttgattacttttgttttaaacagtacaaaggggacactataattacaaaaacatccttaactgatttgagttgtttttatttctttggatatattttcagagtggtaaattgtgtgtgagaattacaaatgattattcttttagtggtttcttagcctctcttacagcccacggggatagtactgtacatcaataccttcatatgaaatttttatatgcaatgaaaataaaagcatgggttgattctgcctatttatgactcaatcttttacaaataaaagattattcattttaaattatagttcaatcagcatgtctcttaggatactgaacgtggttgaaatgaaaggatagtgacatcataagttagtactgatattcataaccaaataaagccaacttgagtaattttgctacattaaaaattaccaaaattacttagatggcctataagattaagcatggtgttttctaagcaagctttgaaaggggccttccatacttacttaattgaatattctgggatattgaaaattattcagatacttgacaattatttttggttacctactccgcaaactacaaagttttaaggactcaacaataagttaatgagacacagtgtttgctttcatggagcttacagtctggaggggacaaaggcttaaacaatactcatataattatatatgtgatcagtacaatgaaggagctcagtggggtaaataagcaggaacctgaacttgatctgttccggagggccacagaaggcttccttgaggccttgagaaagtgatttgcatctgagttctgaaggattgtaagaggtaactagggaaaaagttgacaggaagaggaaggggatccagacaagaaacatttgcaaagatcttgaggcataaatgagcttgagacatctggagaaactgaggaaaagtgagagagtaggcagggcctggagccgcagagccattgctaaccatcctgtgtgagatatcccccattctgtagctttattctcataaccctgctcaattttctttataacacttctcacagatttatatacgtgtttgtttttgttatctgtctctcccaccagaccacagctccatgagagcaaggtctttgcttaccaatatatcactagcacttaaaactatgcctggtacacagtaggttcttaatatgtgttgaatatagccatcaaattgatattggatataattcaatctgataagatattttgagatattaaagagtttttaacttgataccataaaaa

SEQ ID NO: 72 - protein, 679 aa, Homo sapiens
MSIIMKPRSRSTSSLRTAEAVCFDVDNGTSAGRSPLDPMTSPGSGLILQANFVHSQRRESFLYRSDSDYDLSPKSMSRNSSIASDIHGDDLIVTPFAQVLASLRTVRNNFAALTNLQDRAPSKRSPMCNQPSINKATITEEAYQKLASETLEELDWCLDQLETLQTRHSVSEMASNKFKRMLNRELTHLSEMSRSGNQVSEFISNTFLDKQHEVEIPSPTQKEKEKKKRPMSQISGVKKLMHSSSLTNSSIPRFGVKTEQEDVLAKELEDVNKWGLHVFRIAELSGNRPLTVIMHTIFQERDLLKTFKIPVDTLITYLMTLEDHYHADVAYHNNIHAADVVQSTHVLLSTPALEAVFTDLEILAAIFASAIHDVDHPGVSNQFLINTNSELALMYNDSSVLENHHLAVGFKLLQEENCDIFQNLTKKQRQSLRKMVIDIVLATDMSKHMNLLADLKTMVETKKVTSSGVLLLDNYSDRIQVLQNMVHCADLSNPTKPLQLYRQWTDRIMEEFFRQGDRERERGMEISPMCDKHNASVEKSQVGFIDYIVHPLWETWADLVHPDAQDILDTLEDNREWYQSTIPQSPSPAPDDPEEGRQGQTEKFQFELTLEEDGESDTEKDSGSQVEEDTSCSDSKTLCTQDSESTEIPLDEQVEEEAVGEEEESQPEACVIDDRSPDT

SEQ ID NO: 73 - DNA, 8159 bp, Homo sapiens
  source 1..8159: mol_type = other DNA
ctatagttggcgtaccctgaggcctgccagttcctgccttaatgcatatgtagtcgtaattgagttctgacacggccttggatgtttctgtcctaaatagctgacattgcatcttcaagactgtcattccagttggcttttgagtggatacgtgcagtgagatcattgacactggaaacactagttcccattttaattacttaaaacaccacgatgaaaagaaatacctgtgatttgctttctcggagcaaaagtgacttgagcatctgaagattttggtttctgcagagggtgggaaaggttgaaccaatcccccatggataccaaggcctctgaggaaacactacattccagtaatgaagaggaagaccctttccgcggaatggaaccctatcttgtccggagactttcatgtcgcaatattcagcttccccctctcgccttcagacagttggaacaagctgacttgaaaagtgaatcagagaacattcaacgaccaaccagcctccccctgaagattctgccgctgattgctatcacttctgcagaatccagtggttttgatgtggacaatggcacatctgcgggacggagtcccttggatcccatgaccagcccaggatccgggctaattctccaagcaaattttgtccacagtcaacgacgggagtccttcctgtatcgatccgacagcgattatgacctctctccaaagtctatgtcccggaactcctccattgccagtgatatacacggagatgacttgattgtgactccatttgctcaggtcttggccagtctgcgaactgtacgaaacaactttgctgcattaactaatttgcaagatcgagcacctagcaaaagatcacccatgtgcaaccaaccatccatcaacaaagccaccataacagaggaggcctaccagaaactggccagcgagaccctggaggagctggactggtgtctggaccagctagagaccctacagaccaggcactccgtcagtgagatggcctccaacaagtttaaaaggatgcttaatcgggagctcacccatctctctgaaatgagtcggtctggaaatcaagtgtcagagtttatatcaaacacattcttagataagcaacatgaagtggaaattccttctccaactcagaaggaaaaggagaaaaagaaaagaccaatgtctcagatcagtggagtcaagaaattgatgcacagctctagtctgactaattcaagtatcccaaggtttggagttaaaactgaacaagaagatgtccttgccaaggaactagaagatgtgaacaaatggggtcttcatgttttcagaatagcagagttgtctggtaaccggcccttgactgttatcatgcacaccatttttcaggaacgggatttattaaaaacatttaaaattccagtagatactttaattacatatcttatgactctcgaagaccattaccatgctgatgtggcctatcacaacaatatccatgctgcagatgttgtccagtctactcatgtgctattatctacacctgctttggaggctgtgtttacagatttggagattcttgcagcaatttttgccagtgcaatacatgatgtagatcatcctggtgtgtccaatcaatttctgatcaatacaaactctgaacttgccttgatgtacaatgattcctcagtcttagagaaccatcatttggctgtgggctttaaattgcttcaggaagaaaactgtgacattttccagaatttgaccaaaaaacaaagacaatctttaaggaaaatggtcattgacatcgtacttgcaacagatatgtcaaaacacatgaatctactggctgatttgaagactatggttgaaactaagaaagtgacaagctctggagttcttcttcttgataattattccgataggattcaggttcttcagaatatggtgcactgtgcagatctgagcaacccaacaaagcctctccagctgtaccgccagtggacggaccggataatggaggagttcttccgccaaggagaccgagagagggaacgtggcatggagataagccccatgtgtgacaagcacaatgcttccgtggaaaaatcacaggtgggcttcatagactatattgttcatcccctctgggagacatgggcagacctcgtccaccctgacgcccaggatattttggacactttggaggacaatcgtgaatggtaccagagcacaatccctcagagcccctctcctgcacctgatgacccagaggagggccggcagggtcaaactgagaaattccagtttgaactaactttagaggaagatggtgagtcagacacggaaaaggacagtggcagtcaagtggaagaagacactagctgcagtgactccaagactctttgtactcaagactcagagtctactgaaattccccttgatgaacaggttgaagaggaggcagtaggggaagaagaggaaagccagcctgaagcctgtgtcatagatgatcgttctcctgacacgtaacagtgcaaaaactttcatgccttttttttttttaagtagaaaaattgtttccaaagtgcatgtcacatgccacaaccacggtcacacctcactgtcatctgccaggacgtttgttgaacaaaactgaccttgactactcagtccagcgctcaggaatatcgtaaccagttttttcacctccatgtcatccgagcaaggtggacatcttcacgaacagcgtttttaacaagatttcagcttggtagagctgacaaagcagataaaatctactccaaattattttcaagagagtgtgactcatcaggcagcccaaaagtttattggacttggggtttctattcctttttatttgtttgcaatattttcagaagaaaggcattgcacagagtgaacttaatggacgaagcaacaaatatgtcaagaacaggacatagcacgaatctgttaccagtaggaggaggatgagccacagaaattgcataattttctaatttcaagtcttcctgatacatgactgaatagtgtggttcagtgagctgcactgacctctacattttgtatgatatgtaaaacagattttttgtagagcttacttttattattaaatgtattgaggtattatatttaaaaaaaactatgttcagaacttcatctgccactggttatttttttctaaggagtaacttgcaagttttcagtacaaatctgtgctacactggataaaaatctaatttatgaattttacttgcaccttatagttcatagcaattaactgatttgtagtgattcattgtttgttttatataccaatgacttccatattttaaaagagaaaaacaactttatgttgcaggaaaccctttttgtaagtctttattatttactttgcattttgtttcactctttccagataagcagagttgctcttcaccagtgtttttcttcatgtgcaaagtgactatttgttctataatacttttatgtgtgttatatcaaatgtgtcttaagcttcatgcaaactcagtcatcagttcgtgttgtctgaagcaagtgggagatatataaatacccagtagctaaaatggtcagtcttttttagatgttttcctacttagtatctcctaataacgttttgctgtgtcactagatgttcatttcacaagtgcatgtctttctaataatccacacatttcatgctctaataatccacacatttcatgctcatttttattgtttttacagccagttatagtaagaaaaaggtttttccccttgtgctgctttataatttagcgtgtgtctgaaccttatccatgtttgctagatgaggtcttgtcaaatatatcactaccattgtcaccggtgaaaagaaacaggtagttaagttagggttaacattcatttcaaccacgaggttgtatatcatgactagcttttactcttggtttacagagaaaagttaaacagccaactaggcagtttttaagaatattaacaatatattaacaaacaccaatacaactaatcctatttggttttaatgatttcaccatgggattaagaactatatcaggaacatccctgagaaacggttttaagtgtagcaactactcttccttaatggacagccacataacgtgtaggaagtcctttatcacttatcctcgatccataagcatatcttgcagaggggaactacttctttaaacacatggagggaaagaagatgatgccactggcaccagagggttagtactgtgatgcatcctaaaatatttattatattggtaaaaattctggttaaataaaaaattagagatcactcttggctgatttcagcaccaggaactgtattacagttttagagattaattcctagtgtttacctgattatagcagttggcatcatggggcatttaattctgactttatccccacgtcagccttaataaagtcttctttaccttctctatgaagactttaaagcccaaataatcatttttcacattgatattcaagaattgagatagatagaagccaaagtgggtatctgacaagtggaaaatcaaacgtttaagaagaattacaactctgaaaagcatttatatgtggaacttctcaaggagcctcctggggactggaaagtaagtcatcagccaggcaaatgactcatgctgaagagagtccccatttcagtcccctgagatctagctgatgcttagatcctttgaaataaaaattatgtctttataactctgatcttttacataaagcagaagaggaatcaactagttaattgcaaggtttctactctgtttcctctgtaaagatcagatggtaatctttcaaataagaaaaaaataaagacgtatgtttgaccaagtagtttcacaagaatatttgggaacttgtttcttttaattttatttgtccctgagtgaagtctagaaagaaaggtaaagagtctagagtttattcctctttccaaaacattctcattcctctcctccctacacttagtatttcccccacagagtgcctagaatcttaataatgaataaaataaaaagcagcaatatgtcattaacaaatccagacctgaaagggtaaagggtttataactgcactaataaagagaggctctttttttttcttccagtttgttggtttttaatggtaccgtgttgtaaagatacccactaatggacaatcaaattgcagaaaaggctcaatatccaagagacagggactaatgcactgtacaatctgcttatccttgcccttctctcttgccaaagtgtgcttcagaaatatatactgctttaaaaaagaataaaagaatatccttttacaagtggctttacatttcctaaaatgccataagaaaatgcaatatctgggtactgtatggggaaaaaaatgtccaagtttgtgtaaaaccagtgcatttcagcttgcaagttactgaacacaataatgctgttttaattttgttttatatcagttaaaattcacaataatgtagatagaacaaattacagacaaggaaagaaaaaacttgaatgaaatggattttacagaaagctttatgataatttttgaatgcattatttattttttgtgccatgcattttttttctcaccaaatgaccttacctgtaatacagtcttgtttgtctgtttacaaccatgtatttattgcaatgtacatactgtaatgttaattgtaaattatctgttcttattaaaacatcatcccatgatgggatggtgttgatatatttggaaactcttggtgagagaatgaatggtgtgtatacatactctgtacatttttcttttctcctgtaatatagtcttgtcaccttagagcttgtttatggaagattcaagaaaactataaaatacttaaagatatataaatttaaaaaaacatagctgcaggtctttggtcccagggctgtgccttaactttaaccaatattttcttctgttttgctgcatttgaaaggtaacagtggagctagggctgggcattttacatccaggcttttaattgattagaattctgccaataggtggattttacaaaaccacagacaacctctgaaagattctgagacccttttgagacagaagctcttaagtacttcttgccagggagcagcactgcatgtgtgatggttgtttgccatctgttgatcaggaactacttcagctacttgcatttgattatttcctttttttttttttttaactcggaaacacaactggggaaatatattctttcccagtgattataaacaatctttttcttttttttaagtccttttggcttctagagctcataggaaaatggacttgatttgaaattggagccagagtttactcgtgttggttatctattcatcagcttcctgacatgttaagagaatacattaaagagaaaatactgttttttaatcctaaaatttttcttccactaagataaaccaaatgtccttacatatatgtaaacccatctatttaaacgcaaaggtgggttgatgtcagtttacatagcagaaagcattcactatcctctaagatttgtttctgcaaaactttcattgctttagaattttaaaatttcaccttgtacaatggccagcccctaaagcaggaaacatttataatggattatatggaaacatcctcccagtacttgcccagcccttgaatcatgtggcttttcagtgaaaggaaagattctttttctaggaaaaatgagcctattttattttattttattttattttttgacacaaactgtagattttagcagccctggcccaaaggaatttgattacttttgttttaaacagtacaaaggggacactataattacaaaaacatccttaactgatttgagttgtttttatttctttggatatattttcagagtggtaaattgtgtgtgagaattacaaatgattattcttttagtggtttcttagcctctcttacagcccacggggatagtactgtacatcaataccttcatatgaaatttttatatgcaatgaaaataaaagcatgggttgattctgcctatttatgactcaatcttttacaaataaaagattattcattttaaattatagttcaatcagcatgtctcttaggatactgaacgtggttgaaatgaaaggatagtgacatcataagttagtactgatattcataaccaaataaagccaacttgagtaattttgctacattaaaaattaccaaaattacttagatggcctataagattaagcatggtgttttctaagcaagctttgaaaggggccttccatacttacttaattgaatattctgggatattgaaaattattcagatacttgacaattatttttggttacctactccgcaaactacaaagttttaaggactcaacaataagttaatgagacacagtgtttgctttcatggagcttacagtctggaggggacaaaggcttaaacaatactcatataattatatatgtgatcagtacaatgaaggagctcagtggggtaaataagcaggaacctgaacttgatctgttccggagggccacagaaggcttccttgaggccttgagaaagtgatttgcatctgagttctgaaggattgtaagaggtaactagggaaaaagttgacaggaagaggaaggggatccagacaagaaacatttgcaaagatcttgaggcataaatgagcttgagacatctggagaaactgaggaaaagtgagagagtaggcagggcctggagccgcagagccattgctaaccatcctgtgtgagatatcccccattctgtagctttattctcataaccctgctcaattttctttataacacttctcacagatttatatacgtgtttgtttttgttatctgtctctcccaccagaccacagctccatgagagcaaggtctttgcttaccaatatatcactagcacttaaaactatgcctggtacacagtaggttcttaatatgtgttgaatatagccatcaaattgatattggatataattcaatctgataagatattttgagatattaaagagtttttaacttgataccataaaaa

SEQ ID NO: 74 - protein, 738 aa, Homo sapiens
MDTKASEETLHSSNEEEDPFRGMEPYLVRRLSCRNIQLPPLAFRQLEQADLKSESENIQRPTSLPLKILPLIAITSAESSGFDVDNGTSAGRSPLDPMTSPGSGLILQANFVHSQRRESFLYRSDSDYDLSPKSMSRNSSIASDIHGDDLIVTPFAQVLASLRTVRNNFAALTNLQDRAPSKRSPMCNQPSINKATITEEAYQKLASETLEELDWCLDQLETLQTRHSVSEMASNKFKRMLNRELTHLSEMSRSGNQVSEFISNTFLDKQHEVEIPSPTQKEKEKKKRPMSQISGVKKLMHSSSLTNSSIPRFGVKTEQEDVLAKELEDVNKWGLHVFRIAELSGNRPLTVIMHTIFQERDLLKTFKIPVDTLITYLMTLEDHYHADVAYHNNIHAADVVQSTHVLLSTPALEAVFTDLEILAAIFASAIHDVDHPGVSNQFLINTNSELALMYNDSSVLENHHLAVGFKLLQEENCDIFQNLTKKQRQSLRKMVIDIVLATDMSKHMNLLADLKTMVETKKVTSSGVLLLDNYSDRIQVLQNMVHCADLSNPTKPLQLYRQWTDRIMEEFFRQGDRERERGMEISPMCDKHNASVEKSQVGFIDYIVHPLWETWADLVHPDAQDILDTLEDNREWYQSTIPQSPSPAPDDPEEGRQGQTEKFQFELTLEEDGESDTEKDSGSQVEEDTSCSDSKTLCTQDSESTEIPLDEQVEEEAVGEEEESQPEACVIDDRSPDT

SEQ ID NO: 75 - DNA, 8147 bp, Homo sapiens
  source 1..8147: mol_type = other DNA
ggattcaatacttgttgcaataattgcccacgatagctgctcaaacaagagagttggaattcatctgtaaaaatcactacatgtaacgtaggagacaagaaaaatattaatgacagaagatctgcgaacatgatgcacgtgaataattttccctttagaaggcattcctggatatgctgatggtaacagcagaaaaatgtgaactctgaataaagaggtgggagtttttcagcacataaagaatatttaaagccaattcattggatgcattgaccagtaagtgtagagatcaaaatcaagaacaactccaagaattgagagcagatgcaaaccccaatttttgtgggtctccagtccagccttcccaggaatgctggtctgactactcagatttgcttttacttcttgccttttggatataatgagtttgccaagcagctgtgagtacctgactctggggaaggtggctagattccgaagcgcttatgttcatggatcaccatacgcgatcaacatgccaattgatattaagccacagaggagacgttttgatgtggacaatggcacatctgcgggacggagtcccttggatcccatgaccagcccaggatccgggctaattctccaagcaaattttgtccacagtcaacgacgggagtccttcctgtatcgatccgacagcgattatgacctctctccaaagtctatgtcccggaactcctccattgccagtgatatacacggagatgacttgattgtgactccatttgctcaggtcttggccagtctgcgaactgtacgaaacaactttgctgcattaactaatttgcaagatcgagcacctagcaaaagatcacccatgtgcaaccaaccatccatcaacaaagccaccataacagaggaggcctaccagaaactggccagcgagaccctggaggagctggactggtgtctggaccagctagagaccctacagaccaggcactccgtcagtgagatggcctccaacaagtttaaaaggatgcttaatcgggagctcacccatctctctgaaatgagtcggtctggaaatcaagtgtcagagtttatatcaaacacattcttagataagcaacatgaagtggaaattccttctccaactcagaaggaaaaggagaaaaagaaaagaccaatgtctcagatcagtggagtcaagaaattgatgcacagctctagtctgactaattcaagtatcccaaggtttggagttaaaactgaacaagaagatgtccttgccaaggaactagaagatgtgaacaaatggggtcttcatgttttcagaatagcagagttgtctggtaaccggcccttgactgttatcatgcacaccatttttcaggaacgggatttattaaaaacatttaaaattccagtagatactttaattacatatcttatgactctcgaagaccattaccatgctgatgtggcctatcacaacaatatccatgctgcagatgttgtccagtctactcatgtgctattatctacacctgctttggaggctgtgtttacagatttggagattcttgcagcaatttttgccagtgcaatacatgatgtagatcatcctggtgtgtccaatcaatttctgatcaatacaaactctgaacttgccttgatgtacaatgattcctcagtcttagagaaccatcatttggctgtgggctttaaattgcttcaggaagaaaactgtgacattttccagaatttgaccaaaaaacaaagacaatctttaaggaaaatggtcattgacatcgtacttgcaacagatatgtcaaaacacatgaatctactggctgatttgaagactatggttgaaactaagaaagtgacaagctctggagttcttcttcttgataattattccgataggattcaggttcttcagaatatggtgcactgtgcagatctgagcaacccaacaaagcctctccagctgtaccgccagtggacggaccggataatggaggagttcttccgccaaggagaccgagagagggaacgtggcatggagataagccccatgtgtgacaagcacaatgcttccgtggaaaaatcacaggtgggcttcatagactatattgttcatcccctctgggagacatgggcagacctcgtccaccctgacgcccaggatattttggacactttggaggacaatcgtgaatggtaccagagcacaatccctcagagcccctctcctgcacctgatgacccagaggagggccggcagggtcaaactgagaaattccagtttgaactaactttagaggaagatggtgagtcagacacggaaaaggacagtggcagtcaagtggaagaagacactagctgcagtgactccaagactctttgtactcaagactcagagtctactgaaattccccttgatgaacaggttgaagaggaggcagtaggggaagaagaggaaagccagcctgaagcctgtgtcatagatgatcgttctcctgacacgtaacagtgcaaaaactttcatgccttttttttttttaagtagaaaaattgtttccaaagtgcatgtcacatgccacaaccacggtcacacctcactgtcatctgccaggacgtttgttgaacaaaactgaccttgactactcagtccagcgctcaggaatatcgtaaccagttttttcacctccatgtcatccgagcaaggtggacatcttcacgaacagcgtttttaacaagatttcagcttggtagagctgacaaagcagataaaatctactccaaattattttcaagagagtgtgactcatcaggcagcccaaaagtttattggacttggggtttctattcctttttatttgtttgcaatattttcagaagaaaggcattgcacagagtgaacttaatggacgaagcaacaaatatgtcaagaacaggacatagcacgaatctgttaccagtaggaggaggatgagccacagaaattgcataattttctaatttcaagtcttcctgatacatgactgaatagtgtggttcagtgagctgcactgacctctacattttgtatgatatgtaaaacagattttttgtagagcttacttttattattaaatgtattgaggtattatatttaaaaaaaactatgttcagaacttcatctgccactggttatttttttctaaggagtaacttgcaagttttcagtacaaatctgtgctacactggataaaaatctaatttatgaattttacttgcaccttatagttcatagcaattaactgatttgtagtgattcattgtttgttttatataccaatgacttccatattttaaaagagaaaaacaactttatgttgcaggaaaccctttttgtaagtctttattatttactttgcattttgtttcactctttccagataagcagagttgctcttcaccagtgtttttcttcatgtgcaaagtgactatttgttctataatacttttatgtgtgttatatcaaatgtgtcttaagcttcatgcaaactcagtcatcagttcgtgttgtctgaagcaagtgggagatatataaatacccagtagctaaaatggtcagtcttttttagatgttttcctacttagtatctcctaataacgttttgctgtgtcactagatgttcatttcacaagtgcatgtctttctaataatccacacatttcatgctctaataatccacacatttcatgctcatttttattgtttttacagccagttatagtaagaaaaaggtttttccccttgtgctgctttataatttagcgtgtgtctgaaccttatccatgtttgctagatgaggtcttgtcaaatatatcactaccattgtcaccggtgaaaagaaacaggtagttaagttagggttaacattcatttcaaccacgaggttgtatatcatgactagcttttactcttggtttacagagaaaagttaaacagccaactaggcagtttttaagaatattaacaatatattaacaaacaccaatacaactaatcctatttggttttaatgatttcaccatgggattaagaactatatcaggaacatccctgagaaacggttttaagtgtagcaactactcttccttaatggacagccacataacgtgtaggaagtcctttatcacttatcctcgatccataagcatatcttgcagaggggaactacttctttaaacacatggagggaaagaagatgatgccactggcaccagagggttagtactgtgatgcatcctaaaatatttattatattggtaaaaattctggttaaataaaaaattagagatcactcttggctgatttcagcaccaggaactgtattacagttttagagattaattcctagtgtttacctgattatagcagttggcatcatggggcatttaattctgactttatccccacgtcagccttaataaagtcttctttaccttctctatgaagactttaaagcccaaataatcatttttcacattgatattcaagaattgagatagatagaagccaaagtgggtatctgacaagtggaaaatcaaacgtttaagaagaattacaactctgaaaagcatttatatgtggaacttctcaaggagcctcctggggactggaaagtaagtcatcagccaggcaaatgactcatgctgaagagagtccccatttcagtcccctgagatctagctgatgcttagatcctttgaaataaaaattatgtctttataactctgatcttttacataaagcagaagaggaatcaactagttaattgcaaggtttctactctgtttcctctgtaaagatcagatggtaatctttcaaataagaaaaaaataaagacgtatgtttgaccaagtagtttcacaagaatatttgggaacttgtttcttttaattttatttgtccctgagtgaagtctagaaagaaaggtaaagagtctagagtttattcctctttccaaaacattctcattcctctcctccctacacttagtatttcccccacagagtgcctagaatcttaataatgaataaaataaaaagcagcaatatgtcattaacaaatccagacctgaaagggtaaagggtttataactgcactaataaagagaggctctttttttttcttccagtttgttggtttttaatggtaccgtgttgtaaagatacccactaatggacaatcaaattgcagaaaaggctcaatatccaagagacagggactaatgcactgtacaatctgcttatccttgcccttctctcttgccaaagtgtgcttcagaaatatatactgctttaaaaaagaataaaagaatatccttttacaagtggctttacatttcctaaaatgccataagaaaatgcaatatctgggtactgtatggggaaaaaaatgtccaagtttgtgtaaaaccagtgcatttcagcttgcaagttactgaacacaataatgctgttttaattttgttttatatcagttaaaattcacaataatgtagatagaacaaattacagacaaggaaagaaaaaacttgaatgaaatggattttacagaaagctttatgataatttttgaatgcattatttattttttgtgccatgcattttttttctcaccaaatgaccttacctgtaatacagtcttgtttgtctgtttacaaccatgtatttattgcaatgtacatactgtaatgttaattgtaaattatctgttcttattaaaacatcatcccatgatgggatggtgttgatatatttggaaactcttggtgagagaatgaatggtgtgtatacatactctgtacatttttcttttctcctgtaatatagtcttgtcaccttagagcttgtttatggaagattcaagaaaactataaaatacttaaagatatataaatttaaaaaaacatagctgcaggtctttggtcccagggctgtgccttaactttaaccaatattttcttctgttttgctgcatttgaaaggtaacagtggagctagggctgggcattttacatccaggcttttaattgattagaattctgccaataggtggattttacaaaaccacagacaacctctgaaagattctgagacccttttgagacagaagctcttaagtacttcttgccagggagcagcactgcatgtgtgatggttgtttgccatctgttgatcaggaactacttcagctacttgcatttgattatttcctttttttttttttttaactcggaaacacaactggggaaatatattctttcccagtgattataaacaatctttttcttttttttaagtccttttggcttctagagctcataggaaaatggacttgatttgaaattggagccagagtttactcgtgttggttatctattcatcagcttcctgacatgttaagagaatacattaaagagaaaatactgttttttaatcctaaaatttttcttccactaagataaaccaaatgtccttacatatatgtaaacccatctatttaaacgcaaaggtgggttgatgtcagtttacatagcagaaagcattcactatcctctaagatttgtttctgcaaaactttcattgctttagaattttaaaatttcaccttgtacaatggccagcccctaaagcaggaaacatttataatggattatatggaaacatcctcccagtacttgcccagcccttgaatcatgtggcttttcagtgaaaggaaagattctttttctaggaaaaatgagcctattttattttattttattttattttttgacacaaactgtagattttagcagccctggcccaaaggaatttgattacttttgttttaaacagtacaaaggggacactataattacaaaaacatccttaactgatttgagttgtttttatttctttggatatattttcagagtggtaaattgtgtgtgagaattacaaatgattattcttttagtggtttcttagcctctcttacagcccacggggatagtactgtacatcaataccttcatatgaaatttttatatgcaatgaaaataaaagcatgggttgattctgcctatttatgactcaatcttttacaaataaaagattattcattttaaattatagttcaatcagcatgtctcttaggatactgaacgtggttgaaatgaaaggatagtgacatcataagttagtactgatattcataaccaaataaagccaacttgagtaattttgctacattaaaaattaccaaaattacttagatggcctataagattaagcatggtgttttctaagcaagctttgaaaggggccttccatacttacttaattgaatattctgggatattgaaaattattcagatacttgacaattatttttggttacctactccgcaaactacaaagttttaaggactcaacaataagttaatgagacacagtgtttgctttcatggagcttacagtctggaggggacaaaggcttaaacaatactcatataattatatatgtgatcagtacaatgaaggagctcagtggggtaaataagcaggaacctgaacttgatctgttccggagggccacagaaggcttccttgaggccttgagaaagtgatttgcatctgagttctgaaggattgtaagaggtaactagggaaaaagttgacaggaagaggaaggggatccagacaagaaacatttgcaaagatcttgaggcataaatgagcttgagacatctggagaaactgaggaaaagtgagagagtaggcagggcctggagccgcagagccattgctaaccatcctgtgtgagatatcccccattctgtagctttattctcataaccctgctcaattttctttataacacttctcacagatttatatacgtgtttgtttttgttatctgtctctcccaccagaccacagctccatgagagcaaggtctttgcttaccaatatatcactagcacttaaaactatgcctggtacacagtaggttcttaatatgtgttgaatatagccatcaaattgatattggatataattcaatctgataagatattttgagatattaaagagtttttaacttgataccataaaaa

SEQ ID NO: 76 - protein, 699 aa, Homo sapiens
MSLPSSCEYLTLGKVARFRSAYVHGSPYAINMPIDIKPQRRRFDVDNGTSAGRSPLDPMTSPGSGLILQANFVHSQRRESFLYRSDSDYDLSPKSMSRNSSIASDIHGDDLIVTPFAQVLASLRTVRNNFAALTNLQDRAPSKRSPMCNQPSINKATITEEAYQKLASETLEELDWCLDQLETLQTRHSVSEMASNKFKRMLNRELTHLSEMSRSGNQVSEFISNTFLDKQHEVEIPSPTQKEKEKKKRPMSQISGVKKLMHSSSLTNSSIPRFGVKTEQEDVLAKELEDVNKWGLHVFRIAELSGNRPLTVIMHTIFQERDLLKTFKIPVDTLITYLMTLEDHYHADVAYHNNIHAADVVQSTHVLLSTPALEAVFTDLEILAAIFASAIHDVDHPGVSNQFLINTNSELALMYNDSSVLENHHLAVGFKLLQEENCDIFQNLTKKQRQSLRKMVIDIVLATDMSKHMNLLADLKTMVETKKVTSSGVLLLDNYSDRIQVLQNMVHCADLSNPTKPLQLYRQWTDRIMEEFFRQGDRERERGMEISPMCDKHNASVEKSQVGFIDYIVHPLWETWADLVHPDAQDILDTLEDNREWYQSTIPQSPSPAPDDPEEGRQGQTEKFQFELTLEEDGESDTEKDSGSQVEEDTSCSDSKTLCTQDSESTEIPLDEQVEEEAVGEEEESQPEACVIDDRSPDT

SEQ ID NO: 77 - DNA, 8085 bp, Homo sapiens
  source 1..8085: mol_type = other DNA
ctatagttggcgtaccctgaggcctgccagttcctgccttaatgcatatgtagtcgtaattgagttctgacacggccttggatgtttctgtcctaaatagctgacattgcatcttcaagactgtcattccagttggcttttgagtggatacgtgcagtgagatcattgacactggaaacactagttcccattttaattacttaaaacaccacgatgaaaagaaatacctgtgatttgctttctcggagcaaaagtgacttgagcatctgaagattttggtttctgcagagggtgggaaaggttgaaccaatcccccatggataccaaggcctctgaggaaacactacattccagtaatgaagaggaagaccctttccgcggaatggaaccctatcttgtccggagactttcatgtcgcaatattcagcttccccctctcgccttcagacagttggaacaagctgacttgaaaagtgaatcagagaacattcaacgaccaaccagcctccccctgaagattctgccgctgattgctatcacttctgcagaatccagtggttttgatgtggacaatggcacatctgcgggacggagtcccttggatcccatgaccagcccaggatccgggctaattctccaagcaaattttgtccacagtcaacgacgggagtccttcctgtatcgatccgacagcgattatgacctctctccaaagtctatgtcccggaactcctccattgccagtgatatacacggagatgacttgattgtgactccatttgctcagaagatcacccatgtgcaaccaaccatccatcaacaaagccaccataacagaggaggcctaccagaaactggccagcgagaccctggaggagctggactggtgtctggaccagctagagaccctacagaccaggcactccgtcagtgagatggcctccaacaagtttaaaaggatgcttaatcgggagctcacccatctctctgaaatgagtcggtctggaaatcaagtgtcagagtttatatcaaacacattcttagataagcaacatgaagtggaaattccttctccaactcagaaggaaaaggagaaaaagaaaagaccaatgtctcagatcagtggagtcaagaaattgatgcacagctctagtctgactaattcaagtatcccaaggtttggagttaaaactgaacaagaagatgtccttgccaaggaactagaagatgtgaacaaatggggtcttcatgttttcagaatagcagagttgtctggtaaccggcccttgactgttatcatgcacaccatttttcaggaacgggatttattaaaaacatttaaaattccagtagatactttaattacatatcttatgactctcgaagaccattaccatgctgatgtggcctatcacaacaatatccatgctgcagatgttgtccagtctactcatgtgctattatctacacctgctttggaggctgtgtttacagatttggagattcttgcagcaatttttgccagtgcaatacatgatgtagatcatcctggtgtgtccaatcaatttctgatcaatacaaactctgaacttgccttgatgtacaatgattcctcagtcttagagaaccatcatttggctgtgggctttaaattgcttcaggaagaaaactgtgacattttccagaatttgaccaaaaaacaaagacaatctttaaggaaaatggtcattgacatcgtacttgcaacagatatgtcaaaacacatgaatctactggctgatttgaagactatggttgaaactaagaaagtgacaagctctggagttcttcttcttgataattattccgataggattcaggttcttcagaatatggtgcactgtgcagatctgagcaacccaacaaagcctctccagctgtaccgccagtggacggaccggataatggaggagttcttccgccaaggagaccgagagagggaacgtggcatggagataagccccatgtgtgacaagcacaatgcttccgtggaaaaatcacaggtgggcttcatagactatattgttcatcccctctgggagacatgggcagacctcgtccaccctgacgcccaggatattttggacactttggaggacaatcgtgaatggtaccagagcacaatccctcagagcccctctcctgcacctgatgacccagaggagggccggcagggtcaaactgagaaattccagtttgaactaactttagaggaagatggtgagtcagacacggaaaaggacagtggcagtcaagtggaagaagacactagctgcagtgactccaagactctttgtactcaagactcagagtctactgaaattccccttgatgaacaggttgaagaggaggcagtaggggaagaagaggaaagccagcctgaagcctgtgtcatagatgatcgttctcctgacacgtaacagtgcaaaaactttcatgccttttttttttttaagtagaaaaattgtttccaaagtgcatgtcacatgccacaaccacggtcacacctcactgtcatctgccaggacgtttgttgaacaaaactgaccttgactactcagtccagcgctcaggaatatcgtaaccagttttttcacctccatgtcatccgagcaaggtggacatcttcacgaacagcgtttttaacaagatttcagcttggtagagctgacaaagcagataaaatctactccaaattattttcaagagagtgtgactcatcaggcagcccaaaagtttattggacttggggtttctattcctttttatttgtttgcaatattttcagaagaaaggcattgcacagagtgaacttaatggacgaagcaacaaatatgtcaagaacaggacatagcacgaatctgttaccagtaggaggaggatgagccacagaaattgcataattttctaatttcaagtcttcctgatacatgactgaatagtgtggttcagtgagctgcactgacctctacattttgtatgatatgtaaaacagattttttgtagagcttacttttattattaaatgtattgaggtattatatttaaaaaaaactatgttcagaacttcatctgccactggttatttttttctaaggagtaacttgcaagttttcagtacaaatctgtgctacactggataaaaatctaatttatgaattttacttgcaccttatagttcatagcaattaactgatttgtagtgattcattgtttgttttatataccaatgacttccatattttaaaagagaaaaacaactttatgttgcaggaaaccctttttgtaagtctttattatttactttgcattttgtttcactctttccagataagcagagttgctcttcaccagtgtttttcttcatgtgcaaagtgactatttgttctataatacttttatgtgtgttatatcaaatgtgtcttaagcttcatgcaaactcagtcatcagttcgtgttgtctgaagcaagtgggagatatataaatacccagtagctaaaatggtcagtcttttttagatgttttcctacttagtatctcctaataacgttttgctgtgtcactagatgttcatttcacaagtgcatgtctttctaataatccacacatttcatgctctaataatccacacatttcatgctcatttttattgtttttacagccagttatagtaagaaaaaggtttttccccttgtgctgctttataatttagcgtgtgtctgaaccttatccatgtttgctagatgaggtcttgtcaaatatatcactaccattgtcaccggtgaaaagaaacaggtagttaagttagggttaacattcatttcaaccacgaggttgtatatcatgactagcttttactcttggtttacagagaaaagttaaacagccaactaggcagtttttaagaatattaacaatatattaacaaacaccaatacaactaatcctatttggttttaatgatttcaccatgggattaagaactatatcaggaacatccctgagaaacggttttaagtgtagcaactactcttccttaatggacagccacataacgtgtaggaagtcctttatcacttatcctcgatccataagcatatcttgcagaggggaactacttctttaaacacatggagggaaagaagatgatgccactggcaccagagggttagtactgtgatgcatcctaaaatatttattatattggtaaaaattctggttaaataaaaaattagagatcactcttggctgatttcagcaccaggaactgtattacagttttagagattaattcctagtgtttacctgattatagcagttggcatcatggggcatttaattctgactttatccccacgtcagccttaataaagtcttctttaccttctctatgaagactttaaagcccaaataatcatttttcacattgatattcaagaattgagatagatagaagccaaagtgggtatctgacaagtggaaaatcaaacgtttaagaagaattacaactctgaaaagcatttatatgtggaacttctcaaggagcctcctggggactggaaagtaagtcatcagccaggcaaatgactcatgctgaagagagtccccatttcagtcccctgagatctagctgatgcttagatcctttgaaataaaaattatgtctttataactctgatcttttacataaagcagaagaggaatcaactagttaattgcaaggtttctactctgtttcctctgtaaagatcagatggtaatctttcaaataagaaaaaaataaagacgtatgtttgaccaagtagtttcacaagaatatttgggaacttgtttcttttaattttatttgtccctgagtgaagtctagaaagaaaggtaaagagtctagagtttattcctctttccaaaacattctcattcctctcctccctacacttagtatttcccccacagagtgcctagaatcttaataatgaataaaataaaaagcagcaatatgtcattaacaaatccagacctgaaagggtaaagggtttataactgcactaataaagagaggctctttttttttcttccagtttgttggtttttaatggtaccgtgttgtaaagatacccactaatggacaatcaaattgcagaaaaggctcaatatccaagagacagggactaatgcactgtacaatctgcttatccttgcccttctctcttgccaaagtgtgcttcagaaatatatactgctttaaaaaagaataaaagaatatccttttacaagtggctttacatttcctaaaatgccataagaaaatgcaatatctgggtactgtatggggaaaaaaatgtccaagtttgtgtaaaaccagtgcatttcagcttgcaagttactgaacacaataatgctgttttaattttgttttatatcagttaaaattcacaataatgtagatagaacaaattacagacaaggaaagaaaaaacttgaatgaaatggattttacagaaagctttatgataatttttgaatgcattatttattttttgtgccatgcattttttttctcaccaaatgaccttacctgtaatacagtcttgtttgtctgtttacaaccatgtatttattgcaatgtacatactgtaatgttaattgtaaattatctgttcttattaaaacatcatcccatgatgggatggtgttgatatatttggaaactcttggtgagagaatgaatggtgtgtatacatactctgtacatttttcttttctcctgtaatatagtcttgtcaccttagagcttgtttatggaagattcaagaaaactataaaatacttaaagatatataaatttaaaaaaacatagctgcaggtctttggtcccagggctgtgccttaactttaaccaatattttcttctgttttgctgcatttgaaaggtaacagtggagctagggctgggcattttacatccaggcttttaattgattagaattctgccaataggtggattttacaaaaccacagacaacctctgaaagattctgagacccttttgagacagaagctcttaagtacttcttgccagggagcagcactgcatgtgtgatggttgtttgccatctgttgatcaggaactacttcagctacttgcatttgattatttcctttttttttttttttaactcggaaacacaactggggaaatatattctttcccagtgattataaacaatctttttcttttttttaagtccttttggcttctagagctcataggaaaatggacttgatttgaaattggagccagagtttactcgtgttggttatctattcatcagcttcctgacatgttaagagaatacattaaagagaaaatactgttttttaatcctaaaatttttcttccactaagataaaccaaatgtccttacatatatgtaaacccatctatttaaacgcaaaggtgggttgatgtcagtttacatagcagaaagcattcactatcctctaagatttgtttctgcaaaactttcattgctttagaattttaaaatttcaccttgtacaatggccagcccctaaagcaggaaacatttataatggattatatggaaacatcctcccagtacttgcccagcccttgaatcatgtggcttttcagtgaaaggaaagattctttttctaggaaaaatgagcctattttattttattttattttattttttgacacaaactgtagattttagcagccctggcccaaaggaatttgattacttttgttttaaacagtacaaaggggacactataattacaaaaacatccttaactgatttgagttgtttttatttctttggatatattttcagagtggtaaattgtgtgtgagaattacaaatgattattcttttagtggtttcttagcctctcttacagcccacggggatagtactgtacatcaataccttcatatgaaatttttatatgcaatgaaaataaaagcatgggttgattctgcctatttatgactcaatcttttacaaataaaagattattcattttaaattatagttcaatcagcatgtctcttaggatactgaacgtggttgaaatgaaaggatagtgacatcataagttagtactgatattcataaccaaataaagccaacttgagtaattttgctacattaaaaattaccaaaattacttagatggcctataagattaagcatggtgttttctaagcaagctttgaaaggggccttccatacttacttaattgaatattctgggatattgaaaattattcagatacttgacaattatttttggttacctactccgcaaactacaaagttttaaggactcaacaataagttaatgagacacagtgtttgctttcatggagcttacagtctggaggggacaaaggcttaaacaatactcatataattatatatgtgatcagtacaatgaaggagctcagtggggtaaataagcaggaacctgaacttgatctgttccggagggccacagaaggcttccttgaggccttgagaaagtgatttgcatctgagttctgaaggattgtaagaggtaactagggaaaaagttgacaggaagaggaaggggatccagacaagaaacatttgcaaagatcttgaggcataaatgagcttgagacatctggagaaactgaggaaaagtgagagagtaggcagggcctggagccgcagagccattgctaaccatcctgtgtgagatatcccccattctgtagctttattctcataaccctgctcaattttctttataacacttctcacagatttatatacgtgtttgtttttgttatctgtctctcccaccagaccacagctccatgagagcaaggtctttgcttaccaatatatcactagcacttaaaactatgcctggtacacagtaggttcttaatatgtgttgaatatagccatcaaattgatattggatataattcaatctgataagatattttgagatattaaagagtttttaacttgataccataaaaa

SEQ ID NO: 78 - protein, 553 aa, Homo sapiens
MCNQPSINKATITEEAYQKLASETLEELDWCLDQLETLQTRHSVSEMASNKFKRMLNRELTHLSEMSRSGNQVSEFISNTFLDKQHEVEIPSPTQKEKEKKKRPMSQISGVKKLMHSSSLTNSSIPRFGVKTEQEDVLAKELEDVNKWGLHVFRIAELSGNRPLTVIMHTIFQERDLLKTFKIPVDTLITYLMTLEDHYHADVAYHNNIHAADVVQSTHVLLSTPALEAVFTDLEILAAIFASAIHDVDHPGVSNQFLINTNSELALMYNDSSVLENHHLAVGFKLLQEENCDIFQNLTKKQRQSLRKMVIDIVLATDMSKHMNLLADLKTMVETKKVTSSGVLLLDNYSDRIQVLQNMVHCADLSNPTKPLQLYRQWTDRIMEEFFRQGDRERERGMEISPMCDKHNASVEKSQVGFIDYIVHPLWETWADLVHPDAQDILDTLEDNREWYQSTIPQSPSPAPDDPEEGRQGQTEKFQFELTLEEDGESDTEKDSGSQVEEDTSCSDSKTLCTQDSESTEIPLDEQVEEEAVGEEEESQPEACVIDDRSPDT

SEQ ID NO: 79 - DNA, 8110 bp, Homo sapiens
  source 1..8110: mol_type = other DNA
acagtttccctctcggtttggaagaacaaagcttttgttatttatgttcttaaacaacagcgctttgtcctatactcaggagcgtgcaaagcaaacagaagatttcctgaacggccatcccatttatggtgaggagtcagtccaagagcattccagttggcttttgagtggatacgtgcagtgagatcattgacactggaaacactagttcccattttaattacttaaaacaccacgatgaaaagaaatacctgtgatttgctttctcggagcaaaagtgcctctgaggaaacactacattccagtaatgaagaggaagaccctttccgcggaatggaaccctatcttgtccggagactttcatgtcgcaatattcagcttccccctctcgccttcagacagttggaacaagctgacttgaaaagtgaatcagagaacattcaacgaccaaccagcctccccctgaagattctgccgctgattgctatcacttctgcagaatccagtggttttgatgtggacaatggcacatctgcgggacggagtcccttggatcccatgaccagcccaggatccgggctaattctccaagcaaattttgtccacagtcaacgacgggagtccttcctgtatcgatccgacagcgattatgacctctctccaaagtctatgtcccggaactcctccattgccagtgatatacacggagatgacttgattgtgactccatttgctcaggtcttggccagtctgcgaactgtacgaaacaactttgctgcattaactaatttgcaagatcgagcacctagcaaaagatcacccatgtgcaaccaaccatccatcaacaaagccaccataacagaggaggcctaccagaaactggccagcgagaccctggaggagctggactggtgtctggaccagctagagaccctacagaccaggcactccgtcagtgagatggcctccaacaagtttaaaaggatgcttaatcgggagctcacccatctctctgaaatgagtcggtctggaaatcaagtgtcagagtttatatcaaacacattcttagataagcaacatgaagtggaaattccttctccaactcagaaggaaaaggagaaaaagaaaagaccaatgtctcagatcagtggagtcaagaaattgatgcacagctctagtctgactaattcaagtatcccaaggtttggagttaaaactgaacaagaagatgtccttgccaaggaactagaagatgtgaacaaatggggtcttcatgttttcagaatagcagagttgtctggtaaccggcccttgactgttatcatgcacaccatttttcaggaacgggatttattaaaaacatttaaaattccagtagatactttaattacatatcttatgactctcgaagaccattaccatgctgatgtggcctatcacaacaatatccatgctgcagatgttgtccagtctactcatgtgctattatctacacctgctttggaggctgtgtttacagatttggagattcttgcagcaatttttgccagtgcaatacatgatgtagatcatcctggtgtgtccaatcaatttctgatcaatacaaactctgaacttgccttgatgtacaatgattcctcagtcttagagaaccatcatttggctgtgggctttaaattgcttcaggaagaaaactgtgacattttccagaatttgaccaaaaaacaaagacaatctttaaggaaaatggtcattgacatcgtacttgcaacagatatgtcaaaacacatgaatctactggctgatttgaagactatggttgaaactaagaaagtgacaagctctggagttcttcttcttgataattattccgataggattcaggttcttcagaatatggtgcactgtgcagatctgagcaacccaacaaagcctctccagctgtaccgccagtggacggaccggataatggaggagttcttccgccaaggagaccgagagagggaacgtggcatggagataagccccatgtgtgacaagcacaatgcttccgtggaaaaatcacaggtgggcttcatagactatattgttcatcccctctgggagacatgggcagacctcgtccaccctgacgcccaggatattttggacactttggaggacaatcgtgaatggtaccagagcacaatccctcagagcccctctcctgcacctgatgacccagaggagggccggcagggtcaaactgagaaattccagtttgaactaactttagaggaagatggtgagtcagacacggaaaaggacagtggcagtcaagtggaagaagacactagctgcagtgactccaagactctttgtactcaagactcagagtctactgaaattccccttgatgaacaggttgaagaggaggcagtaggggaagaagaggaaagccagcctgaagcctgtgtcatagatgatcgttctcctgacacgtaacagtgcaaaaactttcatgccttttttttttttaagtagaaaaattgtttccaaagtgcatgtcacatgccacaaccacggtcacacctcactgtcatctgccaggacgtttgttgaacaaaactgaccttgactactcagtccagcgctcaggaatatcgtaaccagttttttcacctccatgtcatccgagcaaggtggacatcttcacgaacagcgtttttaacaagatttcagcttggtagagctgacaaagcagataaaatctactccaaattattttcaagagagtgtgactcatcaggcagcccaaaagtttattggacttggggtttctattcctttttatttgtttgcaatattttcagaagaaaggcattgcacagagtgaacttaatggacgaagcaacaaatatgtcaagaacaggacatagcacgaatctgttaccagtaggaggaggatgagccacagaaattgcataattttctaatttcaagtcttcctgatacatgactgaatagtgtggttcagtgagctgcactgacctctacattttgtatgatatgtaaaacagattttttgtagagcttacttttattattaaatgtattgaggtattatatttaaaaaaaactatgttcagaacttcatctgccactggttatttttttctaaggagtaacttgcaagttttcagtacaaatctgtgctacactggataaaaatctaatttatgaattttacttgcaccttatagttcatagcaattaactgatttgtagtgattcattgtttgttttatataccaatgacttccatattttaaaagagaaaaacaactttatgttgcaggaaaccctttttgtaagtctttattatttactttgcattttgtttcactctttccagataagcagagttgctcttcaccagtgtttttcttcatgtgcaaagtgactatttgttctataatacttttatgtgtgttatatcaaatgtgtcttaagcttcatgcaaactcagtcatcagttcgtgttgtctgaagcaagtgggagatatataaatacccagtagctaaaatggtcagtcttttttagatgttttcctacttagtatctcctaataacgttttgctgtgtcactagatgttcatttcacaagtgcatgtctttctaataatccacacatttcatgctctaataatccacacatttcatgctcatttttattgtttttacagccagttatagtaagaaaaaggtttttccccttgtgctgctttataatttagcgtgtgtctgaaccttatccatgtttgctagatgaggtcttgtcaaatatatcactaccattgtcaccggtgaaaagaaacaggtagttaagttagggttaacattcatttcaaccacgaggttgtatatcatgactagcttttactcttggtttacagagaaaagttaaacagccaactaggcagtttttaagaatattaacaatatattaacaaacaccaatacaactaatcctatttggttttaatgatttcaccatgggattaagaactatatcaggaacatccctgagaaacggttttaagtgtagcaactactcttccttaatggacagccacataacgtgtaggaagtcctttatcacttatcctcgatccataagcatatcttgcagaggggaactacttctttaaacacatggagggaaagaagatgatgccactggcaccagagggttagtactgtgatgcatcctaaaatatttattatattggtaaaaattctggttaaataaaaaattagagatcactcttggctgatttcagcaccaggaactgtattacagttttagagattaattcctagtgtttacctgattatagcagttggcatcatggggcatttaattctgactttatccccacgtcagccttaataaagtcttctttaccttctctatgaagactttaaagcccaaataatcatttttcacattgatattcaagaattgagatagatagaagccaaagtgggtatctgacaagtggaaaatcaaacgtttaagaagaattacaactctgaaaagcatttatatgtggaacttctcaaggagcctcctggggactggaaagtaagtcatcagccaggcaaatgactcatgctgaagagagtccccatttcagtcccctgagatctagctgatgcttagatcctttgaaataaaaattatgtctttataactctgatcttttacataaagcagaagaggaatcaactagttaattgcaaggtttctactctgtttcctctgtaaagatcagatggtaatctttcaaataagaaaaaaataaagacgtatgtttgaccaagtagtttcacaagaatatttgggaacttgtttcttttaattttatttgtccctgagtgaagtctagaaagaaaggtaaagagtctagagtttattcctctttccaaaacattctcattcctctcctccctacacttagtatttcccccacagagtgcctagaatcttaataatgaataaaataaaaagcagcaatatgtcattaacaaatccagacctgaaagggtaaagggtttataactgcactaataaagagaggctctttttttttcttccagtttgttggtttttaatggtaccgtgttgtaaagatacccactaatggacaatcaaattgcagaaaaggctcaatatccaagagacagggactaatgcactgtacaatctgcttatccttgcccttctctcttgccaaagtgtgcttcagaaatatatactgctttaaaaaagaataaaagaatatccttttacaagtggctttacatttcctaaaatgccataagaaaatgcaatatctgggtactgtatggggaaaaaaatgtccaagtttgtgtaaaaccagtgcatttcagcttgcaagttactgaacacaataatgctgttttaattttgttttatatcagttaaaattcacaataatgtagatagaacaaattacagacaaggaaagaaaaaacttgaatgaaatggattttacagaaagctttatgataatttttgaatgcattatttattttttgtgccatgcattttttttctcaccaaatgaccttacctgtaatacagtcttgtttgtctgtttacaaccatgtatttattgcaatgtacatactgtaatgttaattgtaaattatctgttcttattaaaacatcatcccatgatgggatggtgttgatatatttggaaactcttggtgagagaatgaatggtgtgtatacatactctgtacatttttcttttctcctgtaatatagtcttgtcaccttagagcttgtttatggaagattcaagaaaactataaaatacttaaagatatataaatttaaaaaaacatagctgcaggtctttggtcccagggctgtgccttaactttaaccaatattttcttctgttttgctgcatttgaaaggtaacagtggagctagggctgggcattttacatccaggcttttaattgattagaattctgccaataggtggattttacaaaaccacagacaacctctgaaagattctgagacccttttgagacagaagctcttaagtacttcttgccagggagcagcactgcatgtgtgatggttgtttgccatctgttgatcaggaactacttcagctacttgcatttgattatttcctttttttttttttttaactcggaaacacaactggggaaatatattctttcccagtgattataaacaatctttttcttttttttaagtccttttggcttctagagctcataggaaaatggacttgatttgaaattggagccagagtttactcgtgttggttatctattcatcagcttcctgacatgttaagagaatacattaaagagaaaatactgttttttaatcctaaaatttttcttccactaagataaaccaaatgtccttacatatatgtaaacccatctatttaaacgcaaaggtgggttgatgtcagtttacatagcagaaagcattcactatcctctaagatttgtttctgcaaaactttcattgctttagaattttaaaatttcaccttgtacaatggccagcccctaaagcaggaaacatttataatggattatatggaaacatcctcccagtacttgcccagcccttgaatcatgtggcttttcagtgaaaggaaagattctttttctaggaaaaatgagcctattttattttattttattttattttttgacacaaactgtagattttagcagccctggcccaaaggaatttgattacttttgttttaaacagtacaaaggggacactataattacaaaaacatccttaactgatttgagttgtttttatttctttggatatattttcagagtggtaaattgtgtgtgagaattacaaatgattattcttttagtggtttcttagcctctcttacagcccacggggatagtactgtacatcaataccttcatatgaaatttttatatgcaatgaaaataaaagcatgggttgattctgcctatttatgactcaatcttttacaaataaaagattattcattttaaattatagttcaatcagcatgtctcttaggatactgaacgtggttgaaatgaaaggatagtgacatcataagttagtactgatattcataaccaaataaagccaacttgagtaattttgctacattaaaaattaccaaaattacttagatggcctataagattaagcatggtgttttctaagcaagctttgaaaggggccttccatacttacttaattgaatattctgggatattgaaaattattcagatacttgacaattatttttggttacctactccgcaaactacaaagttttaaggactcaacaataagttaatgagacacagtgtttgctttcatggagcttacagtctggaggggacaaaggcttaaacaatactcatataattatatatgtgatcagtacaatgaaggagctcagtggggtaaataagcaggaacctgaacttgatctgttccggagggccacagaaggcttccttgaggccttgagaaagtgatttgcatctgagttctgaaggattgtaagaggtaactagggaaaaagttgacaggaagaggaaggggatccagacaagaaacatttgcaaagatcttgaggcataaatgagcttgagacatctggagaaactgaggaaaagtgagagagtaggcagggcctggagccgcagagccattgctaaccatcctgtgtgagatatcccccattctgtagctttattctcataaccctgctcaattttctttataacacttctcacagatttatatacgtgtttgtttttgttatctgtctctcccaccagaccacagctccatgagagcaaggtctttgcttaccaatatatcactagcacttaaaactatgcctggtacacagtaggttcttaatatgtgttgaatatagccatcaaattgatattggatataattcaatctgataagatattttgagatattaaagagtttttaacttgataccataaaaa

SEQ ID NO: 80 - protein, 748 aa, Homo sapiens; identical to SEQ ID NO: 68

SEQ ID NO: 81 - DNA, 1487 bp, Homo sapiens
  source 1..1487: mol_type = other DNA
agtgattacaggttttagagaagaggaacaatgcttcctctgagcctgaagaaaagaatgaaataagggctgcaagggaacatgcaggtttcacactacaggagcttgtctgtcttggtgcaagtgggagcattccagttggcttttgagtggatacgtgcagtgagatcattgacactggaaacactagttcccattttaattacttaaaacaccacgatgaaaagaaatacctgtgatttgctttctcggagcaaaagtgcctctgaggaaacactacattccagtaatgaagaggaagaccctttccgcggaatggaaccctatcttgtccggagactttcatgtcgcaatattcagcttccccctctcgccttcagacagttggaacaagctgacttgaaaagtgaatcagagaacattcaacgaccaaccagcctccccctgaagattctgccgctgattgctatcacttctgcagaatccagtggttttgatgtggacaatggcacatctgcgggacggagtcccttggatcccatgaccagcccaggatccgggctaattctccaagcaaattttgtccacagtcaacgacgggagtccttcctgtatcgatccgacagcgattatgacctctctccaaagtctatgtcccggaactcctccattgccagtgatatacacggagatgacttgattgtgactccatttgctcaggtcttggccagtctgcgaactgtacgaaacaactttgctgcattaactaatttgcaagatcgagcacctagcaaaagatcacccatgtgcaaccaaccatccatcaacaaagccaccataacaggatcctggatggaattgaacccatatacgttacttgacatgtgaaacacgtgtgaccctggcagatgatttggctgaccttgaaaactacagctgtttagtcactttgaaaacaatgcaatacaagtgatttactaggcttcagttttaaccattttatgctgactggtggaaattctaacccttcagaaagaaaaaaaaattgtgaagcaatggaaatgtaccatcctgggtattaatgtcattaattttcaatacattttctcacaaaaagtataaagaagtctttgcttgaccttacgggaaaaaacaacatacatgtggctttattttgcctttttttttttttaattaatgaagaaatccaagatttgacttttgtttcttctctacccaaatcaaaagcagtctataatctcctgcaaagatcaaagctttttgcttactataaagtatgtgccctgcttaggcattacatggtagaaagatagcattctgttccaagaaatctctattcgttctctagttgctgtgtatatattctcttttagctagaatatggttagtaaatgagtcctgaaaatttcgctgtatataccaaaacatgttgtataccataaatatataaaatatttttatttcaa

SEQ ID NO: 82 - protein, 222 aa, Homo sapiens
MKRNTCDLLSRSKSASEETLHSSNEEEDPFRGMEPYLVRRLSCRNIQLPPLAFRQLEQADLKSESENIQRPTSLPLKILPLIAITSAESSGFDVDNGTSAGRSPLDPMTSPGSGLILQANFVHSQRRESFLYRSDSDYDLSPKSMSRNSSIASDIHGDDLIVTPFAQVLASLRTVRNNFAALTNLQDRAPSKRSPMCNQPSINKATITGSWMELNPYTLLDM

SEQ ID NO: 83 - DNA, 3388 bp, Homo sapiens
  source 1..3388: mol_type = other DNA
gcggcgcattagttccaatagtttaacaggctgctttgtagcacggacaaagccgtgcgagcgcggtgctttccctccttgttcatttgctatgcgagcttgtcagtgatctttggcaggggcttgggagaggaggggtgacgtttaatacgcttccgcggaggagtgcgctcgcctcctctgcacccagccccaggctctacagagagactgaggcaggcgactgaatgcactaacagcagcaggctcagacctgcttccctggacatttccgggaccgtgagcgagggaaccacgttgccctggattcttgccagctgtacaaagttgaccaggaaaatggctcagcagacaagcccggacactttaacagtacctgaagtggataatccgcattgtccaaacccgtggctgaacgaagaccttgtgaaatccttgcgagaaaacctgttgcagcatgagaagtccaagacagcgaggaaatcggtttctcccaagctctctccagtgatctctccgagaaattcccccaggcttctgcgcagaatgcttctcagcagcaacatccccaaacagcggcgtttcacggtggcacatacatgttttgatgtggacaatggcacatctgcgggacggagtcccttggatcccatgaccagcccaggatccgggctaattctccaagcaaattttgtccacagtcaacgacgggagtccttcctgtatcgatccgacagcgattatgacctctctccaaagtctatgtcccggaactcctccattgccagtgatatgtaagtacaagggcaggcaaagagagagaaaaccgagtaaatttatatctagagctgatgacataataaaactaatgacttttgttcaactgtatcactctcctccaatgtagaaagaatatgaataaaattatacaagctagaaatgaatggtagatttaacctgagtgcactgtcactcttgattaacacacacacacacacacacacacacacacacacacgcatgtatttattttcccagaaaatactttataggaaaactgagaattaaatttttaatggaaactaacacttaaatcattagcttatatttatgtagagcctgagttttagctacctaactacatggatattttctaatattttgaaaagctttcaactccattgaaaagtcctgtgataatagactgtatagcattttgaatatatttcaattaatgtatgtacagatgttagcactggtttgccagatcatttaagaaatctttgtgggactttgccaaaattaaaccaacttttaaggatcatgagaggcaagcacagaaaacattagacagacttgaatatcatttaagatatagtacagcttgaaaaacaatgaaaactgacaagcaggtttgcagatcctgtaccatcactagctcattttctcagtgcatttcattcttgtggtagtgtgcatgtttttctacataggtctttattctcactcaatacctatactatcattcgtggcacatctgcctctgtatagaatcgatcttcatctttctctcttggtctatacatttgtccaataacattcaccatcttttcatgacacccatctcaaaaactcataacaggctgcaatttatcttataagaattagtctgtatggaacccctgagtgtctagtgttattcttgccattctaacagagcatcagttgtattgcaataggtctacatggggttctagaaatgaaattatatttcactcatttttacaaactatggttgctattttagcagttgtattattgacgtctacccttcttcatctctaaacaactttctattcctagtggccctatttttacattatttttatctcacttccttagatttgaaattcatgacacttacttattcattcacacataatgagaatgcttcttgagcaaatatggtgtatttaaagctctgaatctgtggagcagtgaggtctggcattttagaccattgtaataaaatatggtgagcacaatccttgaggcatttatcatgtactgcaggaacagagagaggagatggagagttttccacccaagggaaagatacagaaaataccgggctaagggaacaacatttactaaatgtgaggcatggaaaattatggctgaactaaggaatgacaatctgcttgatgtgaatagcgaaacctggcaagagagaagaaaatttcaaatacagtctatgggacctgagagccacagaggtttttagctgagttttggcatgatcatattcttgtttttattgcatcttgattactctattgttgaatgattgcatagcgaagtcactacagggaagtatttcatgtcgaaattcacagaagtaaggcaggctaaatatgatgaagacctaagtcaagggagtgatggcagtggagcaaagagctggtttagatgcaagaggcttatagaatggttgtgtgtgtgtgtgtgtgtgtgtgtgtgtgtgtgtgtgtgtgtgtgaagtatgtatgtatgttgggggacagccagtggagaaggagaatcaaagagagtgctgatttttgtccatgaatgagtacgtacatggtgatgtacgtacatggtgatgaggaacaaagggcagagagtagaaaacatgacagataacaggtgatgaattggtttgtacatgataaggctaggggaaacaagacaacagttaaagtactgggacagcaaacagaaataacagtccagaggaccaggagaaatagaacagttaccttctataattactaggtttttgaatgacagttgagtggtgcgttgtattcaggtaatagcattaggagcccctgggttaaggagtgaattgaaagtggaaatgtgagcaaatgcaggcatctctttaaaaggctgatgggtggagtaggaagaaagaactaaggctgcctgacagagaattaggttcaagcggaatttttttgaattcaggttacttgagctgagggaaggctccaggagatagaaagagactaaaaattcaaggggaaagagggtttaaagatggagctgtagttgctgacaaaaacatgatcatgagccaaagtaaggaggctatccttggaaaagtagtaaataccagaactgtattctttaggaaggacaaagaagacctgccttggcaacatagtgagaccttgtccttactaaaaatccaaaaaaatagctgggcatggtggcacatgcctttagtcccagctactctggagaggtaggaggattggttgagcctgggagttcagggttgcagtgagctacgatcatgccactgcagtccagcctgggtgacagaggaagacaagactgt

SEQ ID NO: 84 - protein, 152 aa, Homo sapiens
MAQQTSPDTLTVPEVDNPHCPNPWLNEDLVKSLRENLLQHEKSKTARKSVSPKLSPVISPRNSPRLLRRMLLSSNIPKQRRFTVAHTCFDVDNGTSAGRSPLDPMTSPGSGLILQANFVHSQRRESFLYRSDSDYDLSPKSMSRNSSIASDM

SEQ ID NO: 85 - DNA, 1598 bp, Homo sapiens
  source 1..1598: mol_type = other DNA
gcggcgcattagttccaatagtttaacaggctgctttgtagcacggacaaagccgtgcgagcgcggtgctttccctccttgttcatttgctatgcgagcttgtcagtgatctttggcaggggcttgggagaggaggggtgacgtttaatacgcttccgcggaggagtgcgctcgcctcctctgcacccagccccaggctctacagagagactgaggcaggcgactgaatgcactaacagcagcaggctcagacctgcttccctggacatttccgggaccgtgagcgagggaaccacgttgccctggattcttgccagctgtacaaagttgaccaggaaaatggctcagcagacaagcccggacactttaacagtacctgaagtggataatccgcattgtccaaacccgtggctgaacgaagaccttgtgaaatccttgcgagaaaacctgttgcagcatgagaagtccaagacagcgaggaaatcggtttctcccaagctctctccagtgatctctccgagaaattcccccaggcttctgcgcagaatgcttctcagcagcaacatccccaaacagcggcgtttcacggtggcacatacatgttttgatgtggacaatggcacatctgcgggacggagtcccttggatcccatgaccagcccaggatccgggctaattctccaagcaaattttgtccacagtcaacgacgggagtccttcctgtatcgatccgacagcgattatgacctctctccaaagtctatgtcccggaactcctccattgccagtgatatacacggagatgacttgattgtgactccatttgctcaggtcttggccagtctgcgaactgtacgaaacaactttgctgcattaactaatttgcaagatcgagcacctagcaaaagatcacccatgtgcaaccaaccatccatcaacaaagccaccataacaggatcctggatggaattgaacccatatacgttacttgacatgtgaaacacgtgtgaccctggcagatgatttggctgaccttgaaaactacagctgtttagtcactttgaaaacaatgcaatacaagtgatttactaggcttcagttttaaccattttatgctgactggtggaaattctaacccttcagaaagaaaaaaaaattgtgaagcaatggaaatgtaccatcctgggtattaatgtcattaattttcaatacattttctcacaaaaagtataaagaagtctttgcttgaccttacgggaaaaaacaacatacatgtggctttattttgcctttttttttttttaattaatgaagaaatccaagatttgacttttgtttcttctctacccaaatcaaaagcagtctataatctcctgcaaagatcaaagctttttgcttactataaagtatgtgccctgcttaggcattacatggtagaaagatagcattctgttccaagaaatctctattcgttctctagttgctgtgtatatattctcttttagctagaatatggttagtaaatgagtcctgaaaatttcgctgtatataccaaaacatgttgtataccataaatatataaaatatttttatttcaa

SEQ ID NO: 86 - protein, 219 aa, Homo sapiens
MAQQTSPDTLTVPEVDNPHCPNPWLNEDLVKSLRENLLQHEKSKTARKSVSPKLSPVISPRNSPRLLRRMLLSSNIPKQRRFTVAHTCFDVDNGTSAGRSPLDPMTSPGSGLILQANFVHSQRRESFLYRSDSDYDLSPKSMSRNSSIASDIHGDDLIVTPFAQVLASLRTVRNNFAALTNLQDRAPSKRSPMCNQPSINKATITGSWMELNPYTLLDM

SEQ ID NO: 87 - DNA, 8247 bp, Homo sapiens
  source 1..8247: mol_type = other DNA
gcggcgcattagttccaatagtttaacaggctgctttgtagcacggacaaagccgtgcgagcgcggtgctttccctccttgttcatttgctatgcgagcttgtcagtgatctttggcaggggcttgggagaggaggggtgacgtttaatacgcttccgcggaggagtgcgctcgcctcctctgcacccagccccaggctctacagagagactgaggcaggcgactgaatgcactaacagcagcaggctcagacctgcttccctggacatttccgggaccgtgagcgagggaaccacgttgccctggattcttgccagctgtacaaagttgaccaggaaaatggctcagcagacaagcccggacactttaacagtacctgaagtggataatccgcattgtccaaacccgtggctgaacgaagaccttgtgaaatccttgcgagaaaacctgttgcagcatgagaagtccaagacagcgaggaaatcggtttctcccaagctctctccagtgatctctccgagaaattcccccaggcttctgcgcagaatgcttctcagcagcaacatccccaaacagcggcgtttcacggtggcacatacatgttttgatgtggacaatggcacatctgcgggacggagtcccttggatcccatgaccagcccaggatccgggctaattctccaagcaaattttgtccacagtcaacgacgggagtccttcctgtatcgatccgacagcgattatgacctctctccaaagtctatgtcccggaactcctccattgccagtgatatacacggagatgacttgattgtgactccatttgctcaggtcttggccagtctgcgaactgtacgaaacaactttgctgcattaactaatttgcaagatcgagcacctagcaaaagatcacccatgtgcaaccaaccatccatcaacaaagccaccataacagggctctataatgggatcattgcatttctctgattactaatgagaaggaggcctaccagaaactggccagcgagaccctggaggagctggactggtgtctggaccagctagagaccctacagaccaggcactccgtcagtgagatggcctccaacaagtttaaaaggatgcttaatcgggagctcacccatctctctgaaatgagtcggtctggaaatcaagtgtcagagtttatatcaaacacattcttagataagcaacatgaagtggaaattccttctccaactcagaaggaaaaggagaaaaagaaaagaccaatgtctcagatcagtggagtcaagaaattgatgcacagctctagtctgactaattcaagtatcccaaggtttggagttaaaactgaacaagaagatgtccttgccaaggaactagaagatgtgaacaaatggggtcttcatgttttcagaatagcagagttgtctggtaaccggcccttgactgttatcatgcacaccatttttcaggaacgggatttattaaaaacatttaaaattccagtagatactttaattacatatcttatgactctcgaagaccattaccatgctgatgtggcctatcacaacaatatccatgctgcagatgttgtccagtctactcatgtgctattatctacacctgctttggaggctgtgtttacagatttggagattcttgcagcaatttttgccagtgcaatacatgatgtagatcatcctggtgtgtccaatcaatttctgatcaatacaaactctgaacttgccttgatgtacaatgattcctcagtcttagagaaccatcatttggctgtgggctttaaattgcttcaggaagaaaactgtgacattttccagaatttgaccaaaaaacaaagacaatctttaaggaaaatggtcattgacatcgtacttgcaacagatatgtcaaaacacatgaatctactggctgatttgaagactatggttgaaactaagaaagtgacaagctctggagttcttcttcttgataattattccgataggattcaggttcttcagaatatggtgcactgtgcagatctgagcaacccaacaaagcctctccagctgtaccgccagtggacggaccggataatggaggagttcttccgccaaggagaccgagagagggaacgtggcatggagataagccccatgtgtgacaagcacaatgcttccgtggaaaaatcacaggtgggcttcatagactatattgttcatcccctctgggagacatgggcagacctcgtccaccctgacgcccaggatattttggacactttggaggacaatcgtgaatggtaccagagcacaatccctcagagcccctctcctgcacctgatgacccagaggagggccggcagggtcaaactgagaaattccagtttgaactaactttagaggaagatggtgagtcagacacggaaaaggacagtggcagtcaagtggaagaagacactagctgcagtgactccaagactctttgtactcaagactcagagtctactgaaattccccttgatgaacaggttgaagaggaggcagtaggggaagaagaggaaagccagcctgaagcctgtgtcatagatgatcgttctcctgacacgtaacagtgcaaaaactttcatgccttttttttttttaagtagaaaaattgtttccaaagtgcatgtcacatgccacaaccacggtcacacctcactgtcatctgccaggacgtttgttgaacaaaactgaccttgactactcagtccagcgctcaggaatatcgtaaccagttttttcacctccatgtcatccgagcaaggtggacatcttcacgaacagcgtttttaacaagatttcagcttggtagagctgacaaagcagataaaatctactccaaattattttcaagagagtgtgactcatcaggcagcccaaaagtttattggacttggggtttctattcctttttatttgtttgcaatattttcagaagaaaggcattgcacagagtgaacttaatggacgaagcaacaaatatgtcaagaacaggacatagcacgaatctgttaccagtaggaggaggatgagccacagaaattgcataattttctaatttcaagtcttcctgatacatgactgaatagtgtggttcagtgagctgcactgacctctacattttgtatgatatgtaaaacagattttttgtagagcttacttttattattaaatgtattgaggtattatatttaaaaaaaactatgttcagaacttcatctgccactggttatttttttctaaggagtaacttgcaagttttcagtacaaatctgtgctacactggataaaaatctaatttatgaattttacttgcaccttatagttcatagcaattaactgatttgtagtgattcattgtttgttttatataccaatgacttccatattttaaaagagaaaaacaactttatgttgcaggaaaccctttttgtaagtctttattatttactttgcattttgtttcactctttccagataagcagagttgctcttcaccagtgtttttcttcatgtgcaaagtgactatttgttctataatacttttatgtgtgttatatcaaatgtgtcttaagcttcatgcaaactcagtcatcagttcgtgttgtctgaagcaagtgggagatatataaatacccagtagctaaaatggtcagtcttttttagatgttttcctacttagtatctcctaataacgttttgctgtgtcactagatgttcatttcacaagtgcatgtctttctaataatccacacatttcatgctctaataatccacacatttcatgctcatttttattgtttttacagccagttatagtaagaaaaaggtttttccccttgtgctgctttataatttagcgtgtgtctgaaccttatccatgtttgctagatgaggtcttgtcaaatatatcactaccattgtcaccggtgaaaagaaacaggtagttaagttagggttaacattcatttcaaccacgaggttgtatatcatgactagcttttactcttggtttacagagaaaagttaaacagccaactaggcagtttttaagaatattaacaatatattaacaaacaccaatacaactaatcctatttggttttaatgatttcaccatgggattaagaactatatcaggaacatccctgagaaacggttttaagtgtagcaactactcttccttaatggacagccacataacgtgtaggaagtcctttatcacttatcctcgatccataagcatatcttgcagaggggaactacttctttaaacacatggagggaaagaagatgatgccactggcaccagagggttagtactgtgatgcatcctaaaatatttattatattggtaaaaattctggttaaataaaaaattagagatcactcttggctgatttcagcaccaggaactgtattacagttttagagattaattcctagtgtttacctgattatagcagttggcatcatggggcatttaattctgactttatccccacgtcagccttaataaagtcttctttaccttctctatgaagactttaaagcccaaataatcatttttcacattgatattcaagaattgagatagatagaagccaaagtgggtatctgacaagtggaaaatcaaacgtttaagaagaattacaactctgaaaagcatttatatgtggaacttctcaaggagcctcctggggactggaaagtaagtcatcagccaggcaaatgactcatgctgaagagagtccccatttcagtcccctgagatctagctgatgcttagatcctttgaaataaaaattatgtctttataactctgatcttttacataaagcagaagaggaatcaactagttaattgcaaggtttctactctgtttcctctgtaaagatcagatggtaatctttcaaataagaaaaaaataaagacgtatgtttgaccaagtagtttcacaagaatatttgggaacttgtttcttttaattttatttgtccctgagtgaagtctagaaagaaaggtaaagagtctagagtttattcctctttccaaaacattctcattcctctcctccctacacttagtatttcccccacagagtgcctagaatcttaataatgaataaaataaaaagcagcaatatgtcattaacaaatccagacctgaaagggtaaagggtttataactgcactaataaagagaggctctttttttttcttccagtttgttggtttttaatggtaccgtgttgtaaagatacccactaatggacaatcaaattgcagaaaaggctcaatatccaagagacagggactaatgcactgtacaatctgcttatccttgcccttctctcttgccaaagtgtgcttcagaaatatatactgctttaaaaaagaataaaagaatatccttttacaagtggctttacatttcctaaaatgccataagaaaatgcaatatctgggtactgtatggggaaaaaaatgtccaagtttgtgtaaaaccagtgcatttcagcttgcaagttactgaacacaataatgctgttttaattttgttttatatcagttaaaattcacaataatgtagatagaacaaattacagacaaggaaagaaaaaacttgaatgaaatggattttacagaaagctttatgataatttttgaatgcattatttattttttgtgccatgcattttttttctcaccaaatgaccttacctgtaatacagtcttgtttgtctgtttacaaccatgtatttattgcaatgtacatactgtaatgttaattgtaaattatctgttcttattaaaacatcatcccatgatgggatggtgttgatatatttggaaactcttggtgagagaatgaatggtgtgtatacatactctgtacatttttcttttctcctgtaatatagtcttgtcaccttagagcttgtttatggaagattcaagaaaactataaaatacttaaagatatataaatttaaaaaaacatagctgcaggtctttggtcccagggctgtgccttaactttaaccaatattttcttctgttttgctgcatttgaaaggtaacagtggagctagggctgggcattttacatccaggcttttaattgattagaattctgccaataggtggattttacaaaaccacagacaacctctgaaagattctgagacccttttgagacagaagctcttaagtacttcttgccagggagcagcactgcatgtgtgatggttgtttgccatctgttgatcaggaactacttcagctacttgcatttgattatttcctttttttttttttttaactcggaaacacaactggggaaatatattctttcccagtgattataaacaatctttttcttttttttaagtccttttggcttctagagctcataggaaaatggacttgatttgaaattggagccagagtttactcgtgttggttatctattcatcagcttcctgacatgttaagagaatacattaaagagaaaatactgttttttaatcctaaaatttttcttccactaagataaaccaaatgtccttacatatatgtaaacccatctatttaaacgcaaaggtgggttgatgtcagtttacatagcagaaagcattcactatcctctaagatttgtttctgcaaaactttcattgctttagaattttaaaatttcaccttgtacaatggccagcccctaaagcaggaaacatttataatggattatatggaaacatcctcccagtacttgcccagcccttgaatcatgtggcttttcagtgaaaggaaagattctttttctaggaaaaatgagcctattttattttattttattttattttttgacacaaactgtagattttagcagccctggcccaaaggaatttgattacttttgttttaaacagtacaaaggggacactataattacaaaaacatccttaactgatttgagttgtttttatttctttggatatattttcagagtggtaaattgtgtgtgagaattacaaatgattattcttttagtggtttcttagcctctcttacagcccacggggatagtactgtacatcaataccttcatatgaaatttttatatgcaatgaaaataaaagcatgggttgattctgcctatttatgactcaatcttttacaaataaaagattattcattttaaattatagttcaatcagcatgtctcttaggatactgaacgtggttgaaatgaaaggatagtgacatcataagttagtactgatattcataaccaaataaagccaacttgagtaattttgctacattaaaaattaccaaaattacttagatggcctataagattaagcatggtgttttctaagcaagctttgaaaggggccttccatacttacttaattgaatattctgggatattgaaaattattcagatacttgacaattatttttggttacctactccgcaaactacaaagttttaaggactcaacaataagttaatgagacacagtgtttgctttcatggagcttacagtctggaggggacaaaggcttaaacaatactcatataattatatatgtgatcagtacaatgaaggagctcagtggggtaaataagcaggaacctgaacttgatctgttccggagggccacagaaggcttccttgaggccttgagaaagtgatttgcatctgagttctgaaggattgtaagaggtaactagggaaaaagttgacaggaagaggaaggggatccagacaagaaacatttgcaaagatcttgaggcataaatgagcttgagacatctggagaaactgaggaaaagtgagagagtaggcagggcctggagccgcagagccattgctaaccatcctgtgtgagatatcccccattctgtagctttattctcataaccctgctcaattttctttataacacttctcacagatttatatacgtgtttgtttttgttatctgtctctcccaccagaccacagctccatgagagcaaggtctttgcttaccaatatatcactagcacttaaaactatgcctggtacacagtaggttcttaatatgtgttgaatatagccatcaaattgatattggatataattcaatctgataagatattttgagatattaaagagtttttaacttgataccataaaaa

SEQ ID NO: 88 - protein, 507 aa, Homo sapiens; identical to SEQ ID NO: 58

SEQ ID NO: 89 - DNA, 8824 bp, Homo sapiens
  source 1..8824: mol_type = other DNA
agagttaatgtacagtaccacggagcctgcaagtgtcctgagctgatcagagctggggcggcacagcccagggcagacaaggcggctgcgaggattccaaaggttctgctggaaattcggcgctgggggactccagcaggagcctgttgccattgtgttttaaaagcatgcaaggtctgtatagcttgggcatgagaatctttcagaagatgtcagagcatcagaataaatgacacctattggaaaactgaatttggggtgaaaaacaaaagagattgagagaggaaaaaaaagaaaagaaagacatcgggggaagaattcttagacaacgtctgacttgcagctgtgaaattcattttctttccaaggcaaaatatgaaaagctcccacatggttttgataataacaaaataaaggggattctgcagtgaaaagatcaatagcttagtcattttacttaaagagaacagccagccttattatggggttaggcagcagaaatgaatttcatcgtgacagcatcttctgaagtcatgatggtagttaatggtaatcttgtcctgcagagcagaaattactcattgccttcctacttttgcagttgaaccagcaattctgaaatctgggaaagaagttggctttggtgatacatggtttctagcccctctgcccaggcctttgtccgacacgtctcagacggtagcactgcgttaaagtgaccatacatgaatatgtgcctaagaaagaagaaaaagcaatattcatttctaaaggacagcatggcaaagcaacctgaagttttccatttcccttctaacacttctttaacaaggatatcaagaaactgtcttttgactcctttcttcccacattccagagtccttccttaaggatgcattaatttacactcaaggcggttagattttaccaggacaatatttgccaccatttaggattattagttgaactggttattttagtatgttgactaactagtggaacctaaatggatggacccatacctgcagtgctctgtgatgtttcttttttcaaatcctggaaggccttttgtaattgctatttgtttttattggtggggggagattttttttttttttttgggattcaatacttgttgcaataattgcccacgatagctgctcaaacaagagagttggaattcatctgtaaaaatcactacatgtaacgtaggagacaagaaaaatattaatgacagaagatctgcgaacatgatgcacgtgaataattttccctttagaaggcattcctggatatgttttgatgtggacaatggcacatctgcgggacggagtcccttggatcccatgaccagcccaggatccgggctaattctccaagcaaattttgtccacagtcaacgacgggagtccttcctgtatcgatccgacagcgattatgacctctctccaaagtctatgtcccggaactcctccattgccagtgatatacacggagatgacttgattgtgactccatttgctcagaagatcacccatgtgcaaccaaccatccatcaacaaagccaccataacagaggaggcctaccagaaactggccagcgagaccctggaggagctggactggtgtctggaccagctagagaccctacagaccaggcactccgtcagtgagatggcctccaacaagtttaaaaggatgcttaatcgggagctcacccatctctctgaaatgagtcggtctggaaatcaagtgtcagagtttatatcaaacacattcttagataagcaacatgaagtggaaattccttctccaactcagaaggaaaaggagaaaaagaaaagaccaatgtctcagatcagtggagtcaagaaattgatgcacagctctagtctgactaattcaagtatcccaaggtttggagttaaaactgaacaagaagatgtccttgccaaggaactagaagatgtgaacaaatggggtcttcatgttttcagaatagcagagttgtctggtaaccggcccttgactgttatcatgcacaccatttttcaggaacgggatttattaaaaacatttaaaattccagtagatactttaattacatatcttatgactctcgaagaccattaccatgctgatgtggcctatcacaacaatatccatgctgcagatgttgtccagtctactcatgtgctattatctacacctgctttggaggctgtgtttacagatttggagattcttgcagcaatttttgccagtgcaatacatgatgtagatcatcctggtgtgtccaatcaatttctgatcaatacaaactctgaacttgccttgatgtacaatgattcctcagtcttagagaaccatcatttggctgtgggctttaaattgcttcaggaagaaaactgtgacattttccagaatttgaccaaaaaacaaagacaatctttaaggaaaatggtcattgacatcgtacttgcaacagatatgtcaaaacacatgaatctactggctgatttgaagactatggttgaaactaagaaagtgacaagctctggagttcttcttcttgataattattccgataggattcaggttcttcagaatatggtgcactgtgcagatctgagcaacccaacaaagcctctccagctgtaccgccagtggacggaccggataatggaggagttcttccgccaaggagaccgagagagggaacgtggcatggagataagccccatgtgtgacaagcacaatgcttccgtggaaaaatcacaggtgggcttcatagactatattgttcatcccctctgggagacatgggcagacctcgtccaccctgacgcccaggatattttggacactttggaggacaatcgtgaatggtaccagagcacaatccctcagagcccctctcctgcacctgatgacccagaggagggccggcagggtcaaactgagaaattccagtttgaactaactttagaggaagatggtgagtcagacacggaaaaggacagtggcagtcaagtggaagaagacactagctgcagtgactccaagactctttgtactcaagactcagagtctactgaaattccccttgatgaacaggttgaagaggaggcagtaggggaagaagaggaaagccagcctgaagcctgtgtcatagatgatcgttctcctgacacgtaacagtgcaaaaactttcatgccttttttttttttaagtagaaaaattgtttccaaagtgcatgtcacatgccacaaccacggtcacacctcactgtcatctgccaggacgtttgttgaacaaaactgaccttgactactcagtccagcgctcaggaatatcgtaaccagttttttcacctccatgtcatccgagcaaggtggacatcttcacgaacagcgtttttaacaagatttcagcttggtagagctgacaaagcagataaaatctactccaaattattttcaagagagtgtgactcatcaggcagcccaaaagtttattggacttggggtttctattcctttttatttgtttgcaatattttcagaagaaaggcattgcacagagtgaacttaatggacgaagcaacaaatatgtcaagaacaggacatagcacgaatctgttaccagtaggaggaggatgagccacagaaattgcataattttctaatttcaagtcttcctgatacatgactgaatagtgtggttcagtgagctgcactgacctctacattttgtatgatatgtaaaacagattttttgtagagcttacttttattattaaatgtattgaggtattatatttaaaaaaaactatgttcagaacttcatctgccactggttatttttttctaaggagtaacttgcaagttttcagtacaaatctgtgctacactggataaaaatctaatttatgaattttacttgcaccttatagttcatagcaattaactgatttgtagtgattcattgtttgttttatataccaatgacttccatattttaaaagagaaaaacaactttatgttgcaggaaaccctttttgtaagtctttattatttactttgcattttgtttcactctttccagataagcagagttgctcttcaccagtgtttttcttcatgtgcaaagtgactatttgttctataatacttttatgtgtgttatatcaaatgtgtcttaagcttcatgcaaactcagtcatcagttcgtgttgtctgaagcaagtgggagatatataaatacccagtagctaaaatggtcagtcttttttagatgttttcctacttagtatctcctaataacgttttgctgtgtcactagatgttcatttcacaagtgcatgtctttctaataatccacacatttcatgctctaataatccacacatttcatgctcatttttattgtttttacagccagttatagtaagaaaaaggtttttccccttgtgctgctttataatttagcgtgtgtctgaaccttatccatgtttgctagatgaggtcttgtcaaatatatcactaccattgtcaccggtgaaaagaaacaggtagttaagttagggttaacattcatttcaaccacgaggttgtatatcatgactagcttttactcttggtttacagagaaaagttaaacagccaactaggcagtttttaagaatattaacaatatattaacaaacaccaatacaactaatcctatttggttttaatgatttcaccatgggattaagaactatatcaggaacatccctgagaaacggttttaagtgtagcaactactcttccttaatggacagccacataacgtgtaggaagtcctttatcacttatcctcgatccataagcatatcttgcagaggggaactacttctttaaacacatggagggaaagaagatgatgccactggcaccagagggttagtactgtgatgcatcctaaaatatttattatattggtaaaaattctggttaaataaaaaattagagatcactcttggctgatttcagcaccaggaactgtattacagttttagagattaattcctagtgtttacctgattatagcagttggcatcatggggcatttaattctgactttatccccacgtcagccttaataaagtcttctttaccttctctatgaagactttaaagcccaaataatcatttttcacattgatattcaagaattgagatagatagaagccaaagtgggtatctgacaagtggaaaatcaaacgtttaagaagaattacaactctgaaaagcatttatatgtggaacttctcaaggagcctcctggggactggaaagtaagtcatcagccaggcaaatgactcatgctgaagagagtccccatttcagtcccctgagatctagctgatgcttagatcctttgaaataaaaattatgtctttataactctgatcttttacataaagcagaagaggaatcaactagttaattgcaaggtttctactctgtttcctctgtaaagatcagatggtaatctttcaaataagaaaaaaataaagacgtatgtttgaccaagtagtttcacaagaatatttgggaacttgtttcttttaattttatttgtccctgagtgaagtctagaaagaaaggtaaagagtctagagtttattcctctttccaaaacattctcattcctctcctccctacacttagtatttcccccacagagtgcctagaatcttaataatgaataaaataaaaagcagcaatatgtcattaacaaatccagacctgaaagggtaaagggtttataactgcactaataaagagaggctctttttttttcttccagtttgttggtttttaatggtaccgtgttgtaaagatacccactaatggacaatcaaattgcagaaaaggctcaatatccaagagacagggactaatgcactgtacaatctgcttatccttgcccttctctcttgccaaagtgtgcttcagaaatatatactgctttaaaaaagaataaaagaatatccttttacaagtggctttacatttcctaaaatgccataagaaaatgcaatatctgggtactgtatggggaaaaaaatgtccaagtttgtgtaaaaccagtgcatttcagcttgcaagttactgaacacaataatgctgttttaattttgttttatatcagttaaaattcacaataatgtagatagaacaaattacagacaaggaaagaaaaaacttgaatgaaatggattttacagaaagctttatgataatttttgaatgcattatttattttttgtgccatgcattttttttctcaccaaatgaccttacctgtaatacagtcttgtttgtctgtttacaaccatgtatttattgcaatgtacatactgtaatgttaattgtaaattatctgttcttattaaaacatcatcccatgatgggatggtgttgatatatttggaaactcttggtgagagaatgaatggtgtgtatacatactctgtacatttttcttttctcctgtaatatagtcttgtcaccttagagcttgtttatggaagattcaagaaaactataaaatacttaaagatatataaatttaaaaaaacatagctgcaggtctttggtcccagggctgtgccttaactttaaccaatattttcttctgttttgctgcatttgaaaggtaacagtggagctagggctgggcattttacatccaggcttttaattgattagaattctgccaataggtggattttacaaaaccacagacaacctctgaaagattctgagacccttttgagacagaagctcttaagtacttcttgccagggagcagcactgcatgtgtgatggttgtttgccatctgttgatcaggaactacttcagctacttgcatttgattatttcctttttttttttttttaactcggaaacacaactggggaaatatattctttcccagtgattataaacaatctttttcttttttttaagtccttttggcttctagagctcataggaaaatggacttgatttgaaattggagccagagtttactcgtgttggttatctattcatcagcttcctgacatgttaagagaatacattaaagagaaaatactgttttttaatcctaaaatttttcttccactaagataaaccaaatgtccttacatatatgtaaacccatctatttaaacgcaaaggtgggttgatgtcagtttacatagcagaaagcattcactatcctctaagatttgtttctgcaaaactttcattgctttagaattttaaaatttcaccttgtacaatggccagcccctaaagcaggaaacatttataatggattatatggaaacatcctcccagtacttgcccagcccttgaatcatgtggcttttcagtgaaaggaaagattctttttctaggaaaaatgagcctattttattttattttattttattttttgacacaaactgtagattttagcagccctggcccaaaggaatttgattacttttgttttaaacagtacaaaggggacactataattacaaaaacatccttaactgatttgagttgtttttatttctttggatatattttcagagtggtaaattgtgtgtgagaattacaaatgattattcttttagtggtttcttagcctctcttacagcccacggggatagtactgtacatcaataccttcatatgaaatttttatatgcaatgaaaataaaagcatgggttgattctgcctatttatgactcaatcttttacaaataaaagattattcattttaaattatagttcaatcagcatgtctcttaggatactgaacgtggttgaaatgaaaggatagtgacatcataagttagtactgatattcataaccaaataaagccaacttgagtaattttgctacattaaaaattaccaaaattacttagatggcctataagattaagcatggtgttttctaagcaagctttgaaaggggccttccatacttacttaattgaatattctgggatattgaaaattattcagatacttgacaattatttttggttacctactccgcaaactacaaagttttaaggactcaacaataagttaatgagacacagtgtttgctttcatggagcttacagtctggaggggacaaaggcttaaacaatactcatataattatatatgtgatcagtacaatgaaggagctcagtggggtaaataagcaggaacctgaacttgatctgttccggagggccacagaaggcttccttgaggccttgagaaagtgatttgcatctgagttctgaaggattgtaagaggtaactagggaaaaagttgacaggaagaggaaggggatccagacaagaaacatttgcaaagatcttgaggcataaatgagcttgagacatctggagaaactgaggaaaagtgagagagtaggcagggcctggagccgcagagccattgctaaccatcctgtgtgagatatcccccattctgtagctttattctcataaccctgctcaattttctttataacacttctcacagatttatatacgtgtttgtttttgttatctgtctctcccaccagaccacagctccatgagagcaaggtctttgcttaccaatatatcactagcacttaaaactatgcctggtacacagtaggttcttaatatgtgttgaatatagccatcaaattgatattggatataattcaatctgataagatattttgagatattaaagagtttttaacttgataccataaaaa

SEQ ID NO: 90 - protein, 553 aa, Homo sapiens; identical to SEQ ID NO: 78

SEQ ID NO: 91 - DNA, 6959 bp, Homo sapiens
  source 1..6959: mol_type = other DNA
gtcgaaagccggcccgactggagcaggacgaagggggagggtctcgaggccgagtcctgttcttctgagggacggaccccagctggggtggaaaagcagtaccagagagcctccgaggcgcgcggtgccaaccatggagcgggccggccccagcttcgggcagcagcgacagcagcagcagccccagcagcagaagcagcagcagagggatcaggactcggtcgaagcatggctggacgatcactgggactttaccttctcatactttgttagaaaagccaccagagaaatggtcaatgcatggtttgctgagagagttcacaccatccctgtgtgcaaggaaggtatcagaggccacaccgaatcttgctcttgtcccttgcagcagagtcctcgtgcagataacagtgcccctggaacaccaaccaggaaaatctctgcctctgaatttgaccggcctcttagacccattgttgtcaaggattctgagggaactgtgagcttcctctctgactcagaaaagaaggaacagatgcctctaacccctccaaggtttgatcatgatgaaggggaccagtgctcaagactcttggaattagtgaaggatatttctagtcatttggatgtcacagccttatgtcacaaaattttcttgcatatccatggactgatatctgctgaccgctattccctgttccttgtctgtgaagacagctccaatgacaagtttcttatcagccgcctctttgatgttgctgaaggttcaacactggaagaagtttcaaataactgtatccgcttagaatggaacaaaggcattgtgggacatgtggcagcgcttggtgagcccttgaacatcaaagatgcatatgaggatcctcggttcaatgcagaagttgaccaaattacaggctacaagacacaaagcattctttgtatgccaattaagaatcatagggaagaggttgttggtgtagcccaggccatcaacaagaaatcaggaaacggtgggacatttactgaaaaagatgaaaaggactttgctgcttatttggcattttgtggtattgttcttcataatgctcagctctatgagacttcactgctggagaacaagagaaatcaggtgctgcttgaccttgctagtttaatttttgaagaacaacaatcattagaagtaattttgaagaaaatagctgccactattatctctttcatgcaagtgcagaaatgcaccattttcatagtggatgaagattgctccgattctttttctagtgtgtttcacatggagtgtgaggaattagaaaaatcatctgatacattaacaagggaacatgatgcaaacaaaatcaattacatgtatgctcagtatgtcaaaaatactatggaaccacttaatatcccagatgtcagtaaggataaaagatttccctggacaactgaaaatacaggaaatgtaaaccagcagtgcattagaagtttgctttgtacacctataaaaaatggaaagaagaataaagttataggggtttgccaacttgttaataagatggaggagaatactggcaaggttaagcctttcaaccgaaatgacgaacagtttctggaagcttttgtcatcttttgtggcttggggatccagaacacgcagatgtatgaagcagtggagagagccatggccaagcaaatggtcacattggaggttctgtcgtatcatgcttcagcagcagaggaagaaacaagagagctacagtcgttagcggctgctgtggtgccatctgcccagacccttaaaattactgactttagcttcagtgactttgagctgtctgatctggaaacagcactgtgtacaattcggatgtttactgacctcaaccttgtgcagaacttccagatgaaacatgaggttctttgcagatggattttaagtgttaagaagaattatcggaagaatgttgcctatcataattggagacatgcctttaatacagctcagtgcatgtttgctgctctaaaagcaggcaaaattcagaacaagctgactgacctggagatacttgcattgctgattgctgcactaagccacgatttggatcaccgtggtgtgaataactcttacatacagcgaagtgaacatccacttgcccagctttactgccattcaatcatggaacaccatcattttgaccagtgcctgatgattcttaatagtccaggcaatcagattctcagtggcctctccattgaagaatataagaccacgttgaaaataatcaagcaagctattttagctacagacctagcactgtacattaagaggcgaggagaattttttgaacttataagaaaaaatcaattcaatttggaagatcctcatcaaaaggagttgtttttggcaatgctgatgacagcttgtgatctttctgcaattacaaaaccctggcctattcaacaacggatagcagaacttgtagcaactgaattttttgatcaaggagacagagagagaaaagaactcaacatagaacccactgatctaatgaacagggagaagaaaaacaaaatcccaagtatgcaagttgggttcatagatgccatctgcttgcaactgtatgaggccctgacccacgtgtcagaggactgtttccctttgctagatggctgcagaaagaacaggcagaaatggcaggcccttgcagaacagcaggagaagatgctgattaatggggaaagcggccaggccaagcggaactgagtggcctatttcatgcagagttgaagtttacagagatggtgtgttctgcaatatgcctagtttcttacacactgtctgtatagtgtctgtatttggtatatactttgccactgctgtatttttatttttgcacaacttttgagagtatagcatgaatgtttttagaggactattacatattttttgtatatttgttttatgctactgaactgaaaggatcaacaacatccactgttagcacattgataaaagcattgtttgtgatatttcgtgtactgcaaagtgtatgcagtattcttgcactgaggtttttttgcttggggattattttaaataattggtttttgtgttttctgaattaccattttttcaagaatgtttggaatctttcctttttcaaaagtaggttaggagcaaattatcatacattctgtgacatttaaagcctttataggatagtgaaaaatgctggctgagtggattttaagagaaataattgtatttgttaacagtgtctttttttaaaaagttaaggcactctgaaacaaatggaaagtcctatgaaactgtattgtaaagaaaacattatttaattgatatgctgttttgtgagagaacaggcaagacagaactttgtcacttcagtgcagtacatttttctgaaagctacccataaaatcactttcatctcacctacctgatgcaaagcaggtgaaaccttaggagatgatccagtcactgacttgattgagggataagtgtgatttagaaatggaatggccttggatgtctatcagtgaagaaaaatgttctgttagaagatctctctaagagtttttttccttctgagcttccttttcaaaataaaagtgacaattgtagcattgacttgaagtgagacatggttatagataagagagtacaaaatgactctttttcctgtcaattgaaatttaaagaaaagttttaattatataaatagcaaagggctattgccaatactagggtcaaaaatgaatttgagggaacagtgggtaagaaactttatgcctgaataacatttagcagtattgtgattgaaaaattgccatattttgatgtataggacaagtcaactgagatccagagaatcctggatgtgaatgctaaacactggcccttaactcacattcaatgtattttcttcccataacatttagtatagttaatattttcttagaatttgagcccatttaagtggattaatattctacatgtgtgcccctaaagacacatttactcaatattggagaagtagataatgaattaagcaactggtctaggaaaggaaaatttgtttcaaatatgcaggaatgtttggatttggggagagtagaaggagagatttgcttgatttgttaacttctacctccaacccacaaaaaagatatttgatctgagtttctatcactaatttggatagaaaatttctaagggacatggtaatccagcattctcaaggacctttcgccaaaatgtgttttccatctatgtcccgattcccctaaattttgcctaaaattcagtatgttccttaagtttttaaaattctgagtgtgtacaaatatcttgacataatgcagttttatttttatcattctggtaaaaaaacaaaaaatagaagcaaaacacattgtattgccattattttgtatttggtaaaggttaatctaggaagttaccaactgtttaatgctatatgtattgtatacttgtattttcaggatattttattttttttgccatacagataaaatttgtaaggttgcccctttgtggcactggtgtgtaaaatacacagactatcactaaaataatagttatatatacatacaggtgtatacttatgcatgcatacataaatccttagtatagaaaaattgcataaagaatagcaatctttaataaacctttttattacattgtgatttagcagttatgctaaaatatgtacttatgctttagtagtttgtttggtcccctctagtatgtgtcactgagaaattttttaaagacatggtagatcgtgtttagaggctttgtatgtgtgtcattttaataagcaagaagatatatttagattagaaatggtttggtctgcctttgaatattgtttattttactttactagttgagacattaaaggaagctgggcaatgcctattttatttctttgttggatattttagttcatacaaagcagagtacttctttagggctggttaattggttcaaataatttttaatttcctttctagtatcttctcaagttggaaaaatatacatacagtcctccttcaccttactctgtatttatattacccataactagcaagaagttcttgttctagattttttgtttgtttagttataacagagtaacataccatttaattacaatttttagccagaaaagtccccactattttactaacttgttaaaagatatctatataattgcctggccttatatttttcagtagattagaccgtgccaatcacaatcctgggtggatttgtgtaagtcacttaacctctgtgtgcctaaacaagttgtgcttttttaaaaggagttatgtttgggcaaagcctttgtcttcaagcagaatgtcacagaaggcagctactttataagccccaatgggccatggagaccactgtcagaaatgggatattagtctagagagaaggtgatctattcccacatgtcatttctaatgttgagtttccatgactgaacaaagagaatatatttattcagcttcacttgcagatcactagtgaatgtgagatttagagctcattgagtatattgcttcaaggtacaaacccaggatgatgatgttgtcaccactgtctcttaattttgaataatagtttcctttaataggagtattagagataagaaagtatatgaaaatatactggaaatattggattcttggagaaaactgttcagtcacagatatattcttgcctagcagtgaagtgcctttattttcagcatagcaaataaatattagacctgttccaatttgatctacaatttttttctgtgtttttcaccagattgtactcctaaaacttaacaggccatcacaagcaattgtcttttgtttacaagattgatttaatatgagaggatacaaaatgtcatcgttatcctctcttatgaacaactgtagtcaaaataaggtggcacaatttaattgttttgtatcagaaatacactgacccaccttttattgagtcctgccacatgttaggtaccgtgctctgctgtggagacagagcagtgaccccaaggagctcacggtccctgaaggaggtgctagagaagagacttagcttctgatactgccaatttaatgtgagaacatggggtatactgcatcatttccattttcatcaataacatatgttttatgcaccttctttacctgaaacttactaagaatctaccagtaaacaaacatcctgtctttttgcaagtatgaatcacttaacctgctgatagttgaagaacactttaggagttttgtattcttgtatatagtttattttttccatgtgctagccaggtaaagattacacagttcttctggactgttaaattgtgcatggttttggaccccttctgctctactacagagagtgaagaagaaagtattaaagctcactttaccattccatatacttactaaaagcctgtgtaaacatgtcttaatgaatgttgttgaaagcaatgtaaatagttgaaaatataaatttatattacagtttaagaaaaccttatgaggcatcactagccactgttaatatctatttgtattcttataccttttcaatatatttgaacaaatatagtttctggcactatttttatactaggaaaaggagttactatgtatattatgcttagcttttaaggcattttaaataaccatgaatgttgatttcattactttcctttcctccatcacgagagtcatttcagatgactctttcatgacaaaatcactttaaaggaacacttacctccgattcctgtataaagtcatgagatggtcaaggtggttttccattgtgcaaattcttcacctgtcagtggtttcctcattttgccatgctttgtaaaaataaaaagaatgatcaagta

SEQ ID NO: 92 - protein, 875 aa, Homo sapiens
MERAGPSFGQQRQQQQPQQQKQQQRDQDSVEAWLDDHWDFTFSYFVRKATREMVNAWFAERVHTIPVCKEGIRGHTESCSCPLQQSPRADNSAPGTPTRKISASEFDRPLRPIVVKDSEGTVSFLSDSEKKEQMPLTPPRFDHDEGDQCSRLLELVKDISSHLDVTALCHKIFLHIHGLISADRYSLFLVCEDSSNDKFLISRLFDVAEGSTLEEVSNNCIRLEWNKGIVGHVAALGEPLNIKDAYEDPRFNAEVDQITGYKTQSILCMPIKNHREEVVGVAQAINKKSGNGGTFTEKDEKDFAAYLAFCGIVLHNAQLYETSLLENKRNQVLLDLASLIFEEQQSLEVILKKIAATIISFMQVQKCTIFIVDEDCSDSFSSVFHMECEELEKSSDTLTREHDANKINYMYAQYVKNTMEPLNIPDVSKDKRFPWTTENTGNVNQQCIRSLLCTPIKNGKKNKVIGVCQLVNKMEENTGKVKPFNRNDEQFLEAFVIFCGLGIQNTQMYEAVERAMAKQMVTLEVLSYHASAAEEETRELQSLAAAVVPSAQTLKITDFSFSDFELSDLETALCTIRMFTDLNLVQNFQMKHEVLCRWILSVKKNYRKNVAYHNWRHAFNTAQCMFAALKAGKIQNKLTDLEILALLIAALSHDLDHRGVNNSYIQRSEHPLAQLYCHSIMEHHHFDQCLMILNSPGNQILSGLSIEEYKTTLKIIKQAILATDLALYIKRRGEFFELIRKNQFNLEDPHQKELFLAMLMTACDLSAITKPWPIQQRIAELVATEFFDQGDRERKELNIEPTDLMNREKKNKIPSMQVGFIDAICLQLYEALTHVSEDCFPLLDGCRKNRQKWQALAEQQEKMLINGESGQAKRN

SEQ ID NO: 93 - DNA, 5645 bp, Homo sapiens
  source 1..5645: mol_type = other DNA
agtatgttttgcagacaagacccagagaagtccagactggacttgttgcagactgcaaaactgccattggaaggcctccgtcccagtccttctacagagtagccagtgggattcccagccatgggcgaggtgacagcagaggaggtggagaagttcctggactcgaatattggctttgccaaacagtactacaacctccactaccgggccaagctcatctccgacctccttggggccaaggaggctgccgtggacttcagcaactaccactccccgagcagcatggaggagagcgaaatcatctttgatctcctgcgggactttcaggagaatttacagacagagaaatgcatcttcaatgtcatgaagaagctgtgcttcctcctgcaggcagaccgcatgagcctgttcatgtaccggacccgcaatggcatcgcagagctggccaccaggcttttcaatgtccacaaggatgctgtcctcgaggactgcctggtgatgcccgaccaagagatcgtcttccctttggacatgggcatcgtgggccatgtcgcacactctaagaagattgctaacgtccccaacacagaggaggatgagcatttctgtgactttgtggacatcctcacagagtacaagaccaagaacatcttggcttcccccataatgaatgggaaggatgtggtggccataatcatggctgtgaataaagtggatggatcccacttcaccaagagagatgaagagattcttctcaagtacctcaattttgcaaatctaatcatgaaggtgtaccacctgagttacctgcacaactgtgaaactcgacgtggccagatactgctgtggtctgggagcaaagtctttgaagaacttacggacatcgaacgacagttccacaaagccctgtacacagtccgtgctttcctcaactgtgacagatactctgtgggtctcttagacatgaccaagcagaaggaattttttgatgtgtggccggttctgatgggtgaagttccaccttactctggtcccaggactccggatggaagagaaattaacttttacaaggtcattgactacatcctgcatggcaaagaggacatcaaagtcatcccgaatccacctcctgaccattgggctttagtaagcggtctcccagcttatgttgcccagaatggcctgatttgcaacatcatgaatgcgcctgcggaggacttttttgcatttcagaaagaacctctggatgagtctggatggatgattaaaaatgtgctttcaatgccgattgtgaacaagaaggaagaaattgttggagtggccacattttacaatcgtaaagatgggaagccctttgatgaaatggatgagacgctcatggagtctttgactcaatttctgggctggtctgtcttaaatcctgacacctatgagtcaatgaataaacttgaaaataggaaggatattttccaggacatagtaaaatatcatgtgaagtgtgacaatgaagaaattcagaaaatcttgaaaaccagagaggtgtatgggaaggagccatgggagtgtgaggaagaggagctggctgagatcctgcaagcggagctgccagatgcagataaatacgaaattaataaatttcacttcagtgacttacccctaacagaactggagctggtaaaatgtggaatacagatgtattatgagctcaaagtggtggataaatttcacattccacaagaggccctggtgcggttcatgtactccctgagtaagggctaccgcaagatcacctaccacaactggcggcacggcttcaacgtggggcagaccatgttctccctgctggtgacgggaaagctgaagcgctacttcacggacctagaggccttggccatggtcactgctgctttctgccatgacattgaccacagaggcaccaataacctctaccagatgaaatcccagaacccactggccaagctccatgggtcctctatcttggaaagacaccacttggagtttggcaaaacactgctcagagacgagagcctgaatatctttcaaaacctcaatcgtcgacagcatgagcatgccatccacatgatggacattgcaatcattgccacagacctcgccctgtatttcaagaagaggacgatgttccaaaagatcgtggatcagtctaagacatatgagagtgaacaggagtggacacagtacatgatgctggagcagacacggaaggaaatcgttatggccatgatgatgaccgcctgtgatctctcagccatcaccaaaccctgggaggtgcagagccaggtagctctgctggtggctgctgaattctgggaacaaggtgacctggagcgcacggtgctgcaacagaatcccattcccatgatggacagaaacaaagcagatgaactccctaagcttcaagtcggcttcattgactttgtttgcaccttcgtctacaaggaattctcccgtttccacgaggagatcaccccaatgttggacgggatcaccaacaatcgcaaggagtggaaggcgcttgctgatgagtacgatgccaagatgaaggtgcaggaggagaagaagcagaaacagcagtcggccaagtcagcagccgcaggaaatcagccggggggaaaccccagcccagggggtgcaactacatccaagtcctgctgcatccagtaacaccactggggatgtgctggctggacggcaccaccctttcctgggaagagatgactcaagccagtggaagaccacacaccttgagaagtagaagagtcataggatttgaaagctgttagagaatttagcttccaggactgttcaatcttttggcttccctgggccacattggaagaattgtcttgggtcacacataaaatacagtaacactaatgatagctgttgaacttaaaaaaaaaaatcgccaaaaaaaaaaatttcataatgttttaagaaagtttatgaatttgtgttgggccgcattcaaagccgtcctgggctgcatgtggcccacgggccgtgggttgaacaagcttggcttataccttatccagtggcttttaaacattcttttagtcttgagaactgcctattgagctaaaaccaatattctagctttcatagacatcagttaaacatttaattacatttaattaatgccagattcactggcttgcttagaatcatttttgttcttatactttcagttaatgtattgtaaaaattttcaatcattttcaaaagtagagaattgtacgttgaatccccacatacccatcacccagattccaatatcaagattttgctacatgcatttcgtctgtcctttttacattttcttttcaattttttttcttacctgaagtgtttaaaggcaaatcctggccaggcgtggtggctcacacctgtaatcccagcacttcaggaggctgaggtgggcagactgcatgagcccaggagtctgagaccaacctgagcaaaatggcaaaaccctgtctctacaaaaaatacaaaaattagcactcacctgtagtctcagctacctgggaggcagaggtgagaggatctcttgaacccaggaggcggaagttgcagtgagctgagatcatgctactgcactccagcttgggcgaccgagcgagactctgactcaaacaaaagcaaaagaaaaggcaaatcccaaacatatcatttcacacctctactatctcatctttaaagaaataagtatgttttctaacataaccacatcactggcccatgcaaccaatgcctgcctaatacccagctgtgatctatgctttgatgggctgcacagaccccaagcttcagcaaaggacttgggaccccaccagctttgagtgctgttgacagacccttagtatcaaccccatcaggtgttactgcagccttccccagggtggcctacacccaatgactgatccatgccaggtggagaggcctggccatcttggctgagcatgggataactgtgcagggctgttccagctccacgactcctcgtggggtccactaaggctgtcgctgggctcacatcccaactcgacttctccctctgcccactcctatttccttcccttccccaagcatcggtccccagggcactgcttaataagcatcctgcagactaagtccattttagagtctgctttctgggacacccaacttgtgatgccagcccttaatcaaccttccttcattctcatgaacgttttcaatggttggcttgcctgaatctgatccaaacaaattcacatattgaatttagttgtttctttttgttggtttttagaaaaaagaagatgtactttttattcttggatttttcattgatttcacagagtataaattaagtcagattattctcaattccagaacttctgtttcttaaattagcaggcattctgttggtttaaaaagatagatgttggccgggcgcggtggctcacgcctgtaattccagcactttgggaggccaaggtgggtggatcacctgaggtcaggagttcaagaccagcctggccaacatggtgaaaccccatctctactaaaaatacaaaaattagctgggtgtggtggtgtgcacctgtaatcccagctactcaggaggctgaggcaggagaatcgcttgaacctgggaggcgaaggttgcagtgagctgagatcatgccactgcactccagcctgggcaacaagagcaagactccgtctcaaaaaaaaaaaaaagaaaaaaaaaagatgtggcagatagaatttctctctttctctatctttcatgacgaggtctcactctgtcgcccaggctggagtgcagtggtatgaccatagctcactggagccccagctgcccgggctcaagcaatcctccatctcagcttaccaagcagcggtgaccacaggcatgcaccaccatgcccagctaattttttaaaacctatctttgtagacatggggtctcattctgttgcccaggctggcctcaaactcctgacttcaagcaatcctcctgcctcagcctcccaaagtgttgggattacaggcgtgagccactgcacctggccaggacttatttcttttaaaccgaatctaagtatgttctggcaagtatgcaatacctagcggaatgcactggcctgatcagcattcataccatagtaactgatgttgaaaacagcacaaataaaccagaagttgaaaatggcaataacatgctaaaaatttgcaagtcaatttgttacacttgtccaaatcttgattttttttccttctctatcgttccccccccaccaccagctttatggaggtataattagcaaataaaaagtatacatatttaaggtatacactgtgatgttttgatatacattgtgaaatggttaccataattaagctaattaatatatccatcacctcacatagccatggttaagtttctgaagtctcttttaatctacaaagtactccttccttttttccattgtcatcaccttgcagaaacagagtcagttttcccacattctgtatttatctgtttgtttctttgtggccgcatgtaacacattcctctgtctcattctaataaatggacattagctctagaa

SEQ ID NO: 94 - protein, 860 aa, Homo sapiens
MGEVTAEEVEKFLDSNIGFAKQYYNLHYRAKLISDLLGAKEAAVDFSNYHSPSSMEESEIIFDLLRDFQENLQTEKCIFNVMKKLCFLLQADRMSLFMYRTRNGIAELATRLFNVHKDAVLEDCLVMPDQEIVFPLDMGIVGHVAHSKKIANVPNTEEDEHFCDFVDILTEYKTKNILASPIMNGKDVVAIIMAVNKVDGSHFTKRDEEILLKYLNFANLIMKVYHLSYLHNCETRRGQILLWSGSKVFEELTDIERQFHKALYTVRAFLNCDRYSVGLLDMTKQKEFFDVWPVLMGEVPPYSGPRTPDGREINFYKVIDYILHGKEDIKVIPNPPPDHWALVSGLPAYVAQNGLICNIMNAPAEDFFAFQKEPLDESGWMIKNVLSMPIVNKKEEIVGVATFYNRKDGKPFDEMDETLMESLTQFLGWSVLNPDTYESMNKLENRKDIFQDIVKYHVKCDNEEIQKILKTREVYGKEPWECEEEELAEILQAELPDADKYEINKFHFSDLPLTELELVKCGIQMYYELKVVDKFHIPQEALVRFMYSLSKGYRKITYHNWRHGFNVGQTMFSLLVTGKLKRYFTDLEALAMVTAAFCHDIDHRGTNNLYQMKSQNPLAKLHGSSILERHHLEFGKTLLRDESLNIFQNLNRRQHEHAIHMMDIAIIATDLALYFKKRTMFQKIVDQSKTYESEQEWTQYMMLEQTRKEIVMAMMMTACDLSAITKPWEVQSQVALLVAAEFWEQGDLERTVLQQNPIPMMDRNKADELPKLQVGFIDFVCTFVYKEFSRFHEEITPMLDGITNNRKEWKALADEYDAKMKVQEEKKQKQQSAKSAAAGNQPGGNPSPGGATTSKSCCIQ

SEQ ID NO: 95 - DNA, 3294 bp, Homo sapiens
  source 1..3294: mol_type = other DNA
ctgggagtccatgcgtgcctggagcagcagcgtctccagggacaggcagccaccatgagcctcagtgaggagcaggcccggagctttctggaccagaaccccgattttgcccgccagtactttgggaagaaactgagccctgagaatgtggccgcggcctgcgaggacgggtgcccgccggactgcgacagcctccgggacctctgccaggtggaggagagcacggcgctgctggagctggtgcaggatatgcaggagagcatcaacatggagcgcgtggtcttcaaggtcctgcggcgcctctgcaccctcctgcaggccgaccgctgcagcctcttcatgtaccgccagcgcaacggcgtggccgagctggccaccaggcttttcagcgtgcagccggacagcgtcctggaggactgcctggtgccccccgactccgagatcgtcttcccactggacatcggggtcgtgggccacgtggctcagaccaaaaagatggtgaacgtcgaggacgtggccgagtgccctcacttcagctcatttgctgacgagctcactgactacaagacaaagaatatgctggccacacccatcatgaatggcaaagacgtcgtggcggtgatcatggcagtgaacaagctcaacggcccattcttcaccagcgaagacgaagatgtgttcttgaagtacctgaattttgccacgttgtacctgaagatctatcacctgagctacctccacaactgcgagacgcgccgcggccaggtgctgctgtggtcggccaacaaggtgtttgaggagctgacggacatcgagaggcagttccacaaggccttctacacggtgcgggcctacctcaactgcgagcggtactccgtgggcctcctggacatgaccaaggagaaggaattttttgacgtgtggtctgtgctgatgggagagtcccagccgtactcgggcccacgcacgcctgatggccgggaaattgtcttctacaaagtgatcgactacgtcctccacggcaaggaggagatcaaggtcattcccacaccctcagccgatcactgggccctggccagcggccttccaagctacgtggcagaaagcggctttatttgtaacatcatgaatgcttccgctgacgaaatgttcaaatttcaggaaggggccctggacgactccgggtggctcatcaagaatgtgctgtccatgcccatcgtcaacaagaaggaggagattgtgggagtcgccacattttacaacaggaaagacgggaagccctttgacgaacaggacgaggttctcatggagtccctgacacagttcctgggctggtcagtgatgaacaccgacacctacgacaagatgaacaagctggagaaccgcaaggacatcgcacaggacatggtcctttaccacgtgaagtgcgacagggacgagatccagctcatcctgccaaccagagcgcgcctggggaaggagcctgctgactgcgatgaggacgagctgggcgaaatcctgaaggaggagctgccagggcccaccacatttgacatctacgaattccacttctctgacctggagtgcaccgaactggacctggtcaaatgtggcatccagatgtactacgagctgggcgtggtccgaaagttccagatcccccaggaggtcctggtgcggttcctgttctccatcagcaaagggtaccggagaatcacctaccacaactggcgccacggcttcaacgtggcccagacgatgttcacgctgctcatgaccggcaaactgaagagctactacacggacctggaggccttcgccatggtgacagccggcctgtgccatgacatcgaccaccgcggcaccaacaacctgtaccagatgaagtcccagaaccccttggctaagctccacggctcctcgattttggagcggcaccacctggagtttgggaagttcctgctctcggaggagaccctgaacatctaccagaacctgaaccggcggcagcacgagcacgtgatccacctgatggacatcgccatcatcgccacggacctggccctgtacttcaagaagagagcgatgtttcagaagatcgtggatgagtccaagaactaccaggacaagaagagctgggtggagtacctgtccctggagacgacccggaaggagatcgtcatggccatgatgatgacagcctgcgacctgtctgccatcaccaagccctgggaagtccagagcaaggtcgcacttctcgtggctgctgagttctgggagcaaggtgacttggaaaggacagtcttggatcagcagcccattcctatgatggaccggaacaaggcggccgagctccccaagctgcaagtgggcttcatcgacttcgtgtgcacattcgtgtacaaggagttctctcgtttccacgaagagatcctgcccatgttcgaccgactgcagaacaataggaaagagtggaaggcgctggctgatgagtatgaggccaaagtgaaggctctggaggagaaggaggaggaggagagggtggcagccaagaaagtaggcacagaaatttgcaatggcggcccagcacccaagtcttcaacctgctgtatcctgtgagcactggtcccatggggaccctatggctccctcaatcttcacccactaggatttgggttctgcctgtggctatttgctacaagaggttaggaagcccaagaaaatgactgaagatcattctggatattttaatttttttttttttttttttttgagatggagtcttgctctgtcacccaggctggagtgccgtggcacgatctcagctcactgcaacctccacctcccaggttcaagcgattctcgtgcctcagcctcctgagtagctgggactacaggcgcccaccaccacacatggctaatttttgtattttcagtacagatggggtttcaccatattgggcaggctggtctcgaactcctgacctcaggtgatcacccgcctcagcttcctgaagtgctgggattacaggcatgagccaccacgcccagcctgtttttataaactgaagccaactgtgaataaactgtagcctacattactcatccatttttggatagttaccactgggagacctttgaaaagggtccatgaactctgaaatcactgagaacatttgcagccacacatgtacatatgtgtacacaggtagacagatggacacaggccgtttctcatccagtttaggaaaacacacatgctcaggaattcagaataaaataaacagaaaacta

SEQ ID NO: 96 - protein, 854 aa, Homo sapiens
MSLSEEQARSFLDQNPDFARQYFGKKLSPENVAAACEDGCPPDCDSLRDLCQVEESTALLELVQDMQESINMERVVFKVLRRLCTLLQADRCSLFMYRQRNGVAELATRLFSVQPDSVLEDCLVPPDSEIVFPLDIGVVGHVAQTKKMVNVEDVAECPHFSSFADELTDYKTKNMLATPIMNGKDVVAVIMAVNKLNGPFFTSEDEDVFLKYLNFATLYLKIYHLSYLHNCETRRGQVLLWSANKVFEELTDIERQFHKAFYTVRAYLNCERYSVGLLDMTKEKEFFDVWSVLMGESQPYSGPRTPDGREIVFYKVIDYVLHGKEEIKVIPTPSADHWALASGLPSYVAESGFICNIMNASADEMFKFQEGALDDSGWLIKNVLSMPIVNKKEEIVGVATFYNRKDGKPFDEQDEVLMESLTQFLGWSVMNTDTYDKMNKLENRKDIAQDMVLYHVKCDRDEIQLILPTRARLGKEPADCDEDELGEILKEELPGPTTFDIYEFHFSDLECTELDLVKCGIQMYYELGVVRKFQIPQEVLVRFLFSISKGYRRITYHNWRHGFNVAQTMFTLLMTGKLKSYYTDLEAFAMVTAGLCHDIDHRGTNNLYQMKSQNPLAKLHGSSILERHHLEFGKFLLSEETLNIYQNLNRRQHEHVIHLMDIAIIATDLALYFKKRAMFQKIVDESKNYQDKKSWVEYLSLETTRKEIVMAMMMTACDLSAITKPWEVQSKVALLVAAEFWEQGDLERTVLDQQPIPMMDRNKAAELPKLQVGFIDFVCTFVYKEFSRFHEEILPMFDRLQNNRKEWKALADEYEAKVKALEEKEEEERVAAKKVGTEICNGGPAPKSSTCCIL

SEQ ID NO: 97 - DNA, 3358 bp, Homo sapiens
  source 1..3358: mol_type = other DNA
gtcacatcccaagagttacaggcagtttgaaagctctgctttctgcttgacctttggaagtcctatgagggaccatttacggtttcctcagtaatttccaccaggatgaatttccttctcatcactctgcctcaggtagtgctctgaaggtcgtcctttctgaacaaacgcagcaaagcaagccacaccatgggtgagatcaaccaagttgccgtggagaaatacctggaggagaaccctcagtttgccaaggagtactttgacaggaagttgcgggtggaggtgctgggagaaatcttcaagaacagccaggtgccagtccagtccagcatgtccttctctgagctgacccaggtggaggagtcagccctgtgcttggagctgctgtggaccgtgcaggaggaggggggcaccccagagcagggggttcacagggccctgcagaggctggcccacctgctccaggctgaccgctgcagcatgttcctgtgccggtcccggaacggcatacctgaggtggcctctaggttgctggatgtcacccccacctccaagtttgaggacaacctggtgggccctgacaaagaagttgtgtttccattggacattgggatagtgggttgggctgctcacacgaagaaaactcataatgtcccagatgtgaaaaagaacagccatttttctgacttcatggacaagcaaactgggtatgtcactaagaacctgctggcaaccccgatcgtggtgggcaaggaggttcttgctgtgatcatggcagttaacaaagtaaatgcatctgaattttccaaacaggatgaagaggtcttttccaaatacctcaactttgtgtctatcatcctaaggcttcatcacaccagctacatgtacaatattgaatcccgaagaagccagatccttatgtggtcagccaataaagtatttgaagaactcacagatgttgagcgacagtttcacaaagcgctctacacggttagatcatatctgaactgtgaacgatactccattggactgctggacatgaccaaggagaaggaattctacgatgaatggccaatcaagcttggagaagtagagccttataaaggtccaaagacacctgatggcagggaagtcaacttttataaaatcattgattacattttacatggaaaagaagagatcaaagtgattccgacgcctcctgcagaccactggacactcattagtgggttgccaacatatgttgctgaaaatggatttatctgtaacatgatgaatgcccctgcggatgaatacttcacatttcagaaaggacctgtagacgaaactggttgggtcattaagaatgttttgtccctgcctattgtcaacaagaaagaagatattgtgggagtggctacattttacaacaggaaggatggaaaacctttcgatgagcatgatgaatacattaccgagactctcacacaatttcttggatggtctcttttaaatactgacacctacgataagatgaataagctagaaaacagaaaggacattgctcaggaaatgctcatgaaccaaaccaaagccactcctgaagaaattaagtccattttgaaatttcaagagaagttaaatgttgatgtaattgacgactgtgaagaaaaacaacttgttgcaattttgaaagaggacttgccagacccacgctcagcagaactgtacgaattccgcttcagtgacttcccccttacagagcacggattgattaaatgtggaatacgactgttttttgaaataaatgtggtggagaaattcaaagtacctgtagaggttcttaccagatggatgtacactgtgaggaaagggtaccgagctgtcacttaccacaattggcggcatgggttcaacgtggggcagaccatgtttactttgctgatgacaggaagattaaagaagtactacacagatctcgaagcctttgccatgcttgctgctgctttctgccatgatattgaccacagaggcaccaataatttgtaccagatgaaatccacgtctccattagcaagacttcatggttcttctattttggagaggcaccacctggagtacagtaagactctgttgcaggatgagagtttaaacatcttccagaacctaaataagcggcagtttgaaacagttattcatttgttcgaggtcgcaataatagcaactgacctggctttatatttcaagaagaggaccatgtttcaaaaaattgttgatgcctgtgaacaaatgcaaacggaagaagaagccatcaaatatgtaactgttgatccaaccaagaaagagattatcatggcaatgatgatgacggcatgtgacttgtctgctattaccaagccctgggaggtgcaaagtcaggtagcacttatggttgcaaatgaattttgggaacaaggagatctggagagaacagtgttgcagcaacaacccattcctatgatggacagaaacaaaagagatgaattacctaaacttcaagttggatttattgattttgtttgtacttttgtatataaggagttctcacggtttcacaaagaaatcacacctatgctgagtggtcttcagaataacagagtagaatggaaatcactagctgatgagtatgatgcaaagatgaaggtcattgaagaggaggcaaaaaagcaagaaggaggagccgaaaaagctgctgaagattcaggaggtggtgatgacaaaaagtccaaaacatgtttaatgttgtaatattatctaactggtctaaacttcaaatatcattttacctttgaagaaaaccagaaaacattcaaaagaacttcaacaaatcatcacgtaacaggatcttcagaaaaactaccctgtgactatgaagaaaatatatattgctagcccaaaaatcccaggggcaaaataaagttcaacaaaagtgcaaaatatgacaaaaataggtacatttttggtgccaatttattttaaattaaaaaatatgcaatcctgaaactagtcacaaattcttttttaaaacattaattgtatttatttgctaaggctgctataacaaagtaccacagactgggtgcttaaccaatagaaatgtattttctcaaagtcctgggggctggaagttcaagatcaaggagttggcagggttggtttcttgggaggcctctcaacttggtttgcagatggccatcttctccctgtgtcttcacatggtcttccctctgtgtgtctgtgtcctaatctccttttcttataaggactccagtaggactggattagggcctacccatgtgacctcattttagtcttaattacctcgttaatggccttatct

SEQ ID NO: 98 - protein, 858 aa, Homo sapiens
MGEINQVAVEKYLEENPQFAKEYFDRKLRVEVLGEIFKNSQVPVQSSMSFSELTQVEESALCLELLWTVQEEGGTPEQGVHRALQRLAHLLQADRCSMFLCRSRNGIPEVASRLLDVTPTSKFEDNLVGPDKEVVFPLDIGIVGWAAHTKKTHNVPDVKKNSHFSDFMDKQTGYVTKNLLATPIVVGKEVLAVIMAVNKVNASEFSKQDEEVFSKYLNFVSIILRLHHTSYMYNIESRRSQILMWSANKVFEELTDVERQFHKALYTVRSYLNCERYSIGLLDMTKEKEFYDEWPIKLGEVEPYKGPKTPDGREVNFYKIIDYILHGKEEIKVIPTPPADHWTLISGLPTYVAENGFICNMMNAPADEYFTFQKGPVDETGWVIKNVLSLPIVNKKEDIVGVATFYNRKDGKPFDEHDEYITETLTQFLGWSLLNTDTYDKMNKLENRKDIAQEMLMNQTKATPEEIKSILKFQEKLNVDVIDDCEEKQLVAILKEDLPDPRSAELYEFRFSDFPLTEHGLIKCGIRLFFEINVVEKFKVPVEVLTRWMYTVRKGYRAVTYHNWRHGFNVGQTMFTLLMTGRLKKYYTDLEAFAMLAAAFCHDIDHRGTNNLYQMKSTSPLARLHGSSILERHHLEYSKTLLQDESLNIFQNLNKRQFETVIHLFEVAIIATDLALYFKKRTMFQKIVDACEQMQTEEEAIKYVTVDPTKKEIIMAMMMTACDLSAITKPWEVQSQVALMVANEFWEQGDLERTVLQQQPIPMMDRNKRDELPKLQVGFIDFVCTFVYKEFSRFHKEITPMLSGLQNNRVEWKSLADEYDAKMKVIEEEAKKQEGGAEKAAEDSGGGDDKKSKTCLML

SEQ ID NO: 99 - DNA, 1140 bp, Homo sapiens
  source 1..1140: mol_type = other DNA
atcagaagcgggagctgaggggagagagaggccggtcctggtctggccgctgcggctgctagcccgaggtctccaagccgggctgcggctccatcctcggctcctgggcaccgtctgcgaggctccgccgaccagagtgagaaagccgcgggcggcgaccgccgcatcatgtcagccaaggacgagcgggccagggagatcctgaggggcttcaaactaaattggatgaaccttcgggatgctgagacagggaagatactctggcaaggaacagaagacctgtctgtccctggtgtggagcatgaagcccgtgttcccaagaaaatcctcaagtgcaaggcagtgtctcgagaacttaatttttcttcgacagaacaaatggaaaaattccgcctggaacaaaaagtttacttcaaagggcaatgcctagaagaatggttcttcgagtttggctttgtgatccctaactccacaaatacctggcagtccttgatagaggcagcacccgagtcccagatgatgccagcaagcgtcttaactgggaacgttatcatagaaacaaagttttttgacgacgatcttcttgtaagcacatccagagtgagacttttctatgtttgaaagaagaatgtgtgtacatttcaagaatttgggttttttggagggaggaggaaactgtttacttttttcctccacacgtttgatttttgacacatacacccctaattccctcaacagcagaacctacctgcagccaccaggggaccagctctgtgtaggtaaccagatggctctttttcccaagccaccatcttccagctgaccagactaaactcccaaccccagaccagggcaggggacaggtctcaagtccttcccagcatacacacagggaacaaacacataccacaaaccggtaactgtacctgtcaccctccttgtctcctccttgggccctacaggctacacatctacctttggcccctggttttggaaaaattccgtgttcctgacccatgtttagttttttcctaccatttctatttcatacattctcatacatttaacttgtaaaatagactgtgatattattacataatgtaattaaaaatatgaattaaaatattcctacagtcttta

SEQ ID NO: 100 - protein, 150 aa, Homo sapiens
MSAKDERAREILRGFKLNWMNLRDAETGKILWQGTEDLSVPGVEHEARVPKKILKCKAVSRELNFSSTEQMEKFRLEQKVYFKGQCLEEWFFEFGFVIPNSTNTWQSLIEAAPESQMMPASVLTGNVIIETKFFDDDLLVSTSRVRLFYV

SEQ ID NO: 101 - DNA, 988 bp, Homo sapiens
  source 1..988: mol_type = other DNA
gggaggcccagcactcacagcacagccccctgagacccgccctgcacttgaccgcagcaggagggagtccaggagccaaggttgccgcggtgtctccgtcagcctcaccatgaacctggaaccgcccaaggctgagttccggtcagccaccagggtggccgggggacctgtcacccccaggaaagggccccctaaatttaagcagcgacagaccaggcagttcaagagcaagcccccaaagaaaggcgttcaagggtttggggacgacatccctggaatggaaggcctgggaacagacatcacagtcatctgcccttgggaggccttcaaccacctggagctgcacgagctggcccaatatggcatcatctagcacgaggccctgctgaagtccagaccctccccctcctgcccactgtgctctaaaccctgctcaggattcctgttgaggagatgcctccctagcccagatggcacctggacaccaggatgggactgcaacctcaggtctccccctacatattaataccagtcaccaggagcccaccacctccctctaggatgccccctcaggggctggccaggccctgctcaacatctggagatacaggcccacccctcagtcctgcccacagagaggcttggtcggtctccactcccagggagaacgggaagtggaccccagcccgggagcctgctggaccccagatcgtcccctcctcccagctggaaagctagggcaggtctccccagagtgcttctgcaccccagccccctgtcctgcctgtaaggggatacagagaagctccccgtctctgcatcccttcccaggggggtgcccttagtttggacatgctgggtagcaggactccagggcgtgcacggtgagcagatgaggccccaagctcatcacaccagggggccatccttctcaatacagcctgcccttgcagtccctatttcaaaataaaattagtgtgtccttgcc

SEQ ID NO: 102 - protein, 87 aa, Homo sapiens
MNLEPPKAEFRSATRVAGGPVTPRKGPPKFKQRQTRQFKSKPPKKGVQGFGDDIPGMEGLGTDITVICPWEAFNHLELHELAQYGII

SEQ ID NO: 103 - DNA, 727 bp, Homo sapiens
  source 1..727: mol_type = other DNA
gcaaagaaggcagctgggcagctgataggaacaacattcagctccgaggctgaaagggaaacatcagccgcccggggggagttaaaatgagtgacaacactactctgcctgctccagcttcaaaccagggtcctaccaccccacgcaaaggccctcccaagttcaagcagaggcagactcgccaattcaagagtaaacctccaaagaaaggtgtgaaaggatttggagatgacattccaggaatggaggggctaggaacagatatcacagtgatttgtccatgggaggcattcagccacctggaattgcatgagctcgctcagtttgggattatctgaagtgccagaggttctgccactctcaatgacatctgctgtaattttggttgcttttgccctgttgatctgccggagtcttgaaattcagctgattggaagtggtttctttgactttcaaggtcattccctatcagttactactaagagttctcttactgtcagaatctctcttgcagtacagctcaaaatagtggatgcatttcaaacttgaccaccttttcctaccagctagttagaagtcatcaatatttctctacattttgtttatctgtaagtcctttaaatctatttttgctaggcattcattatgattaatagtagacttttaagacaacatttatgtcactccccacctcctcatatttaataaaggagatatttaccttgaa

SEQ ID NO: 104 - protein, 83 aa, Homo sapiens
MSDNTTLPAPASNQGPTTPRKGPPKFKQRQTRQFKSKPPKKGVKGFGDDIPGMEGLGTDITVICPWEAFSHLELHELAQFGII

SEQ ID NO: 105 - DNA, 6443 bp, Homo sapiens
  source 1..6443: mol_type = other DNA
agtcagtgtcccctctcttttgcctcgggacagctggtatttatcagactcctaagaagttttccttgctccctagtagaagagagagattatgcagcgggcttttgattgatccaatgggaattacattgatctggtgtctggccttggttcttatcaagtggatcacctctaagaggcgtggagctatttcctatgacagttctgatcagactgcattatacattcgtatgctaggagatgtacgtgtaaggagccgagcaggatttgaatcagaaagaagaggttctcacccatatattgattttcgtattttccactctcaatctgaaattgaagtgtctgtctctgcaaggaatatcagaaggctactaagtttccagcgatatcttagatcttcacgcttttttcgtggtactgcggtttcaaattccctaaacattttagatgatgattataatggacaagccaagtgtatgctggaaaaagttggaaattggaattttgatatctttctatttgatagactaacaaatggaaatagtctagtaagcttaacctttcatttatttagtcttcatggattaattgagtacttccatttagatatgatgaaacttcgtagatttttagttatgattcaagaagattaccacagtcaaaatccttaccataacgcagtccacgctgcggatgttactcaggccatgcactgttacttaaaggaacctaagcttgccaattctgtaactccttgggatatcttgctgagcttaattgcagctgccactcatgatctggatcatccaggtgttaatcaacctttccttattaaaactaaccattacttggcaactttatacaagaatacctcagtactggaaaatcaccactggagatctgcagtgggcttattgagagaatcaggcttattctcacatctgccattagaaagcaggcaacaaatggagacacagataggtgctctgatactagccacagacatcagtcgccagaatgagtatctgtctttgtttaggtcccatttggatagaggtgatttatgcctagaagacaccagacacagacatttggttttacagatggctttgaaatgtgctgatatttgtaacccatgtcggacgtgggaattaagcaagcagtggagtgaaaaagtaacggaggaattcttccatcaaggagatatagaaaaaaaatatcatttgggtgtgagtccactttgcgatcgtcacactgaatctattgccaacatccagattggttttatgacttacctagtggagcctttatttacagaatgggccaggttttccaatacaaggctatcccagacaatgcttggacacgtggggctgaataaagccagctggaagggactgcagagagaacagtcgagcagtgaggacactgatgctgcatttgagttgaactcacagttattacctcaggaaaatcggttatcataacccccagaaccagtgggacaaactgcctcctggaggtttttagaaatgtgaaatggggtcttgaggtgagagaacttaactcttgactgccaaggtttccaagtgagtgatgccagccagcattatttatttccaagatttcctctgttggatcatttgaacccacttgttaattgcaagacccgaacatacagcaatatgaatttggctttcatgtgaaaccttgaatatgcaaagcccagcaggagagaatccgaaaggagtaacaaaggaagttttgatatgtgccacgactttttcaaagcatctaatcttcaaaacgtgaaacttgaattgttcagcaacaatctcttggaatttaaccagtctgatgcaacaatgtgtatcttgtaccttccactaagttctctctgagaaaatggaaatgtgaagtgcccagcctctgctgcctctggcaagacaatgtttacaaatcaactctgaaaatattggttctaaattgccttggagcatgattgtgaaggaaccactcaaacaaatttaaagatcaaactttagactgcagctctttccccctggtttgcctttttcttctttggatgccaccaaagcctcccatttgctatagttttatttcatgcactggaaactgagcatttatcgtagagtaccgccaagctttcactccagtgccgtttggcaatgcaattttttttagcaattagtttttaatttggggtgggaggggaagaacaccaatgtcctagctgtattatgattctgcagtgaagacattgcatgttgttttcactactgtacacttgacctgcacatgcgagaaaaaggtggaatgtttaaaacaccataatcagctcagggtatttgccaatctgaaataaaagtgggatgggagagtgtgtccttcagatcaagggtactaaagtccctttcgctgcagtgagtgagaggtatgttgtgtgtgaatgtacggatgtgtgtttgcgtgcatgtttgtgcatgtgtgactgtgcatgttatgtttctccatgtgggcaaagatttgaaatgtaagcttttatttattattttagaatgtgacataatgagcagccacactcgggggaggggaaggttggtaggtaagctgtaacagattgctccagttgccttaaactatgcacatagctaagtgaccaaacttcttgttttgatttgaaaaaagtgcattgttttcttgtccctccctttgatgaaacgttaccctttgacgggccttttgatgtgaacagatgttttctaggacaaactataaggactaattttaaacttcaaacattccacttttgtaatttgttttaaattgttttatgtatagtaagcacaactgtaatctagttttaagagaaaccggtgctttcttttagttcatttgtatttcccttgttactgtaaaagactgtttattaattgtttacagtttgttgcaacagccattttcttgggagaaagcttgagtgtaaagccatttgtaaaaggctttgccatactcattttaatatgtgcctgttgctgttaacttttgatgaataaaaacctatcttttcatatttttatctttgacatttaccttataactcaatcttttggaaaacacaatgctaaattacaaggaaatcaaagttagcttcttggctcttgtaattcatccctcagatgtttactcagtccgagcttatctactaatgactcaccttgcaagtgagtaagcagaagcccagttagggctgttggagtcctgactaacacaggggagaggtcagctttgagccaggccttttgttcctacagtggtgaactgcataagacatcagcaagtcttgcaagtactaaaatactagttgtatttatttctatcaatcattggcctttttaaagtgataagaaaaggccactccactctacttgattgatatcagttgtaaacaaggtaccactgtgccattccctatatcttcccaggtccaactcattagaagggatatggtgcaaacttctaaatcaaacacattaacatattatttgtacagaagagtgttgatgtccaatagaaacagaatccaagccacataattttcggttttctagtagccacatttagaaaacatggaattaattttagtaacatctattccaatacgtccaaaatattgtatcactttaaaatgtcaatataaaaacaattagatgtttttacattcttttggggggtactaagtctttgaaatccagtgtatattgtgtacttacagcacatctcaatttggactagtcatatctcaggcacccaatatccacatgtggctagtggctaccatattggacagtgtgggtatagaggtctgagggtagtagaggaatatggtcagctggtcactctcgtgagatggccataccttggcctatatttaatgtgtacagaaagtctgataactcagatccttaaaaattcaggcccactgtttcagtacatagagagtggaactatcatggcaaacccacattaaccaagctcacagtaactatttttttaaaacactatcaatattttaatttacagtgagaaatgtaactatcaattattctctccctttaggcaaatcttcctgggaagccaaattatgagcagctggtgagcatggattctgagcaagggaagcaagttgcctcgtgcacccatgtccctttgggtgcacagaagacccatgtcttctgtgatattcatgtttgtggaccagggtaccctcttcccctggaaggtgctagagattctctgccagtagttgcttctctacatcagcttctgattggcacatgcattaaataacgtcattacctcaagccttgtttcagttgagcttacctgggctccattctgcctgtatacatgattgcttctgctctgatccattgtttctcttatagtttgaaactgaaaagatcatcctatttccacattctcaggggaactgtgggtgtggctcccatttcctgcctacacatataataaacccattgaaaagttgttttattatgtatatgtgggaatcaccttctatagcccttttgtttttttttttttttgagacagggtctcgctgctaactaggctggagtgcagtggcatgatcactgcagcctccacctcctaggctcaagcaatcctcccacctcagcctcctgagtgccaccacaccacccagctaatttttttttttttttttttttttttttttgagacagagccttgctctgtcgcccaggctggagtgcagtgccgcgatattggctcactgcaagttccgcctcccgggttcacgccattctcctcattctcctgcctcagtctcccaggtcgctgggactacaggcgcccgccaccaggccctgctaatttttttgtactttattagtagagttagggtttcaccatgttagccaggatggtctcaatctcctgacctcgtgatccgcccgcctcggcctcccatagtgctgggattacaggcgtgagccaccgtgcccggccagctaattttttaagaacatttttgtggccgggcatggtggctcacacctgtaatcccagcactttgggaggctgaggtgggtggatcacctgaggtcgggagttcgagaccagtctggccaacatggtgaaaccccatctctactaaaaatgcaaaaattagctgggcgtggtggcgcattcctgtaatcccagctactcgggaggctgaggcggaagaattgcttgaacccaggtggcggaggttgcaaggagcagagattgtgctactgcactccagcctaggtgacagagcaagactctgtctcaaaaaaaaaaaaaaaacttttttatagagacagggtctctctttgttggcttggctggtcttgaactcttgggctcaagcagtcctgccaccgtggcctctcaaagtgctgggattacaggtgtgagacactgcatcaggcctatagctccacttaaatacgacctatattactggaatatttttttctaaaaaattttaggaaacagttaaatatttaaaagattacttttttaaaaagcaagtaaatattacagaacagaatgcaaaatttattttacatgggagactaaaaattttcacacacatggccaccctttgggcctcttggctcaacatttcaggggctgagggagtctctgctctaggagtaaaaggtccttggagagaaaattttgacaagtcctaactttaaaaaagaaaaattggttcctggtcaatatttgtactcactgtaaatgtgatggttggtaatgatactctgtataaaagtaaaaatcatattttatgtcctttgcaaacaaatatatttgtacctgaggtacagattagaggtgctagtaattccttgaagattctgaaaatgatctttttttccaaaatgctttcttggtttttattaaactttctattttcttaaaactctcacatcaggtatttccagtgttttcaagcatgtataaatattttaatgtataaatgttgtttaaaatcccctcaatcggtatctcctgattgagaaaatacacagtgaccaatagctaataggaattcagtattgctttcaaagaaatgtgcatattaatcactgtagcatctgcatacatttgaaacacggagtaatacaggtctgtgcaagaattagcagcttgttccttgctaataatgacttgtgtcatctggaaggcccccaagagcccatggtctacaggtggaatgaccaccacttgggagtgagctgatggagagcacccagcaggtctcctccatcttcctggttcctgtgctcaccatagggctggtgtacattgggccattaataaacgtttgttgaacaaattaa

SEQ ID NO: 106 - protein, 456 aa, Homo sapiens
MGITLIWCLALVLIKWITSKRRGAISYDSSDQTALYIRMLGDVRVRSRAGFESERRGSHPYIDFRIFHSQSEIEVSVSARNIRRLLSFQRYLRSSRFFRGTAVSNSLNILDDDYNGQAKCMLEKVGNWNFDIFLFDRLTNGNSLVSLTFHLFSLHGLIEYFHLDMMKLRRFLVMIQEDYHSQNPYHNAVHAADVTQAMHCYLKEPKLANSVTPWDILLSLIAAATHDLDHPGVNQPFLIKTNHYLATLYKNTSVLENHHWRSAVGLLRESGLFSHLPLESRQQMETQIGALILATDISRQNEYLSLFRSHLDRGDLCLEDTRHRHLVLQMALKCADICNPCRTWELSKQWSEKVTEEFFHQGDIEKKYHLGVSPLCDRHTESIANIQIGFMTYLVEPLFTEWARFSNTRLSQTMLGHVGLNKASWKGLQREQSSSEDTDAAFELNSQLLPQENRLS

SEQ ID NO: 107 - DNA, 5385 bp, Homo sapiens
  source 1..5385: mol_type = other DNA
agttggtctgggcactgcagcaggctcggctctgtcccagcacttgtctgggagaaaagtggtgttactcacccagggagagtctctctttctaccttccttctttctcgatctccttgtgtgcttttgtgtttctttatttcttttccttttttttctttttttttttttgttacttaattatattcctaatcctggatgaagttgctggattctgcagcacaagtcttcatgaacaagcagcaccgctcagagatttcacggcattcaaaggtcacagaactgccactatggttaaatgtcttgtttaatggttgagaggtgtggcgaaatcttgtttgagaaccccgatcagaatgccaaatgtgtttgcatgctgggagatatacgactaaggggtcagacgggggttcgtgctgaacgccgtggctcctacccattcattgacttccgcctacttaacagtacaacatactcaggggagattggcaccaagaaaaaggtgaaaagactattaagctttcaaagatacttccatgcatcaaggctgcttcgtggaattataccacaagcccctctgcacctgctggatgaagactaccttggacaagcaaggcatatgctctccaaagtgggaatgtgggattttgacattttcttgtttgatcgcttgacaaatggaaacagcctggtaacactgttgtgccacctcttcaatacccatggactcattcaccatttcaagttagatatggtgaccttacaccgatttttagtcatggttcaagaagattaccacagccaaaacccgtatcacaatgctgttcacgcagccgacgtcacccaggccatgcactgctacctgaaagagccaaagcttgccagcttcctcacgcctctggacatcatgcttggactgctggctgcagcagcacacgatgtggaccacccaggggtgaaccagccatttttgataaaaactaaccaccatcttgcaaacctatatcagaatatgtctgtgctggagaatcatcactggcgatctacaattggcatgcttcgagaatcaaggcttcttgctcatttgccaaaggaaatgacacaggatattgaacagcagctgggctccttgatcttggcaacagacatcaacaggcagaatgaatttttgaccagattgaaagctcacctccacaataaagacttaagactggaggatgcacaggacaggcactttatgcttcagatcgccttgaagtgtgctgacatttgcaatccttgtagaatctgggagatgagcaagcagtggagtgaaagggtctgtgaagaattctacaggcaaggtgaacttgaacagaaatttgaactggaaatcagtcctctttgtaatcaacagaaagattccatccctagtatacaaattggtttcatgagctacatcgtggagccgctcttccgggaatgggcccatttcacgggtaacagcaccctgtcggagaacatgctgggccacctcgcacacaacaaggcccagtggaagagcctgttgcccaggcagcacagaagcaggggcagcagtggcagcgggcctgaccacgaccacgcaggccaagggactgagagcgaggagcaggaaggcgacagcccctaggggccggcccaacttagacgcggctctcctccggcagggcccccagagggcagaagcagcgtggaggggccctcacgcagcagcccagccactttctgagtgttgtcctggggctctttggaacgccatcttcctcccacttacctgcctcccctccttttcgcaaatgtacagaagccatttgtcacctcagcattcgctgccgaaatgagcaactccattcagtaacgtgggagctgatcccacgggcaggctctccctgctccaggagaagactaggaggaagaatgaggtgctcctgccgtgtccgccttgttccgggtcgcactggaacaggcagcaattcctaagtccggagcgtttgagcgtttgctatctgactgctgatctgcgtgacagaaacaccagcatatttgcaacgccaaggatattggtcttaagtgcaagagcacaaatgagagtgtgagagaaagtaccttctattttaataataatattattataaaaataataaatctttttaacttttatattttatgcactagacaatggatctgcaactttggactaaggtcattcaatgtacccaaacttgaacagggggttcattgttttgctattgactttattatgccactttggggcagagacttggcatcttcgcagtttaagaaaccacgtttcctatccaatccgaagggaaggtgctgtacagttcattcctttgcaccattagccaatctgtcttttatggattctgtgacatgtttatattcacccatgtacattttctgtaaataccaaacgctactgattcccatgccaaaatacatgagtattatgggattgctacctgtataaacaatggcactgtgaaaatactgttagttttaatacaagagaatgcatttgtaaatatggtatagagtttattaatatactattgtttgcagataaaggccttaactttaaacatctttcatcttctgaaagctgcccaacttaaatcctcatagatgtctttctcaactgccttcccatgttcatctgtatgttttccagctaaggtcacaaaccaaaactgaataaagtctttgaggaaacattttggaaacttcacatgcattccgcttgagaccatagtgtttaatctatggcaccaagcatcgtttcctcagattaatgagacccttcaacaagcctgaatcagtcacttttcaacacagcgatgttttaacaagccagctgctaagcttgtgtttatgtgactcttgttacagatcatggcggtgcgtcagcctcacaggagacatagcaggtctcagaaaccttctatgaccctgtcatctaaccatcagggaattccctgctcccatgccacacatttgtctattatggctatagtaccaaagtacttttggtgtttggttggtgtgcatttctttagtgtcgatagtaactggatttttctttttccttaatctcatgtgaacaactacccaactgtttagctgaagttcatattatttaagtaaagaaaatatttcagttttataacagactttaccttcctggcaggtcattgtagttaattatgtctctagcttggagtgtcaccttggaatttcgttgccattttttctcagacacctggccgtaaaatcagtttgttacagcattcttctctaggctgctaaacgctgtgcattgaaccttttctttagaagtttcagcgtaactaatgttagatgaaaattgttgatgcccctttctttttactttaaacaatgtggtagtgggagaatgactgtttctgccactatcaacctgatcctcatgctgatagaatgacagctagcacttatttcctaagtgcaactgttttagagatttttctcctaacatgcaaaggaaatactgattggcctataataagttcctatagggagactgaggcttgcagaattaaggttcaggggaaattttggaaagttggttgtattttcattgaagtaggagagattatcagatggtgctaaagaaagtgtgaagatcttatgaaataggtggatggtaagttgaaattattgatgtgggtaagaagggaggttgtggaaagttaacactagctttgtatttttttttctgtaaaactgtgaactgatatattttcctttatcactttagtattctgcagttctcagcttggtgaggctccaaaagagaatatgtcagatgtattcctacttccaaacctgtcttactttggtttgatggtacacatagggcttttgaacagtctatttttaatgtatatgaggtcaaatcaaggaaggcaattgctggggacaagaaaagtagaggtaggaaagaagacactattttagctaatggggtttcttgggactaaaaaatggctttgtttaaattataattatataataatttaaataaatgagattggaggtattcttagtagttctgagttgatagtttacattacaattaggtcttgaagaagagctcacagagaaaaaactaccaaatatccaatgggtaagcccatgatgtagccactagtacaataaaaatctgaagtaaaatgaggcataaacttgatgcagctgcctccctcattcaactggggagttcttgagttcctcatttgttggtaaaaagaaaaagaatgtgaaaatgtctctttttttcttggctattagtggctgtcttgcaatatttcaataggagtccaattactagttaaaacactggcggggtgcggtggctcacgcctgtaatcctagcactttgggaggccaagttgggcagatcacaagttcaagagatcgagaccattctggccaacatggtgaaaccccgtctctactaaaaatacaaaaattagctgggcatggcagtgcgtgcctgcaatcccagctactcaggaagctgaggcaggagaatcgcttgaacctgggaggtggaagttgtagtgaactgagatcgcaccactgcactccagcctggcaacagagctagaatccgtctcaaacaaacaaacaaaaaatcccacagctattggatcatccacagattttttctttacaatcttgttctccttgtccatggaccatcaatagttgacttgccaggtttaattctttcattgcttgagaagaaaggaatcaaaggactgtgtgtagtaagctgacggtaaagttaagattaaattaagacagagagagaatacatatcactgccaggcctgataggaaaaatctgctcttccttttaataacagtgatgaattgtcaggaccttatttaggaaaccctgacctacccataactccctgctaggctaagtagaaaccaggttatttctccctgcttatggctccccgcaaagggacttgcagcgtgtcctgcaactttgtcttcagatagtgcttcctacaaaactaggtcttgttttgtaatcttttctcgtgttgaatcagatctgcttacttatttaggtttggttatgagcttgtatctcactgtatttctcatgctttgttcttttaaacaaatcctttaaactgtgtcattttgtatacacatgtgaggtttgaaaaaaaaaaaaaaaaaaaaaagaactaccttgtgagttttgctcaaaatgtggcctaagtagccattggcatgtctagatgaacaaataaaaataaagataatttctttaaaatatca

SEQ ID NO: 108 - protein, 450 aa, Homo sapiens
MSCLMVERCGEILFENPDQNAKCVCMLGDIRLRGQTGVRAERRGSYPFIDFRLLNSTTYSGEIGTKKKVKRLLSFQRYFHASRLLRGIIPQAPLHLLDEDYLGQARHMLSKVGMWDFDIFLFDRLTNGNSLVTLLCHLFNTHGLIHHFKLDMVTLHRFLVMVQEDYHSQNPYHNAVHAADVTQAMHCYLKEPKLASFLTPLDIMLGLLAAAAHDVDHPGVNQPFLIKTNHHLANLYQNMSVLENHHWRSTIGMLRESRLLAHLPKEMTQDIEQQLGSLILATDINRQNEFLTRLKAHLHNKDLRLEDAQDRHFMLQIALKCADICNPCRIWEMSKQWSERVCEEFYRQGELEQKFELEISPLCNQQKDSIPSIQIGFMSYIVEPLFREWAHFTGNSTLSENMLGHLAHNKAQWKSLLPRQHRSRGSSGSGPDHDHAGQGTESEEQEGDSP

SEQ ID NO: 109 - DNA, 4036 bp, Homo sapiens
  source 1..4036: mol_type = other DNA
gcggccgaggcgagcccggcgatgtgagaggcggccgtcggctcctgcctcaggaagggcatgttcggaggggcggcctcggcacgccacccgcctaagcgcccccttcccaccgcagccgccgccgccgcagcgcccgcaccgcgataaaaggggcggccgcgtttcctgacgcgagatccgcgctcgccgccgcccgcccaggcggcgatgacacggcgcccgcggcggcccggaggcgccgggtgggccgtttgctgaccggatcgcggctacccgccagcgtgtccgcggcgccgccgccagcatgggctgtgccccgagcatccacatttccgagcgcctggtggccgaggacgcgcctagccccgcggcaccgccgctgtcgtccggcgggccgcgcctcccgcagggccagaagacggccgccttgccccggacccgcggcgccggcctcttggagtcggagcttcgcgacggcagcggcaagaaggtagcagtagctgatgtgcagtttggccccatgagatttcatcaagatcaacttcaggtacttttagtgtttaccaaagaagataaccaatgtaatggattctgcagggcatgtgaaaaagcagggtttaagtgtacagttaccaaggaggctcaggctgtccttgcctgtttcctggacaaacatcatgacattatcatcatagaccacagaaatcctcgacagctggatgcagaggcactgtgcaggtctatcagatcatcaaaactctcagaaaacacagttattgttggtgtagtacgcagggtggatagagaagagttgtccgtaatgcctttcatttctgctggatttacaaggaggtatgtagaaaaccccaacatcatggcctgctacaatgaactgctccagctggagtttggagaggtgcgatcacaactgaaactcagggcttgtaactcagtattcactgcattagaaaacagtgaagatgcaattgaaattacaagcgaagaccgttttatacagtatgcaaatcctgcatttgaaacaacaatgggctatcagtcaggtgaattaatagggaaggagttaggagaagtgcctataaatgaaaaaaaggctgacttgctcgatactataaattcatgcatcaggataggcaaggagtggcaaggaatttactatgccaaaaagaaaaacggagataatatacaacaaaatgtgaagataatacctgtcattggacagggaggaaaaattagacactatgtgtccattatcagagtgtgcaatggcaacaataaggctgagaaaatatccgaatgtgttcagtctgacactcatacagataatcagacaggcaaacataaagacaggagaaaaggctcactagacgtcaaagctgttgcctcccgtgcaactgaagtttccagccagagacgacactcttccatggcccggatacattccatgacaattgaggcgcccatcaccaaggtaatcaatattatcaatgctgcccaggaaagtagtcccatgcctgtgacagaagccctagaccgtgtgctggaaattctaagaaccactgagttatattcaccacagtttggtgctaaagatgatgatccccatgccaatgaccttgttgggggcttaatgtctgatggtttgcgaagactatcagggaatgaatatgttctttcaacaaaaaacactcaaatggtttcaagcaatataatcactcccatctcccttgatgatgtcccaccacggatagctcgggccatggaaaatgaggaatactgggactttgatatttttgaactggaggctgccacccacaataggcctttgatttatcttggtctcaaaatgtttgctcgctttggaatctgtgaattcttacactgctccgagtcaacgctaagatcatggttacaaattatcgaagccaattatcattcctccaatccctaccacaattctacacattctgctgatgtgcttcatgccactgcctattttctctccaaggagaggataaaggaaactttagatccaattgatgaggtcgctgcactcatcgcagccaccattcatgatgtggatcaccctgggagaaccaactccttcctgtgtaatgctggaagtgagctggccattttgtacaatgacactgctgtgctggagagccaccatgcggccttggccttccagctgaccactggagatgataaatgcaatatatttaaaaacatggagaggaatgattatcggacactgcgccaggggattatcgacatggtcttagccacagaaatgacaaagcactttgagcatgtcaacaaatttgtcaacagcatcaacaaacccttggcaacactagaagaaaatggggaaactgataaaaaccaggaagtgataaacactatgcttaggactccagagaaccggaccctaatcaaacgaatgctgattaaatgtgctgatgtgtccaatccctgccgacccctgcagtactgcatcgagtgggctgcacgcatttcggaagaatatttttctcagactgatgaagagaagcagcagggcttacctgtggtgatgccagtgtttgacagaaatacctgcagcatccccaaatcccaaatctctttcattgattacttcatcacagacatgtttgatgcttgggatgcctttgtagacctgcctgatttaatgcagcatcttgacaacaactttaaatactggaaaggactggacgaaatgaagctgcggaacctccgaccacctcctgaatagtgggagacaccacccagagccctgaagctttgttccttcggtcatttggaattcctgagggcagccagagctccttggtcctttcagtactaggcagaacagcccccgatctgcatagcctgtgaaagcccacggggacatcagtaaccttctgcagccaccatccaatgccattactgtcaagtgagacttggccactgtagcctgggcctgctgcaggagctcttcagaaaggcacatgaggaccacggtttgcctcagtttctggtaaaacacaaggtctggagtgcccctgcaaagggtattgatggacttcctgccagtgacagagcatgtctattgcaaacaattctctcagttacgttcagcacttaagaacggctaatggcaataggatctttagcaactttttcacatcatagaaggtgcaatcgctcacttgggaacactactgagagtgacttctcttttaaaattgagtagcagatgaaaaattaaaatttgaacttgattattaatatcaattaaaatgttttatttattttattaaaagctcaatattttctatgaattcaaaaatacttcagagccaaagccaacttcaaataccgtgaccaaatttacatgattcatattcattatgcattacttggtatacagacttattttcataatgcaaattaataaaatgacacttttactgcactatagaaatattcatgtatgttaaacttttctgattgaggctaactggaaaaagctggggtcgtattctaagtgctaaagaaggctgcttctactgtatagaacccagggctctgaaacagctctagccgcctaatgcacttcacaggtaactccccaaggtaaaactagactctcttgttggttcgcaaagaaaagttaggacttaacacttttttctaaaattttataattcaatttccaaaagtctactctattttatactgtttctacaaaatattccttataaaaacaaagaacaaaaattgaatatttaatgaattgacattttataaccaacctgtttttatctacggtgggaatctttgatgccagaaatttataaagaggttctgtatcttcacaccttgaataagcataataccataaaaaatgacacttgacatgtcaatgtatttgtcatttcattttaaactcgtatttgtggtttttttcccagataaaaatgaaattaaaccatttctttttaagaaa

SEQ ID NO: 110 - protein, 829 aa, Homo sapiens
MGCAPSIHISERLVAEDAPSPAAPPLSSGGPRLPQGQKTAALPRTRGAGLLESELRDGSGKKVAVADVQFGPMRFHQDQLQVLLVFTKEDNQCNGFCRACEKAGFKCTVTKEAQAVLACFLDKHHDIIIIDHRNPRQLDAEALCRSIRSSKLSENTVIVGVVRRVDREELSVMPFISAGFTRRYVENPNIMACYNELLQLEFGEVRSQLKLRACNSVFTALENSEDAIEITSEDRFIQYANPAFETTMGYQSGELIGKELGEVPINEKKADLLDTINSCIRIGKEWQGIYYAKKKNGDNIQQNVKIIPVIGQGGKIRHYVSIIRVCNGNNKAEKISECVQSDTHTDNQTGKHKDRRKGSLDVKAVASRATEVSSQRRHSSMARIHSMTIEAPITKVINIINAAQESSPMPVTEALDRVLEILRTTELYSPQFGAKDDDPHANDLVGGLMSDGLRRLSGNEYVLSTKNTQMVSSNIITPISLDDVPPRIARAMENEEYWDFDIFELEAATHNRPLIYLGLKMFARFGICEFLHCSESTLRSWLQIIEANYHSSNPYHNSTHSADVLHATAYFLSKERIKETLDPIDEVAALIAATIHDVDHPGRTNSFLCNAGSELAILYNDTAVLESHHAALAFQLTTGDDKCNIFKNMERNDYRTLRQGIIDMVLATEMTKHFEHVNKFVNSINKPLATLEENGETDKNQEVINTMLRTPENRTLIKRMLIKCADVSNPCRPLQYCIEWAARISEEYFSQTDEEKQQGLPVVMPVFDRNTCSIPKSQISFIDYFITDMFDAWDAFVDLPDLMQHLDNNFKYWKGLDEMKLRNLRPPPE

SEQ ID NO: 111 - DNA, 4606 bp, Homo sapiens
  source 1..4606: mol_type = other DNA
gtgtatgcgcgctcccccgctcggggaggaagatggcccaaaagggaaagttggggtgacgcgcgcggtccccggaggctcggcggggggcaccgcggccagcccgacggagcggcggacacacaggccggggggcgcgcagtccgggcgccgccgcggccgccccctcactgcaggtggcagcgggtgcgctgggtcccggcggccgcgggcgcgggcgggcgcgcgggggagcccggccgagggatgggctgcgcccccagcatccatgtctcgcagagcggcgtgatctactgccgggactcggacgagtccagctcgccccgccagaccaccagcgtgtcgcagggcccggcggcacccctgcccggcctcttcgtccagaccgacgccgccgacgccatccccccgagccgcgcgtcgggaccccccagcgtagcccgcgtccgcagggcccgcaccgagctgggcagcggtagcagcgcgggttccgcagcccccgccgcgaccaccagcaggggccggaggcgccactgctgcagcagcgccgaggccgagactcagacctgctacaccagcgtgaagcaggtgtcttctgcggaggtgcgcatcgggcccatgagactgacgcaggaccctattcaggttttgctgatctttgcaaaggaagatagtcagagcgatggcttctggtgggcctgcgacagagctggttatagatgcaatattgctcggactccagagtcagcccttgaatgctttcttgataagcatcatgaaattattgtaattgatcatagacaaactcagaacttcgatgcagaagcagtgtgcaggtcgatccgggccacaaatccctccgagcacacggtgatcctcgcagtggtttcgcgagtatcggatgaccatgaagaggcgtcagtccttcctcttctccacgcaggcttcaacaggagatttatggagaatagcagcataattgcttgctataatgaactgattcaaatagaacatggggaagttcgctcccagttcaaattacgggcctgtaattcagtgtttacagcattagatcactgtcatgaagccatagaaataacaagcgatgaccacgtgattcagtatgtcaacccagccttcgaaaggatgatgggctaccacaaaggtgagctcctgggaaaagaactcgctgatctgcccaaaagcgataagaaccgggcagaccttctcgacaccatcaatacatgcatcaagaagggaaaggagtggcagggggtttactatgccagacggaaatccggggacagcatccaacagcacgtgaagatcaccccagtgattggccaaggagggaaaattaggcattttgtctcgctcaagaaactgtgttgtaccactgacaataataagcagattcacaagattcatcgtgattcaggagacaattctcagacagagcctcattcattcagatataagaacaggaggaaagagtccattgacgtgaaatcgatatcatctcgaggcagtgatgcaccaagcctgcagaatcgtcgctatccgtccatggcgaggatccactccatgaccatcgaggctcccatcacaaaggttataaatataatcaatgcagcccaagaaaacagcccagtcacagtagcggaagccttggacagagttctagagattttacggaccacagaactgtactcccctcagctgggtaccaaagatgaagatccccacaccagtgatcttgttggaggcctgatgactgacggcttgagaagactgtcaggaaacgagtatgtgtttactaagaatgtgcaccagagtcacagtcaccttgcaatgccaataaccatcaatgatgttcccccttgtatctctcaattacttgataatgaggagagttgggacttcaacatctttgaattggaagccattacgcataaaaggccattggtttatctgggcttaaaggtcttctctcggtttggagtatgtgaatttttaaactgttctgaaaccactcttcgggcctggttccaagtgatcgaagccaactaccactcttccaatgcctaccacaactccacccatgctgccgacgtcctgcacgccaccgctttctttcttggaaaggaaagagtaaagggaagcctcgatcagttggatgaggtggcagccctcattgctgccacagtccatgacgtggatcacccgggaaggaccaactctttcctctgcaatgcaggcagtgagcttgctgtgctctacaatgacactgctgttctggagagtcaccacaccgccctggccttccagctcacggtcaaggacaccaaatgcaacattttcaagaatattgacaggaaccattatcgaacgctgcgccaggctattattgacatggttttggcaacagagatgacaaaacactttgaacatgtgaataagtttgtgaacagcatcaacaagccaatggcagctgagattgaaggcagcgactgtgaatgcaaccctgctgggaagaacttccctgaaaaccaaatcctgatcaaacgcatgatgattaagtgtgctgacgtggccaacccatgccgccccttggacctgtgcattgaatgggctgggaggatctctgaggagtattttgcacagactgatgaagagaagagacagggactacctgtggtgatgccagtgtttgaccggaatacctgtagcatccccaagtctcagatctctttcattgactacttcataacagacatgtttgatgcttgggatgcctttgcacatctgccagccctgatgcaacatttggctgacaactacaaacactggaagacactagatgacctaaagtgcaaaagtttgaggcttccatctgacagctaaagccaagccacagagggggcctcttgaccgacaaaggacactgtgaatcacagtagcgtaaacgagaggccttcctttctaatgacaatgacaggtattggtgaaggagctaatgtttaatatttgaccttgaatcattcaagtccccaaatttcattcttagaaagttatgttccatgaagaaaaatatatgttcttttgaatacttaatgacagaacaaatacttggcaaactcctttgctctgctgtcatcctgtgtacccttgtcaatccatggagctggttcactgtaactagcaggccacaggaagcaaagccttggtgcctgtgagctcatctcccaggatggtgactaagtagcttagctagtgatcagctcatcctttaccataaaagtcatcattgctgtttagcttgactgttttcctcaagaacatcgatctgaaggattcataaggagcttatctgaacagatttatctaagaaaaaaaaaaaacgacataaaataagtgaaacaactaggaccaaattacagataaactagttagcttcacagcctctatggctacatggttcttctggccgatggtatgacacctaagttagaacacagccttggctggtgggtgccctctctagactggtatcagcagcctgtgtaacccctttcctgtaaaaggggttcatcttaacaaagtcatccatgatgagggaaaaagtggcatttcatttttggggaatccatgagcttcctttatttctggctcacagaggcagccacgaggcactacaccaagtattatataaaagccattaaatttgaatgcccttggacaagcttttcttaaaaaaaaaaaaaaaaagtttatatacatgtttaaaatttttattaaaatccaaattttctgggtgtaagcccatgcagtatgttgtgccatgcaccatctatacgtaatattttgggaggggataggggaagtttcaaggttcagatatttttaaccagtctatatttgaaatcatgccattagctttaacaatgttaaaattgtgtggtgtaaatatatcagaaaataggcatatggggaggcagtaaatactattttaagctattaattgtatgctaaaagcttctaaagcacaagtgcatatttttatactgctcttttcacaactccctgtgatctacataaagtcagactcgagattttcctttctcttttaccagctgatccttcctatgtattataaatattagactccgtaaacaaacttcatttttctttctctgtacttcatgctgcatttttaaaaggtataaacaaacagagactgaattaattgaatcagtaattacttttttccaatacaaattggaatgcagaatacttggaacttgtacatggggaaaaaatgacttatcactacataatgtgccaatgtttttttctatgttttgtaccaaaaatggaaaaatatgacaattccatgcaaagaaatgtatctaaattatttttgttagatgataagagaacttgcttggtcaggacagcagccagctttgtattgtaatgctatattatgtaaatgtgatgaaaatgtttttgtgaagtacttgtaactaaattcctacagccatttttcactcccaacagctgtttttattttacctctttggcctaaagttttcataatttcaaa

SEQ ID NO: 112 - protein, 885 aa, Homo sapiens
MGCAPSIHVSQSGVIYCRDSDESSSPRQTTSVSQGPAAPLPGLFVQTDAADAIPPSRASGPPSVARVRRARTELGSGSSAGSAAPAATTSRGRRRHCCSSAEAETQTCYTSVKQVSSAEVRIGPMRLTQDPIQVLLIFAKEDSQSDGFWWACDRAGYRCNIARTPESALECFLDKHHEIIVIDHRQTQNFDAEAVCRSIRATNPSEHTVILAVVSRVSDDHEEASVLPLLHAGFNRRFMENSSIIACYNELIQIEHGEVRSQFKLRACNSVFTALDHCHEAIEITSDDHVIQYVNPAFERMMGYHKGELLGKELADLPKSDKNRADLLDTINTCIKKGKEWQGVYYARRKSGDSIQQHVKITPVIGQGGKIRHFVSLKKLCCTTDNNKQIHKIHRDSGDNSQTEPHSFRYKNRRKESIDVKSISSRGSDAPSLQNRRYPSMARIHSMTIEAPITKVINIINAAQENSPVTVAEALDRVLEILRTTELYSPQLGTKDEDPHTSDLVGGLMTDGLRRLSGNEYVFTKNVHQSHSHLAMPITINDVPPCISQLLDNEESWDFNIFELEAITHKRPLVYLGLKVFSRFGVCEFLNCSETTLRAWFQVIEANYHSSNAYHNSTHAADVLHATAFFLGKERVKGSLDQLDEVAALIAATVHDVDHPGRTNSFLCNAGSELAVLYNDTAVLESHHTALAFQLTVKDTKCNIFKNIDRNHYRTLRQAIIDMVLATEMTKHFEHVNKFVNSINKPMAAEIEGSDCECNPAGKNFPENQILIKRMMIKCADVANPCRPLDLCIEWAGRISEEYFAQTDEEKRQGLPVVMPVFDRNTCSIPKSQISFIDYFITDMFDAWDAFAHLPALMQHLADNYKHWKTLDDLKCKSLRLPSDS

SEQ ID NO: 113 - DNA, 2192 bp, Homo sapiens
  source 1..2192: mol_type = other DNA
gagcggaggagaccctgcggcgcgcggcggcggctcccgggcgtcccgggcccggtggcggcgcggctgtggttggctgagcgccgcgggccgccccccgcccgccccctcccctgctcccctcccccgcctcccgcggcggctggcgtcgggaaagtacagtaaaaagtccgagtgcagccgccgggcgcaggatgggatccggctcctccagctaccggcccaaggccatctacctggacatcgatggacgcattcagaaggtaatcttcagcaagtactgcaactccagcgacatcatggacctgttctgcatcgccaccggcctgcctcggaacacgaccatctccctgctgaccaccgacgacgccatggtctccatcgaccccaccatgcccgcgaattcagaacgcactccgtacaaagtgagacctgtggccatcaagcaactctccgctggtgtcgaggacaagagaaccacaagccgtggccagtctgctgagagaccactgagggacagacgggttgtgggcctggagcagccccggagggaaggagcatttgaaagtggacaggtagagcccaggcccagagagccccagggctgctaccaggaaggccagcgcatccctccagagagagaagaattaatccagagcgtgctggcgcaggttgcagagcagttctcaagagcattcaaaatcaatgaactgaaagctgaagttgcaaatcacttggctgtcctagagaaacgcgtggaattggaaggactaaaagtggtggagattgagaaatgcaagagtgacattaagaagatgagggaggagctggcggccagaagcagcaggaccaactgcccctgtaagtacagttttttggataaccacaagaagttgactcctcgacgcgatgttcccacttaccccaagtacctgctctctccagagaccatcgaggccctgcggaagccgacctttgacgtctggctttgggagcccaatgagatgctgagctgcctggagcacatgtaccacgacctcgggctggtcagggacttcagcatcaaccctgtcaccctcaggaggtggctgttctgcgtccacgacaactacagaaacaaccccttccacaacttccggcactgcttctgcgtggcccagatgatgtacagcatggtctggctctgcagtctccaggagaagttctcacaaacggatatcctgatcctaatgacagcggccatctgccacgatctggaccatcccggctacaacaacacgtaccagatcaatgcccgcacagagctggcggtccgctacaatgacatctcaccgctggagaaccaccactgcgccgtggccttccagatcctcgccgagcctgagtgcaacatcttctccaacatcccacctgatgggttcaagcagatccgacagggaatgatcacattaatcttggccactgacatggcaagacatgcagaaattatggattctttcaaagagaaaatggagaattttgactacagcaacgaggagcacatgaccctgctgaagatgattttgataaaatgctgtgatatctctaacgaggtccgtccaatggaagtcgcagagccttgggtggactgtttattagaggaatattttatgcagagcgaccgtgagaagtcagaaggccttcctgtggcaccgttcatggaccgagacaaagtgaccaaggccacagcccagattgggttcatcaagtttgtcctgatcccaatgtttgaaacagtgaccaagctcttccccatggttgaggagatcatgctgcagccactttgggaatcccgagatcgctacgaggagctgaagcggatagatgacgccatgaaagagttacagaagaagactgacagcttgacgtctggggccaccgagaagtccagagagagaagcagagatgtgaaaaacagtgaaggagactgtgcctgaggaaagcggggggcgtggctgcagttctggacgggctggccgagctgcgcgggatccttgtgcagggaagagctgccctgggcacctggcaccacaagaccatgttttctaagaaccattttgttcactgatacaaaaaaaaaaaaaggaattcatgatgctgtacagaattttatttttaaactgtcttttaaataatatattcttatacggaaa

SEQ ID NO: 114 - protein, 593 aa, Homo sapiens
MGSGSSSYRPKAIYLDIDGRIQKVIFSKYCNSSDIMDLFCIATGLPRNTTISLLTTDDAMVSIDPTMPANSERTPYKVRPVAIKQLSAGVEDKRTTSRGQSAERPLRDRRVVGLEQPRREGAFESGQVEPRPREPQGCYQEGQRIPPEREELIQSVLAQVAEQFSRAFKINELKAEVANHLAVLEKRVELEGLKVVEIEKCKSDIKKMREELAARSSRTNCPCKYSFLDNHKKLTPRRDVPTYPKYLLSPETIEALRKPTFDVWLWEPNEMLSCLEHMYHDLGLVRDFSINPVTLRRWLFCVHDNYRNNPFHNFRHCFCVAQMMYSMVWLCSLQEKFSQTDILILMTAAICHDLDHPGYNNTYQINARTELAVRYNDISPLENHHCAVAFQILAEPECNIFSNIPPDGFKQIRQGMITLILATDMARHAEIMDSFKEKMENFDYSNEEHMTLLKMILIKCCDISNEVRPMEVAEPWVDCLLEEYFMQSDREKSEGLPVAPFMDRDKVTKATAQIGFIKFVLIPMFETVTKLFPMVEEIMLQPLWESRDRYEELKRIDDAMKELQKKTDSLTSGATEKSRERSRDVKNSEGDCA

SEQ ID NO: 115 - DNA, 8501 bp, Homo sapiens
  source 1..8501: mol_type = other DNA
agcagtagtcaccgcggcggcggtggcagcggcggcgggcggcggcggctcttcctctcgcctgcgctccagggcttgctgcttccagcccgtgccggtccccggccgccgccgccgccccggctcccccttggccaggccgcccgccgcgcgggctcccccggcttccccggcgccggcccaggcggcggcggccaaactccgcggcgtccccagggcgccagcttcgccctcgccgccgcggccgcgctgctcttcggctccgacatggaagatggaccttctaataatgcgagctgcttccgaaggctgaccgagtgcttcctgagccccaaagctaatggtatagatatagaagtcatccacagagatgttacagttgaagagatgggggtagagaagactttgaaggaaaagaatgtagaatgaggatagaagagaggaaatcccaacatttaacaggtttgacagatgaaaaagtgaaggcatatctttctcttcacccccaggtattagatgaatttgtatctgaaagtgttagtgcagagacagtagagaaatggctgaagaggaagaacaacaaatcagaagatgaatcagctcctaaggaagtcagcaggtaccaagatacgaatatgcagggagttgtatatgaactaaacagctatatagaacaacggttggacacaggaggagacaaccagctactcctctatgaactgagcagcatcattaaaatagccacaaaagccgatggatttgcactgtatttccttggagagtgcaataatagcctgtgtatattcacgccacctgggataaaggaaggaaaaccccgcctcatccctgctgggcccatcactcagggcaccaccgtctctgcttatgtggccaagtccaggaaaacactgctagtagaagacatccttggagatgaacgatttccaagaggtactggactggaatcagggactcgtatccagtctgttctttgcttaccaattgtcactgcaattggtgacttgattggtattctcgagctgtatcggcactggggcaaagaagccttctgtcttagtcaccaggaggttgcaacagcaaatcttgcctgggcttcagtagcaatacatcaggtgcaggtatgcagaggccttgccaaacagacagaattgaatgacttcctactcgacgtatcaaaaacatattttgataacatagttgcaatagattctctacttgaacacataatgatatatgcaaaaaacctggtgaatgccgatcgttgtgcgcttttccaggtggaccataagaacaaggagttatattcagacctttttgatattggagaggaaaaggaaggaaaacctgtcttcaagaagaccaaagagataagattttcaattgagaaaggaattgctggccaagtagcaagaacaggggaagtcctgaacattccagatgcctatgcagacccacgctttaacagagaagtagacttgtacacaggctacaccacgcggaacatcctgtgcatgcccatcgtcagccgaggcagcgtgataggtgtggtgcagatggtcaacaaaatcagtggcagtgccttctctaaaacagatgaaaacaacttcaaaatgtttgccgtcttttgtgctttagccttacactgtgctaatatgtatcatagaattcgccactcagagtgcatttaccgggtaacgatggaaaagctgtcctaccatagcatttgtacttcagaagagtggcaaggtctcatgcaattcacccttcccgtgcgtctctgcaaagaaattgaattattccactttgacattggtccttttgaaaacatgtggcctggaatttttgtctacatggttcatcggtcctgtgggacatcctgctttgagcttgaaaagttgtgtcgttttattatgtctgtgaagaagaactatcggcgggttccttatcacaactggaagcatgcggtcactgtagcacactgcatgtatgccatacttcagaacaatcacacgcttttcacagaccttgagcgcaaaggactgctgattgcgtgtctgtgtcatgacctggaccacaggggcttcagtaacagctacctgcagaagttcgaccaccctctggccgctctctactccacttccaccatggagcagcaccacttctcccagactgtgtccatcctccagttggaagggcacaatatcttctccactctgagctccagtgaatatgagcaggtgcttgagatcatccgcaaagccatcattgccacagaccttgctttatactttggaaacaggaagcagttggaagagatgtaccagaccggatcactaaaccttaataatcaatcacatagagaccgtgtaattggtttgatgatgactgcctgtgacctttgttctgtgacaaaactgtggcccgttacaaaattgacggcaaatgatatatatgcagaattctgggctgagggtgatgaaatgaagaaattgggaatacagcctattcctatgatggacagagacaagaaggatgaagtcccccaaggccagcttgggttctacaatgccgtggccattccctgctatacaacccttacccagatcctccctcccacggagcctcttctgaaagcatgcagggataatctcagtcagtgggagaaggtgattcgaggggaggagactgcaacctggatttcatccccatccgtggctcagaaggcagctgcatctgaagattgagcactggtcaccctgacacgctgtcccacctacagatcctcatcttgcttctttgacattcttttcctttttttggggggggtggggggaacctgcacctggtaactggggtgcaaacctcttcaagaaggtaacatcaaataaataagtcaagcagaggacttcctgccaatctcttctgtgaggcatcatagacactgagcaaccaggaccacccccacgttcagaaatcagctggccaagtgactccatttgacttgcaaaccagccttttctaataggctaatattgctgaggccttaaaggaaatggacaaaaattatccagaaggggtacttttccattgtatctttctaataagggtttaaaatggtactattatggtattgtacttgggctttaacatcaatgttgctttgatgttgttggatataaataggaatttttacacattactattgtgaatggtgaatgttcatgtatgacctacttgtaattaacttgagttgtagtccacagcctcaggacaaatgtcgttgaggttacagagtaagaaatgatggcaaaacgtcaaactcttatttcagagcttcatgaatttagttagactaaacataattctttaagttcaacctaaagggctgagatcaataaatttaacactagacgaagtagacttcctgtctttttgagaagagatgaggtatatgttacaataaatctcagaacttcaagtagcagttcaaaagatgtcagtttttaaaattgtttttgttgttgtcttggcagttttactgaaccctttgcataaagaacaaaataaaagctcggcattgtaatttttttaatggacaagtcttatggatacgaagggtacatttttcataatgattcctttatattttcactttgtgtcattgcagaattttagactctcattcacaatgaaaagtttattttaaacattgtttaattaaaataccatacagttctcttttaaacatcaaaccataaaaagtgtattttgtaattttactctgacctgccgcagtcacctctcacttatctcttccacgtactgcacggtcgtatttcatgagctttctgtccatagcacagaaacagagcagaaagtagtacaatcatgttggaccttctttctgttctctttactcttctcacagatcagatcactccatagaagcctgtgggtttcgatggtttcttctatacacctttttggttgaccagtattactatacaatgtaagtgttttaaaaaatacgaaagtaatactctgcaccccttcctacaaagatgataaagcagtcacttctggcgcattttaataatttaaagatttttagtgcaatggcacggtaacctccaaacctgaattagacagagactcactcaggaagtgacaggcccatcatatcaaataacttattcacttttcatgtggcaggaaactggaatatcgcttttaataaaatggaaaaatatgcttctacatatttaccaccataggcgttttgttcatatgagcctggtttgtgcaaaattaaatcagaggcttctacaacatggtttatttatgttgtagcaaagttggctctacataaacattgttcttattttaaaattaacactatgtgttcagttttcttgtgggcttctgaaagttgccatcttccctccgtggagctccatttgctattttcattatacactatgaggtaaaatgtaataacaaaagagagagaagtaccactgtggctagatatatacacacacatatatatatggatggatgtaatatatgtagaacacacacatagatgtatataggatacacactcatgtatgtaaacgtatacatatgtgtatatatgatacatacacatacacacacacgagagacagaaggaaagagaggaagagagaagcaaacatgtaggaaaaaatataaatcagccccattctcccattctttaagaacaatgatttttcttgatggaaaatgcatatcacttgacagttgacaagaaagtgtcatttttgtgttagtgtatcatataattgaatttgaacaagatacatatttttctgcatacaaatttatgaagctggagtctaccaaacacagctttagtcacaaaagttagtttagttatctcatttcgcttggagatggaatttcaggaagggatatattatttaagattattgtttaattacaagaattttaaaagaatgtatgaattctgttttttaatatagaaaataattatggagttaggaatctcatggctacatttacatttttaggttattacagaaaattctcttaatttattatagtcaagtgtattatgtaatctctatttagaacagtttcccaaaggaatgtgattggatttactggttggttaatttcttgtgaaatattgtcataatagaagcacagcttgaacaaaagactgaattctgatataaactgtcaatattgcttttaccatgtgtaagatttacttagtaatcacagatttacctaaaataaaaggacccgggttgcagtgatatttagttaatgatttgttttggaaaacatgcagttaggagtatttttgtattttgtcagatgtttaggagacagactttcgggtcatgtttcttgtcttgttcccagatcttttcttaaaagaacagtgtgacaccagaagccaagagatggtttttactaacaacagctttgatgagttcctattaaggtcgtattgtgtattgtgccaaattttccacccagtataaatttagtaacccgctatgagcatatgtaggatattcaatttgcagatacttttgttggttatgttggtttataatagacaagttttatggtcatatgcaattattccattatctttttggacacagtgaatatgttttttagctaaaaatgtccttggaaacataaatgcctgccaataacatggaatattgaattcgggcaatgtgaattgattaattagaaaagggtcaaaagaaatacaatggatgtggaaactaattctaaaaaatagccctattaatagggcagagactctggtccatttcccagctgtacttctctctaagaggtgtatgaaaaacccatcttgcaaaagagaccaaaatattagacacaatcgttcccattcctgactcttcaatggaaaaggaaggtacagatgtttacagtggtgccccaggtgactcgttctcaccacaacaaaagcaactaattggaaactagatgtgttcaataatagatttcctcttttttggcatgctttttagattttttttcattttgtaaaatctcagttaatttttctttattggtatatttgtgtatgcgagacaaatcctgtattgtacaggatataaatagatgcataaatccttagatacctgggttttttaataggtttaggtttgggtattgtgtttctggtcttttaactcaaaattaaggtttgagctttaataggactaaattattcacctgccttggcctgtgcctttattttaaatactgcaattttacttcttcattcatgtatttattattttgcttttcttgcttaagtataattgaaaatatttgcaggaacgcacaattcattttatcaagttgaatgaataggaccattctctcctcatcagatttctgttctttatttgacttcattgacatataccctggtgactataaccagtgaactgttcagagtcagtcttttcggcaagaacttcagagaactgtgacactggttatgatgtgattttggggggtttcaggtacctaagcatgatttttaaaatcacttctctctttacatatttcgaacatatgtttgctttctacactttgcagattttatttaggatttaattctttaaagactatattcatttagtcactatagtggatctcttctactgcaagtattcatctgatttttaaattatgtaaaatgtaaatcagccaagtatgtcatccgttatagtttccccatgctttcagcgcatggccatgagatttttacatgtgcataagtatttagccaatacacattttgctgacttctttaaccatttatattgtttaaattagtaatatccaatgcagtgcacacttttttgtcttttttccaacggaatattttggttgtctgtagcgttggaagcattttatatgataaaaatagcaagaaaaaattaaaaagtgtcaacggtgtgctggttctaaattaagaagatagaacaaagagaaagacattaatgttacctaagaaacacatttaacatccgaagaagcaatgctgtcctcacttgatgtttctcttctcaacccagcaatggagagcagggcttgcaaagccgtacagagcctacgtgctctttcctgcaagtgggagaaaactaatcaatggcacacagggccaggtgtggccctgtgaggcaaaggataatgtcacctcaggaccaaggtggaaacttacagctgaatccagggcttactaagtagggaagtcagtttacatatttcagttttcctctgatgtttttgaggtactgtgtatttgcagaagtttaagcagaagggttttgtttctattgtaagttaggttctaaaagtgtataatctgatactctagcccaactgaaatattatatcttgggcgttacagcctttgtctttttctttagtcaccttaatacccagtcctatgctgtatctctgatagcctatataaatgacatataggaatattattttccatatgatctgttgtatggtgtatatgctatgtgttcatttcgtgtgcaagttcagagtgtaatagatttacccagagaaggtgtttctatacaatgcccctacctatttgaaattacatgcttgcccaacacactgtgaaatagttaccaaaatttgtacaaatgcagcatcttcattctttctgagaagacaagatggttttctttacatgaacaaatgaacaaaagagatcctagatccataacgtagctaaggcatctaagagtttgctgttgataatcttgctgaccaaaaactactggagagtaacacaggttatatgccatcacaaatacaatgctcatgaagaactgatttgtagagtcaatgaacctgtgtccagaattttaataggctctctattggaaggagaaagaatttcaagttaacagtatctaactttatcatagttgatgttagtaaattttaaaaaatgattttatatgtatgacaaaaatctttgtaaaatgcgcaagtgcaataatttaaagaggtcttaactttgcatttataaattataaatattgtacatgtgtgtaattttttcatgtattcatttgcagtctttgtatttaaaaaacatttactgttatgtttgtataatagaacagtaatcatttattataatctaggcaagttgtaaataaattcataattcaaacagccagtatatatgcatatatgagtgttatattgcaaaatctttgttttacttacatggttaaagcagcaagaattcttttgttgatatgtaattatacacataaaatatatatatgtatgatacatgaaatatatttagaaatgttcataattttaatggatatcctttggtgtgaataattgaatacagagtttttaaaata

SEQ ID NO: 116 - protein, 779 aa, Homo sapiens
MRIEERKSQHLTGLTDEKVKAYLSLHPQVLDEFVSESVSAETVEKWLKRKNNKSEDESAPKEVSRYQDTNMQGVVYELNSYIEQRLDTGGDNQLLLYELSSIIKIATKADGFALYFLGECNNSLCIFTPPGIKEGKPRLIPAGPITQGTTVSAYVAKSRKTLLVEDILGDERFPRGTGLESGTRIQSVLCLPIVTAIGDLIGILELYRHWGKEAFCLSHQEVATANLAWASVAIHQVQVCRGLAKQTELNDFLLDVSKTYFDNIVAIDSLLEHIMIYAKNLVNADRCALFQVDHKNKELYSDLFDIGEEKEGKPVFKKTKEIRFSIEKGIAGQVARTGEVLNIPDAYADPRFNREVDLYTGYTTRNILCMPIVSRGSVIGVVQMVNKISGSAFSKTDENNFKMFAVFCALALHCANMYHRIRHSECIYRVTMEKLSYHSICTSEEWQGLMQFTLPVRLCKEIELFHFDIGPFENMWPGIFVYMVHRSCGTSCFELEKLCRFIMSVKKNYRRVPYHNWKHAVTVAHCMYAILQNNHTLFTDLERKGLLIACLCHDLDHRGFSNSYLQKFDHPLAALYSTSTMEQHHFSQTVSILQLEGHNIFSTLSSSEYEQVLEIIRKAIIATDLALYFGNRKQLEEMYQTGSLNLNNQSHRDRVIGLMMTACDLCSVTKLWPVTKLTANDIYAEFWAEGDEMKKLGIQPIPMMDRDKKDEVPQGQLGFYNAVAIPCYTTLTQILPPTEPLLKACRDNLSQWEKVIRGEETATWISSPSVAQKAAASED

SEQ ID NO: 117 - DNA, 7801 bp, Homo sapiens
  source 1..7801: mol_type = other DNA
aagcctgatgtttgtctgtggaaagatgttacttcatctcccaggtttgctcactgcaaatacaatcctgagaactgaactagggccttaaagtcctgacatgcatggcttggttttgtggattgcctctctcaacaggtggtgaaatttaccaaatcctttgaattgatgtccccaaagtgcagtgctgatgctgagaacagtttcaaagaaagcatggagaaatcatcatactccgactggctaataaataacagcattgctgagctggttgcttcaacaggccttccagtgaacatcagtgatgcctaccaggatccgcgctttgatgcagaggcagaccagatatctggttttcacataagatctgttctttgtgtccctatttggaatagcaaccaccaaataattggagtggctcaagtgttaaacagacttgatgggaaaccttttgatgatgcagatcaacgactttttgaggcttttgtcatcttttgtggacttggcatcaacaacacaattatgtatgatcaagtgaagaagtcctgggccaagcagtctgtggctcttgatgtgctatcataccatgcaacatgttcaaaagctgaagttgacaagtttaaggcagccaacatccctctggtgtcagaacttgccatcgatgacattcattttgatgacttttctctcgacgttgatgccatgatcacagctgctctccggatgttcatggagctggggatggtacagaaatttaaaattgactatgagacactgtgtaggtggcttttgacagtgaggaaaaactatcggatggttctataccacaactggagacatgccttcaacgtgtgtcagctgatgttcgcgatgttaaccactgctgggtttcaagacattctgaccgaggtggaaattttagcggtgattgtgggatgcctgtgtcatgacctcgaccacaggggaaccaacaatgccttccaagctaagagtggctctgccctggcccaactctatggaacctctgctaccttggagcatcaccatttcaaccacgccgtgatgatccttcaaagtgagggtcacaatatctttgctaacctgtcctccaaggaatatagtgaccttatgcagcttttgaagcagtcaatattggcaacagacctcacgctgtactttgagaggagaactgaattctttgaacttgtcagtaaaggagaatacgattggaacatcaaaaaccatcgtgatatatttcgatcaatgttaatgacagcctgtgaccttggagccgtgaccaaaccgtgggagatctccagacaggtggcagaacttgtaaccagtgagttcttcgaacaaggagatcgggagagattagagctcaaactcactccttcagcaatttttgatcggaaccggaaggatgaactgcctcggttgcaactggagtggattgatagcatctgcatgcctttgtatcaggcactggtgaaggtcaacgtgaaactgaagccgatgctagattcagtagctacaaacagaagtaagtgggaagagctacaccaaaaacgactgctggcctcaactgcctcatcctcccctgccagtgttatggtagccaaggaagacaggaactaaacctccaggtcagctgcagctgcaaaatgactacagcctgaagggccattttcagtccagcaatgtcatccttttgttcttttagctcagaaagacctaacatctcaaggatgcactgggaagcatgcctgggctttcaccttgaagcatggtcagcagcagagagagcaacgggaaggacaaagaaagaggtggggcagggagcacaccccaggaccctcacttttccctaatgaacacgcatgggctgaaatgaaggctctgggtaggggactgttttggatccaaggacctgtggacagtcggcctacttactctgagctgagggaacactgaacagtaaaagcgtcattagcgctgcttcgttttgtatagggcttttctgtttgttacaagccaaacactgcctgtctttgcttcctgtccctgaatgcctttttgtgccagactgtcccaagaatcctaatttgtattccatagaggtattttatttttaatcctagagcttcttattgatggatcctttagaattgcctacctaaaaggtaaactatactatccttataaatactgatcaatcccagttctccccctaaaaatgaatacatagtaggactatagcaaatgtgtttgatgggtaattctagactgggactatggtacccttttccagagttttaaaattcaaccttcattacagacaaagttttctcccagaaggaatggattgatagattttgattaaagtaagggtggaaggaaatctgtagctggatttaccacaagtgacatctagaaactatagttcacaggacagagcagagccatggagactaagcattgactaccttgagttctcctagtgaggagttctggtataaaatttaagattactaccagtaaccaacttaaagcaaactataggggtccctaattttggatttttccttaagtgtaagaaacaatgcttcaaatgttaagaaataacagtctgggcaaagaacgcatattctataggaagccaggtttacaataggtaagaataaactgtattaagtagatgtaatgactagaaagctgctttgctccctatattgagaaattgtggacatggtatgtgttatccaaagaacattgggctagaagatagatttctatccttagctttggcattattgactggattgacttgaacaagtcacttaacttctacaagcttgtttccttatttgtcaaattagattacactaggaaacgattctcgaacatgttttaaccttacaactctttgttcaaataaatctttcaatgaatccccaacatataaaacgtcaaaaagctgaattcctatgtgaattataagcagggtttggacatccagagcacctacaaaccttcatctctttgattacgtacatgggggtccacagggactctgaagagtttgaaaatccctggcctagattaaacctgagagccattctagctcttaaaaaaatctgaaatttacaaaccatttttcttgttattgtttttgtttctttgtttgtttgttttttgagactgagttttcactcttgttgcccaggctggagtgcaatggcgtgatctcggcttactgcaacctctgcttcctgggttcaagcaattctccagcctcaacctcctgagaagctgggattacaggtgcctgccaccacgcctggctaatttttgtacttttagtagacacagggtttcaccatgtttgccaggctgatctcaaactcctgacctcaggtgagccacccacctctgcctccgaaagtgctgggattacaggcgtgagccaccgtacccggcccttgttattgttattaatcattatcaatcattaactttacagatattaaagaaataggggccatgttctacatgcgacattgttttcctggcacacagtagacaattcaggaaatgtctgaagaaggaatgggtaaaattaagataccaaaatggaattgaggggagagcaggtaattgtagagaaaaagactctttatggcaagaaacaaagtaaaagaaatgtatagaccgggcgcggtggctcacgcctgtaatcccagcaatttggaaggccgaggcgggcggatcacgaggtcaggagatcgagaccgtcctggctaacacggtgaaaccctgtctctactaaaaaacacaaaacaaattagccaggcgcggtggcaggcgtctgtagtcccagctactggggaggctgaggcaagagaatggcgggaacccgcgaggcggagcttgcagtgagtcgagatcacgtcactgccctccagcctgggcgaccagcgagactccgtctcaaaaaaaaaaaaaaaaaaaaaaaaaaaaaaaaaaagtataaaccagactaagaggggaataaaagcaagaagaaaaagaaacgtaagaacaccagtaaaggaaagacagggaccgagacaggtggttaagggaaatgaaaaaaaaaaaaaaaaggtgaaagtcaatccaaacaaagaaaaatggcacttccaaccaaaaaaaatgaaggtgtagaaccctgtcatcaattgctcagaaaagagagacacttgagcagggaggggtttgagaaaggggagaaggaaggagtgagagccctaaaaaataatgttcctagctaccctttacagctgtctctgcagggaagactggagaaagtagagggggaaatgaatgcaggaagaaactgcctctgcagagcaggtaagaggaggttgttcagatttatggattttattaagccagttttctgtatcactctgctataaaggaaaatagcttctgcagggctgtctctcctccttcaggtggggaacaaagggtgggtggagtcagggacagagtctggtctgcgagatcgtgacgtgtctgcagctccgaagcactgcaggtgtttctgggtaatgtgccacatcatgtttatatcacgaacgggaattgaaaatcagtctgtgtgaggcagagatgagcccacatctgttatcctccccaacaataaataaataaatagcccagacaaatggatgccagtccatctacagcaacattttaaagcatgtgctttatgacaaaactggacccagggtctgacagagactgcaggctgccgtgagcactgtagctatcctgaacattgatgctacatattgctaaggggaacataatttatagcataaaccctacaagcttccactaaggttgagttttcctctcattttcttgccgttttattggcttcactgcatggttgccaatagcaacatccactggtagcaaggggagttcaacaccattgcaatctgccatacagtggagccctgacaatgtcaaccatcaatctagtagctgtttgtaattgcctccatctatttctcctgtcttgaggtatctttcctattgtgggtcaagatttagaaactgctgactaatgccatgggtctgtgtctccatgactatgaagcagtggacaggaaggtagcagcttcctggtgccaacaaccccagaggttagaggttgaactcttgcgggtttcaggcgtttttaatcccttttctaaacaatttataattttgcaagaatgtgaggcatatgcagttatccatataatctgcttttccaaaaaagagaaaggaagtttcccagtccttattattaatgtttatttcctattggagaaagacatttgaaatatgagccttcttgtaaaaactcaaactgaccagattatgtttgcttcctcaggtctcttggcattaattgttgaaataacttcatcctactttttcgatgagatgtatttttttcagacatatttattcttactagtcactatgtagctattatgtgcacaatctacaatgtagtggcaatcctggtgggtagggacagcttcacatactgcaaagggtgccattcagtgcatagcagactggaactccctcctagcttggccaccagctgaacctgtaatcttaggactctccaagtcttagaatctccatctattacataaaagcactgacttttattcagtccccacaccaaaggaccaagacgtgtttagctttaaagaaattttccagataattttcttttttattcttctcaaataaaatagcaacaaacctaaagcagtcatcttcttaataaagacataataaaacttacatatatggggtagatgtaagcacaatcatactacagatgtatcttgagcctgtctctaattatgatgaaagatgtagtcatcaatacaatttaaaaaaagatatgtcctttttttgagacagggtcttgctctgtcacccaggctggagggcagtggcacaatcacagccactgcagccttgacctctccaacttaagtgatctttcctgcctcagcctcatgagtagctgggaccacaggtgtgcaccaccacacccagctaaattttgtattgtttgtaaagacgaggcctcactatgctgaccacactggtctcgaactcctgggctcaagcaatcctcctgccttggcctcccaaagtgttagggttagagatatgaaccaccacacccaccttatatgtccttttatttcataaaaaacaattttagattatctgatatcacacatatcccataaatggtagtcattaatttagaagtgaatttataaagttaagagaagttaaaattgcacatgcattttgtttctaaaatctgagatgtctatgcatttccaggtattgtatatttgcaaatacattgggttagaaatcatctttaacattttgtgttagtgtaataacaatattatctaatattaatgctgccagaatccagttgctttttctgtgtatcaaaatttatcataactttttccacttaacactaggtaattaaacagaatctgcccaatttattctgcagtaaaattattttaaaatctatttttcctgctgactcttagaaattgcagaaagacaaaaaccagtttcatctccagtaatagtgtgaaacaatttccttccagtgggacagaaacctagacatactagggaaagatttaaatataaagaaaaatgccttggctgaaaaaaaaaaaaaccaccaaaacacaaaaaggattcattaaagcaacagaacaaaacctaatttgggaccctaaaaactctggcaatgccactgtaatgaagtttcattatctgcttcagagtaacagtctctgaaattgttattctgctacatgctgtaaagaactcccaaaactcaaatgtatcaggaaatgtaaaggttaagtctgactacaagaaggccaaaattgcaccagcttcctaagtgaagaataatagaataaaacatatagagggcagaaataaaatgaggtgtatctggagaatttcatgatgagcatttagatttagcaatgcccaatgtcatgctgacactgtttgtcatgaccttgtcttcagctagtaatttggggttgtacttttttaaatttaattttgaatgttcttgcatgtttggtacctctctcctcactgctaaagataaattgtttatctgtataacataactacaccaatgtcatttttgtatacgctagtacacaaatgtgtttttttattaagtaatgaagtatttgctgtgaaaaatgtattatttgtgccaccgtttatatctgtgttcattttctgtgtgtatatgcgtgtgtattcgaatctcaatttttcttttactctagtttagattaagacatatttagatgaaattttaaaaataacattggaaataggaggctaagttttgttgagtctcattcccttggggggaaattgcttttgccattttattttcatgtacaataacctaaaaaggatctcctactgacttccttcctaattattattgttttacacgaaagaaaggaaatacgttttcaattgagttgtttgaaatcattcactttgtgtagatttcccagactgatgtttcattgtaagaatattacattatagacaggttggccatttcacaagcaactaatccatagttttggaagcccgctttaagagacctgaatatctttgtttttaataaaatacttagagtttaactaaa

SEQ ID NO: 118 - protein, 489 aa, Homo sapiens
MSPKCSADAENSFKESMEKSSYSDWLINNSIAELVASTGLPVNISDAYQDPRFDAEADQISGFHIRSVLCVPIWNSNHQIIGVAQVLNRLDGKPFDDADQRLFEAFVIFCGLGINNTIMYDQVKKSWAKQSVALDVLSYHATCSKAEVDKFKAANIPLVSELAIDDIHFDDFSLDVDAMITAALRMFMELGMVQKFKIDYETLCRWLLTVRKNYRMVLYHNWRHAFNVCQLMFAMLTTAGFQDILTEVEILAVIVGCLCHDLDHRGTNNAFQAKSGSALAQLYGTSATLEHHHFNHAVMILQSEGHNIFANLSSKEYSDLMQLLKQSILATDLTLYFERRTEFFELVSKGEYDWNIKNHRDIFRSMLMTACDLGAVTKPWEISRQVAELVTSEFFEQGDRERLELKLTPSAIFDRNRKDELPRLQLEWIDSICMPLYQALVKVNVKLKPMLDSVATNRSKWEELHQKRLLASTASSSPASVMVAKEDRN

SEQ ID NO: 119 - protein, 28 aa, synthetic construct
HDSGYEVHHQKLVFFAEDVGSNKGAIIG

SEQ ID NO: 120 - protein, 33 aa, synthetic construct
FRHDSGYEVHHQKLVFFAEDVGSNKGAIIGLMV

SEQ ID NO: 121 - protein, 42 aa, synthetic construct [sequence omitted]

SEQ ID NO: 122 - protein, 40 aa, synthetic construct
DAEFRHDSGYEVHHQKLVFFAEDVGSNKGAIIGLMVGGVV